European Patent Application EP 4 681 728 A2, published January 21, 2026. Title: HERPES ZOSTER mRNA VACCINE, PREPARATION METHOD THEREFOR, AND USE THEREOF. Applicant: Hangzhou Tianlong Pharmaceutical Co., Ltd. Application EP. The sequence listing filed with the application follows.

SEQUENCE LISTING (191 sequences)

SEQ ID NO: 1 - DNA, 2138 bp, Varicella Zoster Virus
  source 1..2138: mol_type = genomic DNA
agaaataagagagaaaagaagagtaagaagaaatataagagccaccatgggcaccgtgaacaagcctgttgtgggcgtgctgatgggcttcggcatcatcacaggcaccctgcggatcaccaatcctgtgcgggctagcgtgctgagatacgacgacttccacatcgacgaggacaagctggacaccaacagcgtgtacgagccctactaccacagcgatcacgccgagtctagctgggtcaacagaggcgagagcagcagaaaggcctacgaccacaacagcccctacatctggccccggaacgactacgatggcttcctggaaaatgcccacgagcaccacggcgtgtacaatcaaggcagaggcatcgacagcggcgagagactgatgcagcctacacagatgagcgcccaagaggacctgggagatgataccggcatccacgtgatccccacactgaacggcgacgacagacacaagatcgtgaacgtggaccagcggcagtacggcgacgtgttcaagggcgacctgaatcctaagcctcagggccagcgcctgatcgaggtgtccgtggaagagaatcaccccttcacactgagagcccctatccagagaatctacggcgtgcgctataccgagacatggtcctttctgcccagcctgacatgtaccggggatgccgctcctgccatccagcacatttgcctgaagcacaccacctgtttccaggacgtggtggtggatgtggactgcgccgagaacaccaaagaggatcagctggccgagatcagctaccggttccagggaaagaaagaggccgaccagccttggatcgtggtcaacaccagcacactgttcgacgagctggaactggaccctcctgagattgaacccggggtgctgaaggtgctgagaaccgagaagcagtacctgggagtgtacatctggaacatgagaggcagcgacggcacctctacctacgccacctttctggtcacatggaagggcgacgagaaaacacggaaccccacaccagctgtgacccctcaacctagaggcgccgagtttcacatgtggaattaccacagccacgtgttcagcgtgggcgatacctttagcctggccatgcatctgcagtacaagatccacgaggcccctttcgacctgctgctggaatggctgtacgtgcccatcgatcctacctgccagcctatgcggctgtactccacctgtctgtatcaccccaacgctccccagtgcctgagccacatgaatagcggctgcaccttcacaagccctcacctggctcagcgagtggccagcacagtgtaccagaattgcgagcacgccgacaattacaccgcctactgtctgggcatcagccacatggaacctagcttcggcctgatcctgcacgatggcggcacaaccctgaagttcgtggatacccctgagagcctgagcggcctgtatgtgttcgtggtgtacttcaacggccacgtggaagccgtggcctacaccgtggtgtctaccgtggaccacttcgtgaacgccatcgaggaaagaggcttccctccaactgctggacagcctcctgccaccaccaagcctaaagaaatcacacccgtgaatcccggcacaagcccactgcttagatacgccgcttggacaggcggactggctgctgttgttctgctgtgcctggtcatcttcctgatctgcaccgccaagcggatgagagtgaaggcctacagagtggacaagagcccttacaaccagagcatgtactacgccggcctgcctgtggacgacttcgaggatagcgagagcaccgacaccgaggaagagttcggcaacgccattggaggatctcacggcggcagcagctataccgtgtacatcgacaagacccggtgagctggagcctcggtggccatgcttcttgccccttgggcctccccccagcccctcctccccttcctgcacccgtacccccgtggtctttgaataaagtctgagtgggcggcaaaaaaaaaaaaaaaaaaaaaaaaaaaaaaaaaaaaaaaaaaaaaaaaaaaaaaaaaaaaaaaaaaaaaaaaaaaaaaaaaaaaaaaaaaaaaaaaaaaaaaaaaaaaaa

SEQ ID NO: 2 - DNA, 1872 bp, Varicella Zoster Virus
  source 1..1872: mol_type = other DNA
atgggcaccgtgaacaagcctgttgtgggcgtgctgatgggcttcggcatcatcacaggcaccctgcggatcaccaatcctgtgcgggctagcgtgctgagatacgacgacttccacatcgacgaggacaagctggacaccaacagcgtgtacgagccctactaccacagcgatcacgccgagtctagctgggtcaacagaggcgagagcagcagaaaggcctacgaccacaacagcccctacatctggccccggaacgactacgatggcttcctggaaaatgcccacgagcaccacggcgtgtacaatcaaggcagaggcatcgacagcggcgagagactgatgcagcctacacagatgagcgcccaagaggacctgggagatgataccggcatccacgtgatccccacactgaacggcgacgacagacacaagatcgtgaacgtggaccagcggcagtacggcgacgtgttcaagggcgacctgaatcctaagcctcagggccagcgcctgatcgaggtgtccgtggaagagaatcaccccttcacactgagagcccctatccagagaatctacggcgtgcgctataccgagacatggtcctttctgcccagcctgacatgtaccggggatgccgctcctgccatccagcacatttgcctgaagcacaccacctgtttccaggacgtggtggtggatgtggactgcgccgagaacaccaaagaggatcagctggccgagatcagctaccggttccagggaaagaaagaggccgaccagccttggatcgtggtcaacaccagcacactgttcgacgagctggaactggaccctcctgagattgaacccggggtgctgaaggtgctgagaaccgagaagcagtacctgggagtgtacatctggaacatgagaggcagcgacggcacctctacctacgccacctttctggtcacatggaagggcgacgagaaaacacggaaccccacaccagctgtgacccctcaacctagaggcgccgagtttcacatgtggaattaccacagccacgtgttcagcgtgggcgatacctttagcctggccatgcatctgcagtacaagatccacgaggcccctttcgacctgctgctggaatggctgtacgtgcccatcgatcctacctgccagcctatgcggctgtactccacctgtctgtatcaccccaacgctccccagtgcctgagccacatgaatagcggctgcaccttcacaagccctcacctggctcagcgagtggccagcacagtgtaccagaattgcgagcacgccgacaattacaccgcctactgtctgggcatcagccacatggaacctagcttcggcctgatcctgcacgatggcggcacaaccctgaagttcgtggatacccctgagagcctgagcggcctgtatgtgttcgtggtgtacttcaacggccacgtggaagccgtggcctacaccgtggtgtctaccgtggaccacttcgtgaacgccatcgaggaaagaggcttccctccaactgctggacagcctcctgccaccaccaagcctaaagaaatcacacccgtgaatcccggcacaagcccactgcttagatacgccgcttggacaggcggactggctgctgttgttctgctgtgcctggtcatcttcctgatctgcaccgccaagcggatgagagtgaaggcctacagagtggacaagagcccttacaaccagagcatgtactacgccggcctgcctgtggacgacttcgaggatagcgagagcaccgacaccgaggaagagttcggcaacgccattggaggatctcacggcggcagcagctataccgtgtacatcgacaagacccggtga

SEQ ID NO: 3 - protein, 623 aa, Varicella Zoster Virus
MGTVNKPVVGVLMGFGIITGTLRITNPVRASVLRYDDFHIDEDKLDTNSVYEPYYHSDHAESSWVNRGESSRKAYDHNSPYIWPRNDYDGFLENAHEHHGVYNQGRGIDSGERLMQPTQMSAQEDLGDDTGIHVIPTLNGDDRHKIVNVDQRQYGDVFKGDLNPKPQGQRLIEVSVEENHPFTLRAPIQRIYGVRYTETWSFLPSLTCTGDAAPAIQHICLKHTTCFQDVVVDVDCAENTKEDQLAEISYRFQGKKEADQPWIVVNTSTLFDELELDPPEIEPGVLKVLRTEKQYLGVYIWNMRGSDGTSTYATFLVTWKGDEKTRNPTPAVTPQPRGAEFHMWNYHSHVFSVGDTFSLAMHLQYKIHEAPFDLLLEWLYVPIDPTCQPMRLYSTCLYHPNAPQCLSHMNSGCTFTSPHLAQRVASTVYQNCEHADNYTAYCLGISHMEPSFGLILHDGGTTLKFVDTPESLSGLYVFVVYFNGHVEAVAYTVVSTVDHFVNAIEERGFPPTAGQPPATTKPKEITPVNPGTSPLLRYAAWTGGLAAVVLLCLVIFLICTAKRMRVKAYRVDKSPYNQSMYYAGLPVDDFEDSESTDTEEEFGNAIGGSHGGSSYTVYIDKTR

SEQ ID NO: 4 - RNA, 2138 nt, Varicella Zoster Virus
  source 1..2138: mol_type = mRNA
agaaataagagagaaaagaagagtaagaagaaatataagagccaccatgggcaccgtgaacaagcctgttgtgggcgtgctgatgggcttcggcatcatcacaggcaccctgcggatcaccaatcctgtgcgggctagcgtgctgagatacgacgacttccacatcgacgaggacaagctggacaccaacagcgtgtacgagccctactaccacagcgatcacgccgagtctagctgggtcaacagaggcgagagcagcagaaaggcctacgaccacaacagcccctacatctggccccggaacgactacgatggcttcctggaaaatgcccacgagcaccacggcgtgtacaatcaaggcagaggcatcgacagcggcgagagactgatgcagcctacacagatgagcgcccaagaggacctgggagatgataccggcatccacgtgatccccacactgaacggcgacgacagacacaagatcgtgaacgtggaccagcggcagtacggcgacgtgttcaagggcgacctgaatcctaagcctcagggccagcgcctgatcgaggtgtccgtggaagagaatcaccccttcacactgagagcccctatccagagaatctacggcgtgcgctataccgagacatggtcctttctgcccagcctgacatgtaccggggatgccgctcctgccatccagcacatttgcctgaagcacaccacctgtttccaggacgtggtggtggatgtggactgcgccgagaacaccaaagaggatcagctggccgagatcagctaccggttccagggaaagaaagaggccgaccagccttggatcgtggtcaacaccagcacactgttcgacgagctggaactggaccctcctgagattgaacccggggtgctgaaggtgctgagaaccgagaagcagtacctgggagtgtacatctggaacatgagaggcagcgacggcacctctacctacgccacctttctggtcacatggaagggcgacgagaaaacacggaaccccacaccagctgtgacccctcaacctagaggcgccgagtttcacatgtggaattaccacagccacgtgttcagcgtgggcgatacctttagcctggccatgcatctgcagtacaagatccacgaggcccctttcgacctgctgctggaatggctgtacgtgcccatcgatcctacctgccagcctatgcggctgtactccacctgtctgtatcaccccaacgctccccagtgcctgagccacatgaatagcggctgcaccttcacaagccctcacctggctcagcgagtggccagcacagtgtaccagaattgcgagcacgccgacaattacaccgcctactgtctgggcatcagccacatggaacctagcttcggcctgatcctgcacgatggcggcacaaccctgaagttcgtggatacccctgagagcctgagcggcctgtatgtgttcgtggtgtacttcaacggccacgtggaagccgtggcctacaccgtggtgtctaccgtggaccacttcgtgaacgccatcgaggaaagaggcttccctccaactgctggacagcctcctgccaccaccaagcctaaagaaatcacacccgtgaatcccggcacaagcccactgcttagatacgccgcttggacaggcggactggctgctgttgttctgctgtgcctggtcatcttcctgatctgcaccgccaagcggatgagagtgaaggcctacagagtggacaagagcccttacaaccagagcatgtactacgccggcctgcctgtggacgacttcgaggatagcgagagcaccgacaccgaggaagagttcggcaacgccattggaggatctcacggcggcagcagctataccgtgtacatcgacaagacccggtgagctggagcctcggtggccatgcttcttgccccttgggcctccccccagcccctcctccccttcctgcacccgtacccccgtggtctttgaataaagtctgagtgggcggcaaaaaaaaaaaaaaaaaaaaaaaaaaaaaaaaaaaaaaaaaaaaaaaaaaaaaaaaaaaaaaaaaaaaaaaaaaaaaaaaaaaaaaaaaaaaaaaaaaaaaaaaaaaaaa

SEQ ID NO: 5 - DNA, 1909 bp, synthetic construct
  source 1..1909: mol_type = other DNA
agactcctccccatcctctccctctgtccctctgtccctctgaccctgcactgtcccagcaccgccaccatgggcaccgtgaacaagcctgttgtgggcgtgctgatgggcttcggcatcatcacaggcaccctgcggatcaccaatcctgtgcgggctagcgtgctgagatacgacgacttccacatcgacgaggacaagctggacaccaacagcgtgtacgagccctactaccacagcgatcacgccgagtctagctgggtcaacagaggcgagagcagcagaaaggcctacgaccacaacagcccctacatctggccccggaacgactacgatggcttcctggaaaatgcccacgagcaccacggcgtgtacaatcaaggcagaggcatcgacagcggcgagagactgatgcagcctacacagatgagcgcccaagaggacctgggagatgataccggcatccacgtgatccccacactgaacggcgacgacagacacaagatcgtgaacgtggaccagcggcagtacggcgacgtgttcaagggcgacctgaatcctaagcctcagggccagcgcctgatcgaggtgtccgtggaagagaatcaccccttcacactgagagcccctatccagagaatctacggcgtgcgctataccgagacatggtcctttctgcccagcctgacatgtaccggggatgccgctcctgccatccagcacatttgcctgaagcacaccacctgtttccaggacgtggtggtggatgtggactgcgccgagaacaccaaagaggatcagctggccgagatcagctaccggttccagggaaagaaagaggccgaccagccttggatcgtggtcaacaccagcacactgttcgacgagctggaactggaccctcctgagattgaacccggggtgctgaaggtgctgagaaccgagaagcagtacctgggagtgtacatctggaacatgagaggcagcgacggcacctctacctacgccacctttctggtcacatggaagggcgacgagaaaacacggaaccccacaccagctgtgacccctcaacctagaggcgccgagtttcacatgtggaattaccacagccacgtgttcagcgtgggcgatacctttagcctggccatgcatctgcagtacaagatccacgaggcccctttcgacctgctgctggaatggctgtacgtgcccatcgatcctacctgccagcctatgcggctgtactccacctgtctgtatcaccccaacgctccccagtgcctgagccacatgaatagcggctgcaccttcacaagccctcacctggctcagcgagtggccagcacagtgtaccagaattgcgagcacgccgacaattacaccgcctactgtctgggcatcagccacatggaacctagcttcggcctgatcctgcacgatggcggcacaaccctgaagttcgtggatacccctgagagcctgagcggcctgtatgtgttcgtggtgtacttcaacggccacgtggaagccgtggcctacaccgtggtgtctaccgtggaccacttcgtgaacgccatcgaggaaagaggcttccctccaactgctggacagcctcctgccaccaccaagcctaaagaaatcacacccgtgaatcccggcacaagcccactgctcagatatgcctgagctggagcctcggtggccatgcttcttgccccttgggcctccccccagcccctcctccccttcctgcacccgtacccccgtggtctttgaataaagtctgagtgggcggcaaaaaaaaaaaaaaaaaaaaaaaaaaaaaaaaaaaaaaaaaaaaaaaaaaaaaaaaaaaaaaaaaaaaaaaaaaaaaaaaaaaaaaaaaaaaaaaaaaaaaaaaaaaaaa

SEQ ID NO: 6 - DNA, 1620 bp, synthetic construct
  source 1..1620: mol_type = other DNA
atgggcaccgtgaacaagcctgttgtgggcgtgctgatgggcttcggcatcatcacaggcaccctgcggatcaccaatcctgtgcgggctagcgtgctgagatacgacgacttccacatcgacgaggacaagctggacaccaacagcgtgtacgagccctactaccacagcgatcacgccgagtctagctgggtcaacagaggcgagagcagcagaaaggcctacgaccacaacagcccctacatctggccccggaacgactacgatggcttcctggaaaatgcccacgagcaccacggcgtgtacaatcaaggcagaggcatcgacagcggcgagagactgatgcagcctacacagatgagcgcccaagaggacctgggagatgataccggcatccacgtgatccccacactgaacggcgacgacagacacaagatcgtgaacgtggaccagcggcagtacggcgacgtgttcaagggcgacctgaatcctaagcctcagggccagcgcctgatcgaggtgtccgtggaagagaatcaccccttcacactgagagcccctatccagagaatctacggcgtgcgctataccgagacatggtcctttctgcccagcctgacatgtaccggggatgccgctcctgccatccagcacatttgcctgaagcacaccacctgtttccaggacgtggtggtggatgtggactgcgccgagaacaccaaagaggatcagctggccgagatcagctaccggttccagggaaagaaagaggccgaccagccttggatcgtggtcaacaccagcacactgttcgacgagctggaactggaccctcctgagattgaacccggggtgctgaaggtgctgagaaccgagaagcagtacctgggagtgtacatctggaacatgagaggcagcgacggcacctctacctacgccacctttctggtcacatggaagggcgacgagaaaacacggaaccccacaccagctgtgacccctcaacctagaggcgccgagtttcacatgtggaattaccacagccacgtgttcagcgtgggcgatacctttagcctggccatgcatctgcagtacaagatccacgaggcccctttcgacctgctgctggaatggctgtacgtgcccatcgatcctacctgccagcctatgcggctgtactccacctgtctgtatcaccccaacgctccccagtgcctgagccacatgaatagcggctgcaccttcacaagccctcacctggctcagcgagtggccagcacagtgtaccagaattgcgagcacgccgacaattacaccgcctactgtctgggcatcagccacatggaacctagcttcggcctgatcctgcacgatggcggcacaaccctgaagttcgtggatacccctgagagcctgagcggcctgtatgtgttcgtggtgtacttcaacggccacgtggaagccgtggcctacaccgtggtgtctaccgtggaccacttcgtgaacgccatcgaggaaagaggcttccctccaactgctggacagcctcctgccaccaccaagcctaaagaaatcacacccgtgaatcccggcacaagcccactgctcagatatgcctga

SEQ ID NO: 7 - protein, 539 aa, synthetic construct
MGTVNKPVVGVLMGFGIITGTLRITNPVRASVLRYDDFHIDEDKLDTNSVYEPYYHSDHAESSWVNRGESSRKAYDHNSPYIWPRNDYDGFLENAHEHHGVYNQGRGIDSGERLMQPTQMSAQEDLGDDTGIHVIPTLNGDDRHKIVNVDQRQYGDVFKGDLNPKPQGQRLIEVSVEENHPFTLRAPIQRIYGVRYTETWSFLPSLTCTGDAAPAIQHICLKHTTCFQDVVVDVDCAENTKEDQLAEISYRFQGKKEADQPWIVVNTSTLFDELELDPPEIEPGVLKVLRTEKQYLGVYIWNMRGSDGTSTYATFLVTWKGDEKTRNPTPAVTPQPRGAEFHMWNYHSHVFSVGDTFSLAMHLQYKIHEAPFDLLLEWLYVPIDPTCQPMRLYSTCLYHPNAPQCLSHMNSGCTFTSPHLAQRVASTVYQNCEHADNYTAYCLGISHMEPSFGLILHDGGTTLKFVDTPESLSGLYVFVVYFNGHVEAVAYTVVSTVDHFVNAIEERGFPPTAGQPPATTKPKEITPVNPGTSPLLRYA

SEQ ID NO: 8 - RNA, 1909 nt, synthetic construct
  source 1..1909: mol_type = other RNA
agactcctccccatcctctccctctgtccctctgtccctctgaccctgcactgtcccagcaccgccaccatgggcaccgtgaacaagcctgttgtgggcgtgctgatgggcttcggcatcatcacaggcaccctgcggatcaccaatcctgtgcgggctagcgtgctgagatacgacgacttccacatcgacgaggacaagctggacaccaacagcgtgtacgagccctactaccacagcgatcacgccgagtctagctgggtcaacagaggcgagagcagcagaaaggcctacgaccacaacagcccctacatctggccccggaacgactacgatggcttcctggaaaatgcccacgagcaccacggcgtgtacaatcaaggcagaggcatcgacagcggcgagagactgatgcagcctacacagatgagcgcccaagaggacctgggagatgataccggcatccacgtgatccccacactgaacggcgacgacagacacaagatcgtgaacgtggaccagcggcagtacggcgacgtgttcaagggcgacctgaatcctaagcctcagggccagcgcctgatcgaggtgtccgtggaagagaatcaccccttcacactgagagcccctatccagagaatctacggcgtgcgctataccgagacatggtcctttctgcccagcctgacatgtaccggggatgccgctcctgccatccagcacatttgcctgaagcacaccacctgtttccaggacgtggtggtggatgtggactgcgccgagaacaccaaagaggatcagctggccgagatcagctaccggttccagggaaagaaagaggccgaccagccttggatcgtggtcaacaccagcacactgttcgacgagctggaactggaccctcctgagattgaacccggggtgctgaaggtgctgagaaccgagaagcagtacctgggagtgtacatctggaacatgagaggcagcgacggcacctctacctacgccacctttctggtcacatggaagggcgacgagaaaacacggaaccccacaccagctgtgacccctcaacctagaggcgccgagtttcacatgtggaattaccacagccacgtgttcagcgtgggcgatacctttagcctggccatgcatctgcagtacaagatccacgaggcccctttcgacctgctgctggaatggctgtacgtgcccatcgatcctacctgccagcctatgcggctgtactccacctgtctgtatcaccccaacgctccccagtgcctgagccacatgaatagcggctgcaccttcacaagccctcacctggctcagcgagtggccagcacagtgtaccagaattgcgagcacgccgacaattacaccgcctactgtctgggcatcagccacatggaacctagcttcggcctgatcctgcacgatggcggcacaaccctgaagttcgtggatacccctgagagcctgagcggcctgtatgtgttcgtggtgtacttcaacggccacgtggaagccgtggcctacaccgtggtgtctaccgtggaccacttcgtgaacgccatcgaggaaagaggcttccctccaactgctggacagcctcctgccaccaccaagcctaaagaaatcacacccgtgaatcccggcacaagcccactgctcagatatgcctgagctggagcctcggtggccatgcttcttgccccttgggcctccccccagcccctcctccccttcctgcacccgtacccccgtggtctttgaataaagtctgagtgggcggcaaaaaaaaaaaaaaaaaaaaaaaaaaaaaaaaaaaaaaaaaaaaaaaaaaaaaaaaaaaaaaaaaaaaaaaaaaaaaaaaaaaaaaaaaaaaaaaaaaaaaaaaaaaaaa

SEQ ID NO: 9 - DNA, 1996 bp, synthetic construct
  source 1..1996: mol_type = other DNA
agactcctccccatcctctccctctgtccctctgtccctctgaccctgcactgtcccagcaccgccaccatgggcaccgtgaacaagcctgttgtgggcgtgctgatgggcttcggcatcatcacaggcaccctgcggatcaccaatcctgtgcgggctagcgtgctgagatacgacgacttccacatcgacgaggacaagctggacaccaacagcgtgtacgagccctactaccacagcgatcacgccgagtctagctgggtcaacagaggcgagagcagcagaaaggcctacgaccacaacagcccctacatctggccccggaacgactacgatggcttcctggaaaatgcccacgagcaccacggcgtgtacaatcaaggcagaggcatcgacagcggcgagagactgatgcagcctacacagatgagcgcccaagaggacctgggagatgataccggcatccacgtgatccccacactgaacggcgacgacagacacaagatcgtgaacgtggaccagcggcagtacggcgacgtgttcaagggcgacctgaatcctaagcctcagggccagcgcctgatcgaggtgtccgtggaagagaatcaccccttcacactgagagcccctatccagagaatctacggcgtgcgctataccgagacatggtcctttctgcccagcctgacatgtaccggggatgccgctcctgccatccagcacatttgcctgaagcacaccacctgtttccaggacgtggtggtggatgtggactgcgccgagaacaccaaagaggatcagctggccgagatcagctaccggttccagggaaagaaagaggccgaccagccttggatcgtggtcaacaccagcacactgttcgacgagctggaactggaccctcctgagattgaacccggggtgctgaaggtgctgagaaccgagaagcagtacctgggagtgtacatctggaacatgagaggcagcgacggcacctctacctacgccacctttctggtcacatggaagggcgacgagaaaacacggaaccccacaccagctgtgacccctcaacctagaggcgccgagtttcacatgtggaattaccacagccacgtgttcagcgtgggcgatacctttagcctggccatgcatctgcagtacaagatccacgaggcccctttcgacctgctgctggaatggctgtacgtgcccatcgatcctacctgccagcctatgcggctgtactccacctgtctgtatcaccccaacgctccccagtgcctgagccacatgaatagcggctgcaccttcacaagccctcacctggctcagcgagtggccagcacagtgtaccagaattgcgagcacgccgacaattacaccgcctactgtctgggcatcagccacatggaacctagcttcggcctgatcctgcacgatggcggcacaaccctgaagttcgtggatacccctgagagcctgagcggcctgtatgtgttcgtggtgtacttcaacggccacgtggaagccgtggcctacaccgtggtgtctaccgtggaccacttcgtgaacgccatcgaggaaagaggcttccctccaactgctggacagcctcctgccaccaccaagcctaaagaaatcacacccgtgaatcccggcacaagcccactgcttagatacgccgcttggacaggcggactggctgctgttgttctgctgtgcctggtcatcttcctgatctgcaccgccaagcggatgagagtgaaagcctgagctggagcctcggtggccatgcttcttgccccttgggcctccccccagcccctcctccccttcctgcacccgtacccccgtggtctttgaataaagtctgagtgggcggcaaaaaaaaaaaaaaaaaaaaaaaaaaaaaaaaaaaaaaaaaaaaaaaaaaaaaaaaaaaaaaaaaaaaaaaaaaaaaaaaaaaaaaaaaaaaaaaaaaaaaaaaaaaaaa

SEQ ID NO: 10 - DNA, 1707 bp, synthetic construct
  source 1..1707: mol_type = other DNA
atgggcaccgtgaacaagcctgttgtgggcgtgctgatgggcttcggcatcatcacaggcaccctgcggatcaccaatcctgtgcgggctagcgtgctgagatacgacgacttccacatcgacgaggacaagctggacaccaacagcgtgtacgagccctactaccacagcgatcacgccgagtctagctgggtcaacagaggcgagagcagcagaaaggcctacgaccacaacagcccctacatctggccccggaacgactacgatggcttcctggaaaatgcccacgagcaccacggcgtgtacaatcaaggcagaggcatcgacagcggcgagagactgatgcagcctacacagatgagcgcccaagaggacctgggagatgataccggcatccacgtgatccccacactgaacggcgacgacagacacaagatcgtgaacgtggaccagcggcagtacggcgacgtgttcaagggcgacctgaatcctaagcctcagggccagcgcctgatcgaggtgtccgtggaagagaatcaccccttcacactgagagcccctatccagagaatctacggcgtgcgctataccgagacatggtcctttctgcccagcctgacatgtaccggggatgccgctcctgccatccagcacatttgcctgaagcacaccacctgtttccaggacgtggtggtggatgtggactgcgccgagaacaccaaagaggatcagctggccgagatcagctaccggttccagggaaagaaagaggccgaccagccttggatcgtggtcaacaccagcacactgttcgacgagctggaactggaccctcctgagattgaacccggggtgctgaaggtgctgagaaccgagaagcagtacctgggagtgtacatctggaacatgagaggcagcgacggcacctctacctacgccacctttctggtcacatggaagggcgacgagaaaacacggaaccccacaccagctgtgacccctcaacctagaggcgccgagtttcacatgtggaattaccacagccacgtgttcagcgtgggcgatacctttagcctggccatgcatctgcagtacaagatccacgaggcccctttcgacctgctgctggaatggctgtacgtgcccatcgatcctacctgccagcctatgcggctgtactccacctgtctgtatcaccccaacgctccccagtgcctgagccacatgaatagcggctgcaccttcacaagccctcacctggctcagcgagtggccagcacagtgtaccagaattgcgagcacgccgacaattacaccgcctactgtctgggcatcagccacatggaacctagcttcggcctgatcctgcacgatggcggcacaaccctgaagttcgtggatacccctgagagcctgagcggcctgtatgtgttcgtggtgtacttcaacggccacgtggaagccgtggcctacaccgtggtgtctaccgtggaccacttcgtgaacgccatcgaggaaagaggcttccctccaactgctggacagcctcctgccaccaccaagcctaaagaaatcacacccgtgaatcccggcacaagcccactgcttagatacgccgcttggacaggcggactggctgctgttgttctgctgtgcctggtcatcttcctgatctgcaccgccaagcggatgagagtgaaagcctga

SEQ ID NO: 11 - protein, 568 aa, synthetic construct
MGTVNKPVVGVLMGFGIITGTLRITNPVRASVLRYDDFHIDEDKLDTNSVYEPYYHSDHAESSWVNRGESSRKAYDHNSPYIWPRNDYDGFLENAHEHHGVYNQGRGIDSGERLMQPTQMSAQEDLGDDTGIHVIPTLNGDDRHKIVNVDQRQYGDVFKGDLNPKPQGQRLIEVSVEENHPFTLRAPIQRIYGVRYTETWSFLPSLTCTGDAAPAIQHICLKHTTCFQDVVVDVDCAENTKEDQLAEISYRFQGKKEADQPWIVVNTSTLFDELELDPPEIEPGVLKVLRTEKQYLGVYIWNMRGSDGTSTYATFLVTWKGDEKTRNPTPAVTPQPRGAEFHMWNYHSHVFSVGDTFSLAMHLQYKIHEAPFDLLLEWLYVPIDPTCQPMRLYSTCLYHPNAPQCLSHMNSGCTFTSPHLAQRVASTVYQNCEHADNYTAYCLGISHMEPSFGLILHDGGTTLKFVDTPESLSGLYVFVVYFNGHVEAVAYTVVSTVDHFVNAIEERGFPPTAGQPPATTKPKEITPVNPGTSPLLRYAAWTGGLAAVVLLCLVIFLICTAKRMRVKA

SEQ ID NO: 12 - RNA, 1996 nt, synthetic construct
  source 1..1996: mol_type = other RNA
agactcctccccatcctctccctctgtccctctgtccctctgaccctgcactgtcccagcaccgccaccatgggcaccgtgaacaagcctgttgtgggcgtgctgatgggcttcggcatcatcacaggcaccctgcggatcaccaatcctgtgcgggctagcgtgctgagatacgacgacttccacatcgacgaggacaagctggacaccaacagcgtgtacgagccctactaccacagcgatcacgccgagtctagctgggtcaacagaggcgagagcagcagaaaggcctacgaccacaacagcccctacatctggccccggaacgactacgatggcttcctggaaaatgcccacgagcaccacggcgtgtacaatcaaggcagaggcatcgacagcggcgagagactgatgcagcctacacagatgagcgcccaagaggacctgggagatgataccggcatccacgtgatccccacactgaacggcgacgacagacacaagatcgtgaacgtggaccagcggcagtacggcgacgtgttcaagggcgacctgaatcctaagcctcagggccagcgcctgatcgaggtgtccgtggaagagaatcaccccttcacactgagagcccctatccagagaatctacggcgtgcgctataccgagacatggtcctttctgcccagcctgacatgtaccggggatgccgctcctgccatccagcacatttgcctgaagcacaccacctgtttccaggacgtggtggtggatgtggactgcgccgagaacaccaaagaggatcagctggccgagatcagctaccggttccagggaaagaaagaggccgaccagccttggatcgtggtcaacaccagcacactgttcgacgagctggaactggaccctcctgagattgaacccggggtgctgaaggtgctgagaaccgagaagcagtacctgggagtgtacatctggaacatgagaggcagcgacggcacctctacctacgccacctttctggtcacatggaagggcgacgagaaaacacggaaccccacaccagctgtgacccctcaacctagaggcgccgagtttcacatgtggaattaccacagccacgtgttcagcgtgggcgatacctttagcctggccatgcatctgcagtacaagatccacgaggcccctttcgacctgctgctggaatggctgtacgtgcccatcgatcctacctgccagcctatgcggctgtactccacctgtctgtatcaccccaacgctccccagtgcctgagccacatgaatagcggctgcaccttcacaagccctcacctggctcagcgagtggccagcacagtgtaccagaattgcgagcacgccgacaattacaccgcctactgtctgggcatcagccacatggaacctagcttcggcctgatcctgcacgatggcggcacaaccctgaagttcgtggatacccctgagagcctgagcggcctgtatgtgttcgtggtgtacttcaacggccacgtggaagccgtggcctacaccgtggtgtctaccgtggaccacttcgtgaacgccatcgaggaaagaggcttccctccaactgctggacagcctcctgccaccaccaagcctaaagaaatcacacccgtgaatcccggcacaagcccactgcttagatacgccgcttggacaggcggactggctgctgttgttctgctgtgcctggtcatcttcctgatctgcaccgccaagcggatgagagtgaaagcctgagctggagcctcggtggccatgcttcttgccccttgggcctccccccagcccctcctccccttcctgcacccgtacccccgtggtctttgaataaagtctgagtgggcggcaaaaaaaaaaaaaaaaaaaaaaaaaaaaaaaaaaaaaaaaaaaaaaaaaaaaaaaaaaaaaaaaaaaaaaaaaaaaaaaaaaaaaaaaaaaaaaaaaaaaaaaaaaaaaa

SEQ ID NO: 13 - DNA, 1988 bp, synthetic construct
  source 1..1988: mol_type = other DNA
agaaataagagagaaaagaagagtaagaagaaatataagagccaccatgggcaccgtgaacaagcctgttgtgggcgtgctgatgggcttcggcatcatcacaggcaccctgcggatcaccaatcctgtgcgggctagcgtgctgagatacgacgacttccacatcgacgaggacaagctggacaccaacagcgtgtacgagccctactaccacagcgatcacgccgagtctagctgggtcaacagaggcgagagcagcagaaaggcctacgaccacaacagcccctacatctggccccggaacgactacgatggcttcctggaaaatgcccacgagcaccacggcgtgtacaatcaaggcagaggcatcgacagcggcgagagactgatgcagcctacacagatgagcgcccaagaggacctgggagatgataccggcatccacgtgatccccacactgaacggcgacgacagacacaagatcgtgaacgtggaccagcggcagtacggcgacgtgttcaagggcgacctgaatcctaagcctcagggccagcgcctgatcgaggtgtccgtggaagagaatcaccccttcacactgagagcccctatccagagaatctacggcgtgcgctataccgagacatggtcctttctgcccagcctgacatgtaccggggatgccgctcctgccatccagcacatttgcctgaagcacaccacctgtttccaggacgtggtggtggatgtggactgcgccgagaacaccaaagaggatcagctggccgagatcagctaccggttccagggaaagaaagaggccgaccagccttggatcgtggtcaacaccagcacactgttcgacgagctggaactggaccctcctgagattgaacccggggtgctgaaggtgctgagaaccgagaagcagtacctgggagtgtacatctggaacatgagaggcagcgacggcacctctacctacgccacctttctggtcacatggaagggcgacgagaaaacacggaaccccacaccagctgtgacccctcaacctagaggcgccgagtttcacatgtggaattaccacagccacgtgttcagcgtgggcgatacctttagcctggccatgcatctgcagtacaagatccacgaggcccctttcgacctgctgctggaatggctgtacgtgcccatcgatcctacctgccagcctatgcggctgtactccacctgtctgtatcaccccaacgctccccagtgcctgagccacatgaatagcggctgcaccttcacaagccctcacctggctcagcgagtggccagcacagtgtaccagaattgcgagcacgccgacaattacaccgcctactgtctgggcatcagccacatggaacctagcttcggcctgatcctgcacgatggcggcacaaccctgaagttcgtggatacccctgagagcctgagcggcctgtatgtgttcgtggtgtacttcaacggccacgtggaagccgtggcctacaccgtggtgtctaccgtggaccacttcgtgaacgccatcgaggaaagaggcttccctccaactgctggacagcctcctgccaccaccaagcctaaagaaatcacacccgtgaatcccggcacaagcccactgcttagatacgccgcttggacaggcggactggctgctgttgttctgctgtgcctggtcatcttcctgatctgcaccgccaagcggatgagagtgaaagccgccagagtggacaagtgagctggagcctcggtggccatgcttcttgccccttgggcctccccccagcccctcctccccttcctgcacccgtacccccgtggtctttgaataaagtctgagtgggcggcaaaaaaaaaaaaaaaaaaaaaaaaaaaaaaaaaaaaaaaaaaaaaaaaaaaaaaaaaaaaaaaaaaaaaaaaaaaaaaaaaaaaaaaaaaaaaaaaaaaaaaaaaaaaaa

SEQ ID NO: 14 - DNA, 1722 bp, synthetic construct
  source 1..1722: mol_type = other DNA
atgggcaccgtgaacaagcctgttgtgggcgtgctgatgggcttcggcatcatcacaggcaccctgcggatcaccaatcctgtgcgggctagcgtgctgagatacgacgacttccacatcgacgaggacaagctggacaccaacagcgtgtacgagccctactaccacagcgatcacgccgagtctagctgggtcaacagaggcgagagcagcagaaaggcctacgaccacaacagcccctacatctggccccggaacgactacgatggcttcctggaaaatgcccacgagcaccacggcgtgtacaatcaaggcagaggcatcgacagcggcgagagactgatgcagcctacacagatgagcgcccaagaggacctgggagatgataccggcatccacgtgatccccacactgaacggcgacgacagacacaagatcgtgaacgtggaccagcggcagtacggcgacgtgttcaagggcgacctgaatcctaagcctcagggccagcgcctgatcgaggtgtccgtggaagagaatcaccccttcacactgagagcccctatccagagaatctacggcgtgcgctataccgagacatggtcctttctgcccagcctgacatgtaccggggatgccgctcctgccatccagcacatttgcctgaagcacaccacctgtttccaggacgtggtggtggatgtggactgcgccgagaacaccaaagaggatcagctggccgagatcagctaccggttccagggaaagaaagaggccgaccagccttggatcgtggtcaacaccagcacactgttcgacgagctggaactggaccctcctgagattgaacccggggtgctgaaggtgctgagaaccgagaagcagtacctgggagtgtacatctggaacatgagaggcagcgacggcacctctacctacgccacctttctggtcacatggaagggcgacgagaaaacacggaaccccacaccagctgtgacccctcaacctagaggcgccgagtttcacatgtggaattaccacagccacgtgttcagcgtgggcgatacctttagcctggccatgcatctgcagtacaagatccacgaggcccctttcgacctgctgctggaatggctgtacgtgcccatcgatcctacctgccagcctatgcggctgtactccacctgtctgtatcaccccaacgctccccagtgcctgagccacatgaatagcggctgcaccttcacaagccctcacctggctcagcgagtggccagcacagtgtaccagaattgcgagcacgccgacaattacaccgcctactgtctgggcatcagccacatggaacctagcttcggcctgatcctgcacgatggcggcacaaccctgaagttcgtggatacccctgagagcctgagcggcctgtatgtgttcgtggtgtacttcaacggccacgtggaagccgtggcctacaccgtggtgtctaccgtggaccacttcgtgaacgccatcgaggaaagaggcttccctccaactgctggacagcctcctgccaccaccaagcctaaagaaatcacacccgtgaatcccggcacaagcccactgcttagatacgccgcttggacaggcggactggctgctgttgttctgctgtgcctggtcatcttcctgatctgcaccgccaagcggatgagagtgaaagccgccagagtggacaagtga

SEQ ID NO: 15 - protein, 573 aa, synthetic construct
MGTVNKPVVGVLMGFGIITGTLRITNPVRASVLRYDDFHIDEDKLDTNSVYEPYYHSDHAESSWVNRGESSRKAYDHNSPYIWPRNDYDGFLENAHEHHGVYNQGRGIDSGERLMQPTQMSAQEDLGDDTGIHVIPTLNGDDRHKIVNVDQRQYGDVFKGDLNPKPQGQRLIEVSVEENHPFTLRAPIQRIYGVRYTETWSFLPSLTCTGDAAPAIQHICLKHTTCFQDVVVDVDCAENTKEDQLAEISYRFQGKKEADQPWIVVNTSTLFDELELDPPEIEPGVLKVLRTEKQYLGVYIWNMRGSDGTSTYATFLVTWKGDEKTRNPTPAVTPQPRGAEFHMWNYHSHVFSVGDTFSLAMHLQYKIHEAPFDLLLEWLYVPIDPTCQPMRLYSTCLYHPNAPQCLSHMNSGCTFTSPHLAQRVASTVYQNCEHADNYTAYCLGISHMEPSFGLILHDGGTTLKFVDTPESLSGLYVFVVYFNGHVEAVAYTVVSTVDHFVNAIEERGFPPTAGQPPATTKPKEITPVNPGTSPLLRYAAWTGGLAAVVLLCLVIFLICTAKRMRVKAARVDK

SEQ ID NO: 16 - RNA, 1988 nt, synthetic construct
  source 1..1988: mol_type = other RNA
agaaataagagagaaaagaagagtaagaagaaatataagagccaccatgggcaccgtgaacaagcctgttgtgggcgtgctgatgggcttcggcatcatcacaggcaccctgcggatcaccaatcctgtgcgggctagcgtgctgagatacgacgacttccacatcgacgaggacaagctggacaccaacagcgtgtacgagccctactaccacagcgatcacgccgagtctagctgggtcaacagaggcgagagcagcagaaaggcctacgaccacaacagcccctacatctggccccggaacgactacgatggcttcctggaaaatgcccacgagcaccacggcgtgtacaatcaaggcagaggcatcgacagcggcgagagactgatgcagcctacacagatgagcgcccaagaggacctgggagatgataccggcatccacgtgatccccacactgaacggcgacgacagacacaagatcgtgaacgtggaccagcggcagtacggcgacgtgttcaagggcgacctgaatcctaagcctcagggccagcgcctgatcgaggtgtccgtggaagagaatcaccccttcacactgagagcccctatccagagaatctacggcgtgcgctataccgagacatggtcctttctgcccagcctgacatgtaccggggatgccgctcctgccatccagcacatttgcctgaagcacaccacctgtttccaggacgtggtggtggatgtggactgcgccgagaacaccaaagaggatcagctggccgagatcagctaccggttccagggaaagaaagaggccgaccagccttggatcgtggtcaacaccagcacactgttcgacgagctggaactggaccctcctgagattgaacccggggtgctgaaggtgctgagaaccgagaagcagtacctgggagtgtacatctggaacatgagaggcagcgacggcacctctacctacgccacctttctggtcacatggaagggcgacgagaaaacacggaaccccacaccagctgtgacccctcaacctagaggcgccgagtttcacatgtggaattaccacagccacgtgttcagcgtgggcgatacctttagcctggccatgcatctgcagtacaagatccacgaggcccctttcgacctgctgctggaatggctgtacgtgcccatcgatcctacctgccagcctatgcggctgtactccacctgtctgtatcaccccaacgctccccagtgcctgagccacatgaatagcggctgcaccttcacaagccctcacctggctcagcgagtggccagcacagtgtaccagaattgcgagcacgccgacaattacaccgcctactgtctgggcatcagccacatggaacctagcttcggcctgatcctgcacgatggcggcacaaccctgaagttcgtggatacccctgagagcctgagcggcctgtatgtgttcgtggtgtacttcaacggccacgtggaagccgtggcctacaccgtggtgtctaccgtggaccacttcgtgaacgccatcgaggaaagaggcttccctccaactgctggacagcctcctgccaccaccaagcctaaagaaatcacacccgtgaatcccggcacaagcccactgcttagatacgccgcttggacaggcggactggctgctgttgttctgctgtgcctggtcatcttcctgatctgcaccgccaagcggatgagagtgaaagccgccagagtggacaagtgagctggagcctcggtggccatgcttcttgccccttgggcctccccccagcccctcctccccttcctgcacccgtacccccgtggtctttgaataaagtctgagtgggcggcaaaaaaaaaaaaaaaaaaaaaaaaaaaaaaaaaaaaaaaaaaaaaaaaaaaaaaaaaaaaaaaaaaaaaaaaaaaaaaaaaaaaaaaaaaaaaaaaaaaaaaaaaaaaaa

SEQ ID NO: 17 - DNA, 2161 bp, synthetic construct
  source 1..2161: mol_type = other DNA
agactcctccccatcctctccctctgtccctctgtccctctgaccctgcactgtcccagcaccgccaccatgggcaccgtgaacaagcctgttgtgggcgtgctgatgggcttcggcatcatcacaggcaccctgcggatcaccaatcctgtgcgggctagcgtgctgagatacgacgacttccacatcgacgaggacaagctggacaccaacagcgtgtacgagccctactaccacagcgatcacgccgagtctagctgggtcaacagaggcgagagcagcagaaaggcctacgaccacaacagcccctacatctggccccggaacgactacgatggcttcctggaaaatgcccacgagcaccacggcgtgtacaatcaaggcagaggcatcgacagcggcgagagactgatgcagcctacacagatgagcgcccaagaggacctgggagatgataccggcatccacgtgatccccacactgaacggcgacgacagacacaagatcgtgaacgtggaccagcggcagtacggcgacgtgttcaagggcgacctgaatcctaagcctcagggccagcgcctgatcgaggtgtccgtggaagagaatcaccccttcacactgagagcccctatccagagaatctacggcgtgcgctataccgagacatggtcctttctgcccagcctgacatgtaccggggatgccgctcctgccatccagcacatttgcctgaagcacaccacctgtttccaggacgtggtggtggatgtggactgcgccgagaacaccaaagaggatcagctggccgagatcagctaccggttccagggaaagaaagaggccgaccagccttggatcgtggtcaacaccagcacactgttcgacgagctggaactggaccctcctgagattgaacccggggtgctgaaggtgctgagaaccgagaagcagtacctgggagtgtacatctggaacatgagaggcagcgacggcacctctacctacgccacctttctggtcacatggaagggcgacgagaaaacacggaaccccacaccagctgtgacccctcaacctagaggcgccgagtttcacatgtggaattaccacagccacgtgttcagcgtgggcgatacctttagcctggccatgcatctgcagtacaagatccacgaggcccctttcgacctgctgctggaatggctgtacgtgcccatcgatcctacctgccagcctatgcggctgtactccacctgtctgtatcaccccaacgctccccagtgcctgagccacatgaatagcggctgcaccttcacaagccctcacctggctcagcgagtggccagcacagtgtaccagaattgcgagcacgccgacaattacaccgcctactgtctgggcatcagccacatggaacctagcttcggcctgatcctgcacgatggcggcacaaccctgaagttcgtggatacccctgagagcctgagcggcctgtatgtgttcgtggtgtacttcaacggccacgtggaagccgtggcctacaccgtggtgtctaccgtggaccacttcgtgaacgccatcgaggaaagaggcttccctccaactgctggacagcctcctgccaccaccaagcctaaagaaatcacacccgtgaatcccggcacaagcccactgcttagatacgccgcttggacaggcggactggctgctgttgttctgctgtgcctggtcatcttcctgatctgcaccgccaagcggatgagagtgaaggccgcgagagtggacaagagcccttacaaccagagcatgtactacgccggcctgcctgtggacgatttcgaggatgctgaagccgccgatgccgaggaagagtttggcaacgccattggcggatctcacggcggcagcagctataccgtgtacatcgacaagacccggtgagctggagcctcggtggccatgcttcttgccccttgggcctccccccagcccctcctccccttcctgcacccgtacccccgtggtctttgaataaagtctgagtgggcggcaaaaaaaaaaaaaaaaaaaaaaaaaaaaaaaaaaaaaaaaaaaaaaaaaaaaaaaaaaaaaaaaaaaaaaaaaaaaaaaaaaaaaaaaaaaaaaaaaaaaaaaaaaaaaa

SEQ ID NO: 18 - DNA, 1872 bp, synthetic construct
  source 1..1872: mol_type = other DNA
atgggcaccgtgaacaagcctgttgtgggcgtgctgatgggcttcggcatcatcacaggcaccctgcggatcaccaatcctgtgcgggctagcgtgctgagatacgacgacttccacatcgacgaggacaagctggacaccaacagcgtgtacgagccctactaccacagcgatcacgccgagtctagctgggtcaacagaggcgagagcagcagaaaggcctacgaccacaacagcccctacatctggccccggaacgactacgatggcttcctggaaaatgcccacgagcaccacggcgtgtacaatcaaggcagaggcatcgacagcggcgagagactgatgcagcctacacagatgagcgcccaagaggacctgggagatgataccggcatccacgtgatccccacactgaacggcgacgacagacacaagatcgtgaacgtggaccagcggcagtacggcgacgtgttcaagggcgacctgaatcctaagcctcagggccagcgcctgatcgaggtgtccgtggaagagaatcaccccttcacactgagagcccctatccagagaatctacggcgtgcgctataccgagacatggtcctttctgcccagcctgacatgtaccggggatgccgctcctgccatccagcacatttgcctgaagcacaccacctgtttccaggacgtggtggtggatgtggactgcgccgagaacaccaaagaggatcagctggccgagatcagctaccggttccagggaaagaaagaggccgaccagccttggatcgtggtcaacaccagcacactgttcgacgagctggaactggaccctcctgagattgaacccggggtgctgaaggtgctgagaaccgagaagcagtacctgggagtgtacatctggaacatgagaggcagcgacggcacctctacctacgccacctttctggtcacatggaagggcgacgagaaaacacggaaccccacaccagctgtgacccctcaacctagaggcgccgagtttcacatgtggaattaccacagccacgtgttcagcgtgggcgatacctttagcctggccatgcatctgcagtacaagatccacgaggcccctttcgacctgctgctggaatggctgtacgtgcccatcgatcctacctgccagcctatgcggctgtactccacctgtctgtatcaccccaacgctccccagtgcctgagccacatgaatagcggctgcaccttcacaagccctcacctggctcagcgagtggccagcacagtgtaccagaattgcgagcacgccgacaattacaccgcctactgtctgggcatcagccacatggaacctagcttcggcctgatcctgcacgatggcggcacaaccctgaagttcgtggatacccctgagagcctgagcggcctgtatgtgttcgtggtgtacttcaacggccacgtggaagccgtggcctacaccgtggtgtctaccgtggaccacttcgtgaacgccatcgaggaaagaggcttccctccaactgctggacagcctcctgccaccaccaagcctaaagaaatcacacccgtgaatcccggcacaagcccactgcttagatacgccgcttggacaggcggactggctgctgttgttctgctgtgcctggtcatcttcctgatctgcaccgccaagcggatgagagtgaaggccgcgagagtggacaagagcccttacaaccagagcatgtactacgccggcctgcctgtggacgatttcgaggatgctgaagccgccgatgccgaggaagagtttggcaacgccattggcggatctcacggcggcagcagctataccgtgtacatcgacaagacccggtga

SEQ ID NO: 19 - protein, 623 aa, synthetic construct
MGTVNKPVVGVLMGFGIITGTLRITNPVRASVLRYDDFHIDEDKLDTNSVYEPYYHSDHAESSWVNRGESSRKAYDHNSPYIWPRNDYDGFLENAHEHHGVYNQGRGIDSGERLMQPTQMSAQEDLGDDTGIHVIPTLNGDDRHKIVNVDQRQYGDVFKGDLNPKPQGQRLIEVSVEENHPFTLRAPIQRIYGVRYTETWSFLPSLTCTGDAAPAIQHICLKHTTCFQDVVVDVDCAENTKEDQLAEISYRFQGKKEADQPWIVVNTSTLFDELELDPPEIEPGVLKVLRTEKQYLGVYIWNMRGSDGTSTYATFLVTWKGDEKTRNPTPAVTPQPRGAEFHMWNYHSHVFSVGDTFSLAMHLQYKIHEAPFDLLLEWLYVPIDPTCQPMRLYSTCLYHPNAPQCLSHMNSGCTFTSPHLAQRVASTVYQNCEHADNYTAYCLGISHMEPSFGLILHDGGTTLKFVDTPESLSGLYVFVVYFNGHVEAVAYTVVSTVDHFVNAIEERGFPPTAGQPPATTKPKEITPVNPGTSPLLRYAAWTGGLAAVVLLCLVIFLICTAKRMRVKAARVDKSPYNQSMYYAGLPVDDFEDAEAADAEEEFGNAIGGSHGGSSYTVYIDKTR

SEQ ID NO: 20 - RNA, 2161 nt, synthetic construct
  source 1..2161: mol_type = other RNA
agactcctccccatcctctccctctgtccctctgtccctctgaccctgcactgtcccagcaccgccaccatgggcaccgtgaacaagcctgttgtgggcgtgctgatgggcttcggcatcatcacaggcaccctgcggatcaccaatcctgtgcgggctagcgtgctgagatacgacgacttccacatcgacgaggacaagctggacaccaacagcgtgtacgagccctactaccacagcgatcacgccgagtctagctgggtcaacagaggcgagagcagcagaaaggcctacgaccacaacagcccctacatctggccccggaacgactacgatggcttcctggaaaatgcccacgagcaccacggcgtgtacaatcaaggcagaggcatcgacagcggcgagagactgatgcagcctacacagatgagcgcccaagaggacctgggagatgataccggcatccacgtgatccccacactgaacggcgacgacagacacaagatcgtgaacgtggaccagcggcagtacggcgacgtgttcaagggcgacctgaatcctaagcctcagggccagcgcctgatcgaggtgtccgtggaagagaatcaccccttcacactgagagcccctatccagagaatctacggcgtgcgctataccgagacatggtcctttctgcccagcctgacatgtaccggggatgccgctcctgccatccagcacatttgcctgaagcacaccacctgtttccaggacgtggtggtggatgtggactgcgccgagaacaccaaagaggatcagctggccgagatcagctaccggttccagggaaagaaagaggccgaccagccttggatcgtggtcaacaccagcacactgttcgacgagctggaactggaccctcctgagattgaacccggggtgctgaaggtgctgagaaccgagaagcagtacctgggagtgtacatctggaacatgagaggcagcgacggcacctctacctacgccacctttctggtcacatggaagggcgacgagaaaacacggaaccccacaccagctgtgacccctcaacctagaggcgccgagtttcacatgtggaattaccacagccacgtgttcagcgtgggcgatacctttagcctggccatgcatctgcagtacaagatccacgaggcccctttcgacctgctgctggaatggctgtacgtgcccatcgatcctacctgccagcctatgcggctgtactccacctgtctgtatcaccccaacgctccccagtgcctgagccacatgaatagcggctgcaccttcacaagccctcacctggctcagcgagtggccagcacagtgtaccagaattgcgagcacgccgacaattacaccgcctactgtctgggcatcagccacatggaacctagcttcggcctgatcctgcacgatggcggcacaaccctgaagttcgtggatacccctgagagcctgagcggcctgtatgtgttcgtggtgtacttcaacggccacgtggaagccgtggcctacaccgtggtgtctaccgtggaccacttcgtgaacgccatcgaggaaagaggcttccctccaactgctggacagcctcctgccaccaccaagcctaaagaaatcacacccgtgaatcccggcacaagcccactgcttagatacgccgcttggacaggcggactggctgctgttgttctgctgtgcctggtcatcttcctgatctgcaccgccaagcggatgagagtgaaggccgctagagtggacaagagcccttacaaccagagcatgtactacgccggcctgcctgtggacgatttcgaggatgctgaagccgccgatgccgaggaagagtttggcaacgccattggcggatctcacggcggcagcagctataccgtgtacatcgacaagacccggtgagctggagcctcggtggccatgcttcttgccccttgggcctccccccagcccctcctccccttcctgcacccgtacccccgtggtctttgaataaagtctgagtgggcggcaaaaaaaaaaaaaaaaaaaaaaaaaaaaaaaaaaaaaaaaaaaaaaaaaaaaaaaaaaaaaaaaaaaaaaaaaaaaaaaaaaaaaaaaaaaaaaaaaaaaaaaaaaaaaa

SEQ ID NO: 21 - DNA, 2161 bp, synthetic construct
  source 1..2161: mol_type = other DNA
agactcctccccatcctctccctctgtccctctgtccctctgaccctgcactgtcccagcaccgccaccatgggcaccgtgaacaagcctgttgtgggcgtgctgatgggcttcggcatcatcacaggcaccctgcggatcaccaatcctgtgcgggctagcgtgctgagatacgacgacttccacatcgacgaggacaagctggacaccaacagcgtgtacgagccctactaccacagcgatcacgccgagtctagctgggtcaacagaggcgagagcagcagaaaggcctacgaccacaacagcccctacatctggccccggaacgactacgatggcttcctggaaaatgcccacgagcaccacggcgtgtacaatcaaggcagaggcatcgacagcggcgagagactgatgcagcctacacagatgagcgcccaagaggacctgggagatgataccggcatccacgtgatccccacactgaacggcgacgacagacacaagatcgtgaacgtggaccagcggcagtacggcgacgtgttcaagggcgacctgaatcctaagcctcagggccagcgcctgatcgaggtgtccgtggaagagaatcaccccttcacactgagagcccctatccagagaatctacggcgtgcgctataccgagacatggtcctttctgcccagcctgacatgtaccggggatgccgctcctgccatccagcacatttgcctgaagcacaccacctgtttccaggacgtggtggtggatgtggactgcgccgagaacaccaaagaggatcagctggccgagatcagctaccggttccagggaaagaaagaggccgaccagccttggatcgtggtcaacaccagcacactgttcgacgagctggaactggaccctcctgagattgaacccggggtgctgaaggtgctgagaaccgagaagcagtacctgggagtgtacatctggaacatgagaggcagcgacggcacctctacctacgccacctttctggtcacatggaagggcgacgagaaaacacggaaccccacaccagctgtgacccctcaacctagaggcgccgagtttcacatgtggaattaccacagccacgtgttcagcgtgggcgatacctttagcctggccatgcatctgcagtacaagatccacgaggcccctttcgacctgctgctggaatggctgtacgtgcccatcgatcctacctgccagcctatgcggctgtactccacctgtctgtatcaccccaacgctccccagtgcctgagccacatgaatagcggctgcaccttcacaagccctcacctggctcagcgagtggccagcacagtgtaccagaattgcgagcacgccgacaattacaccgcctactgtctgggcatcagccacatggaacctagcttcggcctgatcctgcacgatggcggcacaaccctgaagttcgtggatacccctgagagcctgagcggcctgtatgtgttcgtggtgtacttcaacggccacgtggaagccgtggcctacaccgtggtgtctaccgtggaccacttcgtgaacgccatcgaggaaagaggcttccctccaactgctggacagcctcctgccaccaccaagcctaaagaaatcacacccgtgaatcccggcacaagcccactgcttagatacgccgcttggacaggcggactggctgctgttgttctgctgtgcctggtcatcttcctgatctgcaccgccaagcggatgagagtgaaggcctacagagtggacaagagcccttacaaccagtctatgtatgccgccggactgcccgtggacgattttgaggatgctgaagccgccgacgccgaggaagaatttggcaacgccattggcggaagccacggcggcagtagctataccgtgtacatcgacaagacccggtgagctggagcctcggtggccatgcttcttgccccttgggcctccccccagcccctcctccccttcctgcacccgtacccccgtggtctttgaataaagtctgagtgggcggcaaaaaaaaaaaaaaaaaaaaaaaaaaaaaaaaaaaaaaaaaaaaaaaaaaaaaaaaaaaaaaaaaaaaaaaaaaaaaaaaaaaaaaaaaaaaaaaaaaaaaaaaaaaaaa

SEQ ID NO: 22 - DNA, 1872 bp, synthetic construct
  source 1..1872: mol_type = other DNA
atgggcaccgtgaacaagcctgttgtgggcgtgctgatgggcttcggcatcatcacaggcaccctgcggatcaccaatcctgtgcgggctagcgtgctgagatacgacgacttccacatcgacgaggacaagctggacaccaacagcgtgtacgagccctactaccacagcgatcacgccgagtctagctgggtcaacagaggcgagagcagcagaaaggcctacgaccacaacagcccctacatctggccccggaacgactacgatggcttcctggaaaatgcccacgagcaccacggcgtgtacaatcaaggcagaggcatcgacagcggcgagagactgatgcagcctacacagatgagcgcccaagaggacctgggagatgataccggcatccacgtgatccccacactgaacggcgacgacagacacaagatcgtgaacgtggaccagcggcagtacggcgacgtgttcaagggcgacctgaatcctaagcctcagggccagcgcctgatcgaggtgtccgtggaagagaatcaccccttcacactgagagcccctatccagagaatctacggcgtgcgctataccgagacatggtcctttctgcccagcctgacatgtaccggggatgccgctcctgccatccagcacatttgcctgaagcacaccacctgtttccaggacgtggtggtggatgtggactgcgccgagaacaccaaagaggatcagctggccgagatcagctaccggttccagggaaagaaagaggccgaccagccttggatcgtggtcaacaccagcacactgttcgacgagctggaactggaccctcctgagattgaacccggggtgctgaaggtgctgagaaccgagaagcagtacctgggagtgtacatctggaacatgagaggcagcgacggcacctctacctacgccacctttctggtcacatggaagggcgacgagaaaacacggaaccccacaccagctgtgacccctcaacctagaggcgccgagtttcacatgtggaattaccacagccacgtgttcagcgtgggcgatacctttagcctggccatgcatctgcagtacaagatccacgaggcccctttcgacctgctgctggaatggctgtacgtgcccatcgatcctacctgccagcctatgcggctgtactccacctgtctgtatcaccccaacgctccccagtgcctgagccacatgaatagcggctgcaccttcacaagccctcacctggctcagcgagtggccagcacagtgtaccagaattgcgagcacgccgacaattacaccgcctactgtctgggcatcagccacatggaacctagcttcggcctgatcctgcacgatggcggcacaaccctgaagttcgtggatacccctgagagcctgagcggcctgtatgtgttcgtggtgtacttcaacggccacgtggaagccgtggcctacaccgtggtgtctaccgtggaccacttcgtgaacgccatcgaggaaagaggcttccctccaactgctggacagcctcctgccaccaccaagcctaaagaaatcacacccgtgaatcccggcacaagcccactgcttagatacgccgcttggacaggcggactggctgctgttgttctgctgtgcctggtcatcttcctgatctgcaccgccaagcggatgagagtgaaggcctacagagtggacaagagcccttacaaccagtctatgtatgccgccggactgcccgtggacgattttgaggatgctgaagccgccgacgccgaggaagaatttggcaacgccattggcggaagccacggcggcagtagctataccgtgtacatcgacaagacccggtga

SEQ ID NO: 23 - protein, 623 aa, synthetic construct
MGTVNKPVVGVLMGFGIITGTLRITNPVRASVLRYDDFHIDEDKLDTNSVYEPYYHSDHAESSWVNRGESSRKAYDHNSPYIWPRNDYDGFLENAHEHHGVYNQGRGIDSGERLMQPTQMSAQEDLGDDTGIHVIPTLNGDDRHKIVNVDQRQYGDVFKGDLNPKPQGQRLIEVSVEENHPFTLRAPIQRIYGVRYTETWSFLPSLTCTGDAAPAIQHICLKHTTCFQDVVVDVDCAENTKEDQLAEISYRFQGKKEADQPWIVVNTSTLFDELELDPPEIEPGVLKVLRTEKQYLGVYIWNMRGSDGTSTYATFLVTWKGDEKTRNPTPAVTPQPRGAEFHMWNYHSHVFSVGDTFSLAMHLQYKIHEAPFDLLLEWLYVPIDPTCQPMRLYSTCLYHPNAPQCLSHMNSGCTFTSPHLAQRVASTVYQNCEHADNYTAYCLGISHMEPSFGLILHDGGTTLKFVDTPESLSGLYVFVVYFNGHVEAVAYTVVSTVDHFVNAIEERGFPPTAGQPPATTKPKEITPVNPGTSPLLRYAAWTGGLAAVVLLCLVIFLICTAKRMRVKAYRVDKSPYNQSMYAAGLPVDDFEDAEAADAEEEFGNAIGGSHGGSSYTVYIDKTR

SEQ ID NO: 24 - RNA, 2161 nt, synthetic construct
  source 1..2161: mol_type = other RNA
agactcctccccatcctctccctctgtccctctgtccctctgaccctgcactgtcccagcaccgccaccatgggcaccgtgaacaagcctgttgtgggcgtgctgatgggcttcggcatcatcacaggcaccctgcggatcaccaatcctgtgcgggctagcgtgctgagatacgacgacttccacatcgacgaggacaagctggacaccaacagcgtgtacgagccctactaccacagcgatcacgccgagtctagctgggtcaacagaggcgagagcagcagaaaggcctacgaccacaacagcccctacatctggccccggaacgactacgatggcttcctggaaaatgcccacgagcaccacggcgtgtacaatcaaggcagaggcatcgacagcggcgagagactgatgcagcctacacagatgagcgcccaagaggacctgggagatgataccggcatccacgtgatccccacactgaacggcgacgacagacacaagatcgtgaacgtggaccagcggcagtacggcgacgtgttcaagggcgacctgaatcctaagcctcagggccagcgcctgatcgaggtgtccgtggaagagaatcaccccttcacactgagagcccctatccagagaatctacggcgtgcgctataccgagacatggtcctttctgcccagcctgacatgtaccggggatgccgctcctgccatccagcacatttgcctgaagcacaccacctgtttccaggacgtggtggtggatgtggactgcgccgagaacaccaaagaggatcagctggccgagatcagctaccggttccagggaaagaaagaggccgaccagccttggatcgtggtcaacaccagcacactgttcgacgagctggaactggaccctcctgagattgaacccggggtgctgaaggtgctgagaaccgagaagcagtacctgggagtgtacatctggaacatgagaggcagcgacggcacctctacctacgccacctttctggtcacatggaagggcgacgagaaaacacggaaccccacaccagctgtgacccctcaacctagaggcgccgagtttcacatgtggaattaccacagccacgtgttcagcgtgggcgatacctttagcctggccatgcatctgcagtacaagatccacgaggcccctttcgacctgctgctggaatggctgtacgtgcccatcgatcctacctgccagcctatgcggctgtactccacctgtctgtatcaccccaacgctccccagtgcctgagccacatgaatagcggctgcaccttcacaagccctcacctggctcagcgagtggccagcacagtgtaccagaattgcgagcacgccgacaattacaccgcctactgtctgggcatcagccacatggaacctagcttcggcctgatcctgcacgatggcggcacaaccctgaagttcgtggatacccctgagagcctgagcggcctgtatgtgttcgtggtgtacttcaacggccacgtggaagccgtggcctacaccgtggtgtctaccgtggaccacttcgtgaacgccatcgaggaaagaggcttccctccaactgctggacagcctcctgccaccaccaagcctaaagaaatcacacccgtgaatcccggcacaagcccactgcttagatacgccgcttggacaggcggactggctgctgttgttctgctgtgcctggtcatcttcctgatctgcaccgccaagcggatgagagtgaaggcctacagagtggacaagagcccttacaaccagtctatgtatgccgccggactgcccgtggacgattttgaggatgctgaagccgccgacgccgaggaagaatttggcaacgccattggcggaagccacggcggcagtagctataccgtgtacatcgacaagacccggtgagctggagcctcggtggccatgcttcttgccccttgggcctccccccagcccctcctccccttcctgcacccgtacccccgtggtctttgaataaagtctgagtgggcggcaaaaaaaaaaaaaaaaaaaaaaaaaaaaaaaaaaaaaaaaaaaaaaaaaaaaaaaaaaaaaaaaaaaaaaaaaaaaaaaaaaaaaaaaaaaaaaaaaaaaaaaaaaaaaa

SEQ ID NO: 25 - DNA, 2101 bp, synthetic construct
  source 1..2101: mol_type = other DNA
accgccaccatgggcaccgtgaacaagcctgttgtgggcgtgctgatgggcttcggcatcatcacaggcaccctgcggatcaccaatcctgtgcgggctagcgtgctgagatacgacgacttccacatcgacgaggacaagctggacaccaacagcgtgtacgagccctactaccacagcgatcacgccgagtctagctgggtcaacagaggcgagagcagcagaaaggcctacgaccacaacagcccctacatctggccccggaacgactacgatggcttcctggaaaatgcccacgagcaccacggcgtgtacaatcaaggcagaggcatcgacagcggcgagagactgatgcagcctacacagatgagcgcccaagaggacctgggagatgataccggcatccacgtgatccccacactgaacggcgacgacagacacaagatcgtgaacgtggaccagcggcagtacggcgacgtgttcaagggcgacctgaatcctaagcctcagggccagcgcctgatcgaggtgtccgtggaagagaatcaccccttcacactgagagcccctatccagagaatctacggcgtgcgctataccgagacatggtcctttctgcccagcctgacatgtaccggggatgccgctcctgccatccagcacatttgcctgaagcacaccacctgtttccaggacgtggtggtggatgtggactgcgccgagaacaccaaagaggatcagctggccgagatcagctaccggttccagggaaagaaagaggccgaccagccttggatcgtggtcaacaccagcacactgttcgacgagctggaactggaccctcctgagattgaacccggggtgctgaaggtgctgagaaccgagaagcagtacctgggagtgtacatctggaacatgagaggcagcgacggcacctctacctacgccacctttctggtcacatggaagggcgacgagaaaacacggaaccccacaccagctgtgacccctcaacctagaggcgccgagtttcacatgtggaattaccacagccacgtgttcagcgtgggcgatacctttagcctggccatgcatctgcagtacaagatccacgaggcccctttcgacctgctgctggaatggctgtacgtgcccatcgatcctacctgccagcctatgcggctgtactccacctgtctgtatcaccccaacgctccccagtgcctgagccacatgaatagcggctgcaccttcacaagccctcacctggctcagcgagtggccagcacagtgtaccagaattgcgagcacgccgacaattacaccgcctactgtctgggcatcagccacatggaacctagcttcggcctgatcctgcacgatggcggcacaaccctgaagttcgtggatacccctgagagcctgagcggcctgtatgtgttcgtggtgtacttcaacggccacgtggaagccgtggcctacaccgtggtgtctaccgtggaccacttcgtgaacgccatcgaggaaagaggcttccctccaactgctggacagcctcctgccaccaccaagcctaaagaaatcacacccgtgaatcccggcacaagcccactgcttagatacgccgcttggacaggcggactggctgctgttgttctgctgtgcctggtcatcttcctgatctgcaccgccaagcggatgagagtgaaggccaagagagtggacaagagcccttacaaccagtctatgtatgccgccggactgcccgtggacgatttcgaggatagcgagagcaccgacaccgaggaagagttcggcaacgccattggaggatctcacggcggcagcagctataccgtgtacatcgacaagacccggtgagctggagcctcggtggccatgcttcttgccccttgggcctccccccagcccctcctccccttcctgcacccgtacccccgtggtctttgaataaagtctgagtgggcggcaaaaaaaaaaaaaaaaaaaaaaaaaaaaaaaaaaaaaaaaaaaaaaaaaaaaaaaaaaaaaaaaaaaaaaaaaaaaaaaaaaaaaaaaaaaaaaaaaaaaaaaaaaaaaa

SEQ ID NO: 26 - DNA, 1872 bp, synthetic construct
  source 1..1872: mol_type = other DNA
atgggcaccgtgaacaagcctgttgtgggcgtgctgatgggcttcggcatcatcacaggcaccctgcggatcaccaatcctgtgcgggctagcgtgctgagatacgacgacttccacatcgacgaggacaagctggacaccaacagcgtgtacgagccctactaccacagcgatcacgccgagtctagctgggtcaacagaggcgagagcagcagaaaggcctacgaccacaacagcccctacatctggccccggaacgactacgatggcttcctggaaaatgcccacgagcaccacggcgtgtacaatcaaggcagaggcatcgacagcggcgagagactgatgcagcctacacagatgagcgcccaagaggacctgggagatgataccggcatccacgtgatccccacactgaacggcgacgacagacacaagatcgtgaacgtggaccagcggcagtacggcgacgtgttcaagggcgacctgaatcctaagcctcagggccagcgcctgatcgaggtgtccgtggaagagaatcaccccttcacactgagagcccctatccagagaatctacggcgtgcgctataccgagacatggtcctttctgcccagcctgacatgtaccggggatgccgctcctgccatccagcacatttgcctgaagcacaccacctgtttccaggacgtggtggtggatgtggactgcgccgagaacaccaaagaggatcagctggccgagatcagctaccggttccagggaaagaaagaggccgaccagccttggatcgtggtcaacaccagcacactgttcgacgagctggaactggaccctcctgagattgaacccggggtgctgaaggtgctgagaaccgagaagcagtacctgggagtgtacatctggaacatgagaggcagcgacggcacctctacctacgccacctttctggtcacatggaagggcgacgagaaaacacggaaccccacaccagctgtgacccctcaacctagaggcgccgagtttcacatgtggaattaccacagccacgtgttcagcgtgggcgatacctttagcctggccatgcatctgcagtacaagatccacgaggcccctttcgacctgctgctggaatggctgtacgtgcccatcgatcctacctgccagcctatgcggctgtactccacctgtctgtatcaccccaacgctccccagtgcctgagccacatgaatagcggctgcaccttcacaagccctcacctggctcagcgagtggccagcacagtgtaccagaattgcgagcacgccgacaattacaccgcctactgtctgggcatcagccacatggaacctagcttcggcctgatcctgcacgatggcggcacaaccctgaagttcgtggatacccctgagagcctgagcggcctgtatgtgttcgtggtgtacttcaacggccacgtggaagccgtggcctacaccgtggtgtctaccgtggaccacttcgtgaacgccatcgaggaaagaggcttccctccaactgctggacagcctcctgccaccaccaagcctaaagaaatcacacccgtgaatcccggcacaagcccactgcttagatacgccgcttggacaggcggactggctgctgttgttctgctgtgcctggtcatcttcctgatctgcaccgccaagcggatgagagtgaaggccaagagagtggacaagagcccttacaaccagtctatgtatgccgccggactgcccgtggacgatttcgaggatagcgagagcaccgacaccgaggaagagttcggcaacgccattggaggatctcacggcggcagcagctataccgtgtacatcgacaagacccggtga

SEQ ID NO: 27 - protein, 623 aa, synthetic construct
MGTVNKPVVGVLMGFGIITGTLRITNPVRASVLRYDDFHIDEDKLDTNSVYEPYYHSDHAESSWVNRGESSRKAYDHNSPYIWPRNDYDGFLENAHEHHGVYNQGRGIDSGERLMQPTQMSAQEDLGDDTGIHVIPTLNGDDRHKIVNVDQRQYGDVFKGDLNPKPQGQRLIEVSVEENHPFTLRAPIQRIYGVRYTETWSFLPSLTCTGDAAPAIQHICLKHTTCFQDVVVDVDCAENTKEDQLAEISYRFQGKKEADQPWIVVNTSTLFDELELDPPEIEPGVLKVLRTEKQYLGVYIWNMRGSDGTSTYATFLVTWKGDEKTRNPTPAVTPQPRGAEFHMWNYHSHVFSVGDTFSLAMHLQYKIHEAPFDLLLEWLYVPIDPTCQPMRLYSTCLYHPNAPQCLSHMNSGCTFTSPHLAQRVASTVYQNCEHADNYTAYCLGISHMEPSFGLILHDGGTTLKFVDTPESLSGLYVFVVYFNGHVEAVAYTVVSTVDHFVNAIEERGFPPTAGQPPATTKPKEITPVNPGTSPLLRYAAWTGGLAAVVLLCLVIFLICTAKRMRVKAKRVDKSPYNQSMYAAGLPVDDFEDSESTDTEEEFGNAIGGSHGGSSYTVYIDKTR

SEQ ID NO: 28 - RNA, 2161 nt, synthetic construct
  source 1..2161: mol_type = other RNA
agactcctccccatcctctccctctgtccctctgtccctctgaccctgcactgtcccagcaccgccaccatgggcaccgtgaacaagcctgttgtgggcgtgctgatgggcttcggcatcatcacaggcaccctgcggatcaccaatcctgtgcgggctagcgtgctgagatacgacgacttccacatcgacgaggacaagctggacaccaacagcgtgtacgagccctactaccacagcgatcacgccgagtctagctgggtcaacagaggcgagagcagcagaaaggcctacgaccacaacagcccctacatctggccccggaacgactacgatggcttcctggaaaatgcccacgagcaccacggcgtgtacaatcaaggcagaggcatcgacagcggcgagagactgatgcagcctacacagatgagcgcccaagaggacctgggagatgataccggcatccacgtgatccccacactgaacggcgacgacagacacaagatcgtgaacgtggaccagcggcagtacggcgacgtgttcaagggcgacctgaatcctaagcctcagggccagcgcctgatcgaggtgtccgtggaagagaatcaccccttcacactgagagcccctatccagagaatctacggcgtgcgctataccgagacatggtcctttctgcccagcctgacatgtaccggggatgccgctcctgccatccagcacatttgcctgaagcacaccacctgtttccaggacgtggtggtggatgtggactgcgccgagaacaccaaagaggatcagctggccgagatcagctaccggttccagggaaagaaagaggccgaccagccttggatcgtggtcaacaccagcacactgttcgacgagctggaactggaccctcctgagattgaacccggggtgctgaaggtgctgagaaccgagaagcagtacctgggagtgtacatctggaacatgagaggcagcgacggcacctctacctacgccacctttctggtcacatggaagggcgacgagaaaacacggaaccccacaccagctgtgacccctcaacctagaggcgccgagtttcacatgtggaattaccacagccacgtgttcagcgtgggcgatacctttagcctggccatgcatctgcagtacaagatccacgaggcccctttcgacctgctgctggaatggctgtacgtgcccatcgatcctacctgccagcctatgcggctgtactccacctgtctgtatcaccccaacgctccccagtgcctgagccacatgaatagcggctgcaccttcacaagccctcacctggctcagcgagtggccagcacagtgtaccagaattgcgagcacgccgacaattacaccgcctactgtctgggcatcagccacatggaacctagcttcggcctgatcctgcacgatggcggcacaaccctgaagttcgtggatacccctgagagcctgagcggcctgtatgtgttcgtggtgtacttcaacggccacgtggaagccgtggcctacaccgtggtgtctaccgtggaccacttcgtgaacgccatcgaggaaagaggcttccctccaactgctggacagcctcctgccaccaccaagcctaaagaaatcacacccgtgaatcccggcacaagcccactgcttagatacgccgcttggacaggcggactggctgctgttgttctgctgtgcctggtcatcttcctgatctgcaccgccaagcggatgagagtgaaggccaagagagtggacaagagcccttacaaccagtctatgtatgccgccggactgcccgtggacgatttcgaggatagcgagagcaccgacaccgaggaagagttcggcaacgccattggaggatctcacggcggcagcagctataccgtgtacatcgacaagacccggtgagctggagcctcggtggccatgcttcttgccccttgggcctccccccagcccctcctccccttcctgcacccgtacccccgtggtctttgaataaagtctgagtgggcggcaaaaaaaaaaaaaaaaaaaaaaaaaaaaaaaaaaaaaaaaaaaaaaaaaaaaaaaaaaaaaaaaaaaaaaaaaaaaaaaaaaaaaaaaaaaaaaaaaaaaaaaaaaaaaa

SEQ ID NO: 29 - DNA, 2161 bp, synthetic construct
  source 1..2161: mol_type = other DNA
agactcctccccatcctctccctctgtccctctgtccctctgaccctgcactgtcccagcaccgccaccatgggcaccgtgaacaagcctgttgtgggcgtgctgatgggcttcggcatcatcacaggcaccctgcggatcaccaatcctgtgcgggctagcgtgctgagatacgacgacttccacatcgacgaggacaagctggacaccaacagcgtgtacgagccctactaccacagcgatcacgccgagtctagctgggtcaacagaggcgagagcagcagaaaggcctacgaccacaacagcccctacatctggccccggaacgactacgatggcttcctggaaaatgcccacgagcaccacggcgtgtacaatcaaggcagaggcatcgacagcggcgagagactgatgcagcctacacagatgagcgcccaagaggacctgggagatgataccggcatccacgtgatccccacactgaacggcgacgacagacacaagatcgtgaacgtggaccagcggcagtacggcgacgtgttcaagggcgacctgaatcctaagcctcagggccagcgcctgatcgaggtgtccgtggaagagaatcaccccttcacactgagagcccctatccagagaatctacggcgtgcgctataccgagacatggtcctttctgcccagcctgacatgtaccggggatgccgctcctgccatccagcacatttgcctgaagcacaccacctgtttccaggacgtggtggtggatgtggactgcgccgagaacaccaaagaggatcagctggccgagatcagctaccggttccagggaaagaaagaggccgaccagccttggatcgtggtcaacaccagcacactgttcgacgagctggaactggaccctcctgagattgaacccggggtgctgaaggtgctgagaaccgagaagcagtacctgggagtgtacatctggaacatgagaggcagcgacggcacctctacctacgccacctttctggtcacatggaagggcgacgagaaaacacggaaccccacaccagctgtgacccctcaacctagaggcgccgagtttcacatgtggaattaccacagccacgtgttcagcgtgggcgatacctttagcctggccatgcatctgcagtacaagatccacgaggcccctttcgacctgctgctggaatggctgtacgtgcccatcgatcctacctgccagcctatgcggctgtactccacctgtctgtatcaccccaacgctccccagtgcctgagccacatgaatagcggctgcaccttcacaagccctcacctggctcagcgagtggccagcacagtgtaccagaattgcgagcacgccgacaattacaccgcctactgtctgggcatcagccacatggaacctagcttcggcctgatcctgcacgatggcggcacaaccctgaagttcgtggatacccctgagagcctgagcggcctgtatgtgttcgtggtgtacttcaacggccacgtggaagccgtggcctacaccgtggtgtctaccgtggaccacttcgtgaacgccatcgaggaaagaggcttccctccaactgctggacagcctcctgccaccaccaagcctaaagaaatcacacccgtgaatcccggcacaagcccactgcttagatacgccgcttggacaggcggactggctgctgttgttctgctgtgcctggtcatcttcctgatctgcaccgccaagcggatgagagtgaaggccaagagagtggacaagagcccttacaaccagtctatgtatgccgccggactgcccgtggacgattttgaggatgctgaagccgccgacgccgaggaagaatttggcaacgccattggcggaagccacggcggcagtagctataccgtgtacatcgacaagacccggtgagctggagcctcggtggccatgcttcttgccccttgggcctccccccagcccctcctccccttcctgcacccgtacccccgtggtctttgaataaagtctgagtgggcggcaaaaaaaaaaaaaaaaaaaaaaaaaaaaaaaaaaaaaaaaaaaaaaaaaaaaaaaaaaaaaaaaaaaaaaaaaaaaaaaaaaaaaaaaaaaaaaaaaaaaaaaaaaaaaa

SEQ ID NO: 30 - DNA, 1872 bp, synthetic construct
  source 1..1872: mol_type = other DNA
atgggcaccgtgaacaagcctgttgtgggcgtgctgatgggcttcggcatcatcacaggcaccctgcggatcaccaatcctgtgcgggctagcgtgctgagatacgacgacttccacatcgacgaggacaagctggacaccaacagcgtgtacgagccctactaccacagcgatcacgccgagtctagctgggtcaacagaggcgagagcagcagaaaggcctacgaccacaacagcccctacatctggccccggaacgactacgatggcttcctggaaaatgcccacgagcaccacggcgtgtacaatcaaggcagaggcatcgacagcggcgagagactgatgcagcctacacagatgagcgcccaagaggacctgggagatgataccggcatccacgtgatccccacactgaacggcgacgacagacacaagatcgtgaacgtggaccagcggcagtacggcgacgtgttcaagggcgacctgaatcctaagcctcagggccagcgcctgatcgaggtgtccgtggaagagaatcaccccttcacactgagagcccctatccagagaatctacggcgtgcgctataccgagacatggtcctttctgcccagcctgacatgtaccggggatgccgctcctgccatccagcacatttgcctgaagcacaccacctgtttccaggacgtggtggtggatgtggactgcgccgagaacaccaaagaggatcagctggccgagatcagctaccggttccagggaaagaaagaggccgaccagccttggatcgtggtcaacaccagcacactgttcgacgagctggaactggaccctcctgagattgaacccggggtgctgaaggtgctgagaaccgagaagcagtacctgggagtgtacatctggaacatgagaggcagcgacggcacctctacctacgccacctttctggtcacatggaagggcgacgagaaaacacggaaccccacaccagctgtgacccctcaacctagaggcgccgagtttcacatgtggaattaccacagccacgtgttcagcgtgggcgatacctttagcctggccatgcatctgcagtacaagatccacgaggcccctttcgacctgctgctggaatggctgtacgtgcccatcgatcctacctgccagcctatgcggctgtactccacctgtctgtatcaccccaacgctccccagtgcctgagccacatgaatagcggctgcaccttcacaagccctcacctggctcagcgagtggccagcacagtgtaccagaattgcgagcacgccgacaattacaccgcctactgtctgggcatcagccacatggaacctagcttcggcctgatcctgcacgatggcggcacaaccctgaagttcgtggatacccctgagagcctgagcggcctgtatgtgttcgtggtgtacttcaacggccacgtggaagccgtggcctacaccgtggtgtctaccgtggaccacttcgtgaacgccatcgaggaaagaggcttccctccaactgctggacagcctcctgccaccaccaagcctaaagaaatcacacccgtgaatcccggcacaagcccactgcttagatacgccgcttggacaggcggactggctgctgttgttctgctgtgcctggtcatcttcctgatctgcaccgccaagcggatgagagtgaaggccaagagagtggacaagagcccttacaaccagtctatgtatgccgccggactgcccgtggacgattttgaggatgctgaagccgccgacgccgaggaagaatttggcaacgccattggcggaagccacggcggcagtagctataccgtgtacatcgacaagacccggtga

SEQ ID NO: 31 - protein, 623 aa, synthetic construct
MGTVNKPVVGVLMGFGIITGTLRITNPVRASVLRYDDFHIDEDKLDTNSVYEPYYHSDHAESSWVNRGESSRKAYDHNSPYIWPRNDYDGFLENAHEHHGVYNQGRGIDSGERLMQPTQMSAQEDLGDDTGIHVIPTLNGDDRHKIVNVDQRQYGDVFKGDLNPKPQGQRLIEVSVEENHPFTLRAPIQRIYGVRYTETWSFLPSLTCTGDAAPAIQHICLKHTTCFQDVVVDVDCAENTKEDQLAEISYRFQGKKEADQPWIVVNTSTLFDELELDPPEIEPGVLKVLRTEKQYLGVYIWNMRGSDGTSTYATFLVTWKGDEKTRNPTPAVTPQPRGAEFHMWNYHSHVFSVGDTFSLAMHLQYKIHEAPFDLLLEWLYVPIDPTCQPMRLYSTCLYHPNAPQCLSHMNSGCTFTSPHLAQRVASTVYQNCEHADNYTAYCLGISHMEPSFGLILHDGGTTLKFVDTPESLSGLYVFVVYFNGHVEAVAYTVVSTVDHFVNAIEERGFPPTAGQPPATTKPKEITPVNPGTSPLLRYAAWTGGLAAVVLLCLVIFLICTAKRMRVKAKRVDKSPYNQSMYAAGLPVDDFEDAEAADAEEEFGNAIGGSHGGSSYTVYIDKTR

SEQ ID NO: 32 - RNA, 2161 nt, synthetic construct
  source 1..2161: mol_type = other RNA
agactcctccccatcctctccctctgtccctctgtccctctgaccctgcactgtcccagcaccgccaccatgggcaccgtgaacaagcctgttgtgggcgtgctgatgggcttcggcatcatcacaggcaccctgcggatcaccaatcctgtgcgggctagcgtgctgagatacgacgacttccacatcgacgaggacaagctggacaccaacagcgtgtacgagccctactaccacagcgatcacgccgagtctagctgggtcaacagaggcgagagcagcagaaaggcctacgaccacaacagcccctacatctggccccggaacgactacgatggcttcctggaaaatgcccacgagcaccacggcgtgtacaatcaaggcagaggcatcgacagcggcgagagactgatgcagcctacacagatgagcgcccaagaggacctgggagatgataccggcatccacgtgatccccacactgaacggcgacgacagacacaagatcgtgaacgtggaccagcggcagtacggcgacgtgttcaagggcgacctgaatcctaagcctcagggccagcgcctgatcgaggtgtccgtggaagagaatcaccccttcacactgagagcccctatccagagaatctacggcgtgcgctataccgagacatggtcctttctgcccagcctgacatgtaccggggatgccgctcctgccatccagcacatttgcctgaagcacaccacctgtttccaggacgtggtggtggatgtggactgcgccgagaacaccaaagaggatcagctggccgagatcagctaccggttccagggaaagaaagaggccgaccagccttggatcgtggtcaacaccagcacactgttcgacgagctggaactggaccctcctgagattgaacccggggtgctgaaggtgctgagaaccgagaagcagtacctgggagtgtacatctggaacatgagaggcagcgacggcacctctacctacgccacctttctggtcacatggaagggcgacgagaaaacacggaaccccacaccagctgtgacccctcaacctagaggcgccgagtttcacatgtggaattaccacagccacgtgttcagcgtgggcgatacctttagcctggccatgcatctgcagtacaagatccacgaggcccctttcgacctgctgctggaatggctgtacgtgcccatcgatcctacctgccagcctatgcggctgtactccacctgtctgtatcaccccaacgctccccagtgcctgagccacatgaatagcggctgcaccttcacaagccctcacctggctcagcgagtggccagcacagtgtaccagaattgcgagcacgccgacaattacaccgcctactgtctgggcatcagccacatggaacctagcttcggcctgatcctgcacgatggcggcacaaccctgaagttcgtggatacccctgagagcctgagcggcctgtatgtgttcgtggtgtacttcaacggccacgtggaagccgtggcctacaccgtggtgtctaccgtggaccacttcgtgaacgccatcgaggaaagaggcttccctccaactgctggacagcctcctgccaccaccaagcctaaagaaatcacacccgtgaatcccggcacaagcccactgcttagatacgccgcttggacaggcggactggctgctgttgttctgctgtgcctggtcatcttcctgatctgcaccgccaagcggatgagagtgaaggccaagagagtggacaagagcccttacaaccagtctatgtatgccgccggactgcccgtggacgattttgaggatgctgaagccgccgacgccgaggaagaatttggcaacgccattggcggaagccacggcggcagtagctataccgtgtacatcgacaagacccggtgagctggagcctcggtggccatgcttcttgccccttgggcctccccccagcccctcctccccttcctgcacccgtacccccgtggtctttgaataaagtctgagtgggcggcaaaaaaaaaaaaaaaaaaaaaaaaaaaaaaaaaaaaaaaaaaaaaaaaaaaaaaaaaaaaaaaaaaaaaaaaaaaaaaaaaaaaaaaaaaaaaaaaaaaaaaaaaaaaaa

SEQ ID NO: 33 - DNA, 2161 bp, synthetic construct
  source 1..2161: mol_type = other DNA
agactcctccccatcctctccctctgtccctctgtccctctgaccctgcactgtcccagcaccgccaccatgggcaccgtgaacaagcctgttgtgggcgtgctgatgggcttcggcatcatcacaggcaccctgcggatcaccaatcctgtgcgggctagcgtgctgagatacgacgacttccacatcgacgaggacaagctggacaccaacagcgtgtacgagccctactaccacagcgatcacgccgagtctagctgggtcaacagaggcgagagcagcagaaaggcctacgaccacaacagcccctacatctggccccggaacgactacgatggcttcctggaaaatgcccacgagcaccacggcgtgtacaatcaaggcagaggcatcgacagcggcgagagactgatgcagcctacacagatgagcgcccaagaggacctgggagatgataccggcatccacgtgatccccacactgaacggcgacgacagacacaagatcgtgaacgtggaccagcggcagtacggcgacgtgttcaagggcgacctgaatcctaagcctcagggccagcgcctgatcgaggtgtccgtggaagagaatcaccccttcacactgagagcccctatccagagaatctacggcgtgcgctataccgagacatggtcctttctgcccagcctgacatgtaccggggatgccgctcctgccatccagcacatttgcctgaagcacaccacctgtttccaggacgtggtggtggatgtggactgcgccgagaacaccaaagaggatcagctggccgagatcagctaccggttccagggaaagaaagaggccgaccagccttggatcgtggtcaacaccagcacactgttcgacgagctggaactggaccctcctgagattgaacccggggtgctgaaggtgctgagaaccgagaagcagtacctgggagtgtacatctggaacatgagaggcagcgacggcacctctacctacgccacctttctggtcacatggaagggcgacgagaaaacacggaaccccacaccagctgtgacccctcaacctagaggcgccgagtttcacatgtggaattaccacagccacgtgttcagcgtgggcgatacctttagcctggccatgcatctgcagtacaagatccacgaggcccctttcgacctgctgctggaatggctgtacgtgcccatcgatcctacctgccagcctatgcggctgtactccacctgtctgtatcaccccaacgctccccagtgcctgagccacatgaatagcggctgcaccttcacaagccctcacctggctcagcgagtggccagcacagtgtaccagaattgcgagcacgccgacaattacaccgcctactgtctgggcatcagccacatggaacctagcttcggcctgatcctgcacgatggcggcacaaccctgaagttcgtggatacccctgagagcctgagcggcctgtatgtgttcgtggtgtacttcaacggccacgtggaagccgtggcctacaccgtggtgtctaccgtggaccacttcgtgaacgccatcgaggaaagaggcttccctccaactgctggacagcctcctgccaccaccaagcctaaagaaatcacacccgtgaatcccggcacaagcccactgcttagatacgccgcttggacaggcggactggctgctgttgttctgctgtgcctggtcatcttcctgatctgcaccgccaagcggatgcgcgtgaaggacaaagagaaggacaagtccccttacaaccagagcatgtactacgccggcctgcctgtggacgacttcgaggatagcgagagcaccgacaccgaggaagagttcggcaacgccattggaggatctcacggcggcagcagctataccgtgtacatcgacaagacccggtgagctggagcctcggtggccatgcttcttgccccttgggcctccccccagcccctcctccccttcctgcacccgtacccccgtggtctttgaataaagtctgagtgggcggcaaaaaaaaaaaaaaaaaaaaaaaaaaaaaaaaaaaaaaaaaaaaaaaaaaaaaaaaaaaaaaaaaaaaaaaaaaaaaaaaaaaaaaaaaaaaaaaaaaaaaaaaaaaaaa

SEQ ID NO: 34 - DNA, 1872 bp, synthetic construct
  source 1..1872: mol_type = other DNA
atgggcaccgtgaacaagcctgttgtgggcgtgctgatgggcttcggcatcatcacaggcaccctgcggatcaccaatcctgtgcgggctagcgtgctgagatacgacgacttccacatcgacgaggacaagctggacaccaacagcgtgtacgagccctactaccacagcgatcacgccgagtctagctgggtcaacagaggcgagagcagcagaaaggcctacgaccacaacagcccctacatctggccccggaacgactacgatggcttcctggaaaatgcccacgagcaccacggcgtgtacaatcaaggcagaggcatcgacagcggcgagagactgatgcagcctacacagatgagcgcccaagaggacctgggagatgataccggcatccacgtgatccccacactgaacggcgacgacagacacaagatcgtgaacgtggaccagcggcagtacggcgacgtgttcaagggcgacctgaatcctaagcctcagggccagcgcctgatcgaggtgtccgtggaagagaatcaccccttcacactgagagcccctatccagagaatctacggcgtgcgctataccgagacatggtcctttctgcccagcctgacatgtaccggggatgccgctcctgccatccagcacatttgcctgaagcacaccacctgtttccaggacgtggtggtggatgtggactgcgccgagaacaccaaagaggatcagctggccgagatcagctaccggttccagggaaagaaagaggccgaccagccttggatcgtggtcaacaccagcacactgttcgacgagctggaactggaccctcctgagattgaacccggggtgctgaaggtgctgagaaccgagaagcagtacctgggagtgtacatctggaacatgagaggcagcgacggcacctctacctacgccacctttctggtcacatggaagggcgacgagaaaacacggaaccccacaccagctgtgacccctcaacctagaggcgccgagtttcacatgtggaattaccacagccacgtgttcagcgtgggcgatacctttagcctggccatgcatctgcagtacaagatccacgaggcccctttcgacctgctgctggaatggctgtacgtgcccatcgatcctacctgccagcctatgcggctgtactccacctgtctgtatcaccccaacgctccccagtgcctgagccacatgaatagcggctgcaccttcacaagccctcacctggctcagcgagtggccagcacagtgtaccagaattgcgagcacgccgacaattacaccgcctactgtctgggcatcagccacatggaacctagcttcggcctgatcctgcacgatggcggcacaaccctgaagttcgtggatacccctgagagcctgagcggcctgtatgtgttcgtggtgtacttcaacggccacgtggaagccgtggcctacaccgtggtgtctaccgtggaccacttcgtgaacgccatcgaggaaagaggcttccctccaactgctggacagcctcctgccaccaccaagcctaaagaaatcacacccgtgaatcccggcacaagcccactgcttagatacgccgcttggacaggcggactggctgctgttgttctgctgtgcctggtcatcttcctgatctgcaccgccaagcggatgcgcgtgaaggacaaagagaaggacaagtccccttacaaccagagcatgtactacgccggcctgcctgtggacgacttcgaggatagcgagagcaccgacaccgaggaagagttcggcaacgccattggaggatctcacggcggcagcagctataccgtgtacatcgacaagacccggtga

SEQ ID NO: 35 - protein, 623 aa, synthetic construct
MGTVNKPVVGVLMGFGIITGTLRITNPVRASVLRYDDFHIDEDKLDTNSVYEPYYHSDHAESSWVNRGESSRKAYDHNSPYIWPRNDYDGFLENAHEHHGVYNQGRGIDSGERLMQPTQMSAQEDLGDDTGIHVIPTLNGDDRHKIVNVDQRQYGDVFKGDLNPKPQGQRLIEVSVEENHPFTLRAPIQRIYGVRYTETWSFLPSLTCTGDAAPAIQHICLKHTTCFQDVVVDVDCAENTKEDQLAEISYRFQGKKEADQPWIVVNTSTLFDELELDPPEIEPGVLKVLRTEKQYLGVYIWNMRGSDGTSTYATFLVTWKGDEKTRNPTPAVTPQPRGAEFHMWNYHSHVFSVGDTFSLAMHLQYKIHEAPFDLLLEWLYVPIDPTCQPMRLYSTCLYHPNAPQCLSHMNSGCTFTSPHLAQRVASTVYQNCEHADNYTAYCLGISHMEPSFGLILHDGGTTLKFVDTPESLSGLYVFVVYFNGHVEAVAYTVVSTVDHFVNAIEERGFPPTAGQPPATTKPKEITPVNPGTSPLLRYAAWTGGLAAVVLLCLVIFLICTAKRMRVKDKEKDKSPYNQSMYYAGLPVDDFEDSESTDTEEEFGNAIGGSHGGSSYTVYIDKTR

SEQ ID NO: 36 - RNA, 2161 nt, synthetic construct
  source 1..2161: mol_type = other RNA
agactcctccccatcctctccctctgtccctctgtccctctgaccctgcactgtcccagcaccgccaccatgggcaccgtgaacaagcctgttgtgggcgtgctgatgggcttcggcatcatcacaggcaccctgcggatcaccaatcctgtgcgggctagcgtgctgagatacgacgacttccacatcgacgaggacaagctggacaccaacagcgtgtacgagccctactaccacagcgatcacgccgagtctagctgggtcaacagaggcgagagcagcagaaaggcctacgaccacaacagcccctacatctggccccggaacgactacgatggcttcctggaaaatgcccacgagcaccacggcgtgtacaatcaaggcagaggcatcgacagcggcgagagactgatgcagcctacacagatgagcgcccaagaggacctgggagatgataccggcatccacgtgatccccacactgaacggcgacgacagacacaagatcgtgaacgtggaccagcggcagtacggcgacgtgttcaagggcgacctgaatcctaagcctcagggccagcgcctgatcgaggtgtccgtggaagagaatcaccccttcacactgagagcccctatccagagaatctacggcgtgcgctataccgagacatggtcctttctgcccagcctgacatgtaccggggatgccgctcctgccatccagcacatttgcctgaagcacaccacctgtttccaggacgtggtggtggatgtggactgcgccgagaacaccaaagaggatcagctggccgagatcagctaccggttccagggaaagaaagaggccgaccagccttggatcgtggtcaacaccagcacactgttcgacgagctggaactggaccctcctgagattgaacccggggtgctgaaggtgctgagaaccgagaagcagtacctgggagtgtacatctggaacatgagaggcagcgacggcacctctacctacgccacctttctggtcacatggaagggcgacgagaaaacacggaaccccacaccagctgtgacccctcaacctagaggcgccgagtttcacatgtggaattaccacagccacgtgttcagcgtgggcgatacctttagcctggccatgcatctgcagtacaagatccacgaggcccctttcgacctgctgctggaatggctgtacgtgcccatcgatcctacctgccagcctatgcggctgtactccacctgtctgtatcaccccaacgctccccagtgcctgagccacatgaatagcggctgcaccttcacaagccctcacctggctcagcgagtggccagcacagtgtaccagaattgcgagcacgccgacaattacaccgcctactgtctgggcatcagccacatggaacctagcttcggcctgatcctgcacgatggcggcacaaccctgaagttcgtggatacccctgagagcctgagcggcctgtatgtgttcgtggtgtacttcaacggccacgtggaagccgtggcctacaccgtggtgtctaccgtggaccacttcgtgaacgccatcgaggaaagaggcttccctccaactgctggacagcctcctgccaccaccaagcctaaagaaatcacacccgtgaatcccggcacaagcccactgcttagatacgccgcttggacaggcggactggctgctgttgttctgctgtgcctggtcatcttcctgatctgcaccgccaagcggatgcgcgtgaaggacaaagagaaggacaagtccccttacaaccagagcatgtactacgccggcctgcctgtggacgacttcgaggatagcgagagcaccgacaccgaggaagagttcggcaacgccattggaggatctcacggcggcagcagctataccgtgtacatcgacaagacccggtgagctggagcctcggtggccatgcttcttgccccttgggcctccccccagcccctcctccccttcctgcacccgtacccccgtggtctttgaataaagtctgagtgggcggcaaaaaaaaaaaaaaaaaaaaaaaaaaaaaaaaaaaaaaaaaaaaaaaaaaaaaaaaaaaaaaaaaaaaaaaaaaaaaaaaaaaaaaaaaaaaaaaaaaaaaaaaaaaaaa

SEQ ID NO: 37 - DNA, 2161 bp, synthetic construct
  source 1..2161: mol_type = other DNA
agactcctccccatcctctccctctgtccctctgtccctctgaccctgcactgtcccagcaccgccaccatgggcaccgtgaacaagcctgttgtgggcgtgctgatgggcttcggcatcatcacaggcaccctgcggatcaccaatcctgtgcgggctagcgtgctgagatacgacgacttccacatcgacgaggacaagctggacaccaacagcgtgtacgagccctactaccacagcgatcacgccgagtctagctgggtcaacagaggcgagagcagcagaaaggcctacgaccacaacagcccctacatctggccccggaacgactacgatggcttcctggaaaatgcccacgagcaccacggcgtgtacaatcaaggcagaggcatcgacagcggcgagagactgatgcagcctacacagatgagcgcccaagaggacctgggagatgataccggcatccacgtgatccccacactgaacggcgacgacagacacaagatcgtgaacgtggaccagcggcagtacggcgacgtgttcaagggcgacctgaatcctaagcctcagggccagcgcctgatcgaggtgtccgtggaagagaatcaccccttcacactgagagcccctatccagagaatctacggcgtgcgctataccgagacatggtcctttctgcccagcctgacatgtaccggggatgccgctcctgccatccagcacatttgcctgaagcacaccacctgtttccaggacgtggtggtggatgtggactgcgccgagaacaccaaagaggatcagctggccgagatcagctaccggttccagggaaagaaagaggccgaccagccttggatcgtggtcaacaccagcacactgttcgacgagctggaactggaccctcctgagattgaacccggggtgctgaaggtgctgagaaccgagaagcagtacctgggagtgtacatctggaacatgagaggcagcgacggcacctctacctacgccacctttctggtcacatggaagggcgacgagaaaacacggaaccccacaccagctgtgacccctcaacctagaggcgccgagtttcacatgtggaattaccacagccacgtgttcagcgtgggcgatacctttagcctggccatgcatctgcagtacaagatccacgaggcccctttcgacctgctgctggaatggctgtacgtgcccatcgatcctacctgccagcctatgcggctgtactccacctgtctgtatcaccccaacgctccccagtgcctgagccacatgaatagcggctgcaccttcacaagccctcacctggctcagcgagtggccagcacagtgtaccagaattgcgagcacgccgacaattacaccgcctactgtctgggcatcagccacatggaacctagcttcggcctgatcctgcacgatggcggcacaaccctgaagttcgtggatacccctgagagcctgagcggcctgtatgtgttcgtggtgtacttcaacggccacgtggaagccgtggcctacaccgtggtgtctaccgtggaccacttcgtgaacgccatcgaggaaagaggcttccctccaactgctggacagcctcctgccaccaccaagcctaaagaaatcacacccgtgaatcccggcacaagcccactgcttagatacgccgcttggacaggcggactggctgctgttgttctgctgtgcctggtcatcttcctgatctgcaccgccaagcggatgcgcgtgaaggacaaagagaaggacaagtccccttacaaccagagcatgtactacgccggcctgcctgtggacgatttcgaggatgctgaagccgccgatgccgaggaagagtttggcaacgccattggcggatctcacggcggcagcagctataccgtgtacatcgacaagacccggtgagctggagcctcggtggccatgcttcttgccccttgggcctccccccagcccctcctccccttcctgcacccgtacccccgtggtctttgaataaagtctgagtgggcggcaaaaaaaaaaaaaaaaaaaaaaaaaaaaaaaaaaaaaaaaaaaaaaaaaaaaaaaaaaaaaaaaaaaaaaaaaaaaaaaaaaaaaaaaaaaaaaaaaaaaaaaaaaaaaa

SEQ ID NO: 38 - DNA, 1872 bp, synthetic construct
  source 1..1872: mol_type = other DNA
atgggcaccgtgaacaagcctgttgtgggcgtgctgatgggcttcggcatcatcacaggcaccctgcggatcaccaatcctgtgcgggctagcgtgctgagatacgacgacttccacatcgacgaggacaagctggacaccaacagcgtgtacgagccctactaccacagcgatcacgccgagtctagctgggtcaacagaggcgagagcagcagaaaggcctacgaccacaacagcccctacatctggccccggaacgactacgatggcttcctggaaaatgcccacgagcaccacggcgtgtacaatcaaggcagaggcatcgacagcggcgagagactgatgcagcctacacagatgagcgcccaagaggacctgggagatgataccggcatccacgtgatccccacactgaacggcgacgacagacacaagatcgtgaacgtggaccagcggcagtacggcgacgtgttcaagggcgacctgaatcctaagcctcagggccagcgcctgatcgaggtgtccgtggaagagaatcaccccttcacactgagagcccctatccagagaatctacggcgtgcgctataccgagacatggtcctttctgcccagcctgacatgtaccggggatgccgctcctgccatccagcacatttgcctgaagcacaccacctgtttccaggacgtggtggtggatgtggactgcgccgagaacaccaaagaggatcagctggccgagatcagctaccggttccagggaaagaaagaggccgaccagccttggatcgtggtcaacaccagcacactgttcgacgagctggaactggaccctcctgagattgaacccggggtgctgaaggtgctgagaaccgagaagcagtacctgggagtgtacatctggaacatgagaggcagcgacggcacctctacctacgccacctttctggtcacatggaagggcgacgagaaaacacggaaccccacaccagctgtgacccctcaacctagaggcgccgagtttcacatgtggaattaccacagccacgtgttcagcgtgggcgatacctttagcctggccatgcatctgcagtacaagatccacgaggcccctttcgacctgctgctggaatggctgtacgtgcccatcgatcctacctgccagcctatgcggctgtactccacctgtctgtatcaccccaacgctccccagtgcctgagccacatgaatagcggctgcaccttcacaagccctcacctggctcagcgagtggccagcacagtgtaccagaattgcgagcacgccgacaattacaccgcctactgtctgggcatcagccacatggaacctagcttcggcctgatcctgcacgatggcggcacaaccctgaagttcgtggatacccctgagagcctgagcggcctgtatgtgttcgtggtgtacttcaacggccacgtggaagccgtggcctacaccgtggtgtctaccgtggaccacttcgtgaacgccatcgaggaaagaggcttccctccaactgctggacagcctcctgccaccaccaagcctaaagaaatcacacccgtgaatcccggcacaagcccactgcttagatacgccgcttggacaggcggactggctgctgttgttctgctgtgcctggtcatcttcctgatctgcaccgccaagcggatgcgcgtgaaggacaaagagaaggacaagtccccttacaaccagagcatgtactacgccggcctgcctgtggacgatttcgaggatgctgaagccgccgatgccgaggaagagtttggcaacgccattggcggatctcacggcggcagcagctataccgtgtacatcgacaagacccggtga

SEQ ID NO: 39 - protein, 623 aa, synthetic construct
MGTVNKPVVGVLMGFGIITGTLRITNPVRASVLRYDDFHIDEDKLDTNSVYEPYYHSDHAESSWVNRGESSRKAYDHNSPYIWPRNDYDGFLENAHEHHGVYNQGRGIDSGERLMQPTQMSAQEDLGDDTGIHVIPTLNGDDRHKIVNVDQRQYGDVFKGDLNPKPQGQRLIEVSVEENHPFTLRAPIQRIYGVRYTETWSFLPSLTCTGDAAPAIQHICLKHTTCFQDVVVDVDCAENTKEDQLAEISYRFQGKKEADQPWIVVNTSTLFDELELDPPEIEPGVLKVLRTEKQYLGVYIWNMRGSDGTSTYATFLVTWKGDEKTRNPTPAVTPQPRGAEFHMWNYHSHVFSVGDTFSLAMHLQYKIHEAPFDLLLEWLYVPIDPTCQPMRLYSTCLYHPNAPQCLSHMNSGCTFTSPHLAQRVASTVYQNCEHADNYTAYCLGISHMEPSFGLILHDGGTTLKFVDTPESLSGLYVFVVYFNGHVEAVAYTVVSTVDHFVNAIEERGFPPTAGQPPATTKPKEITPVNPGTSPLLRYAAWTGGLAAVVLLCLVIFLICTAKRMRVKDKEKDKSPYNQSMYYAGLPVDDFEDAEAADAEEEFGNAIGGSHGGSSYTVYIDKTR

SEQ ID NO: 40 - RNA, 2161 nt, synthetic construct
  source 1..2161: mol_type = other RNA
agactcctccccatcctctccctctgtccctctgtccctctgaccctgcactgtcccagcaccgccaccatgggcaccgtgaacaagcctgttgtgggcgtgctgatgggcttcggcatcatcacaggcaccctgcggatcaccaatcctgtgcgggctagcgtgctgagatacgacgacttccacatcgacgaggacaagctggacaccaacagcgtgtacgagccctactaccacagcgatcacgccgagtctagctgggtcaacagaggcgagagcagcagaaaggcctacgaccacaacagcccctacatctggccccggaacgactacgatggcttcctggaaaatgcccacgagcaccacggcgtgtacaatcaaggcagaggcatcgacagcggcgagagactgatgcagcctacacagatgagcgcccaagaggacctgggagatgataccggcatccacgtgatccccacactgaacggcgacgacagacacaagatcgtgaacgtggaccagcggcagtacggcgacgtgttcaagggcgacctgaatcctaagcctcagggccagcgcctgatcgaggtgtccgtggaagagaatcaccccttcacactgagagcccctatccagagaatctacggcgtgcgctataccgagacatggtcctttctgcccagcctgacatgtaccggggatgccgctcctgccatccagcacatttgcctgaagcacaccacctgtttccaggacgtggtggtggatgtggactgcgccgagaacaccaaagaggatcagctggccgagatcagctaccggttccagggaaagaaagaggccgaccagccttggatcgtggtcaacaccagcacactgttcgacgagctggaactggaccctcctgagattgaacccggggtgctgaaggtgctgagaaccgagaagcagtacctgggagtgtacatctggaacatgagaggcagcgacggcacctctacctacgccacctttctggtcacatggaagggcgacgagaaaacacggaaccccacaccagctgtgacccctcaacctagaggcgccgagtttcacatgtggaattaccacagccacgtgttcagcgtgggcgatacctttagcctggccatgcatctgcagtacaagatccacgaggcccctttcgacctgctgctggaatggctgtacgtgcccatcgatcctacctgccagcctatgcggctgtactccacctgtctgtatcaccccaacgctccccagtgcctgagccacatgaatagcggctgcaccttcacaagccctcacctggctcagcgagtggccagcacagtgtaccagaattgcgagcacgccgacaattacaccgcctactgtctgggcatcagccacatggaacctagcttcggcctgatcctgcacgatggcggcacaaccctgaagttcgtggatacccctgagagcctgagcggcctgtatgtgttcgtggtgtacttcaacggccacgtggaagccgtggcctacaccgtggtgtctaccgtggaccacttcgtgaacgccatcgaggaaagaggcttccctccaactgctggacagcctcctgccaccaccaagcctaaagaaatcacacccgtgaatcccggcacaagcccactgcttagatacgccgcttggacaggcggactggctgctgttgttctgctgtgcctggtcatcttcctgatctgcaccgccaagcggatgcgcgtgaaggacaaagagaaggacaagtccccttacaaccagagcatgtactacgccggcctgcctgtggacgatttcgaggatgctgaagccgccgatgccgaggaagagtttggcaacgccattggcggatctcacggcggcagcagctataccgtgtacatcgacaagacccggtgagctggagcctcggtggccatgcttcttgccccttgggcctccccccagcccctcctccccttcctgcacccgtacccccgtggtctttgaataaagtctgagtgggcggcaaaaaaaaaaaaaaaaaaaaaaaaaaaaaaaaaaaaaaaaaaaaaaaaaaaaaaaaaaaaaaaaaaaaaaaaaaaaaaaaaaaaaaaaaaaaaaaaaaaaaaaaaaaaaa

SEQ ID NO: 41 - DNA, 2161 bp, synthetic construct
  source 1..2161: mol_type = other DNA
agactcctccccatcctctccctctgtccctctgtccctctgaccctgcactgtcccagcaccgccaccatgggcaccgtgaacaagcctgttgtgggcgtgctgatgggcttcggcatcatcacaggcaccctgcggatcaccaatcctgtgcgggctagcgtgctgagatacgacgacttccacatcgacgaggacaagctggacaccaacagcgtgtacgagccctactaccacagcgatcacgccgagtctagctgggtcaacagaggcgagagcagcagaaaggcctacgaccacaacagcccctacatctggccccggaacgactacgatggcttcctggaaaatgcccacgagcaccacggcgtgtacaatcaaggcagaggcatcgacagcggcgagagactgatgcagcctacacagatgagcgcccaagaggacctgggagatgataccggcatccacgtgatccccacactgaacggcgacgacagacacaagatcgtgaacgtggaccagcggcagtacggcgacgtgttcaagggcgacctgaatcctaagcctcagggccagcgcctgatcgaggtgtccgtggaagagaatcaccccttcacactgagagcccctatccagagaatctacggcgtgcgctataccgagacatggtcctttctgcccagcctgacatgtaccggggatgccgctcctgccatccagcacatttgcctgaagcacaccacctgtttccaggacgtggtggtggatgtggactgcgccgagaacaccaaagaggatcagctggccgagatcagctaccggttccagggaaagaaagaggccgaccagccttggatcgtggtcaacaccagcacactgttcgacgagctggaactggaccctcctgagattgaacccggggtgctgaaggtgctgagaaccgagaagcagtacctgggagtgtacatctggaacatgagaggcagcgacggcacctctacctacgccacctttctggtcacatggaagggcgacgagaaaacacggaaccccacaccagctgtgacccctcaacctagaggcgccgagtttcacatgtggaattaccacagccacgtgttcagcgtgggcgatacctttagcctggccatgcatctgcagtacaagatccacgaggcccctttcgacctgctgctggaatggctgtacgtgcccatcgatcctacctgccagcctatgcggctgtactccacctgtctgtatcaccccaacgctccccagtgcctgagccacatgaatagcggctgcaccttcacaagccctcacctggctcagcgagtggccagcacagtgtaccagaattgcgagcacgccgacaattacaccgcctactgtctgggcatcagccacatggaacctagcttcggcctgatcctgcacgatggcggcacaaccctgaagttcgtggatacccctgagagcctgagcggcctgtatgtgttcgtggtgtacttcaacggccacgtggaagccgtggcctacaccgtggtgtctaccgtggaccacttcgtgaacgccatcgaggaaagaggcttccctccaactgctggacagcctcctgccaccaccaagcctaaagaaatcacacccgtgaatcccggcacaagcccactgcttagatacgccgcttggacaggcggactggctgctgttgttctgctgtgcctggtcatcttcctgatctgcaccgccaagcggatgcgcgtgaaggacaaagagaaggacaagtccccttacaaccagtctatgtatgccgccggactgcccgtggacgatttcgaggatagcgagagcaccgacaccgaggaagagttcggcaacgccattggaggatctcacggcggcagcagctataccgtgtacatcgacaagacccggtgagctggagcctcggtggccatgcttcttgccccttgggcctccccccagcccctcctccccttcctgcacccgtacccccgtggtctttgaataaagtctgagtgggcggcaaaaaaaaaaaaaaaaaaaaaaaaaaaaaaaaaaaaaaaaaaaaaaaaaaaaaaaaaaaaaaaaaaaaaaaaaaaaaaaaaaaaaaaaaaaaaaaaaaaaaaaaaaaaaa

SEQ ID NO: 42 - DNA, 1872 bp, synthetic construct
  source 1..1872: mol_type = other DNA
atgggcaccgtgaacaagcctgttgtgggcgtgctgatgggcttcggcatcatcacaggcaccctgcggatcaccaatcctgtgcgggctagcgtgctgagatacgacgacttccacatcgacgaggacaagctggacaccaacagcgtgtacgagccctactaccacagcgatcacgccgagtctagctgggtcaacagaggcgagagcagcagaaaggcctacgaccacaacagcccctacatctggccccggaacgactacgatggcttcctggaaaatgcccacgagcaccacggcgtgtacaatcaaggcagaggcatcgacagcggcgagagactgatgcagcctacacagatgagcgcccaagaggacctgggagatgataccggcatccacgtgatccccacactgaacggcgacgacagacacaagatcgtgaacgtggaccagcggcagtacggcgacgtgttcaagggcgacctgaatcctaagcctcagggccagcgcctgatcgaggtgtccgtggaagagaatcaccccttcacactgagagcccctatccagagaatctacggcgtgcgctataccgagacatggtcctttctgcccagcctgacatgtaccggggatgccgctcctgccatccagcacatttgcctgaagcacaccacctgtttccaggacgtggtggtggatgtggactgcgccgagaacaccaaagaggatcagctggccgagatcagctaccggttccagggaaagaaagaggccgaccagccttggatcgtggtcaacaccagcacactgttcgacgagctggaactggaccctcctgagattgaacccggggtgctgaaggtgctgagaaccgagaagcagtacctgggagtgtacatctggaacatgagaggcagcgacggcacctctacctacgccacctttctggtcacatggaagggcgacgagaaaacacggaaccccacaccagctgtgacccctcaacctagaggcgccgagtttcacatgtggaattaccacagccacgtgttcagcgtgggcgatacctttagcctggccatgcatctgcagtacaagatccacgaggcccctttcgacctgctgctggaatggctgtacgtgcccatcgatcctacctgccagcctatgcggctgtactccacctgtctgtatcaccccaacgctccccagtgcctgagccacatgaatagcggctgcaccttcacaagccctcacctggctcagcgagtggccagcacagtgtaccagaattgcgagcacgccgacaattacaccgcctactgtctgggcatcagccacatggaacctagcttcggcctgatcctgcacgatggcggcacaaccctgaagttcgtggatacccctgagagcctgagcggcctgtatgtgttcgtggtgtacttcaacggccacgtggaagccgtggcctacaccgtggtgtctaccgtggaccacttcgtgaacgccatcgaggaaagaggcttccctccaactgctggacagcctcctgccaccaccaagcctaaagaaatcacacccgtgaatcccggcacaagcccactgcttagatacgccgcttggacaggcggactggctgctgttgttctgctgtgcctggtcatcttcctgatctgcaccgccaagcggatgcgcgtgaaggacaaagagaaggacaagtccccttacaaccagtctatgtatgccgccggactgcccgtggacgatttcgaggatagcgagagcaccgacaccgaggaagagttcggcaacgccattggaggatctcacggcggcagcagctataccgtgtacatcgacaagacccggtga

SEQ ID NO: 43 - protein, 623 aa, synthetic construct
MGTVNKPVVGVLMGFGIITGTLRITNPVRASVLRYDDFHIDEDKLDTNSVYEPYYHSDHAESSWVNRGESSRKAYDHNSPYIWPRNDYDGFLENAHEHHGVYNQGRGIDSGERLMQPTQMSAQEDLGDDTGIHVIPTLNGDDRHKIVNVDQRQYGDVFKGDLNPKPQGQRLIEVSVEENHPFTLRAPIQRIYGVRYTETWSFLPSLTCTGDAAPAIQHICLKHTTCFQDVVVDVDCAENTKEDQLAEISYRFQGKKEADQPWIVVNTSTLFDELELDPPEIEPGVLKVLRTEKQYLGVYIWNMRGSDGTSTYATFLVTWKGDEKTRNPTPAVTPQPRGAEFHMWNYHSHVFSVGDTFSLAMHLQYKIHEAPFDLLLEWLYVPIDPTCQPMRLYSTCLYHPNAPQCLSHMNSGCTFTSPHLAQRVASTVYQNCEHADNYTAYCLGISHMEPSFGLILHDGGTTLKFVDTPESLSGLYVFVVYFNGHVEAVAYTVVSTVDHFVNAIEERGFPPTAGQPPATTKPKEITPVNPGTSPLLRYAAWTGGLAAVVLLCLVIFLICTAKRMRVKDKEKDKSPYNQSMYAAGLPVDDFEDSESTDTEEEFGNAIGGSHGGSSYTVYIDKTR

SEQ ID NO: 44 - RNA, 2161 nt, synthetic construct
  source 1..2161: mol_type = other RNA
agactcctccccatcctctccctctgtccctctgtccctctgaccctgcactgtcccagcaccgccaccatgggcaccgtgaacaagcctgttgtgggcgtgctgatgggcttcggcatcatcacaggcaccctgcggatcaccaatcctgtgcgggctagcgtgctgagatacgacgacttccacatcgacgaggacaagctggacaccaacagcgtgtacgagccctactaccacagcgatcacgccgagtctagctgggtcaacagaggcgagagcagcagaaaggcctacgaccacaacagcccctacatctggccccggaacgactacgatggcttcctggaaaatgcccacgagcaccacggcgtgtacaatcaaggcagaggcatcgacagcggcgagagactgatgcagcctacacagatgagcgcccaagaggacctgggagatgataccggcatccacgtgatccccacactgaacggcgacgacagacacaagatcgtgaacgtggaccagcggcagtacggcgacgtgttcaagggcgacctgaatcctaagcctcagggccagcgcctgatcgaggtgtccgtggaagagaatcaccccttcacactgagagcccctatccagagaatctacggcgtgcgctataccgagacatggtcctttctgcccagcctgacatgtaccggggatgccgctcctgccatccagcacatttgcctgaagcacaccacctgtttccaggacgtggtggtggatgtggactgcgccgagaacaccaaagaggatcagctggccgagatcagctaccggttccagggaaagaaagaggccgaccagccttggatcgtggtcaacaccagcacactgttcgacgagctggaactggaccctcctgagattgaacccggggtgctgaaggtgctgagaaccgagaagcagtacctgggagtgtacatctggaacatgagaggcagcgacggcacctctacctacgccacctttctggtcacatggaagggcgacgagaaaacacggaaccccacaccagctgtgacccctcaacctagaggcgccgagtttcacatgtggaattaccacagccacgtgttcagcgtgggcgatacctttagcctggccatgcatctgcagtacaagatccacgaggcccctttcgacctgctgctggaatggctgtacgtgcccatcgatcctacctgccagcctatgcggctgtactccacctgtctgtatcaccccaacgctccccagtgcctgagccacatgaatagcggctgcaccttcacaagccctcacctggctcagcgagtggccagcacagtgtaccagaattgcgagcacgccgacaattacaccgcctactgtctgggcatcagccacatggaacctagcttcggcctgatcctgcacgatggcggcacaaccctgaagttcgtggatacccctgagagcctgagcggcctgtatgtgttcgtggtgtacttcaacggccacgtggaagccgtggcctacaccgtggtgtctaccgtggaccacttcgtgaacgccatcgaggaaagaggcttccctccaactgctggacagcctcctgccaccaccaagcctaaagaaatcacacccgtgaatcccggcacaagcccactgcttagatacgccgcttggacaggcggactggctgctgttgttctgctgtgcctggtcatcttcctgatctgcaccgccaagcggatgcgcgtgaaggacaaagagaaggacaagtccccttacaaccagtctatgtatgccgccggactgcccgtggacgatttcgaggatagcgagagcaccgacaccgaggaagagttcggcaacgccattggaggatctcacggcggcagcagctataccgtgtacatcgacaagacccggtgagctggagcctcggtggccatgcttcttgccccttgggcctccccccagcccctcctccccttcctgcacccgtacccccgtggtctttgaataaagtctgagtgggcggcaaaaaaaaaaaaaaaaaaaaaaaaaaaaaaaaaaaaaaaaaaaaaaaaaaaaaaaaaaaaaaaaaaaaaaaaaaaaaaaaaaaaaaaaaaaaaaaaaaaaaaaaaaaaaa

SEQ ID NO: 45 - DNA, 2161 bp, synthetic construct
  source 1..2161: mol_type = other DNA
agactcctccccatcctctccctctgtccctctgtccctctgaccctgcactgtcccagcaccgccaccatgggcaccgtgaacaagcctgttgtgggcgtgctgatgggcttcggcatcatcacaggcaccctgcggatcaccaatcctgtgcgggctagcgtgctgagatacgacgacttccacatcgacgaggacaagctggacaccaacagcgtgtacgagccctactaccacagcgatcacgccgagtctagctgggtcaacagaggcgagagcagcagaaaggcctacgaccacaacagcccctacatctggccccggaacgactacgatggcttcctggaaaatgcccacgagcaccacggcgtgtacaatcaaggcagaggcatcgacagcggcgagagactgatgcagcctacacagatgagcgcccaagaggacctgggagatgataccggcatccacgtgatccccacactgaacggcgacgacagacacaagatcgtgaacgtggaccagcggcagtacggcgacgtgttcaagggcgacctgaatcctaagcctcagggccagcgcctgatcgaggtgtccgtggaagagaatcaccccttcacactgagagcccctatccagagaatctacggcgtgcgctataccgagacatggtcctttctgcccagcctgacatgtaccggggatgccgctcctgccatccagcacatttgcctgaagcacaccacctgtttccaggacgtggtggtggatgtggactgcgccgagaacaccaaagaggatcagctggccgagatcagctaccggttccagggaaagaaagaggccgaccagccttggatcgtggtcaacaccagcacactgttcgacgagctggaactggaccctcctgagattgaacccggggtgctgaaggtgctgagaaccgagaagcagtacctgggagtgtacatctggaacatgagaggcagcgacggcacctctacctacgccacctttctggtcacatggaagggcgacgagaaaacacggaaccccacaccagctgtgacccctcaacctagaggcgccgagtttcacatgtggaattaccacagccacgtgttcagcgtgggcgatacctttagcctggccatgcatctgcagtacaagatccacgaggcccctttcgacctgctgctggaatggctgtacgtgcccatcgatcctacctgccagcctatgcggctgtactccacctgtctgtatcaccccaacgctccccagtgcctgagccacatgaatagcggctgcaccttcacaagccctcacctggctcagcgagtggccagcacagtgtaccagaattgcgagcacgccgacaattacaccgcctactgtctgggcatcagccacatggaacctagcttcggcctgatcctgcacgatggcggcacaaccctgaagttcgtggatacccctgagagcctgagcggcctgtatgtgttcgtggtgtacttcaacggccacgtggaagccgtggcctacaccgtggtgtctaccgtggaccacttcgtgaacgccatcgaggaaagaggcttccctccaactgctggacagcctcctgccaccaccaagcctaaagaaatcacacccgtgaatcccggcacaagcccactgcttagatacgccgcttggacaggcggactggctgctgttgttctgctgtgcctggtcatcttcctgatctgcaccgccaagcggatgcgcgtgaaggacaaagagaaggacaagtccccttacaaccagtctatgtatgccgccggactgcccgtggacgattttgaggatgctgaagccgccgacgccgaggaagaatttggcaacgccattggcggaagccacggcggcagtagctataccgtgtacatcgacaagacccggtgagctggagcctcggtggccatgcttcttgccccttgggcctccccccagcccctcctccccttcctgcacccgtacccccgtggtctttgaataaagtctgagtgggcggcaaaaaaaaaaaaaaaaaaaaaaaaaaaaaaaaaaaaaaaaaaaaaaaaaaaaaaaaaaaaaaaaaaaaaaaaaaaaaaaaaaaaaaaaaaaaaaaaaaaaaaaaaaaaaa

SEQ ID NO: 46 - DNA, 1872 bp, synthetic construct
  source 1..1872: mol_type = other DNA
atgggcaccgtgaacaagcctgttgtgggcgtgctgatgggcttcggcatcatcacaggcaccctgcggatcaccaatcctgtgcgggctagcgtgctgagatacgacgacttccacatcgacgaggacaagctggacaccaacagcgtgtacgagccctactaccacagcgatcacgccgagtctagctgggtcaacagaggcgagagcagcagaaaggcctacgaccacaacagcccctacatctggccccggaacgactacgatggcttcctggaaaatgcccacgagcaccacggcgtgtacaatcaaggcagaggcatcgacagcggcgagagactgatgcagcctacacagatgagcgcccaagaggacctgggagatgataccggcatccacgtgatccccacactgaacggcgacgacagacacaagatcgtgaacgtggaccagcggcagtacggcgacgtgttcaagggcgacctgaatcctaagcctcagggccagcgcctgatcgaggtgtccgtggaagagaatcaccccttcacactgagagcccctatccagagaatctacggcgtgcgctataccgagacatggtcctttctgcccagcctgacatgtaccggggatgccgctcctgccatccagcacatttgcctgaagcacaccacctgtttccaggacgtggtggtggatgtggactgcgccgagaacaccaaagaggatcagctggccgagatcagctaccggttccagggaaagaaagaggccgaccagccttggatcgtggtcaacaccagcacactgttcgacgagctggaactggaccctcctgagattgaacccggggtgctgaaggtgctgagaaccgagaagcagtacctgggagtgtacatctggaacatgagaggcagcgacggcacctctacctacgccacctttctggtcacatggaagggcgacgagaaaacacggaaccccacaccagctgtgacccctcaacctagaggcgccgagtttcacatgtggaattaccacagccacgtgttcagcgtgggcgatacctttagcctggccatgcatctgcagtacaagatccacgaggcccctttcgacctgctgctggaatggctgtacgtgcccatcgatcctacctgccagcctatgcggctgtactccacctgtctgtatcaccccaacgctccccagtgcctgagccacatgaatagcggctgcaccttcacaagccctcacctggctcagcgagtggccagcacagtgtaccagaattgcgagcacgccgacaattacaccgcctactgtctgggcatcagccacatggaacctagcttcggcctgatcctgcacgatggcggcacaaccctgaagttcgtggatacccctgagagcctgagcggcctgtatgtgttcgtggtgtacttcaacggccacgtggaagccgtggcctacaccgtggtgtctaccgtggaccacttcgtgaacgccatcgaggaaagaggcttccctccaactgctggacagcctcctgccaccaccaagcctaaagaaatcacacccgtgaatcccggcacaagcccactgcttagatacgccgcttggacaggcggactggctgctgttgttctgctgtgcctggtcatcttcctgatctgcaccgccaagcggatgcgcgtgaaggacaaagagaaggacaagtccccttacaaccagtctatgtatgccgccggactgcccgtggacgattttgaggatgctgaagccgccgacgccgaggaagaatttggcaacgccattggcggaagccacggcggcagtagctataccgtgtacatcgacaagacccggtga

SEQ ID NO: 47 - protein, 623 aa, synthetic construct
MGTVNKPVVGVLMGFGIITGTLRITNPVRASVLRYDDFHIDEDKLDTNSVYEPYYHSDHAESSWVNRGESSRKAYDHNSPYIWPRNDYDGFLENAHEHHGVYNQGRGIDSGERLMQPTQMSAQEDLGDDTGIHVIPTLNGDDRHKIVNVDQRQYGDVFKGDLNPKPQGQRLIEVSVEENHPFTLRAPIQRIYGVRYTETWSFLPSLTCTGDAAPAIQHICLKHTTCFQDVVVDVDCAENTKEDQLAEISYRFQGKKEADQPWIVVNTSTLFDELELDPPEIEPGVLKVLRTEKQYLGVYIWNMRGSDGTSTYATFLVTWKGDEKTRNPTPAVTPQPRGAEFHMWNYHSHVFSVGDTFSLAMHLQYKIHEAPFDLLLEWLYVPIDPTCQPMRLYSTCLYHPNAPQCLSHMNSGCTFTSPHLAQRVASTVYQNCEHADNYTAYCLGISHMEPSFGLILHDGGTTLKFVDTPESLSGLYVFVVYFNGHVEAVAYTVVSTVDHFVNAIEERGFPPTAGQPPATTKPKEITPVNPGTSPLLRYAAWTGGLAAVVLLCLVIFLICTAKRMRVKDKEKDKSPYNQSMYAAGLPVDDFEDAEAADAEEEFGNAIGGSHGGSSYTVYIDKTR

SEQ ID NO: 48 - RNA, 2161 nt, synthetic construct
  source 1..2161: mol_type = other RNA
agactcctccccatcctctccctctgtccctctgtccctctgaccctgcactgtcccagcaccgccaccatgggcaccgtgaacaagcctgttgtgggcgtgctgatgggcttcggcatcatcacaggcaccctgcggatcaccaatcctgtgcgggctagcgtgctgagatacgacgacttccacatcgacgaggacaagctggacaccaacagcgtgtacgagccctactaccacagcgatcacgccgagtctagctgggtcaacagaggcgagagcagcagaaaggcctacgaccacaacagcccctacatctggccccggaacgactacgatggcttcctggaaaatgcccacgagcaccacggcgtgtacaatcaaggcagaggcatcgacagcggcgagagactgatgcagcctacacagatgagcgcccaagaggacctgggagatgataccggcatccacgtgatccccacactgaacggcgacgacagacacaagatcgtgaacgtggaccagcggcagtacggcgacgtgttcaagggcgacctgaatcctaagcctcagggccagcgcctgatcgaggtgtccgtggaagagaatcaccccttcacactgagagcccctatccagagaatctacggcgtgcgctataccgagacatggtcctttctgcccagcctgacatgtaccggggatgccgctcctgccatccagcacatttgcctgaagcacaccacctgtttccaggacgtggtggtggatgtggactgcgccgagaacaccaaagaggatcagctggccgagatcagctaccggttccagggaaagaaagaggccgaccagccttggatcgtggtcaacaccagcacactgttcgacgagctggaactggaccctcctgagattgaacccggggtgctgaaggtgctgagaaccgagaagcagtacctgggagtgtacatctggaacatgagaggcagcgacggcacctctacctacgccacctttctggtcacatggaagggcgacgagaaaacacggaaccccacaccagctgtgacccctcaacctagaggcgccgagtttcacatgtggaattaccacagccacgtgttcagcgtgggcgatacctttagcctggccatgcatctgcagtacaagatccacgaggcccctttcgacctgctgctggaatggctgtacgtgcccatcgatcctacctgccagcctatgcggctgtactccacctgtctgtatcaccccaacgctccccagtgcctgagccacatgaatagcggctgcaccttcacaagccctcacctggctcagcgagtggccagcacagtgtaccagaattgcgagcacgccgacaattacaccgcctactgtctgggcatcagccacatggaacctagcttcggcctgatcctgcacgatggcggcacaaccctgaagttcgtggatacccctgagagcctgagcggcctgtatgtgttcgtggtgtacttcaacggccacgtggaagccgtggcctacaccgtggtgtctaccgtggaccacttcgtgaacgccatcgaggaaagaggcttccctccaactgctggacagcctcctgccaccaccaagcctaaagaaatcacacccgtgaatcccggcacaagcccactgcttagatacgccgcttggacaggcggactggctgctgttgttctgctgtgcctggtcatcttcctgatctgcaccgccaagcggatgcgcgtgaaggacaaagagaaggacaagtccccttacaaccagtctatgtatgccgccggactgcccgtggacgattttgaggatgctgaagccgccgacgccgaggaagaatttggcaacgccattggcggaagccacggcggcagtagctataccgtgtacatcgacaagacccggtgagctggagcctcggtggccatgcttcttgccccttgggcctccccccagcccctcctccccttcctgcacccgtacccccgtggtctttgaataaagtctgagtgggcggcaaaaaaaaaaaaaaaaaaaaaaaaaaaaaaaaaaaaaaaaaaaaaaaaaaaaaaaaaaaaaaaaaaaaaaaaaaaaaaaaaaaaaaaaaaaaaaaaaaaaaaaaaaaaaa

SEQ ID NO: 49 - DNA, 2128 bp, synthetic construct
  source 1..2128: mol_type = other DNA
agactcctccccatcctctccctctgtccctctgtccctctgaccctgcactgtcccagcaccgccaccatgggcaccgtgaacaagcctgttgtgggcgtgctgatgggcttcggcatcatcacaggcaccctgcggatcaccaatcctgtgcgggctagcgtgctgagatacgacgacttccacatcgacgaggacaagctggacaccaacagcgtgtacgagccctactaccacagcgatcacgccgagtctagctgggtcaacagaggcgagagcagcagaaaggcctacgaccacaacagcccctacatctggccccggaacgactacgatggcttcctggaaaatgcccacgagcaccacggcgtgtacaatcaaggcagaggcatcgacagcggcgagagactgatgcagcctacacagatgagcgcccaagaggacctgggagatgataccggcatccacgtgatccccacactgaacggcgacgacagacacaagatcgtgaacgtggaccagcggcagtacggcgacgtgttcaagggcgacctgaatcctaagcctcagggccagcgcctgatcgaggtgtccgtggaagagaatcaccccttcacactgagagcccctatccagagaatctacggcgtgcgctataccgagacatggtcctttctgcccagcctgacatgtaccggggatgccgctcctgccatccagcacatttgcctgaagcacaccacctgtttccaggacgtggtggtggatgtggactgcgccgagaacaccaaagaggatcagctggccgagatcagctaccggttccagggaaagaaagaggccgaccagccttggatcgtggtcaacaccagcacactgttcgacgagctggaactggaccctcctgagattgaacccggggtgctgaaggtgctgagaaccgagaagcagtacctgggagtgtacatctggaacatgagaggcagcgacggcacctctacctacgccacctttctggtcacatggaagggcgacgagaaaacacggaaccccacaccagctgtgacccctcaacctagaggcgccgagtttcacatgtggaattaccacagccacgtgttcagcgtgggcgatacctttagcctggccatgcatctgcagtacaagatccacgaggcccctttcgacctgctgctggaatggctgtacgtgcccatcgatcctacctgccagcctatgcggctgtactccacctgtctgtatcaccccaacgctccccagtgcctgagccacatgaatagcggctgcaccttcacaagccctcacctggctcagcgagtggccagcacagtgtaccagaattgcgagcacgccgacaattacaccgcctactgtctgggcatcagccacatggaacctagcttcggcctgatcctgcacgatggcggcacaaccctgaagttcgtggatacccctgagagcctgagcggcctgtatgtgttcgtggtgtacttcaacggccacgtggaagccgtggcctacaccgtggtgtctaccgtggaccacttcgtgaacgccatcgaggaaagaggcttccctccaactgctggacagcctcctgccaccaccaagcctaaagaaatcacacccgtgaatcccggcacaagcccactgcttagatacgccgcttggacaggcggactggctgctgttgttctgctgtgcctggtcatcttcctgatctgcaccgccaagcggatgagagtgaaggccatgtactatgccggcctgcctgtggacgacttcgaggatagcgagagcaccgacaccgaggaagagttcggcaacgccattggaggatctcacggcggcagcagctataccgtgtacatcgacaagacccggtgagctggagcctcggtggccatgcttcttgccccttgggcctccccccagcccctcctccccttcctgcacccgtacccccgtggtctttgaataaagtctgagtgggcggcaaaaaaaaaaaaaaaaaaaaaaaaaaaaaaaaaaaaaaaaaaaaaaaaaaaaaaaaaaaaaaaaaaaaaaaaaaaaaaaaaaaaaaaaaaaaaaaaaaaaaaaaaaaaaa

SEQ ID NO: 50 - DNA, 1839 bp, synthetic construct
  source 1..1839: mol_type = other DNA
atgggcaccgtgaacaagcctgttgtgggcgtgctgatgggcttcggcatcatcacaggcaccctgcggatcaccaatcctgtgcgggctagcgtgctgagatacgacgacttccacatcgacgaggacaagctggacaccaacagcgtgtacgagccctactaccacagcgatcacgccgagtctagctgggtcaacagaggcgagagcagcagaaaggcctacgaccacaacagcccctacatctggccccggaacgactacgatggcttcctggaaaatgcccacgagcaccacggcgtgtacaatcaaggcagaggcatcgacagcggcgagagactgatgcagcctacacagatgagcgcccaagaggacctgggagatgataccggcatccacgtgatccccacactgaacggcgacgacagacacaagatcgtgaacgtggaccagcggcagtacggcgacgtgttcaagggcgacctgaatcctaagcctcagggccagcgcctgatcgaggtgtccgtggaagagaatcaccccttcacactgagagcccctatccagagaatctacggcgtgcgctataccgagacatggtcctttctgcccagcctgacatgtaccggggatgccgctcctgccatccagcacatttgcctgaagcacaccacctgtttccaggacgtggtggtggatgtggactgcgccgagaacaccaaagaggatcagctggccgagatcagctaccggttccagggaaagaaagaggccgaccagccttggatcgtggtcaacaccagcacactgttcgacgagctggaactggaccctcctgagattgaacccggggtgctgaaggtgctgagaaccgagaagcagtacctgggagtgtacatctggaacatgagaggcagcgacggcacctctacctacgccacctttctggtcacatggaagggcgacgagaaaacacggaaccccacaccagctgtgacccctcaacctagaggcgccgagtttcacatgtggaattaccacagccacgtgttcagcgtgggcgatacctttagcctggccatgcatctgcagtacaagatccacgaggcccctttcgacctgctgctggaatggctgtacgtgcccatcgatcctacctgccagcctatgcggctgtactccacctgtctgtatcaccccaacgctccccagtgcctgagccacatgaatagcggctgcaccttcacaagccctcacctggctcagcgagtggccagcacagtgtaccagaattgcgagcacgccgacaattacaccgcctactgtctgggcatcagccacatggaacctagcttcggcctgatcctgcacgatggcggcacaaccctgaagttcgtggatacccctgagagcctgagcggcctgtatgtgttcgtggtgtacttcaacggccacgtggaagccgtggcctacaccgtggtgtctaccgtggaccacttcgtgaacgccatcgaggaaagaggcttccctccaactgctggacagcctcctgccaccaccaagcctaaagaaatcacacccgtgaatcccggcacaagcccactgcttagatacgccgcttggacaggcggactggctgctgttgttctgctgtgcctggtcatcttcctgatctgcaccgccaagcggatgagagtgaaggccatgtactatgccggcctgcctgtggacgacttcgaggatagcgagagcaccgacaccgaggaagagttcggcaacgccattggaggatctcacggcggcagcagctataccgtgtacatcgacaagacccggtga

SEQ ID NO: 51 - protein, 612 aa, synthetic construct
MGTVNKPVVGVLMGFGIITGTLRITNPVRASVLRYDDFHIDEDKLDTNSVYEPYYHSDHAESSWVNRGESSRKAYDHNSPYIWPRNDYDGFLENAHEHHGVYNQGRGIDSGERLMQPTQMSAQEDLGDDTGIHVIPTLNGDDRHKIVNVDQRQYGDVFKGDLNPKPQGQRLIEVSVEENHPFTLRAPIQRIYGVRYTETWSFLPSLTCTGDAAPAIQHICLKHTTCFQDVVVDVDCAENTKEDQLAEISYRFQGKKEADQPWIVVNTSTLFDELELDPPEIEPGVLKVLRTEKQYLGVYIWNMRGSDGTSTYATFLVTWKGDEKTRNPTPAVTPQPRGAEFHMWNYHSHVFSVGDTFSLAMHLQYKIHEAPFDLLLEWLYVPIDPTCQPMRLYSTCLYHPNAPQCLSHMNSGCTFTSPHLAQRVASTVYQNCEHADNYTAYCLGISHMEPSFGLILHDGGTTLKFVDTPESLSGLYVFVVYFNGHVEAVAYTVVSTVDHFVNAIEERGFPPTAGQPPATTKPKEITPVNPGTSPLLRYAAWTGGLAAVVLLCLVIFLICTAKRMRVKAMYYAGLPVDDFEDSESTDTEEEFGNAIGGSHGGSSYTVYIDKTR

SEQ ID NO: 52 - RNA, 2128 nt, synthetic construct
  source 1..2128: mol_type = other RNA
agactcctccccatcctctccctctgtccctctgtccctctgaccctgcactgtcccagcaccgccaccatgggcaccgtgaacaagcctgttgtgggcgtgctgatgggcttcggcatcatcacaggcaccctgcggatcaccaatcctgtgcgggctagcgtgctgagatacgacgacttccacatcgacgaggacaagctggacaccaacagcgtgtacgagccctactaccacagcgatcacgccgagtctagctgggtcaacagaggcgagagcagcagaaaggcctacgaccacaacagcccctacatctggccccggaacgactacgatggcttcctggaaaatgcccacgagcaccacggcgtgtacaatcaaggcagaggcatcgacagcggcgagagactgatgcagcctacacagatgagcgcccaagaggacctgggagatgataccggcatccacgtgatccccacactgaacggcgacgacagacacaagatcgtgaacgtggaccagcggcagtacggcgacgtgttcaagggcgacctgaatcctaagcctcagggccagcgcctgatcgaggtgtccgtggaagagaatcaccccttcacactgagagcccctatccagagaatctacggcgtgcgctataccgagacatggtcctttctgcccagcctgacatgtaccggggatgccgctcctgccatccagcacatttgcctgaagcacaccacctgtttccaggacgtggtggtggatgtggactgcgccgagaacaccaaagaggatcagctggccgagatcagctaccggttccagggaaagaaagaggccgaccagccttggatcgtggtcaacaccagcacactgttcgacgagctggaactggaccctcctgagattgaacccggggtgctgaaggtgctgagaaccgagaagcagtacctgggagtgtacatctggaacatgagaggcagcgacggcacctctacctacgccacctttctggtcacatggaagggcgacgagaaaacacggaaccccacaccagctgtgacccctcaacctagaggcgccgagtttcacatgtggaattaccacagccacgtgttcagcgtgggcgatacctttagcctggccatgcatctgcagtacaagatccacgaggcccctttcgacctgctgctggaatggctgtacgtgcccatcgatcctacctgccagcctatgcggctgtactccacctgtctgtatcaccccaacgctccccagtgcctgagccacatgaatagcggctgcaccttcacaagccctcacctggctcagcgagtggccagcacagtgtaccagaattgcgagcacgccgacaattacaccgcctactgtctgggcatcagccacatggaacctagcttcggcctgatcctgcacgatggcggcacaaccctgaagttcgtggatacccctgagagcctgagcggcctgtatgtgttcgtggtgtacttcaacggccacgtggaagccgtggcctacaccgtggtgtctaccgtggaccacttcgtgaacgccatcgaggaaagaggcttccctccaactgctggacagcctcctgccaccaccaagcctaaagaaatcacacccgtgaatcccggcacaagcccactgcttagatacgccgcttggacaggcggactggctgctgttgttctgctgtgcctggtcatcttcctgatctgcaccgccaagcggatgagagtgaaggccatgtactatgccggcctgcctgtggacgacttcgaggatagcgagagcaccgacaccgaggaagagttcggcaacgccattggaggatctcacggcggcagcagctataccgtgtacatcgacaagacccggtgagctggagcctcggtggccatgcttcttgccccttgggcctccccccagcccctcctccccttcctgcacccgtacccccgtggtctttgaataaagtctgagtgggcggcaaaaaaaaaaaaaaaaaaaaaaaaaaaaaaaaaaaaaaaaaaaaaaaaaaaaaaaaaaaaaaaaaaaaaaaaaaaaaaaaaaaaaaaaaaaaaaaaaaaaaaaaaaaaaa

SEQ ID NO: 53 - DNA, 2128 bp, synthetic construct
  source 1..2128: mol_type = other DNA
agactcctccccatcctctccctctgtccctctgtccctctgaccctgcactgtcccagcaccgccaccatgggcaccgtgaacaagcctgttgtgggcgtgctgatgggcttcggcatcatcacaggcaccctgcggatcaccaatcctgtgcgggctagcgtgctgagatacgacgacttccacatcgacgaggacaagctggacaccaacagcgtgtacgagccctactaccacagcgatcacgccgagtctagctgggtcaacagaggcgagagcagcagaaaggcctacgaccacaacagcccctacatctggccccggaacgactacgatggcttcctggaaaatgcccacgagcaccacggcgtgtacaatcaaggcagaggcatcgacagcggcgagagactgatgcagcctacacagatgagcgcccaagaggacctgggagatgataccggcatccacgtgatccccacactgaacggcgacgacagacacaagatcgtgaacgtggaccagcggcagtacggcgacgtgttcaagggcgacctgaatcctaagcctcagggccagcgcctgatcgaggtgtccgtggaagagaatcaccccttcacactgagagcccctatccagagaatctacggcgtgcgctataccgagacatggtcctttctgcccagcctgacatgtaccggggatgccgctcctgccatccagcacatttgcctgaagcacaccacctgtttccaggacgtggtggtggatgtggactgcgccgagaacaccaaagaggatcagctggccgagatcagctaccggttccagggaaagaaagaggccgaccagccttggatcgtggtcaacaccagcacactgttcgacgagctggaactggaccctcctgagattgaacccggggtgctgaaggtgctgagaaccgagaagcagtacctgggagtgtacatctggaacatgagaggcagcgacggcacctctacctacgccacctttctggtcacatggaagggcgacgagaaaacacggaaccccacaccagctgtgacccctcaacctagaggcgccgagtttcacatgtggaattaccacagccacgtgttcagcgtgggcgatacctttagcctggccatgcatctgcagtacaagatccacgaggcccctttcgacctgctgctggaatggctgtacgtgcccatcgatcctacctgccagcctatgcggctgtactccacctgtctgtatcaccccaacgctccccagtgcctgagccacatgaatagcggctgcaccttcacaagccctcacctggctcagcgagtggccagcacagtgtaccagaattgcgagcacgccgacaattacaccgcctactgtctgggcatcagccacatggaacctagcttcggcctgatcctgcacgatggcggcacaaccctgaagttcgtggatacccctgagagcctgagcggcctgtatgtgttcgtggtgtacttcaacggccacgtggaagccgtggcctacaccgtggtgtctaccgtggaccacttcgtgaacgccatcgaggaaagaggcttccctccaactgctggacagcctcctgccaccaccaagcctaaagaaatcacacccgtgaatcccggcacaagcccactgcttagatacgccgcttggacaggcggactggctgctgttgttctgctgtgcctggtcatcttcctgatctgcaccgccaagcggatgagagtgaaggccatgtactatgccggcctgcctgtggacgatttcgaagatgctgaagccgccgacgccgaggaagagtttggaaacgccattggcggaagccacggcggcagcagctacactgtgtacatcgacaagacccggtgagctggagcctcggtggccatgcttcttgccccttgggcctccccccagcccctcctccccttcctgcacccgtacccccgtggtctttgaataaagtctgagtgggcggcaaaaaaaaaaaaaaaaaaaaaaaaaaaaaaaaaaaaaaaaaaaaaaaaaaaaaaaaaaaaaaaaaaaaaaaaaaaaaaaaaaaaaaaaaaaaaaaaaaaaaaaaaaaaaa

SEQ ID NO: 54 - DNA, 1839 bp, synthetic construct
  source 1..1839: mol_type = other DNA
atgggcaccgtgaacaagcctgttgtgggcgtgctgatgggcttcggcatcatcacaggcaccctgcggatcaccaatcctgtgcgggctagcgtgctgagatacgacgacttccacatcgacgaggacaagctggacaccaacagcgtgtacgagccctactaccacagcgatcacgccgagtctagctgggtcaacagaggcgagagcagcagaaaggcctacgaccacaacagcccctacatctggccccggaacgactacgatggcttcctggaaaatgcccacgagcaccacggcgtgtacaatcaaggcagaggcatcgacagcggcgagagactgatgcagcctacacagatgagcgcccaagaggacctgggagatgataccggcatccacgtgatccccacactgaacggcgacgacagacacaagatcgtgaacgtggaccagcggcagtacggcgacgtgttcaagggcgacctgaatcctaagcctcagggccagcgcctgatcgaggtgtccgtggaagagaatcaccccttcacactgagagcccctatccagagaatctacggcgtgcgctataccgagacatggtcctttctgcccagcctgacatgtaccggggatgccgctcctgccatccagcacatttgcctgaagcacaccacctgtttccaggacgtggtggtggatgtggactgcgccgagaacaccaaagaggatcagctggccgagatcagctaccggttccagggaaagaaagaggccgaccagccttggatcgtggtcaacaccagcacactgttcgacgagctggaactggaccctcctgagattgaacccggggtgctgaaggtgctgagaaccgagaagcagtacctgggagtgtacatctggaacatgagaggcagcgacggcacctctacctacgccacctttctggtcacatggaagggcgacgagaaaacacggaaccccacaccagctgtgacccctcaacctagaggcgccgagtttcacatgtggaattaccacagccacgtgttcagcgtgggcgatacctttagcctggccatgcatctgcagtacaagatccacgaggcccctttcgacctgctgctggaatggctgtacgtgcccatcgatcctacctgccagcctatgcggctgtactccacctgtctgtatcaccccaacgctccccagtgcctgagccacatgaatagcggctgcaccttcacaagccctcacctggctcagcgagtggccagcacagtgtaccagaattgcgagcacgccgacaattacaccgcctactgtctgggcatcagccacatggaacctagcttcggcctgatcctgcacgatggcggcacaaccctgaagttcgtggatacccctgagagcctgagcggcctgtatgtgttcgtggtgtacttcaacggccacgtggaagccgtggcctacaccgtggtgtctaccgtggaccacttcgtgaacgccatcgaggaaagaggcttccctccaactgctggacagcctcctgccaccaccaagcctaaagaaatcacacccgtgaatcccggcacaagcccactgcttagatacgccgcttggacaggcggactggctgctgttgttctgctgtgcctggtcatcttcctgatctgcaccgccaagcggatgagagtgaaggccatgtactatgccggcctgcctgtggacgatttcgaagatgctgaagccgccgacgccgaggaagagtttggaaacgccattggcggaagccacggcggcagcagctacactgtgtacatcgacaagacccggtga

SEQ ID NO: 55 - protein, 612 aa, synthetic construct
MGTVNKPVVGVLMGFGIITGTLRITNPVRASVLRYDDFHIDEDKLDTNSVYEPYYHSDHAESSWVNRGESSRKAYDHNSPYIWPRNDYDGFLENAHEHHGVYNQGRGIDSGERLMQPTQMSAQEDLGDDTGIHVIPTLNGDDRHKIVNVDQRQYGDVFKGDLNPKPQGQRLIEVSVEENHPFTLRAPIQRIYGVRYTETWSFLPSLTCTGDAAPAIQHICLKHTTCFQDVVVDVDCAENTKEDQLAEISYRFQGKKEADQPWIVVNTSTLFDELELDPPEIEPGVLKVLRTEKQYLGVYIWNMRGSDGTSTYATFLVTWKGDEKTRNPTPAVTPQPRGAEFHMWNYHSHVFSVGDTFSLAMHLQYKIHEAPFDLLLEWLYVPIDPTCQPMRLYSTCLYHPNAPQCLSHMNSGCTFTSPHLAQRVASTVYQNCEHADNYTAYCLGISHMEPSFGLILHDGGTTLKFVDTPESLSGLYVFVVYFNGHVEAVAYTVVSTVDHFVNAIEERGFPPTAGQPPATTKPKEITPVNPGTSPLLRYAAWTGGLAAVVLLCLVIFLICTAKRMRVKAMYYAGLPVDDFEDAEAADAEEEFGNAIGGSHGGSSYTVYIDKTR

SEQ ID NO: 56 - RNA, 2128 nt, synthetic construct
  source 1..2128: mol_type = other RNA
agactcctccccatcctctccctctgtccctctgtccctctgaccctgcactgtcccagcaccgccaccatgggcaccgtgaacaagcctgttgtgggcgtgctgatgggcttcggcatcatcacaggcaccctgcggatcaccaatcctgtgcgggctagcgtgctgagatacgacgacttccacatcgacgaggacaagctggacaccaacagcgtgtacgagccctactaccacagcgatcacgccgagtctagctgggtcaacagaggcgagagcagcagaaaggcctacgaccacaacagcccctacatctggccccggaacgactacgatggcttcctggaaaatgcccacgagcaccacggcgtgtacaatcaaggcagaggcatcgacagcggcgagagactgatgcagcctacacagatgagcgcccaagaggacctgggagatgataccggcatccacgtgatccccacactgaacggcgacgacagacacaagatcgtgaacgtggaccagcggcagtacggcgacgtgttcaagggcgacctgaatcctaagcctcagggccagcgcctgatcgaggtgtccgtggaagagaatcaccccttcacactgagagcccctatccagagaatctacggcgtgcgctataccgagacatggtcctttctgcccagcctgacatgtaccggggatgccgctcctgccatccagcacatttgcctgaagcacaccacctgtttccaggacgtggtggtggatgtggactgcgccgagaacaccaaagaggatcagctggccgagatcagctaccggttccagggaaagaaagaggccgaccagccttggatcgtggtcaacaccagcacactgttcgacgagctggaactggaccctcctgagattgaacccggggtgctgaaggtgctgagaaccgagaagcagtacctgggagtgtacatctggaacatgagaggcagcgacggcacctctacctacgccacctttctggtcacatggaagggcgacgagaaaacacggaaccccacaccagctgtgacccctcaacctagaggcgccgagtttcacatgtggaattaccacagccacgtgttcagcgtgggcgatacctttagcctggccatgcatctgcagtacaagatccacgaggcccctttcgacctgctgctggaatggctgtacgtgcccatcgatcctacctgccagcctatgcggctgtactccacctgtctgtatcaccccaacgctccccagtgcctgagccacatgaatagcggctgcaccttcacaagccctcacctggctcagcgagtggccagcacagtgtaccagaattgcgagcacgccgacaattacaccgcctactgtctgggcatcagccacatggaacctagcttcggcctgatcctgcacgatggcggcacaaccctgaagttcgtggatacccctgagagcctgagcggcctgtatgtgttcgtggtgtacttcaacggccacgtggaagccgtggcctacaccgtggtgtctaccgtggaccacttcgtgaacgccatcgaggaaagaggcttccctccaactgctggacagcctcctgccaccaccaagcctaaagaaatcacacccgtgaatcccggcacaagcccactgcttagatacgccgcttggacaggcggactggctgctgttgttctgctgtgcctggtcatcttcctgatctgcaccgccaagcggatgagagtgaaggccatgtactatgccggcctgcctgtggacgatttcgaagatgctgaagccgccgacgccgaggaagagtttggaaacgccattggcggaagccacggcggcagcagctacactgtgtacatcgacaagacccggtgagctggagcctcggtggccatgcttcttgccccttgggcctccccccagcccctcctccccttcctgcacccgtacccccgtggtctttgaataaagtctgagtgggcggcaaaaaaaaaaaaaaaaaaaaaaaaaaaaaaaaaaaaaaaaaaaaaaaaaaaaaaaaaaaaaaaaaaaaaaaaaaaaaaaaaaaaaaaaaaaaaaaaaaaaaaaaaaaaaa

SEQ ID NO: 57 - DNA, 2017 bp, synthetic construct
  source 1..2017: mol_type = other DNA
agactcctccccatcctctccctctgtccctctgtccctctgaccctgcactgtcccagcaccgccaccatgggcaccgtgaacaagcctgttgtgggcgtgctgatgggcttcggcatcatcacaggcaccctgcggatcaccaatcctgtgcgggctagcgtgctgagatacgacgacttccacatcgacgaggacaagctggacaccaacagcgtgtacgagccctactaccacagcgatcacgccgagtctagctgggtcaacagaggcgagagcagcagaaaggcctacgaccacaacagcccctacatctggccccggaacgactacgatggcttcctggaaaatgcccacgagcaccacggcgtgtacaatcaaggcagaggcatcgacagcggcgagagactgatgcagcctacacagatgagcgcccaagaggacctgggagatgataccggcatccacgtgatccccacactgaacggcgacgacagacacaagatcgtgaacgtggaccagcggcagtacggcgacgtgttcaagggcgacctgaatcctaagcctcagggccagcgcctgatcgaggtgtccgtggaagagaatcaccccttcacactgagagcccctatccagagaatctacggcgtgcgctataccgagacatggtcctttctgcccagcctgacatgtaccggggatgccgctcctgccatccagcacatttgcctgaagcacaccacctgtttccaggacgtggtggtggatgtggactgcgccgagaacaccaaagaggatcagctggccgagatcagctaccggttccagggaaagaaagaggccgaccagccttggatcgtggtcaacaccagcacactgttcgacgagctggaactggaccctcctgagattgaacccggggtgctgaaggtgctgagaaccgagaagcagtacctgggagtgtacatctggaacatgagaggcagcgacggcacctctacctacgccacctttctggtcacatggaagggcgacgagaaaacacggaaccccacaccagctgtgacccctcaacctagaggcgccgagtttcacatgtggaattaccacagccacgtgttcagcgtgggcgatacctttagcctggccatgcatctgcagtacaagatccacgaggcccctttcgacctgctgctggaatggctgtacgtgcccatcgatcctacctgccagcctatgcggctgtactccacctgtctgtatcaccccaacgctccccagtgcctgagccacatgaatagcggctgcaccttcacaagccctcacctggctcagcgagtggccagcacagtgtaccagaattgcgagcacgccgacaattacaccgcctactgtctgggcatcagccacatggaacctagcttcggcctgatcctgcacgatggcggcacaaccctgaagttcgtggatacccctgagagcctgagcggcctgtatgtgttcgtggtgtacttcaacggccacgtggaagccgtggcctacaccgtggtgtctaccgtggaccacttcgtgaacgccatcgaggaaagaggcttccctccaactgctggacagcctcctgccaccaccaagcctaaagaaatcacacccgtgaatcccggcacaagcccactgcttagatacgccgcttggacaggcggactggctgctgttgttctgctgtgcctggtcatcttcctgatctgcaccgccaagcggatgagagtgaaggcctacagagtggacaagtgataataggctggagcctcggtggccatgcttcttgccccttgggcctccccccagcccctcctccccttcctgcacccgtacccccgtggtctttgaataaagtctgagtgggcggcaaaaaaaaaaaaaaaaaaaaaaaaaaaaaaaaaaaaaaaaaaaaaaaaaaaaaaaaaaaaaaaaaaaaaaaaaaaaaaaaaaaaaaaaaaaaaaaaaaaaaaaaaaaaaa

SEQ ID NO: 58 - DNA, 1722 bp, synthetic construct
  source 1..1722: mol_type = other DNA
atgggcaccgtgaacaagcctgttgtgggcgtgctgatgggcttcggcatcatcacaggcaccctgcggatcaccaatcctgtgcgggctagcgtgctgagatacgacgacttccacatcgacgaggacaagctggacaccaacagcgtgtacgagccctactaccacagcgatcacgccgagtctagctgggtcaacagaggcgagagcagcagaaaggcctacgaccacaacagcccctacatctggccccggaacgactacgatggcttcctggaaaatgcccacgagcaccacggcgtgtacaatcaaggcagaggcatcgacagcggcgagagactgatgcagcctacacagatgagcgcccaagaggacctgggagatgataccggcatccacgtgatccccacactgaacggcgacgacagacacaagatcgtgaacgtggaccagcggcagtacggcgacgtgttcaagggcgacctgaatcctaagcctcagggccagcgcctgatcgaggtgtccgtggaagagaatcaccccttcacactgagagcccctatccagagaatctacggcgtgcgctataccgagacatggtcctttctgcccagcctgacatgtaccggggatgccgctcctgccatccagcacatttgcctgaagcacaccacctgtttccaggacgtggtggtggatgtggactgcgccgagaacaccaaagaggatcagctggccgagatcagctaccggttccagggaaagaaagaggccgaccagccttggatcgtggtcaacaccagcacactgttcgacgagctggaactggaccctcctgagattgaacccggggtgctgaaggtgctgagaaccgagaagcagtacctgggagtgtacatctggaacatgagaggcagcgacggcacctctacctacgccacctttctggtcacatggaagggcgacgagaaaacacggaaccccacaccagctgtgacccctcaacctagaggcgccgagtttcacatgtggaattaccacagccacgtgttcagcgtgggcgatacctttagcctggccatgcatctgcagtacaagatccacgaggcccctttcgacctgctgctggaatggctgtacgtgcccatcgatcctacctgccagcctatgcggctgtactccacctgtctgtatcaccccaacgctccccagtgcctgagccacatgaatagcggctgcaccttcacaagccctcacctggctcagcgagtggccagcacagtgtaccagaattgcgagcacgccgacaattacaccgcctactgtctgggcatcagccacatggaacctagcttcggcctgatcctgcacgatggcggcacaaccctgaagttcgtggatacccctgagagcctgagcggcctgtatgtgttcgtggtgtacttcaacggccacgtggaagccgtggcctacaccgtggtgtctaccgtggaccacttcgtgaacgccatcgaggaaagaggcttccctccaactgctggacagcctcctgccaccaccaagcctaaagaaatcacacccgtgaatcccggcacaagcccactgcttagatacgccgcttggacaggcggactggctgctgttgttctgctgtgcctggtcatcttcctgatctgcaccgccaagcggatgagagtgaaggcctacagagtggacaagtga

SEQ ID NO: 59 - protein, 573 aa, synthetic construct
MGTVNKPVVGVLMGFGIITGTLRITNPVRASVLRYDDFHIDEDKLDTNSVYEPYYHSDHAESSWVNRGESSRKAYDHNSPYIWPRNDYDGFLENAHEHHGVYNQGRGIDSGERLMQPTQMSAQEDLGDDTGIHVIPTLNGDDRHKIVNVDQRQYGDVFKGDLNPKPQGQRLIEVSVEENHPFTLRAPIQRIYGVRYTETWSFLPSLTCTGDAAPAIQHICLKHTTCFQDVVVDVDCAENTKEDQLAEISYRFQGKKEADQPWIVVNTSTLFDELELDPPEIEPGVLKVLRTEKQYLGVYIWNMRGSDGTSTYATFLVTWKGDEKTRNPTPAVTPQPRGAEFHMWNYHSHVFSVGDTFSLAMHLQYKIHEAPFDLLLEWLYVPIDPTCQPMRLYSTCLYHPNAPQCLSHMNSGCTFTSPHLAQRVASTVYQNCEHADNYTAYCLGISHMEPSFGLILHDGGTTLKFVDTPESLSGLYVFVVYFNGHVEAVAYTVVSTVDHFVNAIEERGFPPTAGQPPATTKPKEITPVNPGTSPLLRYAAWTGGLAAVVLLCLVIFLICTAKRMRVKAYRVDK

SEQ ID NO: 60 - RNA, 2017 nt, synthetic construct
  source 1..2017: mol_type = other RNA
agactcctccccatcctctccctctgtccctctgtccctctgaccctgcactgtcccagcaccgccaccatgggcaccgtgaacaagcctgttgtgggcgtgctgatgggcttcggcatcatcacaggcaccctgcggatcaccaatcctgtgcgggctagcgtgctgagatacgacgacttccacatcgacgaggacaagctggacaccaacagcgtgtacgagccctactaccacagcgatcacgccgagtctagctgggtcaacagaggcgagagcagcagaaaggcctacgaccacaacagcccctacatctggccccggaacgactacgatggcttcctggaaaatgcccacgagcaccacggcgtgtacaatcaaggcagaggcatcgacagcggcgagagactgatgcagcctacacagatgagcgcccaagaggacctgggagatgataccggcatccacgtgatccccacactgaacggcgacgacagacacaagatcgtgaacgtggaccagcggcagtacggcgacgtgttcaagggcgacctgaatcctaagcctcagggccagcgcctgatcgaggtgtccgtggaagagaatcaccccttcacactgagagcccctatccagagaatctacggcgtgcgctataccgagacatggtcctttctgcccagcctgacatgtaccggggatgccgctcctgccatccagcacatttgcctgaagcacaccacctgtttccaggacgtggtggtggatgtggactgcgccgagaacaccaaagaggatcagctggccgagatcagctaccggttccagggaaagaaagaggccgaccagccttggatcgtggtcaacaccagcacactgttcgacgagctggaactggaccctcctgagattgaacccggggtgctgaaggtgctgagaaccgagaagcagtacctgggagtgtacatctggaacatgagaggcagcgacggcacctctacctacgccacctttctggtcacatggaagggcgacgagaaaacacggaaccccacaccagctgtgacccctcaacctagaggcgccgagtttcacatgtggaattaccacagccacgtgttcagcgtgggcgatacctttagcctggccatgcatctgcagtacaagatccacgaggcccctttcgacctgctgctggaatggctgtacgtgcccatcgatcctacctgccagcctatgcggctgtactccacctgtctgtatcaccccaacgctccccagtgcctgagccacatgaatagcggctgcaccttcacaagccctcacctggctcagcgagtggccagcacagtgtaccagaattgcgagcacgccgacaattacaccgcctactgtctgggcatcagccacatggaacctagcttcggcctgatcctgcacgatggcggcacaaccctgaagttcgtggatacccctgagagcctgagcggcctgtatgtgttcgtggtgtacttcaacggccacgtggaagccgtggcctacaccgtggtgtctaccgtggaccacttcgtgaacgccatcgaggaaagaggcttccctccaactgctggacagcctcctgccaccaccaagcctaaagaaatcacacccgtgaatcccggcacaagcccactgcttagatacgccgcttggacaggcggactggctgctgttgttctgctgtgcctggtcatcttcctgatctgcaccgccaagcggatgagagtgaaggcctacagagtggacaagtgataataggctggagcctcggtggccatgcttcttgccccttgggcctccccccagcccctcctccccttcctgcacccgtacccccgtggtctttgaataaagtctgagtgggcggcaaaaaaaaaaaaaaaaaaaaaaaaaaaaaaaaaaaaaaaaaaaaaaaaaaaaaaaaaaaaaaaaaaaaaaaaaaaaaaaaaaaaaaaaaaaaaaaaaaaaaaaaaaaaaa

SEQ ID NO: 61 - DNA, 2017 bp, synthetic construct
  source 1..2017: mol_type = other DNA
agactcctccccatcctctccctctgtccctctgtccctctgaccctgcactgtcccagcaccgccaccatgggcaccgtgaacaagcctgttgtgggcgtgctgatgggcttcggcatcatcacaggcaccctgcggatcaccaatcctgtgcgggctagcgtgctgagatacgacgacttccacatcgacgaggacaagctggacaccaacagcgtgtacgagccctactaccacagcgatcacgccgagtctagctgggtcaacagaggcgagagcagcagaaaggcctacgaccacaacagcccctacatctggccccggaacgactacgatggcttcctggaaaatgcccacgagcaccacggcgtgtacaatcaaggcagaggcatcgacagcggcgagagactgatgcagcctacacagatgagcgcccaagaggacctgggagatgataccggcatccacgtgatccccacactgaacggcgacgacagacacaagatcgtgaacgtggaccagcggcagtacggcgacgtgttcaagggcgacctgaatcctaagcctcagggccagcgcctgatcgaggtgtccgtggaagagaatcaccccttcacactgagagcccctatccagagaatctacggcgtgcgctataccgagacatggtcctttctgcccagcctgacatgtaccggggatgccgctcctgccatccagcacatttgcctgaagcacaccacctgtttccaggacgtggtggtggatgtggactgcgccgagaacaccaaagaggatcagctggccgagatcagctaccggttccagggaaagaaagaggccgaccagccttggatcgtggtcaacaccagcacactgttcgacgagctggaactggaccctcctgagattgaacccggggtgctgaaggtgctgagaaccgagaagcagtacctgggagtgtacatctggaacatgagaggcagcgacggcacctctacctacgccacctttctggtcacatggaagggcgacgagaaaacacggaaccccacaccagctgtgacccctcaacctagaggcgccgagtttcacatgtggaattaccacagccacgtgttcagcgtgggcgatacctttagcctggccatgcatctgcagtacaagatccacgaggcccctttcgacctgctgctggaatggctgtacgtgcccatcgatcctacctgccagcctatgcggctgtactccacctgtctgtatcaccccaacgctccccagtgcctgagccacatgaatagcggctgcaccttcacaagccctcacctggctcagcgagtggccagcacagtgtaccagaattgcgagcacgccgacaattacaccgcctactgtctgggcatcagccacatggaacctagcttcggcctgatcctgcacgatggcggcacaaccctgaagttcgtggatacccctgagagcctgagcggcctgtatgtgttcgtggtgtacttcaacggccacgtggaagccgtggcctacaccgtggtgtctaccgtggaccacttcgtgaacgccatcgaggaaagaggcttccctccaactgctggacagcctcctgccaccaccaagcctaaagaaatcacacccgtgaatcccggcacaagcccactgcttagatacgccgcttggacaggcggactggctgctgttgttctgctgtgcctggtcatcttcctgatctgcaccgccaagcggatgagagtgaaggactacagagtggacaagtgataataggctggagcctcggtggccatgcttcttgccccttgggcctccccccagcccctcctccccttcctgcacccgtacccccgtggtctttgaataaagtctgagtgggcggcaaaaaaaaaaaaaaaaaaaaaaaaaaaaaaaaaaaaaaaaaaaaaaaaaaaaaaaaaaaaaaaaaaaaaaaaaaaaaaaaaaaaaaaaaaaaaaaaaaaaaaaaaaaaaa

SEQ ID NO: 62 - DNA, 1722 bp, synthetic construct
  source 1..1722: mol_type = other DNA
atgggcaccgtgaacaagcctgttgtgggcgtgctgatgggcttcggcatcatcacaggcaccctgcggatcaccaatcctgtgcgggctagcgtgctgagatacgacgacttccacatcgacgaggacaagctggacaccaacagcgtgtacgagccctactaccacagcgatcacgccgagtctagctgggtcaacagaggcgagagcagcagaaaggcctacgaccacaacagcccctacatctggccccggaacgactacgatggcttcctggaaaatgcccacgagcaccacggcgtgtacaatcaaggcagaggcatcgacagcggcgagagactgatgcagcctacacagatgagcgcccaagaggacctgggagatgataccggcatccacgtgatccccacactgaacggcgacgacagacacaagatcgtgaacgtggaccagcggcagtacggcgacgtgttcaagggcgacctgaatcctaagcctcagggccagcgcctgatcgaggtgtccgtggaagagaatcaccccttcacactgagagcccctatccagagaatctacggcgtgcgctataccgagacatggtcctttctgcccagcctgacatgtaccggggatgccgctcctgccatccagcacatttgcctgaagcacaccacctgtttccaggacgtggtggtggatgtggactgcgccgagaacaccaaagaggatcagctggccgagatcagctaccggttccagggaaagaaagaggccgaccagccttggatcgtggtcaacaccagcacactgttcgacgagctggaactggaccctcctgagattgaacccggggtgctgaaggtgctgagaaccgagaagcagtacctgggagtgtacatctggaacatgagaggcagcgacggcacctctacctacgccacctttctggtcacatggaagggcgacgagaaaacacggaaccccacaccagctgtgacccctcaacctagaggcgccgagtttcacatgtggaattaccacagccacgtgttcagcgtgggcgatacctttagcctggccatgcatctgcagtacaagatccacgaggcccctttcgacctgctgctggaatggctgtacgtgcccatcgatcctacctgccagcctatgcggctgtactccacctgtctgtatcaccccaacgctccccagtgcctgagccacatgaatagcggctgcaccttcacaagccctcacctggctcagcgagtggccagcacagtgtaccagaattgcgagcacgccgacaattacaccgcctactgtctgggcatcagccacatggaacctagcttcggcctgatcctgcacgatggcggcacaaccctgaagttcgtggatacccctgagagcctgagcggcctgtatgtgttcgtggtgtacttcaacggccacgtggaagccgtggcctacaccgtggtgtctaccgtggaccacttcgtgaacgccatcgaggaaagaggcttccctccaactgctggacagcctcctgccaccaccaagcctaaagaaatcacacccgtgaatcccggcacaagcccactgcttagatacgccgcttggacaggcggactggctgctgttgttctgctgtgcctggtcatcttcctgatctgcaccgccaagcggatgagagtgaaggactacagagtggacaagtga

SEQ ID NO: 63 - protein, 573 aa, synthetic construct
MGTVNKPVVGVLMGFGIITGTLRITNPVRASVLRYDDFHIDEDKLDTNSVYEPYYHSDHAESSWVNRGESSRKAYDHNSPYIWPRNDYDGFLENAHEHHGVYNQGRGIDSGERLMQPTQMSAQEDLGDDTGIHVIPTLNGDDRHKIVNVDQRQYGDVFKGDLNPKPQGQRLIEVSVEENHPFTLRAPIQRIYGVRYTETWSFLPSLTCTGDAAPAIQHICLKHTTCFQDVVVDVDCAENTKEDQLAEISYRFQGKKEADQPWIVVNTSTLFDELELDPPEIEPGVLKVLRTEKQYLGVYIWNMRGSDGTSTYATFLVTWKGDEKTRNPTPAVTPQPRGAEFHMWNYHSHVFSVGDTFSLAMHLQYKIHEAPFDLLLEWLYVPIDPTCQPMRLYSTCLYHPNAPQCLSHMNSGCTFTSPHLAQRVASTVYQNCEHADNYTAYCLGISHMEPSFGLILHDGGTTLKFVDTPESLSGLYVFVVYFNGHVEAVAYTVVSTVDHFVNAIEERGFPPTAGQPPATTKPKEITPVNPGTSPLLRYAAWTGGLAAVVLLCLVIFLICTAKRMRVKDYRVDK

SEQ ID NO: 64 - RNA, 2017 nt, synthetic construct
  source 1..2017: mol_type = other RNA
agactcctccccatcctctccctctgtccctctgtccctctgaccctgcactgtcccagcaccgccaccatgggcaccgtgaacaagcctgttgtgggcgtgctgatgggcttcggcatcatcacaggcaccctgcggatcaccaatcctgtgcgggctagcgtgctgagatacgacgacttccacatcgacgaggacaagctggacaccaacagcgtgtacgagccctactaccacagcgatcacgccgagtctagctgggtcaacagaggcgagagcagcagaaaggcctacgaccacaacagcccctacatctggccccggaacgactacgatggcttcctggaaaatgcccacgagcaccacggcgtgtacaatcaaggcagaggcatcgacagcggcgagagactgatgcagcctacacagatgagcgcccaagaggacctgggagatgataccggcatccacgtgatccccacactgaacggcgacgacagacacaagatcgtgaacgtggaccagcggcagtacggcgacgtgttcaagggcgacctgaatcctaagcctcagggccagcgcctgatcgaggtgtccgtggaagagaatcaccccttcacactgagagcccctatccagagaatctacggcgtgcgctataccgagacatggtcctttctgcccagcctgacatgtaccggggatgccgctcctgccatccagcacatttgcctgaagcacaccacctgtttccaggacgtggtggtggatgtggactgcgccgagaacaccaaagaggatcagctggccgagatcagctaccggttccagggaaagaaagaggccgaccagccttggatcgtggtcaacaccagcacactgttcgacgagctggaactggaccctcctgagattgaacccggggtgctgaaggtgctgagaaccgagaagcagtacctgggagtgtacatctggaacatgagaggcagcgacggcacctctacctacgccacctttctggtcacatggaagggcgacgagaaaacacggaaccccacaccagctgtgacccctcaacctagaggcgccgagtttcacatgtggaattaccacagccacgtgttcagcgtgggcgatacctttagcctggccatgcatctgcagtacaagatccacgaggcccctttcgacctgctgctggaatggctgtacgtgcccatcgatcctacctgccagcctatgcggctgtactccacctgtctgtatcaccccaacgctccccagtgcctgagccacatgaatagcggctgcaccttcacaagccctcacctggctcagcgagtggccagcacagtgtaccagaattgcgagcacgccgacaattacaccgcctactgtctgggcatcagccacatggaacctagcttcggcctgatcctgcacgatggcggcacaaccctgaagttcgtggatacccctgagagcctgagcggcctgtatgtgttcgtggtgtacttcaacggccacgtggaagccgtggcctacaccgtggtgtctaccgtggaccacttcgtgaacgccatcgaggaaagaggcttccctccaactgctggacagcctcctgccaccaccaagcctaaagaaatcacacccgtgaatcccggcacaagcccactgcttagatacgccgcttggacaggcggactggctgctgttgttctgctgtgcctggtcatcttcctgatctgcaccgccaagcggatgagagtgaaggactacagagtggacaagtgataataggctggagcctcggtggccatgcttcttgccccttgggcctccccccagcccctcctccccttcctgcacccgtacccccgtggtctttgaataaagtctgagtgggcggcaaaaaaaaaaaaaaaaaaaaaaaaaaaaaaaaaaaaaaaaaaaaaaaaaaaaaaaaaaaaaaaaaaaaaaaaaaaaaaaaaaaaaaaaaaaaaaaaaaaaaaaaaaaaaa

SEQ ID NO: 65 - DNA, 2014 bp, synthetic construct
  source 1..2014: mol_type = other DNA
agactcctccccatcctctccctctgtccctctgtccctctgaccctgcactgtcccagcaccgccaccatgggcaccgtgaacaagcctgttgtgggcgtgctgatgggcttcggcatcatcacaggcaccctgcggatcaccaatcctgtgcgggctagcgtgctgagatacgacgacttccacatcgacgaggacaagctggacaccaacagcgtgtacgagccctactaccacagcgatcacgccgagtctagctgggtcaacagaggcgagagcagcagaaaggcctacgaccacaacagcccctacatctggccccggaacgactacgatggcttcctggaaaatgcccacgagcaccacggcgtgtacaatcaaggcagaggcatcgacagcggcgagagactgatgcagcctacacagatgagcgcccaagaggacctgggagatgataccggcatccacgtgatccccacactgaacggcgacgacagacacaagatcgtgaacgtggaccagcggcagtacggcgacgtgttcaagggcgacctgaatcctaagcctcagggccagcgcctgatcgaggtgtccgtggaagagaatcaccccttcacactgagagcccctatccagagaatctacggcgtgcgctataccgagacatggtcctttctgcccagcctgacatgtaccggggatgccgctcctgccatccagcacatttgcctgaagcacaccacctgtttccaggacgtggtggtggatgtggactgcgccgagaacaccaaagaggatcagctggccgagatcagctaccggttccagggaaagaaagaggccgaccagccttggatcgtggtcaacaccagcacactgttcgacgagctggaactggaccctcctgagattgaacccggggtgctgaaggtgctgagaaccgagaagcagtacctgggagtgtacatctggaacatgagaggcagcgacggcacctctacctacgccacctttctggtcacatggaagggcgacgagaaaacacggaaccccacaccagctgtgacccctcaacctagaggcgccgagtttcacatgtggaattaccacagccacgtgttcagcgtgggcgatacctttagcctggccatgcatctgcagtacaagatccacgaggcccctttcgacctgctgctggaatggctgtacgtgcccatcgatcctacctgccagcctatgcggctgtactccacctgtctgtatcaccccaacgctccccagtgcctgagccacatgaatagcggctgcaccttcacaagccctcacctggctcagcgagtggccagcacagtgtaccagaattgcgagcacgccgacaattacaccgcctactgtctgggcatcagccacatggaacctagcttcggcctgatcctgcacgatggcggcacaaccctgaagttcgtggatacccctgagagcctgagcggcctgtatgtgttcgtggtgtacttcaacggccacgtggaagccgtggcctacaccgtggtgtctaccgtggaccacttcgtgaacgccatcgaggaaagaggcttccctccaactgctggacagcctcctgccaccaccaagcctaaagaaatcacacccgtgaatcccggcacaagcccactgcttagatacgccgcttggacaggcggactggctgctgttgttctgctgtgcctggtcatcttcctgatctgcaccgccaagcggatgagagtgaagtacagagtggacaagtgataataggctggagcctcggtggccatgcttcttgccccttgggcctccccccagcccctcctccccttcctgcacccgtacccccgtggtctttgaataaagtctgagtgggcggcaaaaaaaaaaaaaaaaaaaaaaaaaaaaaaaaaaaaaaaaaaaaaaaaaaaaaaaaaaaaaaaaaaaaaaaaaaaaaaaaaaaaaaaaaaaaaaaaaaaaaaaaaaaaaa

SEQ ID NO: 66 - DNA, 1719 bp, synthetic construct
  source 1..1719: mol_type = other DNA
atgggcaccgtgaacaagcctgttgtgggcgtgctgatgggcttcggcatcatcacaggcaccctgcggatcaccaatcctgtgcgggctagcgtgctgagatacgacgacttccacatcgacgaggacaagctggacaccaacagcgtgtacgagccctactaccacagcgatcacgccgagtctagctgggtcaacagaggcgagagcagcagaaaggcctacgaccacaacagcccctacatctggccccggaacgactacgatggcttcctggaaaatgcccacgagcaccacggcgtgtacaatcaaggcagaggcatcgacagcggcgagagactgatgcagcctacacagatgagcgcccaagaggacctgggagatgataccggcatccacgtgatccccacactgaacggcgacgacagacacaagatcgtgaacgtggaccagcggcagtacggcgacgtgttcaagggcgacctgaatcctaagcctcagggccagcgcctgatcgaggtgtccgtggaagagaatcaccccttcacactgagagcccctatccagagaatctacggcgtgcgctataccgagacatggtcctttctgcccagcctgacatgtaccggggatgccgctcctgccatccagcacatttgcctgaagcacaccacctgtttccaggacgtggtggtggatgtggactgcgccgagaacaccaaagaggatcagctggccgagatcagctaccggttccagggaaagaaagaggccgaccagccttggatcgtggtcaacaccagcacactgttcgacgagctggaactggaccctcctgagattgaacccggggtgctgaaggtgctgagaaccgagaagcagtacctgggagtgtacatctggaacatgagaggcagcgacggcacctctacctacgccacctttctggtcacatggaagggcgacgagaaaacacggaaccccacaccagctgtgacccctcaacctagaggcgccgagtttcacatgtggaattaccacagccacgtgttcagcgtgggcgatacctttagcctggccatgcatctgcagtacaagatccacgaggcccctttcgacctgctgctggaatggctgtacgtgcccatcgatcctacctgccagcctatgcggctgtactccacctgtctgtatcaccccaacgctccccagtgcctgagccacatgaatagcggctgcaccttcacaagccctcacctggctcagcgagtggccagcacagtgtaccagaattgcgagcacgccgacaattacaccgcctactgtctgggcatcagccacatggaacctagcttcggcctgatcctgcacgatggcggcacaaccctgaagttcgtggatacccctgagagcctgagcggcctgtatgtgttcgtggtgtacttcaacggccacgtggaagccgtggcctacaccgtggtgtctaccgtggaccacttcgtgaacgccatcgaggaaagaggcttccctccaactgctggacagcctcctgccaccaccaagcctaaagaaatcacacccgtgaatcccggcacaagcccactgcttagatacgccgcttggacaggcggactggctgctgttgttctgctgtgcctggtcatcttcctgatctgcaccgccaagcggatgagagtgaagtacagagtggacaagtga

SEQ ID NO: 67 - protein, 572 aa, synthetic construct
MGTVNKPVVGVLMGFGIITGTLRITNPVRASVLRYDDFHIDEDKLDTNSVYEPYYHSDHAESSWVNRGESSRKAYDHNSPYIWPRNDYDGFLENAHEHHGVYNQGRGIDSGERLMQPTQMSAQEDLGDDTGIHVIPTLNGDDRHKIVNVDQRQYGDVFKGDLNPKPQGQRLIEVSVEENHPFTLRAPIQRIYGVRYTETWSFLPSLTCTGDAAPAIQHICLKHTTCFQDVVVDVDCAENTKEDQLAEISYRFQGKKEADQPWIVVNTSTLFDELELDPPEIEPGVLKVLRTEKQYLGVYIWNMRGSDGTSTYATFLVTWKGDEKTRNPTPAVTPQPRGAEFHMWNYHSHVFSVGDTFSLAMHLQYKIHEAPFDLLLEWLYVPIDPTCQPMRLYSTCLYHPNAPQCLSHMNSGCTFTSPHLAQRVASTVYQNCEHADNYTAYCLGISHMEPSFGLILHDGGTTLKFVDTPESLSGLYVFVVYFNGHVEAVAYTVVSTVDHFVNAIEERGFPPTAGQPPATTKPKEITPVNPGTSPLLRYAAWTGGLAAVVLLCLVIFLICTAKRMRVKYRVDK

SEQ ID NO: 68 - RNA, 2014 nt, synthetic construct
  source 1..2014: mol_type = other RNA
agactcctccccatcctctccctctgtccctctgtccctctgaccctgcactgtcccagcaccgccaccatgggcaccgtgaacaagcctgttgtgggcgtgctgatgggcttcggcatcatcacaggcaccctgcggatcaccaatcctgtgcgggctagcgtgctgagatacgacgacttccacatcgacgaggacaagctggacaccaacagcgtgtacgagccctactaccacagcgatcacgccgagtctagctgggtcaacagaggcgagagcagcagaaaggcctacgaccacaacagcccctacatctggccccggaacgactacgatggcttcctggaaaatgcccacgagcaccacggcgtgtacaatcaaggcagaggcatcgacagcggcgagagactgatgcagcctacacagatgagcgcccaagaggacctgggagatgataccggcatccacgtgatccccacactgaacggcgacgacagacacaagatcgtgaacgtggaccagcggcagtacggcgacgtgttcaagggcgacctgaatcctaagcctcagggccagcgcctgatcgaggtgtccgtggaagagaatcaccccttcacactgagagcccctatccagagaatctacggcgtgcgctataccgagacatggtcctttctgcccagcctgacatgtaccggggatgccgctcctgccatccagcacatttgcctgaagcacaccacctgtttccaggacgtggtggtggatgtggactgcgccgagaacaccaaagaggatcagctggccgagatcagctaccggttccagggaaagaaagaggccgaccagccttggatcgtggtcaacaccagcacactgttcgacgagctggaactggaccctcctgagattgaacccggggtgctgaaggtgctgagaaccgagaagcagtacctgggagtgtacatctggaacatgagaggcagcgacggcacctctacctacgccacctttctggtcacatggaagggcgacgagaaaacacggaaccccacaccagctgtgacccctcaacctagaggcgccgagtttcacatgtggaattaccacagccacgtgttcagcgtgggcgatacctttagcctggccatgcatctgcagtacaagatccacgaggcccctttcgacctgctgctggaatggctgtacgtgcccatcgatcctacctgccagcctatgcggctgtactccacctgtctgtatcaccccaacgctccccagtgcctgagccacatgaatagcggctgcaccttcacaagccctcacctggctcagcgagtggccagcacagtgtaccagaattgcgagcacgccgacaattacaccgcctactgtctgggcatcagccacatggaacctagcttcggcctgatcctgcacgatggcggcacaaccctgaagttcgtggatacccctgagagcctgagcggcctgtatgtgttcgtggtgtacttcaacggccacgtggaagccgtggcctacaccgtggtgtctaccgtggaccacttcgtgaacgccatcgaggaaagaggcttccctccaactgctggacagcctcctgccaccaccaagcctaaagaaatcacacccgtgaatcccggcacaagcccactgcttagatacgccgcttggacaggcggactggctgctgttgttctgctgtgcctggtcatcttcctgatctgcaccgccaagcggatgagagtgaagtacagagtggacaagtgataataggctggagcctcggtggccatgcttcttgccccttgggcctccccccagcccctcctccccttcctgcacccgtacccccgtggtctttgaataaagtctgagtgggcggcaaaaaaaaaaaaaaaaaaaaaaaaaaaaaaaaaaaaaaaaaaaaaaaaaaaaaaaaaaaaaaaaaaaaaaaaaaaaaaaaaaaaaaaaaaaaaaaaaaaaaaaaaaaaaa

SEQ ID NO: 69 - DNA, 2017 bp, synthetic construct
  source 1..2017: mol_type = other DNA
agactcctccccatcctctccctctgtccctctgtccctctgaccctgcactgtcccagcaccgccaccatgggcaccgtgaacaagcctgttgtgggcgtgctgatgggcttcggcatcatcacaggcaccctgcggatcaccaatcctgtgcgggctagcgtgctgagatacgacgacttccacatcgacgaggacaagctggacaccaacagcgtgtacgagccctactaccacagcgatcacgccgagtctagctgggtcaacagaggcgagagcagcagaaaggcctacgaccacaacagcccctacatctggccccggaacgactacgatggcttcctggaaaatgcccacgagcaccacggcgtgtacaatcaaggcagaggcatcgacagcggcgagagactgatgcagcctacacagatgagcgcccaagaggacctgggagatgataccggcatccacgtgatccccacactgaacggcgacgacagacacaagatcgtgaacgtggaccagcggcagtacggcgacgtgttcaagggcgacctgaatcctaagcctcagggccagcgcctgatcgaggtgtccgtggaagagaatcaccccttcacactgagagcccctatccagagaatctacggcgtgcgctataccgagacatggtcctttctgcccagcctgacatgtaccggggatgccgctcctgccatccagcacatttgcctgaagcacaccacctgtttccaggacgtggtggtggatgtggactgcgccgagaacaccaaagaggatcagctggccgagatcagctaccggttccagggaaagaaagaggccgaccagccttggatcgtggtcaacaccagcacactgttcgacgagctggaactggaccctcctgagattgaacccggggtgctgaaggtgctgagaaccgagaagcagtacctgggagtgtacatctggaacatgagaggcagcgacggcacctctacctacgccacctttctggtcacatggaagggcgacgagaaaacacggaaccccacaccagctgtgacccctcaacctagaggcgccgagtttcacatgtggaattaccacagccacgtgttcagcgtgggcgatacctttagcctggccatgcatctgcagtacaagatccacgaggcccctttcgacctgctgctggaatggctgtacgtgcccatcgatcctacctgccagcctatgcggctgtactccacctgtctgtatcaccccaacgctccccagtgcctgagccacatgaatagcggctgcaccttcacaagccctcacctggctcagcgagtggccagcacagtgtaccagaattgcgagcacgccgacaattacaccgcctactgtctgggcatcagccacatggaacctagcttcggcctgatcctgcacgatggcggcacaaccctgaagttcgtggatacccctgagagcctgagcggcctgtatgtgttcgtggtgtacttcaacggccacgtggaagccgtggcctacaccgtggtgtctaccgtggaccacttcgtgaacgccatcgaggaaagaggcttccctccaactgctggacagcctcctgccaccaccaagcctaaagaaatcacacccgtgaatcccggcacaagcccactgcttagatacgccgcttggacaggcggactggctgctgttgttctgctgtgcctggtcatcttcctgatctgcaccgccaagcggatgagagtgaaggccaagagagtggacaagtgataataggctggagcctcggtggccatgcttcttgccccttgggcctccccccagcccctcctccccttcctgcacccgtacccccgtggtctttgaataaagtctgagtgggcggcaaaaaaaaaaaaaaaaaaaaaaaaaaaaaaaaaaaaaaaaaaaaaaaaaaaaaaaaaaaaaaaaaaaaaaaaaaaaaaaaaaaaaaaaaaaaaaaaaaaaaaaaaaaaaa

SEQ ID NO: 70 - DNA, 1722 bp, synthetic construct
  source 1..1722: mol_type = other DNA
atgggcaccgtgaacaagcctgttgtgggcgtgctgatgggcttcggcatcatcacaggcaccctgcggatcaccaatcctgtgcgggctagcgtgctgagatacgacgacttccacatcgacgaggacaagctggacaccaacagcgtgtacgagccctactaccacagcgatcacgccgagtctagctgggtcaacagaggcgagagcagcagaaaggcctacgaccacaacagcccctacatctggccccggaacgactacgatggcttcctggaaaatgcccacgagcaccacggcgtgtacaatcaaggcagaggcatcgacagcggcgagagactgatgcagcctacacagatgagcgcccaagaggacctgggagatgataccggcatccacgtgatccccacactgaacggcgacgacagacacaagatcgtgaacgtggaccagcggcagtacggcgacgtgttcaagggcgacctgaatcctaagcctcagggccagcgcctgatcgaggtgtccgtggaagagaatcaccccttcacactgagagcccctatccagagaatctacggcgtgcgctataccgagacatggtcctttctgcccagcctgacatgtaccggggatgccgctcctgccatccagcacatttgcctgaagcacaccacctgtttccaggacgtggtggtggatgtggactgcgccgagaacaccaaagaggatcagctggccgagatcagctaccggttccagggaaagaaagaggccgaccagccttggatcgtggtcaacaccagcacactgttcgacgagctggaactggaccctcctgagattgaacccggggtgctgaaggtgctgagaaccgagaagcagtacctgggagtgtacatctggaacatgagaggcagcgacggcacctctacctacgccacctttctggtcacatggaagggcgacgagaaaacacggaaccccacaccagctgtgacccctcaacctagaggcgccgagtttcacatgtggaattaccacagccacgtgttcagcgtgggcgatacctttagcctggccatgcatctgcagtacaagatccacgaggcccctttcgacctgctgctggaatggctgtacgtgcccatcgatcctacctgccagcctatgcggctgtactccacctgtctgtatcaccccaacgctccccagtgcctgagccacatgaatagcggctgcaccttcacaagccctcacctggctcagcgagtggccagcacagtgtaccagaattgcgagcacgccgacaattacaccgcctactgtctgggcatcagccacatggaacctagcttcggcctgatcctgcacgatggcggcacaaccctgaagttcgtggatacccctgagagcctgagcggcctgtatgtgttcgtggtgtacttcaacggccacgtggaagccgtggcctacaccgtggtgtctaccgtggaccacttcgtgaacgccatcgaggaaagaggcttccctccaactgctggacagcctcctgccaccaccaagcctaaagaaatcacacccgtgaatcccggcacaagcccactgcttagatacgccgcttggacaggcggactggctgctgttgttctgctgtgcctggtcatcttcctgatctgcaccgccaagcggatgagagtgaaggccaagagagtggacaagtga

SEQ ID NO: 71 - protein, 573 aa, synthetic construct
MGTVNKPVVGVLMGFGIITGTLRITNPVRASVLRYDDFHIDEDKLDTNSVYEPYYHSDHAESSWVNRGESSRKAYDHNSPYIWPRNDYDGFLENAHEHHGVYNQGRGIDSGERLMQPTQMSAQEDLGDDTGIHVIPTLNGDDRHKIVNVDQRQYGDVFKGDLNPKPQGQRLIEVSVEENHPFTLRAPIQRIYGVRYTETWSFLPSLTCTGDAAPAIQHICLKHTTCFQDVVVDVDCAENTKEDQLAEISYRFQGKKEADQPWIVVNTSTLFDELELDPPEIEPGVLKVLRTEKQYLGVYIWNMRGSDGTSTYATFLVTWKGDEKTRNPTPAVTPQPRGAEFHMWNYHSHVFSVGDTFSLAMHLQYKIHEAPFDLLLEWLYVPIDPTCQPMRLYSTCLYHPNAPQCLSHMNSGCTFTSPHLAQRVASTVYQNCEHADNYTAYCLGISHMEPSFGLILHDGGTTLKFVDTPESLSGLYVFVVYFNGHVEAVAYTVVSTVDHFVNAIEERGFPPTAGQPPATTKPKEITPVNPGTSPLLRYAAWTGGLAAVVLLCLVIFLICTAKRMRVKAKRVDK

SEQ ID NO: 72 - RNA, 2017 nt, synthetic construct
  source 1..2017: mol_type = other RNA
agactcctccccatcctctccctctgtccctctgtccctctgaccctgcactgtcccagcaccgccaccatgggcaccgtgaacaagcctgttgtgggcgtgctgatgggcttcggcatcatcacaggcaccctgcggatcaccaatcctgtgcgggctagcgtgctgagatacgacgacttccacatcgacgaggacaagctggacaccaacagcgtgtacgagccctactaccacagcgatcacgccgagtctagctgggtcaacagaggcgagagcagcagaaaggcctacgaccacaacagcccctacatctggccccggaacgactacgatggcttcctggaaaatgcccacgagcaccacggcgtgtacaatcaaggcagaggcatcgacagcggcgagagactgatgcagcctacacagatgagcgcccaagaggacctgggagatgataccggcatccacgtgatccccacactgaacggcgacgacagacacaagatcgtgaacgtggaccagcggcagtacggcgacgtgttcaagggcgacctgaatcctaagcctcagggccagcgcctgatcgaggtgtccgtggaagagaatcaccccttcacactgagagcccctatccagagaatctacggcgtgcgctataccgagacatggtcctttctgcccagcctgacatgtaccggggatgccgctcctgccatccagcacatttgcctgaagcacaccacctgtttccaggacgtggtggtggatgtggactgcgccgagaacaccaaagaggatcagctggccgagatcagctaccggttccagggaaagaaagaggccgaccagccttggatcgtggtcaacaccagcacactgttcgacgagctggaactggaccctcctgagattgaacccggggtgctgaaggtgctgagaaccgagaagcagtacctgggagtgtacatctggaacatgagaggcagcgacggcacctctacctacgccacctttctggtcacatggaagggcgacgagaaaacacggaaccccacaccagctgtgacccctcaacctagaggcgccgagtttcacatgtggaattaccacagccacgtgttcagcgtgggcgatacctttagcctggccatgcatctgcagtacaagatccacgaggcccctttcgacctgctgctggaatggctgtacgtgcccatcgatcctacctgccagcctatgcggctgtactccacctgtctgtatcaccccaacgctccccagtgcctgagccacatgaatagcggctgcaccttcacaagccctcacctggctcagcgagtggccagcacagtgtaccagaattgcgagcacgccgacaattacaccgcctactgtctgggcatcagccacatggaacctagcttcggcctgatcctgcacgatggcggcacaaccctgaagttcgtggatacccctgagagcctgagcggcctgtatgtgttcgtggtgtacttcaacggccacgtggaagccgtggcctacaccgtggtgtctaccgtggaccacttcgtgaacgccatcgaggaaagaggcttccctccaactgctggacagcctcctgccaccaccaagcctaaagaaatcacacccgtgaatcccggcacaagcccactgcttagatacgccgcttggacaggcggactggctgctgttgttctgctgtgcctggtcatcttcctgatctgcaccgccaagcggatgagagtgaaggccaagagagtggacaagtgataataggctggagcctcggtggccatgcttcttgccccttgggcctccccccagcccctcctccccttcctgcacccgtacccccgtggtctttgaataaagtctgagtgggcggcaaaaaaaaaaaaaaaaaaaaaaaaaaaaaaaaaaaaaaaaaaaaaaaaaaaaaaaaaaaaaaaaaaaaaaaaaaaaaaaaaaaaaaaaaaaaaaaaaaaaaaaaaaaaaa

SEQ ID NO: 73 - DNA, 2017 bp, synthetic construct
  source 1..2017: mol_type = other DNA
agactcctccccatcctctccctctgtccctctgtccctctgaccctgcactgtcccagcaccgccaccatgggcaccgtgaacaagcctgttgtgggcgtgctgatgggcttcggcatcatcacaggcaccctgcggatcaccaatcctgtgcgggctagcgtgctgagatacgacgacttccacatcgacgaggacaagctggacaccaacagcgtgtacgagccctactaccacagcgatcacgccgagtctagctgggtcaacagaggcgagagcagcagaaaggcctacgaccacaacagcccctacatctggccccggaacgactacgatggcttcctggaaaatgcccacgagcaccacggcgtgtacaatcaaggcagaggcatcgacagcggcgagagactgatgcagcctacacagatgagcgcccaagaggacctgggagatgataccggcatccacgtgatccccacactgaacggcgacgacagacacaagatcgtgaacgtggaccagcggcagtacggcgacgtgttcaagggcgacctgaatcctaagcctcagggccagcgcctgatcgaggtgtccgtggaagagaatcaccccttcacactgagagcccctatccagagaatctacggcgtgcgctataccgagacatggtcctttctgcccagcctgacatgtaccggggatgccgctcctgccatccagcacatttgcctgaagcacaccacctgtttccaggacgtggtggtggatgtggactgcgccgagaacaccaaagaggatcagctggccgagatcagctaccggttccagggaaagaaagaggccgaccagccttggatcgtggtcaacaccagcacactgttcgacgagctggaactggaccctcctgagattgaacccggggtgctgaaggtgctgagaaccgagaagcagtacctgggagtgtacatctggaacatgagaggcagcgacggcacctctacctacgccacctttctggtcacatggaagggcgacgagaaaacacggaaccccacaccagctgtgacccctcaacctagaggcgccgagtttcacatgtggaattaccacagccacgtgttcagcgtgggcgatacctttagcctggccatgcatctgcagtacaagatccacgaggcccctttcgacctgctgctggaatggctgtacgtgcccatcgatcctacctgccagcctatgcggctgtactccacctgtctgtatcaccccaacgctccccagtgcctgagccacatgaatagcggctgcaccttcacaagccctcacctggctcagcgagtggccagcacagtgtaccagaattgcgagcacgccgacaattacaccgcctactgtctgggcatcagccacatggaacctagcttcggcctgatcctgcacgatggcggcacaaccctgaagttcgtggatacccctgagagcctgagcggcctgtatgtgttcgtggtgtacttcaacggccacgtggaagccgtggcctacaccgtggtgtctaccgtggaccacttcgtgaacgccatcgaggaaagaggcttccctccaactgctggacagcctcctgccaccaccaagcctaaagaaatcacacccgtgaatcccggcacaagcccactgcttagatacgccgcttggacaggcggactggctgctgttgttctgctgtgcctggtcatcttcctgatctgcaccgccaagcggatgagagtgaaggcctatgaggtggacaagtgataataggctggagcctcggtggccatgcttcttgccccttgggcctccccccagcccctcctccccttcctgcacccgtacccccgtggtctttgaataaagtctgagtgggcggcaaaaaaaaaaaaaaaaaaaaaaaaaaaaaaaaaaaaaaaaaaaaaaaaaaaaaaaaaaaaaaaaaaaaaaaaaaaaaaaaaaaaaaaaaaaaaaaaaaaaaaaaaaaaaa

SEQ ID NO: 74 - DNA, 1722 bp, synthetic construct
  source 1..1722: mol_type = other DNA
atgggcaccgtgaacaagcctgttgtgggcgtgctgatgggcttcggcatcatcacaggcaccctgcggatcaccaatcctgtgcgggctagcgtgctgagatacgacgacttccacatcgacgaggacaagctggacaccaacagcgtgtacgagccctactaccacagcgatcacgccgagtctagctgggtcaacagaggcgagagcagcagaaaggcctacgaccacaacagcccctacatctggccccggaacgactacgatggcttcctggaaaatgcccacgagcaccacggcgtgtacaatcaaggcagaggcatcgacagcggcgagagactgatgcagcctacacagatgagcgcccaagaggacctgggagatgataccggcatccacgtgatccccacactgaacggcgacgacagacacaagatcgtgaacgtggaccagcggcagtacggcgacgtgttcaagggcgacctgaatcctaagcctcagggccagcgcctgatcgaggtgtccgtggaagagaatcaccccttcacactgagagcccctatccagagaatctacggcgtgcgctataccgagacatggtcctttctgcccagcctgacatgtaccggggatgccgctcctgccatccagcacatttgcctgaagcacaccacctgtttccaggacgtggtggtggatgtggactgcgccgagaacaccaaagaggatcagctggccgagatcagctaccggttccagggaaagaaagaggccgaccagccttggatcgtggtcaacaccagcacactgttcgacgagctggaactggaccctcctgagattgaacccggggtgctgaaggtgctgagaaccgagaagcagtacctgggagtgtacatctggaacatgagaggcagcgacggcacctctacctacgccacctttctggtcacatggaagggcgacgagaaaacacggaaccccacaccagctgtgacccctcaacctagaggcgccgagtttcacatgtggaattaccacagccacgtgttcagcgtgggcgatacctttagcctggccatgcatctgcagtacaagatccacgaggcccctttcgacctgctgctggaatggctgtacgtgcccatcgatcctacctgccagcctatgcggctgtactccacctgtctgtatcaccccaacgctccccagtgcctgagccacatgaatagcggctgcaccttcacaagccctcacctggctcagcgagtggccagcacagtgtaccagaattgcgagcacgccgacaattacaccgcctactgtctgggcatcagccacatggaacctagcttcggcctgatcctgcacgatggcggcacaaccctgaagttcgtggatacccctgagagcctgagcggcctgtatgtgttcgtggtgtacttcaacggccacgtggaagccgtggcctacaccgtggtgtctaccgtggaccacttcgtgaacgccatcgaggaaagaggcttccctccaactgctggacagcctcctgccaccaccaagcctaaagaaatcacacccgtgaatcccggcacaagcccactgcttagatacgccgcttggacaggcggactggctgctgttgttctgctgtgcctggtcatcttcctgatctgcaccgccaagcggatgagagtgaaggcctatgaggtggacaagtga

SEQ ID NO: 75 - protein, 573 aa, synthetic construct
MGTVNKPVVGVLMGFGIITGTLRITNPVRASVLRYDDFHIDEDKLDTNSVYEPYYHSDHAESSWVNRGESSRKAYDHNSPYIWPRNDYDGFLENAHEHHGVYNQGRGIDSGERLMQPTQMSAQEDLGDDTGIHVIPTLNGDDRHKIVNVDQRQYGDVFKGDLNPKPQGQRLIEVSVEENHPFTLRAPIQRIYGVRYTETWSFLPSLTCTGDAAPAIQHICLKHTTCFQDVVVDVDCAENTKEDQLAEISYRFQGKKEADQPWIVVNTSTLFDELELDPPEIEPGVLKVLRTEKQYLGVYIWNMRGSDGTSTYATFLVTWKGDEKTRNPTPAVTPQPRGAEFHMWNYHSHVFSVGDTFSLAMHLQYKIHEAPFDLLLEWLYVPIDPTCQPMRLYSTCLYHPNAPQCLSHMNSGCTFTSPHLAQRVASTVYQNCEHADNYTAYCLGISHMEPSFGLILHDGGTTLKFVDTPESLSGLYVFVVYFNGHVEAVAYTVVSTVDHFVNAIEERGFPPTAGQPPATTKPKEITPVNPGTSPLLRYAAWTGGLAAVVLLCLVIFLICTAKRMRVKAYEVDK

SEQ ID NO: 76 - RNA, 2017 nt, synthetic construct
  source 1..2017: mol_type = other RNA
agactcctccccatcctctccctctgtccctctgtccctctgaccctgcactgtcccagcaccgccaccatgggcaccgtgaacaagcctgttgtgggcgtgctgatgggcttcggcatcatcacaggcaccctgcggatcaccaatcctgtgcgggctagcgtgctgagatacgacgacttccacatcgacgaggacaagctggacaccaacagcgtgtacgagccctactaccacagcgatcacgccgagtctagctgggtcaacagaggcgagagcagcagaaaggcctacgaccacaacagcccctacatctggccccggaacgactacgatggcttcctggaaaatgcccacgagcaccacggcgtgtacaatcaaggcagaggcatcgacagcggcgagagactgatgcagcctacacagatgagcgcccaagaggacctgggagatgataccggcatccacgtgatccccacactgaacggcgacgacagacacaagatcgtgaacgtggaccagcggcagtacggcgacgtgttcaagggcgacctgaatcctaagcctcagggccagcgcctgatcgaggtgtccgtggaagagaatcaccccttcacactgagagcccctatccagagaatctacggcgtgcgctataccgagacatggtcctttctgcccagcctgacatgtaccggggatgccgctcctgccatccagcacatttgcctgaagcacaccacctgtttccaggacgtggtggtggatgtggactgcgccgagaacaccaaagaggatcagctggccgagatcagctaccggttccagggaaagaaagaggccgaccagccttggatcgtggtcaacaccagcacactgttcgacgagctggaactggaccctcctgagattgaacccggggtgctgaaggtgctgagaaccgagaagcagtacctgggagtgtacatctggaacatgagaggcagcgacggcacctctacctacgccacctttctggtcacatggaagggcgacgagaaaacacggaaccccacaccagctgtgacccctcaacctagaggcgccgagtttcacatgtggaattaccacagccacgtgttcagcgtgggcgatacctttagcctggccatgcatctgcagtacaagatccacgaggcccctttcgacctgctgctggaatggctgtacgtgcccatcgatcctacctgccagcctatgcggctgtactccacctgtctgtatcaccccaacgctccccagtgcctgagccacatgaatagcggctgcaccttcacaagccctcacctggctcagcgagtggccagcacagtgtaccagaattgcgagcacgccgacaattacaccgcctactgtctgggcatcagccacatggaacctagcttcggcctgatcctgcacgatggcggcacaaccctgaagttcgtggatacccctgagagcctgagcggcctgtatgtgttcgtggtgtacttcaacggccacgtggaagccgtggcctacaccgtggtgtctaccgtggaccacttcgtgaacgccatcgaggaaagaggcttccctccaactgctggacagcctcctgccaccaccaagcctaaagaaatcacacccgtgaatcccggcacaagcccactgcttagatacgccgcttggacaggcggactggctgctgttgttctgctgtgcctggtcatcttcctgatctgcaccgccaagcggatgagagtgaaggcctatgaggtggacaagtgataataggctggagcctcggtggccatgcttcttgccccttgggcctccccccagcccctcctccccttcctgcacccgtacccccgtggtctttgaataaagtctgagtgggcggcaaaaaaaaaaaaaaaaaaaaaaaaaaaaaaaaaaaaaaaaaaaaaaaaaaaaaaaaaaaaaaaaaaaaaaaaaaaaaaaaaaaaaaaaaaaaaaaaaaaaaaaaaaaaaa

SEQ ID NO: 77 - DNA, 2017 bp, synthetic construct
  source 1..2017: mol_type = other DNA
agactcctccccatcctctccctctgtccctctgtccctctgaccctgcactgtcccagcaccgccaccatgggcaccgtgaacaagcctgttgtgggcgtgctgatgggcttcggcatcatcacaggcaccctgcggatcaccaatcctgtgcgggctagcgtgctgagatacgacgacttccacatcgacgaggacaagctggacaccaacagcgtgtacgagccctactaccacagcgatcacgccgagtctagctgggtcaacagaggcgagagcagcagaaaggcctacgaccacaacagcccctacatctggccccggaacgactacgatggcttcctggaaaatgcccacgagcaccacggcgtgtacaatcaaggcagaggcatcgacagcggcgagagactgatgcagcctacacagatgagcgcccaagaggacctgggagatgataccggcatccacgtgatccccacactgaacggcgacgacagacacaagatcgtgaacgtggaccagcggcagtacggcgacgtgttcaagggcgacctgaatcctaagcctcagggccagcgcctgatcgaggtgtccgtggaagagaatcaccccttcacactgagagcccctatccagagaatctacggcgtgcgctataccgagacatggtcctttctgcccagcctgacatgtaccggggatgccgctcctgccatccagcacatttgcctgaagcacaccacctgtttccaggacgtggtggtggatgtggactgcgccgagaacaccaaagaggatcagctggccgagatcagctaccggttccagggaaagaaagaggccgaccagccttggatcgtggtcaacaccagcacactgttcgacgagctggaactggaccctcctgagattgaacccggggtgctgaaggtgctgagaaccgagaagcagtacctgggagtgtacatctggaacatgagaggcagcgacggcacctctacctacgccacctttctggtcacatggaagggcgacgagaaaacacggaaccccacaccagctgtgacccctcaacctagaggcgccgagtttcacatgtggaattaccacagccacgtgttcagcgtgggcgatacctttagcctggccatgcatctgcagtacaagatccacgaggcccctttcgacctgctgctggaatggctgtacgtgcccatcgatcctacctgccagcctatgcggctgtactccacctgtctgtatcaccccaacgctccccagtgcctgagccacatgaatagcggctgcaccttcacaagccctcacctggctcagcgagtggccagcacagtgtaccagaattgcgagcacgccgacaattacaccgcctactgtctgggcatcagccacatggaacctagcttcggcctgatcctgcacgatggcggcacaaccctgaagttcgtggatacccctgagagcctgagcggcctgtatgtgttcgtggtgtacttcaacggccacgtggaagccgtggcctacaccgtggtgtctaccgtggaccacttcgtgaacgccatcgaggaaagaggcttccctccaactgctggacagcctcctgccaccaccaagcctaaagaaatcacacccgtgaatcccggcacaagcccactgcttagatacgccgcttggacaggcggactggctgctgttgttctgctgtgcctggtcatcttcctgatctgcaccgccaagcggatgagagtgaaggcctaccggaaggacaagtgataataggctggagcctcggtggccatgcttcttgccccttgggcctccccccagcccctcctccccttcctgcacccgtacccccgtggtctttgaataaagtctgagtgggcggcaaaaaaaaaaaaaaaaaaaaaaaaaaaaaaaaaaaaaaaaaaaaaaaaaaaaaaaaaaaaaaaaaaaaaaaaaaaaaaaaaaaaaaaaaaaaaaaaaaaaaaaaaaaaaa

SEQ ID NO: 78 - DNA, 1722 bp, synthetic construct
  source 1..1722: mol_type = other DNA
atgggcaccgtgaacaagcctgttgtgggcgtgctgatgggcttcggcatcatcacaggcaccctgcggatcaccaatcctgtgcgggctagcgtgctgagatacgacgacttccacatcgacgaggacaagctggacaccaacagcgtgtacgagccctactaccacagcgatcacgccgagtctagctgggtcaacagaggcgagagcagcagaaaggcctacgaccacaacagcccctacatctggccccggaacgactacgatggcttcctggaaaatgcccacgagcaccacggcgtgtacaatcaaggcagaggcatcgacagcggcgagagactgatgcagcctacacagatgagcgcccaagaggacctgggagatgataccggcatccacgtgatccccacactgaacggcgacgacagacacaagatcgtgaacgtggaccagcggcagtacggcgacgtgttcaagggcgacctgaatcctaagcctcagggccagcgcctgatcgaggtgtccgtggaagagaatcaccccttcacactgagagcccctatccagagaatctacggcgtgcgctataccgagacatggtcctttctgcccagcctgacatgtaccggggatgccgctcctgccatccagcacatttgcctgaagcacaccacctgtttccaggacgtggtggtggatgtggactgcgccgagaacaccaaagaggatcagctggccgagatcagctaccggttccagggaaagaaagaggccgaccagccttggatcgtggtcaacaccagcacactgttcgacgagctggaactggaccctcctgagattgaacccggggtgctgaaggtgctgagaaccgagaagcagtacctgggagtgtacatctggaacatgagaggcagcgacggcacctctacctacgccacctttctggtcacatggaagggcgacgagaaaacacggaaccccacaccagctgtgacccctcaacctagaggcgccgagtttcacatgtggaattaccacagccacgtgttcagcgtgggcgatacctttagcctggccatgcatctgcagtacaagatccacgaggcccctttcgacctgctgctggaatggctgtacgtgcccatcgatcctacctgccagcctatgcggctgtactccacctgtctgtatcaccccaacgctccccagtgcctgagccacatgaatagcggctgcaccttcacaagccctcacctggctcagcgagtggccagcacagtgtaccagaattgcgagcacgccgacaattacaccgcctactgtctgggcatcagccacatggaacctagcttcggcctgatcctgcacgatggcggcacaaccctgaagttcgtggatacccctgagagcctgagcggcctgtatgtgttcgtggtgtacttcaacggccacgtggaagccgtggcctacaccgtggtgtctaccgtggaccacttcgtgaacgccatcgaggaaagaggcttccctccaactgctggacagcctcctgccaccaccaagcctaaagaaatcacacccgtgaatcccggcacaagcccactgcttagatacgccgcttggacaggcggactggctgctgttgttctgctgtgcctggtcatcttcctgatctgcaccgccaagcggatgagagtgaaggcctaccggaaggacaagtga

SEQ ID NO: 79 - protein, 573 aa, synthetic construct
MGTVNKPVVGVLMGFGIITGTLRITNPVRASVLRYDDFHIDEDKLDTNSVYEPYYHSDHAESSWVNRGESSRKAYDHNSPYIWPRNDYDGFLENAHEHHGVYNQGRGIDSGERLMQPTQMSAQEDLGDDTGIHVIPTLNGDDRHKIVNVDQRQYGDVFKGDLNPKPQGQRLIEVSVEENHPFTLRAPIQRIYGVRYTETWSFLPSLTCTGDAAPAIQHICLKHTTCFQDVVVDVDCAENTKEDQLAEISYRFQGKKEADQPWIVVNTSTLFDELELDPPEIEPGVLKVLRTEKQYLGVYIWNMRGSDGTSTYATFLVTWKGDEKTRNPTPAVTPQPRGAEFHMWNYHSHVFSVGDTFSLAMHLQYKIHEAPFDLLLEWLYVPIDPTCQPMRLYSTCLYHPNAPQCLSHMNSGCTFTSPHLAQRVASTVYQNCEHADNYTAYCLGISHMEPSFGLILHDGGTTLKFVDTPESLSGLYVFVVYFNGHVEAVAYTVVSTVDHFVNAIEERGFPPTAGQPPATTKPKEITPVNPGTSPLLRYAAWTGGLAAVVLLCLVIFLICTAKRMRVKAYRKDK

SEQ ID NO: 80 - RNA, 2017 nt, synthetic construct
  source 1..2017: mol_type = other RNA
agactcctccccatcctctccctctgtccctctgtccctctgaccctgcactgtcccagcaccgccaccatgggcaccgtgaacaagcctgttgtgggcgtgctgatgggcttcggcatcatcacaggcaccctgcggatcaccaatcctgtgcgggctagcgtgctgagatacgacgacttccacatcgacgaggacaagctggacaccaacagcgtgtacgagccctactaccacagcgatcacgccgagtctagctgggtcaacagaggcgagagcagcagaaaggcctacgaccacaacagcccctacatctggccccggaacgactacgatggcttcctggaaaatgcccacgagcaccacggcgtgtacaatcaaggcagaggcatcgacagcggcgagagactgatgcagcctacacagatgagcgcccaagaggacctgggagatgataccggcatccacgtgatccccacactgaacggcgacgacagacacaagatcgtgaacgtggaccagcggcagtacggcgacgtgttcaagggcgacctgaatcctaagcctcagggccagcgcctgatcgaggtgtccgtggaagagaatcaccccttcacactgagagcccctatccagagaatctacggcgtgcgctataccgagacatggtcctttctgcccagcctgacatgtaccggggatgccgctcctgccatccagcacatttgcctgaagcacaccacctgtttccaggacgtggtggtggatgtggactgcgccgagaacaccaaagaggatcagctggccgagatcagctaccggttccagggaaagaaagaggccgaccagccttggatcgtggtcaacaccagcacactgttcgacgagctggaactggaccctcctgagattgaacccggggtgctgaaggtgctgagaaccgagaagcagtacctgggagtgtacatctggaacatgagaggcagcgacggcacctctacctacgccacctttctggtcacatggaagggcgacgagaaaacacggaaccccacaccagctgtgacccctcaacctagaggcgccgagtttcacatgtggaattaccacagccacgtgttcagcgtgggcgatacctttagcctggccatgcatctgcagtacaagatccacgaggcccctttcgacctgctgctggaatggctgtacgtgcccatcgatcctacctgccagcctatgcggctgtactccacctgtctgtatcaccccaacgctccccagtgcctgagccacatgaatagcggctgcaccttcacaagccctcacctggctcagcgagtggccagcacagtgtaccagaattgcgagcacgccgacaattacaccgcctactgtctgggcatcagccacatggaacctagcttcggcctgatcctgcacgatggcggcacaaccctgaagttcgtggatacccctgagagcctgagcggcctgtatgtgttcgtggtgtacttcaacggccacgtggaagccgtggcctacaccgtggtgtctaccgtggaccacttcgtgaacgccatcgaggaaagaggcttccctccaactgctggacagcctcctgccaccaccaagcctaaagaaatcacacccgtgaatcccggcacaagcccactgcttagatacgccgcttggacaggcggactggctgctgttgttctgctgtgcctggtcatcttcctgatctgcaccgccaagcggatgagagtgaaggcctaccggaaggacaagtgataataggctggagcctcggtggccatgcttcttgccccttgggcctccccccagcccctcctccccttcctgcacccgtacccccgtggtctttgaataaagtctgagtgggcggcaaaaaaaaaaaaaaaaaaaaaaaaaaaaaaaaaaaaaaaaaaaaaaaaaaaaaaaaaaaaaaaaaaaaaaaaaaaaaaaaaaaaaaaaaaaaaaaaaaaaaaaaaaaaaa

SEQ ID NO: 81 - DNA, 2017 bp, synthetic construct
  source 1..2017: mol_type = other DNA
agactcctccccatcctctccctctgtccctctgtccctctgaccctgcactgtcccagcaccgccaccatgggcaccgtgaacaagcctgttgtgggcgtgctgatgggcttcggcatcatcacaggcaccctgcggatcaccaatcctgtgcgggctagcgtgctgagatacgacgacttccacatcgacgaggacaagctggacaccaacagcgtgtacgagccctactaccacagcgatcacgccgagtctagctgggtcaacagaggcgagagcagcagaaaggcctacgaccacaacagcccctacatctggccccggaacgactacgatggcttcctggaaaatgcccacgagcaccacggcgtgtacaatcaaggcagaggcatcgacagcggcgagagactgatgcagcctacacagatgagcgcccaagaggacctgggagatgataccggcatccacgtgatccccacactgaacggcgacgacagacacaagatcgtgaacgtggaccagcggcagtacggcgacgtgttcaagggcgacctgaatcctaagcctcagggccagcgcctgatcgaggtgtccgtggaagagaatcaccccttcacactgagagcccctatccagagaatctacggcgtgcgctataccgagacatggtcctttctgcccagcctgacatgtaccggggatgccgctcctgccatccagcacatttgcctgaagcacaccacctgtttccaggacgtggtggtggatgtggactgcgccgagaacaccaaagaggatcagctggccgagatcagctaccggttccagggaaagaaagaggccgaccagccttggatcgtggtcaacaccagcacactgttcgacgagctggaactggaccctcctgagattgaacccggggtgctgaaggtgctgagaaccgagaagcagtacctgggagtgtacatctggaacatgagaggcagcgacggcacctctacctacgccacctttctggtcacatggaagggcgacgagaaaacacggaaccccacaccagctgtgacccctcaacctagaggcgccgagtttcacatgtggaattaccacagccacgtgttcagcgtgggcgatacctttagcctggccatgcatctgcagtacaagatccacgaggcccctttcgacctgctgctggaatggctgtacgtgcccatcgatcctacctgccagcctatgcggctgtactccacctgtctgtatcaccccaacgctccccagtgcctgagccacatgaatagcggctgcaccttcacaagccctcacctggctcagcgagtggccagcacagtgtaccagaattgcgagcacgccgacaattacaccgcctactgtctgggcatcagccacatggaacctagcttcggcctgatcctgcacgatggcggcacaaccctgaagttcgtggatacccctgagagcctgagcggcctgtatgtgttcgtggtgtacttcaacggccacgtggaagccgtggcctacaccgtggtgtctaccgtggaccacttcgtgaacgccatcgaggaaagaggcttccctccaactgctggacagcctcctgccaccaccaagcctaaagaaatcacacccgtgaatcccggcacaagcccactgcttagatacgccgcttggacaggcggactggctgctgttgttctgctgtgcctggtcatcttcctgatctgcaccgccaagcggatgcgcgtgaaggacaaagagaaggacaagtgataataggctggagcctcggtggccatgcttcttgccccttgggcctccccccagcccctcctccccttcctgcacccgtacccccgtggtctttgaataaagtctgagtgggcggcaaaaaaaaaaaaaaaaaaaaaaaaaaaaaaaaaaaaaaaaaaaaaaaaaaaaaaaaaaaaaaaaaaaaaaaaaaaaaaaaaaaaaaaaaaaaaaaaaaaaaaaaaaaaaa

SEQ ID NO: 82 - DNA, 1722 bp, synthetic construct
  source 1..1722: mol_type = other DNA
atgggcaccgtgaacaagcctgttgtgggcgtgctgatgggcttcggcatcatcacaggcaccctgcggatcaccaatcctgtgcgggctagcgtgctgagatacgacgacttccacatcgacgaggacaagctggacaccaacagcgtgtacgagccctactaccacagcgatcacgccgagtctagctgggtcaacagaggcgagagcagcagaaaggcctacgaccacaacagcccctacatctggccccggaacgactacgatggcttcctggaaaatgcccacgagcaccacggcgtgtacaatcaaggcagaggcatcgacagcggcgagagactgatgcagcctacacagatgagcgcccaagaggacctgggagatgataccggcatccacgtgatccccacactgaacggcgacgacagacacaagatcgtgaacgtggaccagcggcagtacggcgacgtgttcaagggcgacctgaatcctaagcctcagggccagcgcctgatcgaggtgtccgtggaagagaatcaccccttcacactgagagcccctatccagagaatctacggcgtgcgctataccgagacatggtcctttctgcccagcctgacatgtaccggggatgccgctcctgccatccagcacatttgcctgaagcacaccacctgtttccaggacgtggtggtggatgtggactgcgccgagaacaccaaagaggatcagctggccgagatcagctaccggttccagggaaagaaagaggccgaccagccttggatcgtggtcaacaccagcacactgttcgacgagctggaactggaccctcctgagattgaacccggggtgctgaaggtgctgagaaccgagaagcagtacctgggagtgtacatctggaacatgagaggcagcgacggcacctctacctacgccacctttctggtcacatggaagggcgacgagaaaacacggaaccccacaccagctgtgacccctcaacctagaggcgccgagtttcacatgtggaattaccacagccacgtgttcagcgtgggcgatacctttagcctggccatgcatctgcagtacaagatccacgaggcccctttcgacctgctgctggaatggctgtacgtgcccatcgatcctacctgccagcctatgcggctgtactccacctgtctgtatcaccccaacgctccccagtgcctgagccacatgaatagcggctgcaccttcacaagccctcacctggctcagcgagtggccagcacagtgtaccagaattgcgagcacgccgacaattacaccgcctactgtctgggcatcagccacatggaacctagcttcggcctgatcctgcacgatggcggcacaaccctgaagttcgtggatacccctgagagcctgagcggcctgtatgtgttcgtggtgtacttcaacggccacgtggaagccgtggcctacaccgtggtgtctaccgtggaccacttcgtgaacgccatcgaggaaagaggcttccctccaactgctggacagcctcctgccaccaccaagcctaaagaaatcacacccgtgaatcccggcacaagcccactgcttagatacgccgcttggacaggcggactggctgctgttgttctgctgtgcctggtcatcttcctgatctgcaccgccaagcggatgcgcgtgaaggacaaagagaaggacaagtga

SEQ ID NO: 83 - protein, 573 aa, synthetic construct
MGTVNKPVVGVLMGFGIITGTLRITNPVRASVLRYDDFHIDEDKLDTNSVYEPYYHSDHAESSWVNRGESSRKAYDHNSPYIWPRNDYDGFLENAHEHHGVYNQGRGIDSGERLMQPTQMSAQEDLGDDTGIHVIPTLNGDDRHKIVNVDQRQYGDVFKGDLNPKPQGQRLIEVSVEENHPFTLRAPIQRIYGVRYTETWSFLPSLTCTGDAAPAIQHICLKHTTCFQDVVVDVDCAENTKEDQLAEISYRFQGKKEADQPWIVVNTSTLFDELELDPPEIEPGVLKVLRTEKQYLGVYIWNMRGSDGTSTYATFLVTWKGDEKTRNPTPAVTPQPRGAEFHMWNYHSHVFSVGDTFSLAMHLQYKIHEAPFDLLLEWLYVPIDPTCQPMRLYSTCLYHPNAPQCLSHMNSGCTFTSPHLAQRVASTVYQNCEHADNYTAYCLGISHMEPSFGLILHDGGTTLKFVDTPESLSGLYVFVVYFNGHVEAVAYTVVSTVDHFVNAIEERGFPPTAGQPPATTKPKEITPVNPGTSPLLRYAAWTGGLAAVVLLCLVIFLICTAKRMRVKDKEKDK

SEQ ID NO: 84 - RNA, 2017 nt, synthetic construct
  source 1..2017: mol_type = other RNA
agactcctccccatcctctccctctgtccctctgtccctctgaccctgcactgtcccagcaccgccaccatgggcaccgtgaacaagcctgttgtgggcgtgctgatgggcttcggcatcatcacaggcaccctgcggatcaccaatcctgtgcgggctagcgtgctgagatacgacgacttccacatcgacgaggacaagctggacaccaacagcgtgtacgagccctactaccacagcgatcacgccgagtctagctgggtcaacagaggcgagagcagcagaaaggcctacgaccacaacagcccctacatctggccccggaacgactacgatggcttcctggaaaatgcccacgagcaccacggcgtgtacaatcaaggcagaggcatcgacagcggcgagagactgatgcagcctacacagatgagcgcccaagaggacctgggagatgataccggcatccacgtgatccccacactgaacggcgacgacagacacaagatcgtgaacgtggaccagcggcagtacggcgacgtgttcaagggcgacctgaatcctaagcctcagggccagcgcctgatcgaggtgtccgtggaagagaatcaccccttcacactgagagcccctatccagagaatctacggcgtgcgctataccgagacatggtcctttctgcccagcctgacatgtaccggggatgccgctcctgccatccagcacatttgcctgaagcacaccacctgtttccaggacgtggtggtggatgtggactgcgccgagaacaccaaagaggatcagctggccgagatcagctaccggttccagggaaagaaagaggccgaccagccttggatcgtggtcaacaccagcacactgttcgacgagctggaactggaccctcctgagattgaacccggggtgctgaaggtgctgagaaccgagaagcagtacctgggagtgtacatctggaacatgagaggcagcgacggcacctctacctacgccacctttctggtcacatggaagggcgacgagaaaacacggaaccccacaccagctgtgacccctcaacctagaggcgccgagtttcacatgtggaattaccacagccacgtgttcagcgtgggcgatacctttagcctggccatgcatctgcagtacaagatccacgaggcccctttcgacctgctgctggaatggctgtacgtgcccatcgatcctacctgccagcctatgcggctgtactccacctgtctgtatcaccccaacgctccccagtgcctgagccacatgaatagcggctgcaccttcacaagccctcacctggctcagcgagtggccagcacagtgtaccagaattgcgagcacgccgacaattacaccgcctactgtctgggcatcagccacatggaacctagcttcggcctgatcctgcacgatggcggcacaaccctgaagttcgtggatacccctgagagcctgagcggcctgtatgtgttcgtggtgtacttcaacggccacgtggaagccgtggcctacaccgtggtgtctaccgtggaccacttcgtgaacgccatcgaggaaagaggcttccctccaactgctggacagcctcctgccaccaccaagcctaaagaaatcacacccgtgaatcccggcacaagcccactgcttagatacgccgcttggacaggcggactggctgctgttgttctgctgtgcctggtcatcttcctgatctgcaccgccaagcggatgcgcgtgaaggacaaagagaaggacaagtgataataggctggagcctcggtggccatgcttcttgccccttgggcctccccccagcccctcctccccttcctgcacccgtacccccgtggtctttgaataaagtctgagtgggcggcaaaaaaaaaaaaaaaaaaaaaaaaaaaaaaaaaaaaaaaaaaaaaaaaaaaaaaaaaaaaaaaaaaaaaaaaaaaaaaaaaaaaaaaaaaaaaaaaaaaaaaaaaaaaaa

SEQ ID NO: 85 - DNA, 2017 bp, synthetic construct
  source 1..2017: mol_type = other DNA
agactcctccccatcctctccctctgtccctctgtccctctgaccctgcactgtcccagcaccgccaccatgggcaccgtgaacaagcctgttgtgggcgtgctgatgggcttcggcatcatcacaggcaccctgcggatcaccaatcctgtgcgggctagcgtgctgagatacgacgacttccacatcgacgaggacaagctggacaccaacagcgtgtacgagccctactaccacagcgatcacgccgagtctagctgggtcaacagaggcgagagcagcagaaaggcctacgaccacaacagcccctacatctggccccggaacgactacgatggcttcctggaaaatgcccacgagcaccacggcgtgtacaatcaaggcagaggcatcgacagcggcgagagactgatgcagcctacacagatgagcgcccaagaggacctgggagatgataccggcatccacgtgatccccacactgaacggcgacgacagacacaagatcgtgaacgtggaccagcggcagtacggcgacgtgttcaagggcgacctgaatcctaagcctcagggccagcgcctgatcgaggtgtccgtggaagagaatcaccccttcacactgagagcccctatccagagaatctacggcgtgcgctataccgagacatggtcctttctgcccagcctgacatgtaccggggatgccgctcctgccatccagcacatttgcctgaagcacaccacctgtttccaggacgtggtggtggatgtggactgcgccgagaacaccaaagaggatcagctggccgagatcagctaccggttccagggaaagaaagaggccgaccagccttggatcgtggtcaacaccagcacactgttcgacgagctggaactggaccctcctgagattgaacccggggtgctgaaggtgctgagaaccgagaagcagtacctgggagtgtacatctggaacatgagaggcagcgacggcacctctacctacgccacctttctggtcacatggaagggcgacgagaaaacacggaaccccacaccagctgtgacccctcaacctagaggcgccgagtttcacatgtggaattaccacagccacgtgttcagcgtgggcgatacctttagcctggccatgcatctgcagtacaagatccacgaggcccctttcgacctgctgctggaatggctgtacgtgcccatcgatcctacctgccagcctatgcggctgtactccacctgtctgtatcaccccaacgctccccagtgcctgagccacatgaatagcggctgcaccttcacaagccctcacctggctcagcgagtggccagcacagtgtaccagaattgcgagcacgccgacaattacaccgcctactgtctgggcatcagccacatggaacctagcttcggcctgatcctgcacgatggcggcacaaccctgaagttcgtggatacccctgagagcctgagcggcctgtatgtgttcgtggtgtacttcaacggccacgtggaagccgtggcctacaccgtggtgtctaccgtggaccacttcgtgaacgccatcgaggaaagaggcttccctccaactgctggacagcctcctgccaccaccaagcctaaagaaatcacacccgtgaatcccggcacaagcccactgcttagatacgccgcttggacaggcggactggctgctgttgttctgctgtgcctggtcatcttcctgatctgcaccgccaagcggatgagagtgaaggacgccgagaaggacaagtgataataggctggagcctcggtggccatgcttcttgccccttgggcctccccccagcccctcctccccttcctgcacccgtacccccgtggtctttgaataaagtctgagtgggcggcaaaaaaaaaaaaaaaaaaaaaaaaaaaaaaaaaaaaaaaaaaaaaaaaaaaaaaaaaaaaaaaaaaaaaaaaaaaaaaaaaaaaaaaaaaaaaaaaaaaaaaaaaaaaaa

SEQ ID NO: 86 - DNA, 1722 bp, synthetic construct
  source 1..1722: mol_type = other DNA
atgggcaccgtgaacaagcctgttgtgggcgtgctgatgggcttcggcatcatcacaggcaccctgcggatcaccaatcctgtgcgggctagcgtgctgagatacgacgacttccacatcgacgaggacaagctggacaccaacagcgtgtacgagccctactaccacagcgatcacgccgagtctagctgggtcaacagaggcgagagcagcagaaaggcctacgaccacaacagcccctacatctggccccggaacgactacgatggcttcctggaaaatgcccacgagcaccacggcgtgtacaatcaaggcagaggcatcgacagcggcgagagactgatgcagcctacacagatgagcgcccaagaggacctgggagatgataccggcatccacgtgatccccacactgaacggcgacgacagacacaagatcgtgaacgtggaccagcggcagtacggcgacgtgttcaagggcgacctgaatcctaagcctcagggccagcgcctgatcgaggtgtccgtggaagagaatcaccccttcacactgagagcccctatccagagaatctacggcgtgcgctataccgagacatggtcctttctgcccagcctgacatgtaccggggatgccgctcctgccatccagcacatttgcctgaagcacaccacctgtttccaggacgtggtggtggatgtggactgcgccgagaacaccaaagaggatcagctggccgagatcagctaccggttccagggaaagaaagaggccgaccagccttggatcgtggtcaacaccagcacactgttcgacgagctggaactggaccctcctgagattgaacccggggtgctgaaggtgctgagaaccgagaagcagtacctgggagtgtacatctggaacatgagaggcagcgacggcacctctacctacgccacctttctggtcacatggaagggcgacgagaaaacacggaaccccacaccagctgtgacccctcaacctagaggcgccgagtttcacatgtggaattaccacagccacgtgttcagcgtgggcgatacctttagcctggccatgcatctgcagtacaagatccacgaggcccctttcgacctgctgctggaatggctgtacgtgcccatcgatcctacctgccagcctatgcggctgtactccacctgtctgtatcaccccaacgctccccagtgcctgagccacatgaatagcggctgcaccttcacaagccctcacctggctcagcgagtggccagcacagtgtaccagaattgcgagcacgccgacaattacaccgcctactgtctgggcatcagccacatggaacctagcttcggcctgatcctgcacgatggcggcacaaccctgaagttcgtggatacccctgagagcctgagcggcctgtatgtgttcgtggtgtacttcaacggccacgtggaagccgtggcctacaccgtggtgtctaccgtggaccacttcgtgaacgccatcgaggaaagaggcttccctccaactgctggacagcctcctgccaccaccaagcctaaagaaatcacacccgtgaatcccggcacaagcccactgcttagatacgccgcttggacaggcggactggctgctgttgttctgctgtgcctggtcatcttcctgatctgcaccgccaagcggatgagagtgaaggacgccgagaaggacaagtga

SEQ ID NO: 87 - protein, 573 aa, synthetic construct
MGTVNKPVVGVLMGFGIITGTLRITNPVRASVLRYDDFHIDEDKLDTNSVYEPYYHSDHAESSWVNRGESSRKAYDHNSPYIWPRNDYDGFLENAHEHHGVYNQGRGIDSGERLMQPTQMSAQEDLGDDTGIHVIPTLNGDDRHKIVNVDQRQYGDVFKGDLNPKPQGQRLIEVSVEENHPFTLRAPIQRIYGVRYTETWSFLPSLTCTGDAAPAIQHICLKHTTCFQDVVVDVDCAENTKEDQLAEISYRFQGKKEADQPWIVVNTSTLFDELELDPPEIEPGVLKVLRTEKQYLGVYIWNMRGSDGTSTYATFLVTWKGDEKTRNPTPAVTPQPRGAEFHMWNYHSHVFSVGDTFSLAMHLQYKIHEAPFDLLLEWLYVPIDPTCQPMRLYSTCLYHPNAPQCLSHMNSGCTFTSPHLAQRVASTVYQNCEHADNYTAYCLGISHMEPSFGLILHDGGTTLKFVDTPESLSGLYVFVVYFNGHVEAVAYTVVSTVDHFVNAIEERGFPPTAGQPPATTKPKEITPVNPGTSPLLRYAAWTGGLAAVVLLCLVIFLICTAKRMRVKDAEKDK

SEQ ID NO: 88 - RNA, 2017 nt, synthetic construct
  source 1..2017: mol_type = other RNA
agactcctccccatcctctccctctgtccctctgtccctctgaccctgcactgtcccagcaccgccaccatgggcaccgtgaacaagcctgttgtgggcgtgctgatgggcttcggcatcatcacaggcaccctgcggatcaccaatcctgtgcgggctagcgtgctgagatacgacgacttccacatcgacgaggacaagctggacaccaacagcgtgtacgagccctactaccacagcgatcacgccgagtctagctgggtcaacagaggcgagagcagcagaaaggcctacgaccacaacagcccctacatctggccccggaacgactacgatggcttcctggaaaatgcccacgagcaccacggcgtgtacaatcaaggcagaggcatcgacagcggcgagagactgatgcagcctacacagatgagcgcccaagaggacctgggagatgataccggcatccacgtgatccccacactgaacggcgacgacagacacaagatcgtgaacgtggaccagcggcagtacggcgacgtgttcaagggcgacctgaatcctaagcctcagggccagcgcctgatcgaggtgtccgtggaagagaatcaccccttcacactgagagcccctatccagagaatctacggcgtgcgctataccgagacatggtcctttctgcccagcctgacatgtaccggggatgccgctcctgccatccagcacatttgcctgaagcacaccacctgtttccaggacgtggtggtggatgtggactgcgccgagaacaccaaagaggatcagctggccgagatcagctaccggttccagggaaagaaagaggccgaccagccttggatcgtggtcaacaccagcacactgttcgacgagctggaactggaccctcctgagattgaacccggggtgctgaaggtgctgagaaccgagaagcagtacctgggagtgtacatctggaacatgagaggcagcgacggcacctctacctacgccacctttctggtcacatggaagggcgacgagaaaacacggaaccccacaccagctgtgacccctcaacctagaggcgccgagtttcacatgtggaattaccacagccacgtgttcagcgtgggcgatacctttagcctggccatgcatctgcagtacaagatccacgaggcccctttcgacctgctgctggaatggctgtacgtgcccatcgatcctacctgccagcctatgcggctgtactccacctgtctgtatcaccccaacgctccccagtgcctgagccacatgaatagcggctgcaccttcacaagccctcacctggctcagcgagtggccagcacagtgtaccagaattgcgagcacgccgacaattacaccgcctactgtctgggcatcagccacatggaacctagcttcggcctgatcctgcacgatggcggcacaaccctgaagttcgtggatacccctgagagcctgagcggcctgtatgtgttcgtggtgtacttcaacggccacgtggaagccgtggcctacaccgtggtgtctaccgtggaccacttcgtgaacgccatcgaggaaagaggcttccctccaactgctggacagcctcctgccaccaccaagcctaaagaaatcacacccgtgaatcccggcacaagcccactgcttagatacgccgcttggacaggcggactggctgctgttgttctgctgtgcctggtcatcttcctgatctgcaccgccaagcggatgagagtgaaggacgccgagaaggacaagtgataataggctggagcctcggtggccatgcttcttgccccttgggcctccccccagcccctcctccccttcctgcacccgtacccccgtggtctttgaataaagtctgagtgggcggcaaaaaaaaaaaaaaaaaaaaaaaaaaaaaaaaaaaaaaaaaaaaaaaaaaaaaaaaaaaaaaaaaaaaaaaaaaaaaaaaaaaaaaaaaaaaaaaaaaaaaaaaaaaaaa

SEQ ID NO: 89 - DNA, 2014 bp, synthetic construct
  source 1..2014: mol_type = other DNA
agactcctccccatcctctccctctgtccctctgtccctctgaccctgcactgtcccagcaccgccaccatgggcaccgtgaacaagcctgttgtgggcgtgctgatgggcttcggcatcatcacaggcaccctgcggatcaccaatcctgtgcgggctagcgtgctgagatacgacgacttccacatcgacgaggacaagctggacaccaacagcgtgtacgagccctactaccacagcgatcacgccgagtctagctgggtcaacagaggcgagagcagcagaaaggcctacgaccacaacagcccctacatctggccccggaacgactacgatggcttcctggaaaatgcccacgagcaccacggcgtgtacaatcaaggcagaggcatcgacagcggcgagagactgatgcagcctacacagatgagcgcccaagaggacctgggagatgataccggcatccacgtgatccccacactgaacggcgacgacagacacaagatcgtgaacgtggaccagcggcagtacggcgacgtgttcaagggcgacctgaatcctaagcctcagggccagcgcctgatcgaggtgtccgtggaagagaatcaccccttcacactgagagcccctatccagagaatctacggcgtgcgctataccgagacatggtcctttctgcccagcctgacatgtaccggggatgccgctcctgccatccagcacatttgcctgaagcacaccacctgtttccaggacgtggtggtggatgtggactgcgccgagaacaccaaagaggatcagctggccgagatcagctaccggttccagggaaagaaagaggccgaccagccttggatcgtggtcaacaccagcacactgttcgacgagctggaactggaccctcctgagattgaacccggggtgctgaaggtgctgagaaccgagaagcagtacctgggagtgtacatctggaacatgagaggcagcgacggcacctctacctacgccacctttctggtcacatggaagggcgacgagaaaacacggaaccccacaccagctgtgacccctcaacctagaggcgccgagtttcacatgtggaattaccacagccacgtgttcagcgtgggcgatacctttagcctggccatgcatctgcagtacaagatccacgaggcccctttcgacctgctgctggaatggctgtacgtgcccatcgatcctacctgccagcctatgcggctgtactccacctgtctgtatcaccccaacgctccccagtgcctgagccacatgaatagcggctgcaccttcacaagccctcacctggctcagcgagtggccagcacagtgtaccagaattgcgagcacgccgacaattacaccgcctactgtctgggcatcagccacatggaacctagcttcggcctgatcctgcacgatggcggcacaaccctgaagttcgtggatacccctgagagcctgagcggcctgtatgtgttcgtggtgtacttcaacggccacgtggaagccgtggcctacaccgtggtgtctaccgtggaccacttcgtgaacgccatcgaggaaagaggcttccctccaactgctggacagcctcctgccaccaccaagcctaaagaaatcacacccgtgaatcccggcacaagcccactgcttagatacgccgcttggacaggcggactggctgctgttgttctgctgtgcctggtcatcttcctgatctgcaccgccaagcggatgcgcgtgaagaaagagaaggacaagtgataataggctggagcctcggtggccatgcttcttgccccttgggcctccccccagcccctcctccccttcctgcacccgtacccccgtggtctttgaataaagtctgagtgggcggcaaaaaaaaaaaaaaaaaaaaaaaaaaaaaaaaaaaaaaaaaaaaaaaaaaaaaaaaaaaaaaaaaaaaaaaaaaaaaaaaaaaaaaaaaaaaaaaaaaaaaaaaaaaaaa

SEQ ID NO: 90 - DNA, 1719 bp, synthetic construct
  source 1..1719: mol_type = other DNA
atgggcaccgtgaacaagcctgttgtgggcgtgctgatgggcttcggcatcatcacaggcaccctgcggatcaccaatcctgtgcgggctagcgtgctgagatacgacgacttccacatcgacgaggacaagctggacaccaacagcgtgtacgagccctactaccacagcgatcacgccgagtctagctgggtcaacagaggcgagagcagcagaaaggcctacgaccacaacagcccctacatctggccccggaacgactacgatggcttcctggaaaatgcccacgagcaccacggcgtgtacaatcaaggcagaggcatcgacagcggcgagagactgatgcagcctacacagatgagcgcccaagaggacctgggagatgataccggcatccacgtgatccccacactgaacggcgacgacagacacaagatcgtgaacgtggaccagcggcagtacggcgacgtgttcaagggcgacctgaatcctaagcctcagggccagcgcctgatcgaggtgtccgtggaagagaatcaccccttcacactgagagcccctatccagagaatctacggcgtgcgctataccgagacatggtcctttctgcccagcctgacatgtaccggggatgccgctcctgccatccagcacatttgcctgaagcacaccacctgtttccaggacgtggtggtggatgtggactgcgccgagaacaccaaagaggatcagctggccgagatcagctaccggttccagggaaagaaagaggccgaccagccttggatcgtggtcaacaccagcacactgttcgacgagctggaactggaccctcctgagattgaacccggggtgctgaaggtgctgagaaccgagaagcagtacctgggagtgtacatctggaacatgagaggcagcgacggcacctctacctacgccacctttctggtcacatggaagggcgacgagaaaacacggaaccccacaccagctgtgacccctcaacctagaggcgccgagtttcacatgtggaattaccacagccacgtgttcagcgtgggcgatacctttagcctggccatgcatctgcagtacaagatccacgaggcccctttcgacctgctgctggaatggctgtacgtgcccatcgatcctacctgccagcctatgcggctgtactccacctgtctgtatcaccccaacgctccccagtgcctgagccacatgaatagcggctgcaccttcacaagccctcacctggctcagcgagtggccagcacagtgtaccagaattgcgagcacgccgacaattacaccgcctactgtctgggcatcagccacatggaacctagcttcggcctgatcctgcacgatggcggcacaaccctgaagttcgtggatacccctgagagcctgagcggcctgtatgtgttcgtggtgtacttcaacggccacgtggaagccgtggcctacaccgtggtgtctaccgtggaccacttcgtgaacgccatcgaggaaagaggcttccctccaactgctggacagcctcctgccaccaccaagcctaaagaaatcacacccgtgaatcccggcacaagcccactgcttagatacgccgcttggacaggcggactggctgctgttgttctgctgtgcctggtcatcttcctgatctgcaccgccaagcggatgcgcgtgaagaaagagaaggacaagtga

SEQ ID NO: 91 - protein, 572 aa, synthetic construct
MGTVNKPVVGVLMGFGIITGTLRITNPVRASVLRYDDFHIDEDKLDTNSVYEPYYHSDHAESSWVNRGESSRKAYDHNSPYIWPRNDYDGFLENAHEHHGVYNQGRGIDSGERLMQPTQMSAQEDLGDDTGIHVIPTLNGDDRHKIVNVDQRQYGDVFKGDLNPKPQGQRLIEVSVEENHPFTLRAPIQRIYGVRYTETWSFLPSLTCTGDAAPAIQHICLKHTTCFQDVVVDVDCAENTKEDQLAEISYRFQGKKEADQPWIVVNTSTLFDELELDPPEIEPGVLKVLRTEKQYLGVYIWNMRGSDGTSTYATFLVTWKGDEKTRNPTPAVTPQPRGAEFHMWNYHSHVFSVGDTFSLAMHLQYKIHEAPFDLLLEWLYVPIDPTCQPMRLYSTCLYHPNAPQCLSHMNSGCTFTSPHLAQRVASTVYQNCEHADNYTAYCLGISHMEPSFGLILHDGGTTLKFVDTPESLSGLYVFVVYFNGHVEAVAYTVVSTVDHFVNAIEERGFPPTAGQPPATTKPKEITPVNPGTSPLLRYAAWTGGLAAVVLLCLVIFLICTAKRMRVKKEKDK

SEQ ID NO: 92 - RNA, 2014 nt, synthetic construct
  source 1..2014: mol_type = other RNA
agactcctccccatcctctccctctgtccctctgtccctctgaccctgcactgtcccagcaccgccaccatgggcaccgtgaacaagcctgttgtgggcgtgctgatgggcttcggcatcatcacaggcaccctgcggatcaccaatcctgtgcgggctagcgtgctgagatacgacgacttccacatcgacgaggacaagctggacaccaacagcgtgtacgagccctactaccacagcgatcacgccgagtctagctgggtcaacagaggcgagagcagcagaaaggcctacgaccacaacagcccctacatctggccccggaacgactacgatggcttcctggaaaatgcccacgagcaccacggcgtgtacaatcaaggcagaggcatcgacagcggcgagagactgatgcagcctacacagatgagcgcccaagaggacctgggagatgataccggcatccacgtgatccccacactgaacggcgacgacagacacaagatcgtgaacgtggaccagcggcagtacggcgacgtgttcaagggcgacctgaatcctaagcctcagggccagcgcctgatcgaggtgtccgtggaagagaatcaccccttcacactgagagcccctatccagagaatctacggcgtgcgctataccgagacatggtcctttctgcccagcctgacatgtaccggggatgccgctcctgccatccagcacatttgcctgaagcacaccacctgtttccaggacgtggtggtggatgtggactgcgccgagaacaccaaagaggatcagctggccgagatcagctaccggttccagggaaagaaagaggccgaccagccttggatcgtggtcaacaccagcacactgttcgacgagctggaactggaccctcctgagattgaacccggggtgctgaaggtgctgagaaccgagaagcagtacctgggagtgtacatctggaacatgagaggcagcgacggcacctctacctacgccacctttctggtcacatggaagggcgacgagaaaacacggaaccccacaccagctgtgacccctcaacctagaggcgccgagtttcacatgtggaattaccacagccacgtgttcagcgtgggcgatacctttagcctggccatgcatctgcagtacaagatccacgaggcccctttcgacctgctgctggaatggctgtacgtgcccatcgatcctacctgccagcctatgcggctgtactccacctgtctgtatcaccccaacgctccccagtgcctgagccacatgaatagcggctgcaccttcacaagccctcacctggctcagcgagtggccagcacagtgtaccagaattgcgagcacgccgacaattacaccgcctactgtctgggcatcagccacatggaacctagcttcggcctgatcctgcacgatggcggcacaaccctgaagttcgtggatacccctgagagcctgagcggcctgtatgtgttcgtggtgtacttcaacggccacgtggaagccgtggcctacaccgtggtgtctaccgtggaccacttcgtgaacgccatcgaggaaagaggcttccctccaactgctggacagcctcctgccaccaccaagcctaaagaaatcacacccgtgaatcccggcacaagcccactgcttagatacgccgcttggacaggcggactggctgctgttgttctgctgtgcctggtcatcttcctgatctgcaccgccaagcggatgcgcgtgaagaaagagaaggacaagtgataataggctggagcctcggtggccatgcttcttgccccttgggcctccccccagcccctcctccccttcctgcacccgtacccccgtggtctttgaataaagtctgagtgggcggcaaaaaaaaaaaaaaaaaaaaaaaaaaaaaaaaaaaaaaaaaaaaaaaaaaaaaaaaaaaaaaaaaaaaaaaaaaaaaaaaaaaaaaaaaaaaaaaaaaaaaaaaaaaaaa

SEQ ID NO: 93 - DNA, 2059 bp, synthetic construct
  source 1..2059: mol_type = other DNA
agactcctccccatcctctccctctgtccctctgtccctctgaccctgcactgtcccagcaccgccaccatgggcaccgtgaacaagcctgttgtgggcgtgctgatgggcttcggcatcatcacaggcaccctgcggatcaccaatcctgtgcgggctagcgtgctgagatacgacgacttccacatcgacgaggacaagctggacaccaacagcgtgtacgagccctactaccacagcgatcacgccgagtctagctgggtcaacagaggcgagagcagcagaaaggcctacgaccacaacagcccctacatctggccccggaacgactacgatggcttcctggaaaatgcccacgagcaccacggcgtgtacaatcaaggcagaggcatcgacagcggcgagagactgatgcagcctacacagatgagcgcccaagaggacctgggagatgataccggcatccacgtgatccccacactgaacggcgacgacagacacaagatcgtgaacgtggaccagcggcagtacggcgacgtgttcaagggcgacctgaatcctaagcctcagggccagcgcctgatcgaggtgtccgtggaagagaatcaccccttcacactgagagcccctatccagagaatctacggcgtgcgctataccgagacatggtcctttctgcccagcctgacatgtaccggggatgccgctcctgccatccagcacatttgcctgaagcacaccacctgtttccaggacgtggtggtggatgtggactgcgccgagaacaccaaagaggatcagctggccgagatcagctaccggttccagggaaagaaagaggccgaccagccttggatcgtggtcaacaccagcacactgttcgacgagctggaactggaccctcctgagattgaacccggggtgctgaaggtgctgagaaccgagaagcagtacctgggagtgtacatctggaacatgagaggcagcgacggcacctctacctacgccacctttctggtcacatggaagggcgacgagaaaacacggaaccccacaccagctgtgacccctcaacctagaggcgccgagtttcacatgtggaattaccacagccacgtgttcagcgtgggcgatacctttagcctggccatgcatctgcagtacaagatccacgaggcccctttcgacctgctgctggaatggctgtacgtgcccatcgatcctacctgccagcctatgcggctgtactccacctgtctgtatcaccccaacgctccccagtgcctgagccacatgaatagcggctgcaccttcacaagccctcacctggctcagcgagtggccagcacagtgtaccagaattgcgagcacgccgacaattacaccgcctactgtctgggcatcagccacatggaacctagcttcggcctgatcctgcacgatggcggcacaaccctgaagttcgtggatacccctgagagcctgagcggcctgtatgtgttcgtggtgtacttcaacggccacgtggaagccgtggcctacaccgtggtgtctaccgtggaccacttcgtgaacgccatcgaggaaagaggcttccctccaactgctggacagcctcctgccaccaccaagcctaaagaaatcacacccgtgaatcccggcacaagcccactgcttagatacgccgcttggacaggcggactggctgctgttgttctgctgtgcctggtcatcttcctgatctgcaccgccaagcggatgagagtgaaggcctacagagtggacaagagcccttacaaccagagcatgtactacgccggcctgcctgtttgataataggctggagcctcggtggccatgcttcttgccccttgggcctccccccagcccctcctccccttcctgcacccgtacccccgtggtctttgaataaagtctgagtgggcggcaaaaaaaaaaaaaaaaaaaaaaaaaaaaaaaaaaaaaaaaaaaaaaaaaaaaaaaaaaaaaaaaaaaaaaaaaaaaaaaaaaaaaaaaaaaaaaaaaaaaaaaaaaaaaa

SEQ ID NO: 94 - DNA, 1764 bp, synthetic construct
  source 1..1764: mol_type = other DNA
atgggcaccgtgaacaagcctgttgtgggcgtgctgatgggcttcggcatcatcacaggcaccctgcggatcaccaatcctgtgcgggctagcgtgctgagatacgacgacttccacatcgacgaggacaagctggacaccaacagcgtgtacgagccctactaccacagcgatcacgccgagtctagctgggtcaacagaggcgagagcagcagaaaggcctacgaccacaacagcccctacatctggccccggaacgactacgatggcttcctggaaaatgcccacgagcaccacggcgtgtacaatcaaggcagaggcatcgacagcggcgagagactgatgcagcctacacagatgagcgcccaagaggacctgggagatgataccggcatccacgtgatccccacactgaacggcgacgacagacacaagatcgtgaacgtggaccagcggcagtacggcgacgtgttcaagggcgacctgaatcctaagcctcagggccagcgcctgatcgaggtgtccgtggaagagaatcaccccttcacactgagagcccctatccagagaatctacggcgtgcgctataccgagacatggtcctttctgcccagcctgacatgtaccggggatgccgctcctgccatccagcacatttgcctgaagcacaccacctgtttccaggacgtggtggtggatgtggactgcgccgagaacaccaaagaggatcagctggccgagatcagctaccggttccagggaaagaaagaggccgaccagccttggatcgtggtcaacaccagcacactgttcgacgagctggaactggaccctcctgagattgaacccggggtgctgaaggtgctgagaaccgagaagcagtacctgggagtgtacatctggaacatgagaggcagcgacggcacctctacctacgccacctttctggtcacatggaagggcgacgagaaaacacggaaccccacaccagctgtgacccctcaacctagaggcgccgagtttcacatgtggaattaccacagccacgtgttcagcgtgggcgatacctttagcctggccatgcatctgcagtacaagatccacgaggcccctttcgacctgctgctggaatggctgtacgtgcccatcgatcctacctgccagcctatgcggctgtactccacctgtctgtatcaccccaacgctccccagtgcctgagccacatgaatagcggctgcaccttcacaagccctcacctggctcagcgagtggccagcacagtgtaccagaattgcgagcacgccgacaattacaccgcctactgtctgggcatcagccacatggaacctagcttcggcctgatcctgcacgatggcggcacaaccctgaagttcgtggatacccctgagagcctgagcggcctgtatgtgttcgtggtgtacttcaacggccacgtggaagccgtggcctacaccgtggtgtctaccgtggaccacttcgtgaacgccatcgaggaaagaggcttccctccaactgctggacagcctcctgccaccaccaagcctaaagaaatcacacccgtgaatcccggcacaagcccactgcttagatacgccgcttggacaggcggactggctgctgttgttctgctgtgcctggtcatcttcctgatctgcaccgccaagcggatgagagtgaaggcctacagagtggacaagagcccttacaaccagagcatgtactacgccggcctgcctgtttga

SEQ ID NO: 95 - protein, 587 aa, synthetic construct
MGTVNKPVVGVLMGFGIITGTLRITNPVRASVLRYDDFHIDEDKLDTNSVYEPYYHSDHAESSWVNRGESSRKAYDHNSPYIWPRNDYDGFLENAHEHHGVYNQGRGIDSGERLMQPTQMSAQEDLGDDTGIHVIPTLNGDDRHKIVNVDQRQYGDVFKGDLNPKPQGQRLIEVSVEENHPFTLRAPIQRIYGVRYTETWSFLPSLTCTGDAAPAIQHICLKHTTCFQDVVVDVDCAENTKEDQLAEISYRFQGKKEADQPWIVVNTSTLFDELELDPPEIEPGVLKVLRTEKQYLGVYIWNMRGSDGTSTYATFLVTWKGDEKTRNPTPAVTPQPRGAEFHMWNYHSHVFSVGDTFSLAMHLQYKIHEAPFDLLLEWLYVPIDPTCQPMRLYSTCLYHPNAPQCLSHMNSGCTFTSPHLAQRVASTVYQNCEHADNYTAYCLGISHMEPSFGLILHDGGTTLKFVDTPESLSGLYVFVVYFNGHVEAVAYTVVSTVDHFVNAIEERGFPPTAGQPPATTKPKEITPVNPGTSPLLRYAAWTGGLAAVVLLCLVIFLICTAKRMRVKAYRVDKSPYNQSMYYAGLPV

SEQ ID NO: 96 - RNA, 2059 nt, synthetic construct
  source 1..2059: mol_type = other RNA
agactcctccccatcctctccctctgtccctctgtccctctgaccctgcactgtcccagcaccgccaccatgggcaccgtgaacaagcctgttgtgggcgtgctgatgggcttcggcatcatcacaggcaccctgcggatcaccaatcctgtgcgggctagcgtgctgagatacgacgacttccacatcgacgaggacaagctggacaccaacagcgtgtacgagccctactaccacagcgatcacgccgagtctagctgggtcaacagaggcgagagcagcagaaaggcctacgaccacaacagcccctacatctggccccggaacgactacgatggcttcctggaaaatgcccacgagcaccacggcgtgtacaatcaaggcagaggcatcgacagcggcgagagactgatgcagcctacacagatgagcgcccaagaggacctgggagatgataccggcatccacgtgatccccacactgaacggcgacgacagacacaagatcgtgaacgtggaccagcggcagtacggcgacgtgttcaagggcgacctgaatcctaagcctcagggccagcgcctgatcgaggtgtccgtggaagagaatcaccccttcacactgagagcccctatccagagaatctacggcgtgcgctataccgagacatggtcctttctgcccagcctgacatgtaccggggatgccgctcctgccatccagcacatttgcctgaagcacaccacctgtttccaggacgtggtggtggatgtggactgcgccgagaacaccaaagaggatcagctggccgagatcagctaccggttccagggaaagaaagaggccgaccagccttggatcgtggtcaacaccagcacactgttcgacgagctggaactggaccctcctgagattgaacccggggtgctgaaggtgctgagaaccgagaagcagtacctgggagtgtacatctggaacatgagaggcagcgacggcacctctacctacgccacctttctggtcacatggaagggcgacgagaaaacacggaaccccacaccagctgtgacccctcaacctagaggcgccgagtttcacatgtggaattaccacagccacgtgttcagcgtgggcgatacctttagcctggccatgcatctgcagtacaagatccacgaggcccctttcgacctgctgctggaatggctgtacgtgcccatcgatcctacctgccagcctatgcggctgtactccacctgtctgtatcaccccaacgctccccagtgcctgagccacatgaatagcggctgcaccttcacaagccctcacctggctcagcgagtggccagcacagtgtaccagaattgcgagcacgccgacaattacaccgcctactgtctgggcatcagccacatggaacctagcttcggcctgatcctgcacgatggcggcacaaccctgaagttcgtggatacccctgagagcctgagcggcctgtatgtgttcgtggtgtacttcaacggccacgtggaagccgtggcctacaccgtggtgtctaccgtggaccacttcgtgaacgccatcgaggaaagaggcttccctccaactgctggacagcctcctgccaccaccaagcctaaagaaatcacacccgtgaatcccggcacaagcccactgcttagatacgccgcttggacaggcggactggctgctgttgttctgctgtgcctggtcatcttcctgatctgcaccgccaagcggatgagagtgaaggcctacagagtggacaagagcccttacaaccagagcatgtactacgccggcctgcctgtttgataataggctggagcctcggtggccatgcttcttgccccttgggcctccccccagcccctcctccccttcctgcacccgtacccccgtggtctttgaataaagtctgagtgggcggcaaaaaaaaaaaaaaaaaaaaaaaaaaaaaaaaaaaaaaaaaaaaaaaaaaaaaaaaaaaaaaaaaaaaaaaaaaaaaaaaaaaaaaaaaaaaaaaaaaaaaaaaaaaaaa

SEQ ID NO: 97 - DNA, 2026 bp, synthetic construct
  source 1..2026: mol_type = other DNA
agactcctccccatcctctccctctgtccctctgtccctctgaccctgcactgtcccagcaccgccaccatgggcaccgtgaacaagcctgttgtgggcgtgctgatgggcttcggcatcatcacaggcaccctgcggatcaccaatcctgtgcgggctagcgtgctgagatacgacgacttccacatcgacgaggacaagctggacaccaacagcgtgtacgagccctactaccacagcgatcacgccgagtctagctgggtcaacagaggcgagagcagcagaaaggcctacgaccacaacagcccctacatctggccccggaacgactacgatggcttcctggaaaatgcccacgagcaccacggcgtgtacaatcaaggcagaggcatcgacagcggcgagagactgatgcagcctacacagatgagcgcccaagaggacctgggagatgataccggcatccacgtgatccccacactgaacggcgacgacagacacaagatcgtgaacgtggaccagcggcagtacggcgacgtgttcaagggcgacctgaatcctaagcctcagggccagcgcctgatcgaggtgtccgtggaagagaatcaccccttcacactgagagcccctatccagagaatctacggcgtgcgctataccgagacatggtcctttctgcccagcctgacatgtaccggggatgccgctcctgccatccagcacatttgcctgaagcacaccacctgtttccaggacgtggtggtggatgtggactgcgccgagaacaccaaagaggatcagctggccgagatcagctaccggttccagggaaagaaagaggccgaccagccttggatcgtggtcaacaccagcacactgttcgacgagctggaactggaccctcctgagattgaacccggggtgctgaaggtgctgagaaccgagaagcagtacctgggagtgtacatctggaacatgagaggcagcgacggcacctctacctacgccacctttctggtcacatggaagggcgacgagaaaacacggaaccccacaccagctgtgacccctcaacctagaggcgccgagtttcacatgtggaattaccacagccacgtgttcagcgtgggcgatacctttagcctggccatgcatctgcagtacaagatccacgaggcccctttcgacctgctgctggaatggctgtacgtgcccatcgatcctacctgccagcctatgcggctgtactccacctgtctgtatcaccccaacgctccccagtgcctgagccacatgaatagcggctgcaccttcacaagccctcacctggctcagcgagtggccagcacagtgtaccagaattgcgagcacgccgacaattacaccgcctactgtctgggcatcagccacatggaacctagcttcggcctgatcctgcacgatggcggcacaaccctgaagttcgtggatacccctgagagcctgagcggcctgtatgtgttcgtggtgtacttcaacggccacgtggaagccgtggcctacaccgtggtgtctaccgtggaccacttcgtgaacgccatcgaggaaagaggcttccctccaactgctggacagcctcctgccaccaccaagcctaaagaaatcacacccgtgaatcccggcacaagcccactgcttagatacgccgcttggacaggcggactggctgctgttgttctgctgtgcctggtcatcttcctgatctgcaccgccaagcggatgagagtgaaggccatgtactatgccggcctgcctgtttgataataggctggagcctcggtggccatgcttcttgccccttgggcctccccccagcccctcctccccttcctgcacccgtacccccgtggtctttgaataaagtctgagtgggcggcaaaaaaaaaaaaaaaaaaaaaaaaaaaaaaaaaaaaaaaaaaaaaaaaaaaaaaaaaaaaaaaaaaaaaaaaaaaaaaaaaaaaaaaaaaaaaaaaaaaaaaaaaaaaaa

SEQ ID NO: 98 - DNA, 1731 bp, synthetic construct
  source 1..1731: mol_type = other DNA
atgggcaccgtgaacaagcctgttgtgggcgtgctgatgggcttcggcatcatcacaggcaccctgcggatcaccaatcctgtgcgggctagcgtgctgagatacgacgacttccacatcgacgaggacaagctggacaccaacagcgtgtacgagccctactaccacagcgatcacgccgagtctagctgggtcaacagaggcgagagcagcagaaaggcctacgaccacaacagcccctacatctggccccggaacgactacgatggcttcctggaaaatgcccacgagcaccacggcgtgtacaatcaaggcagaggcatcgacagcggcgagagactgatgcagcctacacagatgagcgcccaagaggacctgggagatgataccggcatccacgtgatccccacactgaacggcgacgacagacacaagatcgtgaacgtggaccagcggcagtacggcgacgtgttcaagggcgacctgaatcctaagcctcagggccagcgcctgatcgaggtgtccgtggaagagaatcaccccttcacactgagagcccctatccagagaatctacggcgtgcgctataccgagacatggtcctttctgcccagcctgacatgtaccggggatgccgctcctgccatccagcacatttgcctgaagcacaccacctgtttccaggacgtggtggtggatgtggactgcgccgagaacaccaaagaggatcagctggccgagatcagctaccggttccagggaaagaaagaggccgaccagccttggatcgtggtcaacaccagcacactgttcgacgagctggaactggaccctcctgagattgaacccggggtgctgaaggtgctgagaaccgagaagcagtacctgggagtgtacatctggaacatgagaggcagcgacggcacctctacctacgccacctttctggtcacatggaagggcgacgagaaaacacggaaccccacaccagctgtgacccctcaacctagaggcgccgagtttcacatgtggaattaccacagccacgtgttcagcgtgggcgatacctttagcctggccatgcatctgcagtacaagatccacgaggcccctttcgacctgctgctggaatggctgtacgtgcccatcgatcctacctgccagcctatgcggctgtactccacctgtctgtatcaccccaacgctccccagtgcctgagccacatgaatagcggctgcaccttcacaagccctcacctggctcagcgagtggccagcacagtgtaccagaattgcgagcacgccgacaattacaccgcctactgtctgggcatcagccacatggaacctagcttcggcctgatcctgcacgatggcggcacaaccctgaagttcgtggatacccctgagagcctgagcggcctgtatgtgttcgtggtgtacttcaacggccacgtggaagccgtggcctacaccgtggtgtctaccgtggaccacttcgtgaacgccatcgaggaaagaggcttccctccaactgctggacagcctcctgccaccaccaagcctaaagaaatcacacccgtgaatcccggcacaagcccactgcttagatacgccgcttggacaggcggactggctgctgttgttctgctgtgcctggtcatcttcctgatctgcaccgccaagcggatgagagtgaaggccatgtactatgccggcctgcctgtttga

SEQ ID NO: 99 - protein, 576 aa, synthetic construct
MGTVNKPVVGVLMGFGIITGTLRITNPVRASVLRYDDFHIDEDKLDTNSVYEPYYHSDHAESSWVNRGESSRKAYDHNSPYIWPRNDYDGFLENAHEHHGVYNQGRGIDSGERLMQPTQMSAQEDLGDDTGIHVIPTLNGDDRHKIVNVDQRQYGDVFKGDLNPKPQGQRLIEVSVEENHPFTLRAPIQRIYGVRYTETWSFLPSLTCTGDAAPAIQHICLKHTTCFQDVVVDVDCAENTKEDQLAEISYRFQGKKEADQPWIVVNTSTLFDELELDPPEIEPGVLKVLRTEKQYLGVYIWNMRGSDGTSTYATFLVTWKGDEKTRNPTPAVTPQPRGAEFHMWNYHSHVFSVGDTFSLAMHLQYKIHEAPFDLLLEWLYVPIDPTCQPMRLYSTCLYHPNAPQCLSHMNSGCTFTSPHLAQRVASTVYQNCEHADNYTAYCLGISHMEPSFGLILHDGGTTLKFVDTPESLSGLYVFVVYFNGHVEAVAYTVVSTVDHFVNAIEERGFPPTAGQPPATTKPKEITPVNPGTSPLLRYAAWTGGLAAVVLLCLVIFLICTAKRMRVKAMYYAGLPV

SEQ ID NO: 100 - RNA, 2026 nt, synthetic construct
  source 1..2026: mol_type = other RNA
agactcctccccatcctctccctctgtccctctgtccctctgaccctgcactgtcccagcaccgccaccatgggcaccgtgaacaagcctgttgtgggcgtgctgatgggcttcggcatcatcacaggcaccctgcggatcaccaatcctgtgcgggctagcgtgctgagatacgacgacttccacatcgacgaggacaagctggacaccaacagcgtgtacgagccctactaccacagcgatcacgccgagtctagctgggtcaacagaggcgagagcagcagaaaggcctacgaccacaacagcccctacatctggccccggaacgactacgatggcttcctggaaaatgcccacgagcaccacggcgtgtacaatcaaggcagaggcatcgacagcggcgagagactgatgcagcctacacagatgagcgcccaagaggacctgggagatgataccggcatccacgtgatccccacactgaacggcgacgacagacacaagatcgtgaacgtggaccagcggcagtacggcgacgtgttcaagggcgacctgaatcctaagcctcagggccagcgcctgatcgaggtgtccgtggaagagaatcaccccttcacactgagagcccctatccagagaatctacggcgtgcgctataccgagacatggtcctttctgcccagcctgacatgtaccggggatgccgctcctgccatccagcacatttgcctgaagcacaccacctgtttccaggacgtggtggtggatgtggactgcgccgagaacaccaaagaggatcagctggccgagatcagctaccggttccagggaaagaaagaggccgaccagccttggatcgtggtcaacaccagcacactgttcgacgagctggaactggaccctcctgagattgaacccggggtgctgaaggtgctgagaaccgagaagcagtacctgggagtgtacatctggaacatgagaggcagcgacggcacctctacctacgccacctttctggtcacatggaagggcgacgagaaaacacggaaccccacaccagctgtgacccctcaacctagaggcgccgagtttcacatgtggaattaccacagccacgtgttcagcgtgggcgatacctttagcctggccatgcatctgcagtacaagatccacgaggcccctttcgacctgctgctggaatggctgtacgtgcccatcgatcctacctgccagcctatgcggctgtactccacctgtctgtatcaccccaacgctccccagtgcctgagccacatgaatagcggctgcaccttcacaagccctcacctggctcagcgagtggccagcacagtgtaccagaattgcgagcacgccgacaattacaccgcctactgtctgggcatcagccacatggaacctagcttcggcctgatcctgcacgatggcggcacaaccctgaagttcgtggatacccctgagagcctgagcggcctgtatgtgttcgtggtgtacttcaacggccacgtggaagccgtggcctacaccgtggtgtctaccgtggaccacttcgtgaacgccatcgaggaaagaggcttccctccaactgctggacagcctcctgccaccaccaagcctaaagaaatcacacccgtgaatcccggcacaagcccactgcttagatacgccgcttggacaggcggactggctgctgttgttctgctgtgcctggtcatcttcctgatctgcaccgccaagcggatgagagtgaaggccatgtactatgccggcctgcctgtttgataataggctggagcctcggtggccatgcttcttgccccttgggcctccccccagcccctcctccccttcctgcacccgtacccccgtggtctttgaataaagtctgagtgggcggcaaaaaaaaaaaaaaaaaaaaaaaaaaaaaaaaaaaaaaaaaaaaaaaaaaaaaaaaaaaaaaaaaaaaaaaaaaaaaaaaaaaaaaaaaaaaaaaaaaaaaaaaaaaaaa

SEQ ID NO: 101 - DNA, 2026 bp, synthetic construct
  source 1..2026: mol_type = other DNA
agactcctccccatcctctccctctgtccctctgtccctctgaccctgcactgtcccagcaccgccaccatgggcaccgtgaacaagcctgttgtgggcgtgctgatgggcttcggcatcatcacaggcaccctgcggatcaccaatcctgtgcgggctagcgtgctgagatacgacgacttccacatcgacgaggacaagctggacaccaacagcgtgtacgagccctactaccacagcgatcacgccgagtctagctgggtcaacagaggcgagagcagcagaaaggcctacgaccacaacagcccctacatctggccccggaacgactacgatggcttcctggaaaatgcccacgagcaccacggcgtgtacaatcaaggcagaggcatcgacagcggcgagagactgatgcagcctacacagatgagcgcccaagaggacctgggagatgataccggcatccacgtgatccccacactgaacggcgacgacagacacaagatcgtgaacgtggaccagcggcagtacggcgacgtgttcaagggcgacctgaatcctaagcctcagggccagcgcctgatcgaggtgtccgtggaagagaatcaccccttcacactgagagcccctatccagagaatctacggcgtgcgctataccgagacatggtcctttctgcccagcctgacatgtaccggggatgccgctcctgccatccagcacatttgcctgaagcacaccacctgtttccaggacgtggtggtggatgtggactgcgccgagaacaccaaagaggatcagctggccgagatcagctaccggttccagggaaagaaagaggccgaccagccttggatcgtggtcaacaccagcacactgttcgacgagctggaactggaccctcctgagattgaacccggggtgctgaaggtgctgagaaccgagaagcagtacctgggagtgtacatctggaacatgagaggcagcgacggcacctctacctacgccacctttctggtcacatggaagggcgacgagaaaacacggaaccccacaccagctgtgacccctcaacctagaggcgccgagtttcacatgtggaattaccacagccacgtgttcagcgtgggcgatacctttagcctggccatgcatctgcagtacaagatccacgaggcccctttcgacctgctgctggaatggctgtacgtgcccatcgatcctacctgccagcctatgcggctgtactccacctgtctgtatcaccccaacgctccccagtgcctgagccacatgaatagcggctgcaccttcacaagccctcacctggctcagcgagtggccagcacagtgtaccagaattgcgagcacgccgacaattacaccgcctactgtctgggcatcagccacatggaacctagcttcggcctgatcctgcacgatggcggcacaaccctgaagttcgtggatacccctgagagcctgagcggcctgtatgtgttcgtggtgtacttcaacggccacgtggaagccgtggcctacaccgtggtgtctaccgtggaccacttcgtgaacgccatcgaggaaagaggcttccctccaactgctggacagcctcctgccaccaccaagcctaaagaaatcacacccgtgaatcccggcacaagcccactgcttagatacgccgcttggacaggcggactggctgctgttgttctgctgtgcctggtcatcttcctgatctgcaccgccaagcggatgagagtgaaggctatgtatgccgccggactgcctgtttgataataggctggagcctcggtggccatgcttcttgccccttgggcctccccccagcccctcctccccttcctgcacccgtacccccgtggtctttgaataaagtctgagtgggcggcaaaaaaaaaaaaaaaaaaaaaaaaaaaaaaaaaaaaaaaaaaaaaaaaaaaaaaaaaaaaaaaaaaaaaaaaaaaaaaaaaaaaaaaaaaaaaaaaaaaaaaaaaaaaaa

SEQ ID NO: 102 - DNA, 1731 bp, synthetic construct
  source 1..1731: mol_type = other DNA
atgggcaccgtgaacaagcctgttgtgggcgtgctgatgggcttcggcatcatcacaggcaccctgcggatcaccaatcctgtgcgggctagcgtgctgagatacgacgacttccacatcgacgaggacaagctggacaccaacagcgtgtacgagccctactaccacagcgatcacgccgagtctagctgggtcaacagaggcgagagcagcagaaaggcctacgaccacaacagcccctacatctggccccggaacgactacgatggcttcctggaaaatgcccacgagcaccacggcgtgtacaatcaaggcagaggcatcgacagcggcgagagactgatgcagcctacacagatgagcgcccaagaggacctgggagatgataccggcatccacgtgatccccacactgaacggcgacgacagacacaagatcgtgaacgtggaccagcggcagtacggcgacgtgttcaagggcgacctgaatcctaagcctcagggccagcgcctgatcgaggtgtccgtggaagagaatcaccccttcacactgagagcccctatccagagaatctacggcgtgcgctataccgagacatggtcctttctgcccagcctgacatgtaccggggatgccgctcctgccatccagcacatttgcctgaagcacaccacctgtttccaggacgtggtggtggatgtggactgcgccgagaacaccaaagaggatcagctggccgagatcagctaccggttccagggaaagaaagaggccgaccagccttggatcgtggtcaacaccagcacactgttcgacgagctggaactggaccctcctgagattgaacccggggtgctgaaggtgctgagaaccgagaagcagtacctgggagtgtacatctggaacatgagaggcagcgacggcacctctacctacgccacctttctggtcacatggaagggcgacgagaaaacacggaaccccacaccagctgtgacccctcaacctagaggcgccgagtttcacatgtggaattaccacagccacgtgttcagcgtgggcgatacctttagcctggccatgcatctgcagtacaagatccacgaggcccctttcgacctgctgctggaatggctgtacgtgcccatcgatcctacctgccagcctatgcggctgtactccacctgtctgtatcaccccaacgctccccagtgcctgagccacatgaatagcggctgcaccttcacaagccctcacctggctcagcgagtggccagcacagtgtaccagaattgcgagcacgccgacaattacaccgcctactgtctgggcatcagccacatggaacctagcttcggcctgatcctgcacgatggcggcacaaccctgaagttcgtggatacccctgagagcctgagcggcctgtatgtgttcgtggtgtacttcaacggccacgtggaagccgtggcctacaccgtggtgtctaccgtggaccacttcgtgaacgccatcgaggaaagaggcttccctccaactgctggacagcctcctgccaccaccaagcctaaagaaatcacacccgtgaatcccggcacaagcccactgcttagatacgccgcttggacaggcggactggctgctgttgttctgctgtgcctggtcatcttcctgatctgcaccgccaagcggatgagagtgaaggctatgtatgccgccggactgcctgtttga

SEQ ID NO: 103 - protein, 576 aa, synthetic construct
MGTVNKPVVGVLMGFGIITGTLRITNPVRASVLRYDDFHIDEDKLDTNSVYEPYYHSDHAESSWVNRGESSRKAYDHNSPYIWPRNDYDGFLENAHEHHGVYNQGRGIDSGERLMQPTQMSAQEDLGDDTGIHVIPTLNGDDRHKIVNVDQRQYGDVFKGDLNPKPQGQRLIEVSVEENHPFTLRAPIQRIYGVRYTETWSFLPSLTCTGDAAPAIQHICLKHTTCFQDVVVDVDCAENTKEDQLAEISYRFQGKKEADQPWIVVNTSTLFDELELDPPEIEPGVLKVLRTEKQYLGVYIWNMRGSDGTSTYATFLVTWKGDEKTRNPTPAVTPQPRGAEFHMWNYHSHVFSVGDTFSLAMHLQYKIHEAPFDLLLEWLYVPIDPTCQPMRLYSTCLYHPNAPQCLSHMNSGCTFTSPHLAQRVASTVYQNCEHADNYTAYCLGISHMEPSFGLILHDGGTTLKFVDTPESLSGLYVFVVYFNGHVEAVAYTVVSTVDHFVNAIEERGFPPTAGQPPATTKPKEITPVNPGTSPLLRYAAWTGGLAAVVLLCLVIFLICTAKRMRVKAMYAAGLPV

SEQ ID NO: 104 - RNA, 2026 nt, synthetic construct
  source 1..2026: mol_type = other RNA
agactcctccccatcctctccctctgtccctctgtccctctgaccctgcactgtcccagcaccgccaccatgggcaccgtgaacaagcctgttgtgggcgtgctgatgggcttcggcatcatcacaggcaccctgcggatcaccaatcctgtgcgggctagcgtgctgagatacgacgacttccacatcgacgaggacaagctggacaccaacagcgtgtacgagccctactaccacagcgatcacgccgagtctagctgggtcaacagaggcgagagcagcagaaaggcctacgaccacaacagcccctacatctggccccggaacgactacgatggcttcctggaaaatgcccacgagcaccacggcgtgtacaatcaaggcagaggcatcgacagcggcgagagactgatgcagcctacacagatgagcgcccaagaggacctgggagatgataccggcatccacgtgatccccacactgaacggcgacgacagacacaagatcgtgaacgtggaccagcggcagtacggcgacgtgttcaagggcgacctgaatcctaagcctcagggccagcgcctgatcgaggtgtccgtggaagagaatcaccccttcacactgagagcccctatccagagaatctacggcgtgcgctataccgagacatggtcctttctgcccagcctgacatgtaccggggatgccgctcctgccatccagcacatttgcctgaagcacaccacctgtttccaggacgtggtggtggatgtggactgcgccgagaacaccaaagaggatcagctggccgagatcagctaccggttccagggaaagaaagaggccgaccagccttggatcgtggtcaacaccagcacactgttcgacgagctggaactggaccctcctgagattgaacccggggtgctgaaggtgctgagaaccgagaagcagtacctgggagtgtacatctggaacatgagaggcagcgacggcacctctacctacgccacctttctggtcacatggaagggcgacgagaaaacacggaaccccacaccagctgtgacccctcaacctagaggcgccgagtttcacatgtggaattaccacagccacgtgttcagcgtgggcgatacctttagcctggccatgcatctgcagtacaagatccacgaggcccctttcgacctgctgctggaatggctgtacgtgcccatcgatcctacctgccagcctatgcggctgtactccacctgtctgtatcaccccaacgctccccagtgcctgagccacatgaatagcggctgcaccttcacaagccctcacctggctcagcgagtggccagcacagtgtaccagaattgcgagcacgccgacaattacaccgcctactgtctgggcatcagccacatggaacctagcttcggcctgatcctgcacgatggcggcacaaccctgaagttcgtggatacccctgagagcctgagcggcctgtatgtgttcgtggtgtacttcaacggccacgtggaagccgtggcctacaccgtggtgtctaccgtggaccacttcgtgaacgccatcgaggaaagaggcttccctccaactgctggacagcctcctgccaccaccaagcctaaagaaatcacacccgtgaatcccggcacaagcccactgcttagatacgccgcttggacaggcggactggctgctgttgttctgctgtgcctggtcatcttcctgatctgcaccgccaagcggatgagagtgaaggctatgtatgccgccggactgcctgtttgataataggctggagcctcggtggccatgcttcttgccccttgggcctccccccagcccctcctccccttcctgcacccgtacccccgtggtctttgaataaagtctgagtgggcggcaaaaaaaaaaaaaaaaaaaaaaaaaaaaaaaaaaaaaaaaaaaaaaaaaaaaaaaaaaaaaaaaaaaaaaaaaaaaaaaaaaaaaaaaaaaaaaaaaaaaaaaaaaaaaa

SEQ ID NO: 105 - DNA, 2026 bp, synthetic construct
  source 1..2026: mol_type = other DNA
agactcctccccatcctctccctctgtccctctgtccctctgaccctgcactgtcccagcaccgccaccatgggcaccgtgaacaagcctgttgtgggcgtgctgatgggcttcggcatcatcacaggcaccctgcggatcaccaatcctgtgcgggctagcgtgctgagatacgacgacttccacatcgacgaggacaagctggacaccaacagcgtgtacgagccctactaccacagcgatcacgccgagtctagctgggtcaacagaggcgagagcagcagaaaggcctacgaccacaacagcccctacatctggccccggaacgactacgatggcttcctggaaaatgcccacgagcaccacggcgtgtacaatcaaggcagaggcatcgacagcggcgagagactgatgcagcctacacagatgagcgcccaagaggacctgggagatgataccggcatccacgtgatccccacactgaacggcgacgacagacacaagatcgtgaacgtggaccagcggcagtacggcgacgtgttcaagggcgacctgaatcctaagcctcagggccagcgcctgatcgaggtgtccgtggaagagaatcaccccttcacactgagagcccctatccagagaatctacggcgtgcgctataccgagacatggtcctttctgcccagcctgacatgtaccggggatgccgctcctgccatccagcacatttgcctgaagcacaccacctgtttccaggacgtggtggtggatgtggactgcgccgagaacaccaaagaggatcagctggccgagatcagctaccggttccagggaaagaaagaggccgaccagccttggatcgtggtcaacaccagcacactgttcgacgagctggaactggaccctcctgagattgaacccggggtgctgaaggtgctgagaaccgagaagcagtacctgggagtgtacatctggaacatgagaggcagcgacggcacctctacctacgccacctttctggtcacatggaagggcgacgagaaaacacggaaccccacaccagctgtgacccctcaacctagaggcgccgagtttcacatgtggaattaccacagccacgtgttcagcgtgggcgatacctttagcctggccatgcatctgcagtacaagatccacgaggcccctttcgacctgctgctggaatggctgtacgtgcccatcgatcctacctgccagcctatgcggctgtactccacctgtctgtatcaccccaacgctccccagtgcctgagccacatgaatagcggctgcaccttcacaagccctcacctggctcagcgagtggccagcacagtgtaccagaattgcgagcacgccgacaattacaccgcctactgtctgggcatcagccacatggaacctagcttcggcctgatcctgcacgatggcggcacaaccctgaagttcgtggatacccctgagagcctgagcggcctgtatgtgttcgtggtgtacttcaacggccacgtggaagccgtggcctacaccgtggtgtctaccgtggaccacttcgtgaacgccatcgaggaaagaggcttccctccaactgctggacagcctcctgccaccaccaagcctaaagaaatcacacccgtgaatcccggcacaagcccactgcttagatacgccgcttggacaggcggactggctgctgttgttctgctgtgcctggtcatcttcctgatctgcaccgccaagcggatgagagtgaaggctatgtatggcgccggactgcctgtttgataataggctggagcctcggtggccatgcttcttgccccttgggcctccccccagcccctcctccccttcctgcacccgtacccccgtggtctttgaataaagtctgagtgggcggcaaaaaaaaaaaaaaaaaaaaaaaaaaaaaaaaaaaaaaaaaaaaaaaaaaaaaaaaaaaaaaaaaaaaaaaaaaaaaaaaaaaaaaaaaaaaaaaaaaaaaaaaaaaaaa

SEQ ID NO: 106 - DNA, 1731 bp, synthetic construct
  source 1..1731: mol_type = other DNA
atgggcaccgtgaacaagcctgttgtgggcgtgctgatgggcttcggcatcatcacaggcaccctgcggatcaccaatcctgtgcgggctagcgtgctgagatacgacgacttccacatcgacgaggacaagctggacaccaacagcgtgtacgagccctactaccacagcgatcacgccgagtctagctgggtcaacagaggcgagagcagcagaaaggcctacgaccacaacagcccctacatctggccccggaacgactacgatggcttcctggaaaatgcccacgagcaccacggcgtgtacaatcaaggcagaggcatcgacagcggcgagagactgatgcagcctacacagatgagcgcccaagaggacctgggagatgataccggcatccacgtgatccccacactgaacggcgacgacagacacaagatcgtgaacgtggaccagcggcagtacggcgacgtgttcaagggcgacctgaatcctaagcctcagggccagcgcctgatcgaggtgtccgtggaagagaatcaccccttcacactgagagcccctatccagagaatctacggcgtgcgctataccgagacatggtcctttctgcccagcctgacatgtaccggggatgccgctcctgccatccagcacatttgcctgaagcacaccacctgtttccaggacgtggtggtggatgtggactgcgccgagaacaccaaagaggatcagctggccgagatcagctaccggttccagggaaagaaagaggccgaccagccttggatcgtggtcaacaccagcacactgttcgacgagctggaactggaccctcctgagattgaacccggggtgctgaaggtgctgagaaccgagaagcagtacctgggagtgtacatctggaacatgagaggcagcgacggcacctctacctacgccacctttctggtcacatggaagggcgacgagaaaacacggaaccccacaccagctgtgacccctcaacctagaggcgccgagtttcacatgtggaattaccacagccacgtgttcagcgtgggcgatacctttagcctggccatgcatctgcagtacaagatccacgaggcccctttcgacctgctgctggaatggctgtacgtgcccatcgatcctacctgccagcctatgcggctgtactccacctgtctgtatcaccccaacgctccccagtgcctgagccacatgaatagcggctgcaccttcacaagccctcacctggctcagcgagtggccagcacagtgtaccagaattgcgagcacgccgacaattacaccgcctactgtctgggcatcagccacatggaacctagcttcggcctgatcctgcacgatggcggcacaaccctgaagttcgtggatacccctgagagcctgagcggcctgtatgtgttcgtggtgtacttcaacggccacgtggaagccgtggcctacaccgtggtgtctaccgtggaccacttcgtgaacgccatcgaggaaagaggcttccctccaactgctggacagcctcctgccaccaccaagcctaaagaaatcacacccgtgaatcccggcacaagcccactgcttagatacgccgcttggacaggcggactggctgctgttgttctgctgtgcctggtcatcttcctgatctgcaccgccaagcggatgagagtgaaggctatgtatggcgccggactgcctgtttga

SEQ ID NO: 107 - protein, 576 aa, synthetic construct
MGTVNKPVVGVLMGFGIITGTLRITNPVRASVLRYDDFHIDEDKLDTNSVYEPYYHSDHAESSWVNRGESSRKAYDHNSPYIWPRNDYDGFLENAHEHHGVYNQGRGIDSGERLMQPTQMSAQEDLGDDTGIHVIPTLNGDDRHKIVNVDQRQYGDVFKGDLNPKPQGQRLIEVSVEENHPFTLRAPIQRIYGVRYTETWSFLPSLTCTGDAAPAIQHICLKHTTCFQDVVVDVDCAENTKEDQLAEISYRFQGKKEADQPWIVVNTSTLFDELELDPPEIEPGVLKVLRTEKQYLGVYIWNMRGSDGTSTYATFLVTWKGDEKTRNPTPAVTPQPRGAEFHMWNYHSHVFSVGDTFSLAMHLQYKIHEAPFDLLLEWLYVPIDPTCQPMRLYSTCLYHPNAPQCLSHMNSGCTFTSPHLAQRVASTVYQNCEHADNYTAYCLGISHMEPSFGLILHDGGTTLKFVDTPESLSGLYVFVVYFNGHVEAVAYTVVSTVDHFVNAIEERGFPPTAGQPPATTKPKEITPVNPGTSPLLRYAAWTGGLAAVVLLCLVIFLICTAKRMRVKAMYGAGLPV

SEQ ID NO: 108 - RNA, 2026 nt, synthetic construct
  source 1..2026: mol_type = other RNA
agactcctccccatcctctccctctgtccctctgtccctctgaccctgcactgtcccagcaccgccaccatgggcaccgtgaacaagcctgttgtgggcgtgctgatgggcttcggcatcatcacaggcaccctgcggatcaccaatcctgtgcgggctagcgtgctgagatacgacgacttccacatcgacgaggacaagctggacaccaacagcgtgtacgagccctactaccacagcgatcacgccgagtctagctgggtcaacagaggcgagagcagcagaaaggcctacgaccacaacagcccctacatctggccccggaacgactacgatggcttcctggaaaatgcccacgagcaccacggcgtgtacaatcaaggcagaggcatcgacagcggcgagagactgatgcagcctacacagatgagcgcccaagaggacctgggagatgataccggcatccacgtgatccccacactgaacggcgacgacagacacaagatcgtgaacgtggaccagcggcagtacggcgacgtgttcaagggcgacctgaatcctaagcctcagggccagcgcctgatcgaggtgtccgtggaagagaatcaccccttcacactgagagcccctatccagagaatctacggcgtgcgctataccgagacatggtcctttctgcccagcctgacatgtaccggggatgccgctcctgccatccagcacatttgcctgaagcacaccacctgtttccaggacgtggtggtggatgtggactgcgccgagaacaccaaagaggatcagctggccgagatcagctaccggttccagggaaagaaagaggccgaccagccttggatcgtggtcaacaccagcacactgttcgacgagctggaactggaccctcctgagattgaacccggggtgctgaaggtgctgagaaccgagaagcagtacctgggagtgtacatctggaacatgagaggcagcgacggcacctctacctacgccacctttctggtcacatggaagggcgacgagaaaacacggaaccccacaccagctgtgacccctcaacctagaggcgccgagtttcacatgtggaattaccacagccacgtgttcagcgtgggcgatacctttagcctggccatgcatctgcagtacaagatccacgaggcccctttcgacctgctgctggaatggctgtacgtgcccatcgatcctacctgccagcctatgcggctgtactccacctgtctgtatcaccccaacgctccccagtgcctgagccacatgaatagcggctgcaccttcacaagccctcacctggctcagcgagtggccagcacagtgtaccagaattgcgagcacgccgacaattacaccgcctactgtctgggcatcagccacatggaacctagcttcggcctgatcctgcacgatggcggcacaaccctgaagttcgtggatacccctgagagcctgagcggcctgtatgtgttcgtggtgtacttcaacggccacgtggaagccgtggcctacaccgtggtgtctaccgtggaccacttcgtgaacgccatcgaggaaagaggcttccctccaactgctggacagcctcctgccaccaccaagcctaaagaaatcacacccgtgaatcccggcacaagcccactgcttagatacgccgcttggacaggcggactggctgctgttgttctgctgtgcctggtcatcttcctgatctgcaccgccaagcggatgagagtgaaggctatgtatggcgccggactgcctgtttgataataggctggagcctcggtggccatgcttcttgccccttgggcctccccccagcccctcctccccttcctgcacccgtacccccgtggtctttgaataaagtctgagtgggcggcaaaaaaaaaaaaaaaaaaaaaaaaaaaaaaaaaaaaaaaaaaaaaaaaaaaaaaaaaaaaaaaaaaaaaaaaaaaaaaaaaaaaaaaaaaaaaaaaaaaaaaaaaaaaaa

SEQ ID NO: 109 - DNA, 2059 bp, synthetic construct
  source 1..2059: mol_type = other DNA
agactcctccccatcctctccctctgtccctctgtccctctgaccctgcactgtcccagcaccgccaccatgggcaccgtgaacaagcctgttgtgggcgtgctgatgggcttcggcatcatcacaggcaccctgcggatcaccaatcctgtgcgggctagcgtgctgagatacgacgacttccacatcgacgaggacaagctggacaccaacagcgtgtacgagccctactaccacagcgatcacgccgagtctagctgggtcaacagaggcgagagcagcagaaaggcctacgaccacaacagcccctacatctggccccggaacgactacgatggcttcctggaaaatgcccacgagcaccacggcgtgtacaatcaaggcagaggcatcgacagcggcgagagactgatgcagcctacacagatgagcgcccaagaggacctgggagatgataccggcatccacgtgatccccacactgaacggcgacgacagacacaagatcgtgaacgtggaccagcggcagtacggcgacgtgttcaagggcgacctgaatcctaagcctcagggccagcgcctgatcgaggtgtccgtggaagagaatcaccccttcacactgagagcccctatccagagaatctacggcgtgcgctataccgagacatggtcctttctgcccagcctgacatgtaccggggatgccgctcctgccatccagcacatttgcctgaagcacaccacctgtttccaggacgtggtggtggatgtggactgcgccgagaacaccaaagaggatcagctggccgagatcagctaccggttccagggaaagaaagaggccgaccagccttggatcgtggtcaacaccagcacactgttcgacgagctggaactggaccctcctgagattgaacccggggtgctgaaggtgctgagaaccgagaagcagtacctgggagtgtacatctggaacatgagaggcagcgacggcacctctacctacgccacctttctggtcacatggaagggcgacgagaaaacacggaaccccacaccagctgtgacccctcaacctagaggcgccgagtttcacatgtggaattaccacagccacgtgttcagcgtgggcgatacctttagcctggccatgcatctgcagtacaagatccacgaggcccctttcgacctgctgctggaatggctgtacgtgcccatcgatcctacctgccagcctatgcggctgtactccacctgtctgtatcaccccaacgctccccagtgcctgagccacatgaatagcggctgcaccttcacaagccctcacctggctcagcgagtggccagcacagtgtaccagaattgcgagcacgccgacaattacaccgcctactgtctgggcatcagccacatggaacctagcttcggcctgatcctgcacgatggcggcacaaccctgaagttcgtggatacccctgagagcctgagcggcctgtatgtgttcgtggtgtacttcaacggccacgtggaagccgtggcctacaccgtggtgtctaccgtggaccacttcgtgaacgccatcgaggaaagaggcttccctccaactgctggacagcctcctgccaccaccaagcctaaagaaatcacacccgtgaatcccggcacaagcccactgcttagatacgccgcttggacaggcggactggctgctgttgttctgctgtgcctggtcatcttcctgatctgcaccgccaagcggatgcgcgtgaaggacaaagagaaggacaagtccccttacaaccagtctatgtatgccgccggactgcccgtttgataataggctggagcctcggtggccatgcttcttgccccttgggcctccccccagcccctcctccccttcctgcacccgtacccccgtggtctttgaataaagtctgagtgggcggcaaaaaaaaaaaaaaaaaaaaaaaaaaaaaaaaaaaaaaaaaaaaaaaaaaaaaaaaaaaaaaaaaaaaaaaaaaaaaaaaaaaaaaaaaaaaaaaaaaaaaaaaaaaaaa

SEQ ID NO: 110 - DNA, 1764 bp, synthetic construct
  source 1..1764: mol_type = other DNA
atgggcaccgtgaacaagcctgttgtgggcgtgctgatgggcttcggcatcatcacaggcaccctgcggatcaccaatcctgtgcgggctagcgtgctgagatacgacgacttccacatcgacgaggacaagctggacaccaacagcgtgtacgagccctactaccacagcgatcacgccgagtctagctgggtcaacagaggcgagagcagcagaaaggcctacgaccacaacagcccctacatctggccccggaacgactacgatggcttcctggaaaatgcccacgagcaccacggcgtgtacaatcaaggcagaggcatcgacagcggcgagagactgatgcagcctacacagatgagcgcccaagaggacctgggagatgataccggcatccacgtgatccccacactgaacggcgacgacagacacaagatcgtgaacgtggaccagcggcagtacggcgacgtgttcaagggcgacctgaatcctaagcctcagggccagcgcctgatcgaggtgtccgtggaagagaatcaccccttcacactgagagcccctatccagagaatctacggcgtgcgctataccgagacatggtcctttctgcccagcctgacatgtaccggggatgccgctcctgccatccagcacatttgcctgaagcacaccacctgtttccaggacgtggtggtggatgtggactgcgccgagaacaccaaagaggatcagctggccgagatcagctaccggttccagggaaagaaagaggccgaccagccttggatcgtggtcaacaccagcacactgttcgacgagctggaactggaccctcctgagattgaacccggggtgctgaaggtgctgagaaccgagaagcagtacctgggagtgtacatctggaacatgagaggcagcgacggcacctctacctacgccacctttctggtcacatggaagggcgacgagaaaacacggaaccccacaccagctgtgacccctcaacctagaggcgccgagtttcacatgtggaattaccacagccacgtgttcagcgtgggcgatacctttagcctggccatgcatctgcagtacaagatccacgaggcccctttcgacctgctgctggaatggctgtacgtgcccatcgatcctacctgccagcctatgcggctgtactccacctgtctgtatcaccccaacgctccccagtgcctgagccacatgaatagcggctgcaccttcacaagccctcacctggctcagcgagtggccagcacagtgtaccagaattgcgagcacgccgacaattacaccgcctactgtctgggcatcagccacatggaacctagcttcggcctgatcctgcacgatggcggcacaaccctgaagttcgtggatacccctgagagcctgagcggcctgtatgtgttcgtggtgtacttcaacggccacgtggaagccgtggcctacaccgtggtgtctaccgtggaccacttcgtgaacgccatcgaggaaagaggcttccctccaactgctggacagcctcctgccaccaccaagcctaaagaaatcacacccgtgaatcccggcacaagcccactgcttagatacgccgcttggacaggcggactggctgctgttgttctgctgtgcctggtcatcttcctgatctgcaccgccaagcggatgcgcgtgaaggacaaagagaaggacaagtccccttacaaccagtctatgtatgccgccggactgcccgtttga

SEQ ID NO: 111 - protein, 587 aa, synthetic construct
MGTVNKPVVGVLMGFGIITGTLRITNPVRASVLRYDDFHIDEDKLDTNSVYEPYYHSDHAESSWVNRGESSRKAYDHNSPYIWPRNDYDGFLENAHEHHGVYNQGRGIDSGERLMQPTQMSAQEDLGDDTGIHVIPTLNGDDRHKIVNVDQRQYGDVFKGDLNPKPQGQRLIEVSVEENHPFTLRAPIQRIYGVRYTETWSFLPSLTCTGDAAPAIQHICLKHTTCFQDVVVDVDCAENTKEDQLAEISYRFQGKKEADQPWIVVNTSTLFDELELDPPEIEPGVLKVLRTEKQYLGVYIWNMRGSDGTSTYATFLVTWKGDEKTRNPTPAVTPQPRGAEFHMWNYHSHVFSVGDTFSLAMHLQYKIHEAPFDLLLEWLYVPIDPTCQPMRLYSTCLYHPNAPQCLSHMNSGCTFTSPHLAQRVASTVYQNCEHADNYTAYCLGISHMEPSFGLILHDGGTTLKFVDTPESLSGLYVFVVYFNGHVEAVAYTVVSTVDHFVNAIEERGFPPTAGQPPATTKPKEITPVNPGTSPLLRYAAWTGGLAAVVLLCLVIFLICTAKRMRVKDKEKDKSPYNQSMYAAGLPV

SEQ ID NO: 112 - RNA, 2059 nt, synthetic construct
  source 1..2059: mol_type = other RNA
agactcctccccatcctctccctctgtccctctgtccctctgaccctgcactgtcccagcaccgccaccatgggcaccgtgaacaagcctgttgtgggcgtgctgatgggcttcggcatcatcacaggcaccctgcggatcaccaatcctgtgcgggctagcgtgctgagatacgacgacttccacatcgacgaggacaagctggacaccaacagcgtgtacgagccctactaccacagcgatcacgccgagtctagctgggtcaacagaggcgagagcagcagaaaggcctacgaccacaacagcccctacatctggccccggaacgactacgatggcttcctggaaaatgcccacgagcaccacggcgtgtacaatcaaggcagaggcatcgacagcggcgagagactgatgcagcctacacagatgagcgcccaagaggacctgggagatgataccggcatccacgtgatccccacactgaacggcgacgacagacacaagatcgtgaacgtggaccagcggcagtacggcgacgtgttcaagggcgacctgaatcctaagcctcagggccagcgcctgatcgaggtgtccgtggaagagaatcaccccttcacactgagagcccctatccagagaatctacggcgtgcgctataccgagacatggtcctttctgcccagcctgacatgtaccggggatgccgctcctgccatccagcacatttgcctgaagcacaccacctgtttccaggacgtggtggtggatgtggactgcgccgagaacaccaaagaggatcagctggccgagatcagctaccggttccagggaaagaaagaggccgaccagccttggatcgtggtcaacaccagcacactgttcgacgagctggaactggaccctcctgagattgaacccggggtgctgaaggtgctgagaaccgagaagcagtacctgggagtgtacatctggaacatgagaggcagcgacggcacctctacctacgccacctttctggtcacatggaagggcgacgagaaaacacggaaccccacaccagctgtgacccctcaacctagaggcgccgagtttcacatgtggaattaccacagccacgtgttcagcgtgggcgatacctttagcctggccatgcatctgcagtacaagatccacgaggcccctttcgacctgctgctggaatggctgtacgtgcccatcgatcctacctgccagcctatgcggctgtactccacctgtctgtatcaccccaacgctccccagtgcctgagccacatgaatagcggctgcaccttcacaagccctcacctggctcagcgagtggccagcacagtgtaccagaattgcgagcacgccgacaattacaccgcctactgtctgggcatcagccacatggaacctagcttcggcctgatcctgcacgatggcggcacaaccctgaagttcgtggatacccctgagagcctgagcggcctgtatgtgttcgtggtgtacttcaacggccacgtggaagccgtggcctacaccgtggtgtctaccgtggaccacttcgtgaacgccatcgaggaaagaggcttccctccaactgctggacagcctcctgccaccaccaagcctaaagaaatcacacccgtgaatcccggcacaagcccactgcttagatacgccgcttggacaggcggactggctgctgttgttctgctgtgcctggtcatcttcctgatctgcaccgccaagcggatgcgcgtgaaggacaaagagaaggacaagtccccttacaaccagtctatgtatgccgccggactgcccgtttgataataggctggagcctcggtggccatgcttcttgccccttgggcctccccccagcccctcctccccttcctgcacccgtacccccgtggtctttgaataaagtctgagtgggcggcaaaaaaaaaaaaaaaaaaaaaaaaaaaaaaaaaaaaaaaaaaaaaaaaaaaaaaaaaaaaaaaaaaaaaaaaaaaaaaaaaaaaaaaaaaaaaaaaaaaaaaaaaaaaaa

SEQ ID NO: 113 - DNA, 2059 bp, synthetic construct
  source 1..2059: mol_type = other DNA
agactcctccccatcctctccctctgtccctctgtccctctgaccctgcactgtcccagcaccgccaccatgggcaccgtgaacaagcctgttgtgggcgtgctgatgggcttcggcatcatcacaggcaccctgcggatcaccaatcctgtgcgggctagcgtgctgagatacgacgacttccacatcgacgaggacaagctggacaccaacagcgtgtacgagccctactaccacagcgatcacgccgagtctagctgggtcaacagaggcgagagcagcagaaaggcctacgaccacaacagcccctacatctggccccggaacgactacgatggcttcctggaaaatgcccacgagcaccacggcgtgtacaatcaaggcagaggcatcgacagcggcgagagactgatgcagcctacacagatgagcgcccaagaggacctgggagatgataccggcatccacgtgatccccacactgaacggcgacgacagacacaagatcgtgaacgtggaccagcggcagtacggcgacgtgttcaagggcgacctgaatcctaagcctcagggccagcgcctgatcgaggtgtccgtggaagagaatcaccccttcacactgagagcccctatccagagaatctacggcgtgcgctataccgagacatggtcctttctgcccagcctgacatgtaccggggatgccgctcctgccatccagcacatttgcctgaagcacaccacctgtttccaggacgtggtggtggatgtggactgcgccgagaacaccaaagaggatcagctggccgagatcagctaccggttccagggaaagaaagaggccgaccagccttggatcgtggtcaacaccagcacactgttcgacgagctggaactggaccctcctgagattgaacccggggtgctgaaggtgctgagaaccgagaagcagtacctgggagtgtacatctggaacatgagaggcagcgacggcacctctacctacgccacctttctggtcacatggaagggcgacgagaaaacacggaaccccacaccagctgtgacccctcaacctagaggcgccgagtttcacatgtggaattaccacagccacgtgttcagcgtgggcgatacctttagcctggccatgcatctgcagtacaagatccacgaggcccctttcgacctgctgctggaatggctgtacgtgcccatcgatcctacctgccagcctatgcggctgtactccacctgtctgtatcaccccaacgctccccagtgcctgagccacatgaatagcggctgcaccttcacaagccctcacctggctcagcgagtggccagcacagtgtaccagaattgcgagcacgccgacaattacaccgcctactgtctgggcatcagccacatggaacctagcttcggcctgatcctgcacgatggcggcacaaccctgaagttcgtggatacccctgagagcctgagcggcctgtatgtgttcgtggtgtacttcaacggccacgtggaagccgtggcctacaccgtggtgtctaccgtggaccacttcgtgaacgccatcgaggaaagaggcttccctccaactgctggacagcctcctgccaccaccaagcctaaagaaatcacacccgtgaatcccggcacaagcccactgcttagatacgccgcttggacaggcggactggctgctgttgttctgctgtgcctggtcatcttcctgatctgcaccgccaagcggatgcgcgtgaaggacaaagagaaggacaagtccccttacaaccagtctatgtatggcgccggactgcccgtttgataataggctggagcctcggtggccatgcttcttgccccttgggcctccccccagcccctcctccccttcctgcacccgtacccccgtggtctttgaataaagtctgagtgggcggcaaaaaaaaaaaaaaaaaaaaaaaaaaaaaaaaaaaaaaaaaaaaaaaaaaaaaaaaaaaaaaaaaaaaaaaaaaaaaaaaaaaaaaaaaaaaaaaaaaaaaaaaaaaaaa

SEQ ID NO: 114 - DNA, 1764 bp, synthetic construct
  source 1..1764: mol_type = other DNA
atgggcaccgtgaacaagcctgttgtgggcgtgctgatgggcttcggcatcatcacaggcaccctgcggatcaccaatcctgtgcgggctagcgtgctgagatacgacgacttccacatcgacgaggacaagctggacaccaacagcgtgtacgagccctactaccacagcgatcacgccgagtctagctgggtcaacagaggcgagagcagcagaaaggcctacgaccacaacagcccctacatctggccccggaacgactacgatggcttcctggaaaatgcccacgagcaccacggcgtgtacaatcaaggcagaggcatcgacagcggcgagagactgatgcagcctacacagatgagcgcccaagaggacctgggagatgataccggcatccacgtgatccccacactgaacggcgacgacagacacaagatcgtgaacgtggaccagcggcagtacggcgacgtgttcaagggcgacctgaatcctaagcctcagggccagcgcctgatcgaggtgtccgtggaagagaatcaccccttcacactgagagcccctatccagagaatctacggcgtgcgctataccgagacatggtcctttctgcccagcctgacatgtaccggggatgccgctcctgccatccagcacatttgcctgaagcacaccacctgtttccaggacgtggtggtggatgtggactgcgccgagaacaccaaagaggatcagctggccgagatcagctaccggttccagggaaagaaagaggccgaccagccttggatcgtggtcaacaccagcacactgttcgacgagctggaactggaccctcctgagattgaacccggggtgctgaaggtgctgagaaccgagaagcagtacctgggagtgtacatctggaacatgagaggcagcgacggcacctctacctacgccacctttctggtcacatggaagggcgacgagaaaacacggaaccccacaccagctgtgacccctcaacctagaggcgccgagtttcacatgtggaattaccacagccacgtgttcagcgtgggcgatacctttagcctggccatgcatctgcagtacaagatccacgaggcccctttcgacctgctgctggaatggctgtacgtgcccatcgatcctacctgccagcctatgcggctgtactccacctgtctgtatcaccccaacgctccccagtgcctgagccacatgaatagcggctgcaccttcacaagccctcacctggctcagcgagtggccagcacagtgtaccagaattgcgagcacgccgacaattacaccgcctactgtctgggcatcagccacatggaacctagcttcggcctgatcctgcacgatggcggcacaaccctgaagttcgtggatacccctgagagcctgagcggcctgtatgtgttcgtggtgtacttcaacggccacgtggaagccgtggcctacaccgtggtgtctaccgtggaccacttcgtgaacgccatcgaggaaagaggcttccctccaactgctggacagcctcctgccaccaccaagcctaaagaaatcacacccgtgaatcccggcacaagcccactgcttagatacgccgcttggacaggcggactggctgctgttgttctgctgtgcctggtcatcttcctgatctgcaccgccaagcggatgcgcgtgaaggacaaagagaaggacaagtccccttacaaccagtctatgtatggcgccggactgcccgtttga

SEQ ID NO: 115 - protein, 587 aa, synthetic construct
MGTVNKPVVGVLMGFGIITGTLRITNPVRASVLRYDDFHIDEDKLDTNSVYEPYYHSDHAESSWVNRGESSRKAYDHNSPYIWPRNDYDGFLENAHEHHGVYNQGRGIDSGERLMQPTQMSAQEDLGDDTGIHVIPTLNGDDRHKIVNVDQRQYGDVFKGDLNPKPQGQRLIEVSVEENHPFTLRAPIQRIYGVRYTETWSFLPSLTCTGDAAPAIQHICLKHTTCFQDVVVDVDCAENTKEDQLAEISYRFQGKKEADQPWIVVNTSTLFDELELDPPEIEPGVLKVLRTEKQYLGVYIWNMRGSDGTSTYATFLVTWKGDEKTRNPTPAVTPQPRGAEFHMWNYHSHVFSVGDTFSLAMHLQYKIHEAPFDLLLEWLYVPIDPTCQPMRLYSTCLYHPNAPQCLSHMNSGCTFTSPHLAQRVASTVYQNCEHADNYTAYCLGISHMEPSFGLILHDGGTTLKFVDTPESLSGLYVFVVYFNGHVEAVAYTVVSTVDHFVNAIEERGFPPTAGQPPATTKPKEITPVNPGTSPLLRYAAWTGGLAAVVLLCLVIFLICTAKRMRVKDKEKDKSPYNQSMYGAGLPV

SEQ ID NO: 116 - RNA, 2059 nt, synthetic construct
  source 1..2059: mol_type = other RNA
agactcctccccatcctctccctctgtccctctgtccctctgaccctgcactgtcccagcaccgccaccatgggcaccgtgaacaagcctgttgtgggcgtgctgatgggcttcggcatcatcacaggcaccctgcggatcaccaatcctgtgcgggctagcgtgctgagatacgacgacttccacatcgacgaggacaagctggacaccaacagcgtgtacgagccctactaccacagcgatcacgccgagtctagctgggtcaacagaggcgagagcagcagaaaggcctacgaccacaacagcccctacatctggccccggaacgactacgatggcttcctggaaaatgcccacgagcaccacggcgtgtacaatcaaggcagaggcatcgacagcggcgagagactgatgcagcctacacagatgagcgcccaagaggacctgggagatgataccggcatccacgtgatccccacactgaacggcgacgacagacacaagatcgtgaacgtggaccagcggcagtacggcgacgtgttcaagggcgacctgaatcctaagcctcagggccagcgcctgatcgaggtgtccgtggaagagaatcaccccttcacactgagagcccctatccagagaatctacggcgtgcgctataccgagacatggtcctttctgcccagcctgacatgtaccggggatgccgctcctgccatccagcacatttgcctgaagcacaccacctgtttccaggacgtggtggtggatgtggactgcgccgagaacaccaaagaggatcagctggccgagatcagctaccggttccagggaaagaaagaggccgaccagccttggatcgtggtcaacaccagcacactgttcgacgagctggaactggaccctcctgagattgaacccggggtgctgaaggtgctgagaaccgagaagcagtacctgggagtgtacatctggaacatgagaggcagcgacggcacctctacctacgccacctttctggtcacatggaagggcgacgagaaaacacggaaccccacaccagctgtgacccctcaacctagaggcgccgagtttcacatgtggaattaccacagccacgtgttcagcgtgggcgatacctttagcctggccatgcatctgcagtacaagatccacgaggcccctttcgacctgctgctggaatggctgtacgtgcccatcgatcctacctgccagcctatgcggctgtactccacctgtctgtatcaccccaacgctccccagtgcctgagccacatgaatagcggctgcaccttcacaagccctcacctggctcagcgagtggccagcacagtgtaccagaattgcgagcacgccgacaattacaccgcctactgtctgggcatcagccacatggaacctagcttcggcctgatcctgcacgatggcggcacaaccctgaagttcgtggatacccctgagagcctgagcggcctgtatgtgttcgtggtgtacttcaacggccacgtggaagccgtggcctacaccgtggtgtctaccgtggaccacttcgtgaacgccatcgaggaaagaggcttccctccaactgctggacagcctcctgccaccaccaagcctaaagaaatcacacccgtgaatcccggcacaagcccactgcttagatacgccgcttggacaggcggactggctgctgttgttctgctgtgcctggtcatcttcctgatctgcaccgccaagcggatgcgcgtgaaggacaaagagaaggacaagtccccttacaaccagtctatgtatggcgccggactgcccgtttgataataggctggagcctcggtggccatgcttcttgccccttgggcctccccccagcccctcctccccttcctgcacccgtacccccgtggtctttgaataaagtctgagtgggcggcaaaaaaaaaaaaaaaaaaaaaaaaaaaaaaaaaaaaaaaaaaaaaaaaaaaaaaaaaaaaaaaaaaaaaaaaaaaaaaaaaaaaaaaaaaaaaaaaaaaaaaaaaaaaaa

SEQ ID NO: 117 - DNA, 2059 bp, synthetic construct
  source 1..2059: mol_type = other DNA
agactcctccccatcctctccctctgtccctctgtccctctgaccctgcactgtcccagcaccgccaccatgggcaccgtgaacaagcctgttgtgggcgtgctgatgggcttcggcatcatcacaggcaccctgcggatcaccaatcctgtgcgggctagcgtgctgagatacgacgacttccacatcgacgaggacaagctggacaccaacagcgtgtacgagccctactaccacagcgatcacgccgagtctagctgggtcaacagaggcgagagcagcagaaaggcctacgaccacaacagcccctacatctggccccggaacgactacgatggcttcctggaaaatgcccacgagcaccacggcgtgtacaatcaaggcagaggcatcgacagcggcgagagactgatgcagcctacacagatgagcgcccaagaggacctgggagatgataccggcatccacgtgatccccacactgaacggcgacgacagacacaagatcgtgaacgtggaccagcggcagtacggcgacgtgttcaagggcgacctgaatcctaagcctcagggccagcgcctgatcgaggtgtccgtggaagagaatcaccccttcacactgagagcccctatccagagaatctacggcgtgcgctataccgagacatggtcctttctgcccagcctgacatgtaccggggatgccgctcctgccatccagcacatttgcctgaagcacaccacctgtttccaggacgtggtggtggatgtggactgcgccgagaacaccaaagaggatcagctggccgagatcagctaccggttccagggaaagaaagaggccgaccagccttggatcgtggtcaacaccagcacactgttcgacgagctggaactggaccctcctgagattgaacccggggtgctgaaggtgctgagaaccgagaagcagtacctgggagtgtacatctggaacatgagaggcagcgacggcacctctacctacgccacctttctggtcacatggaagggcgacgagaaaacacggaaccccacaccagctgtgacccctcaacctagaggcgccgagtttcacatgtggaattaccacagccacgtgttcagcgtgggcgatacctttagcctggccatgcatctgcagtacaagatccacgaggcccctttcgacctgctgctggaatggctgtacgtgcccatcgatcctacctgccagcctatgcggctgtactccacctgtctgtatcaccccaacgctccccagtgcctgagccacatgaatagcggctgcaccttcacaagccctcacctggctcagcgagtggccagcacagtgtaccagaattgcgagcacgccgacaattacaccgcctactgtctgggcatcagccacatggaacctagcttcggcctgatcctgcacgatggcggcacaaccctgaagttcgtggatacccctgagagcctgagcggcctgtatgtgttcgtggtgtacttcaacggccacgtggaagccgtggcctacaccgtggtgtctaccgtggaccacttcgtgaacgccatcgaggaaagaggcttccctccaactgctggacagcctcctgccaccaccaagcctaaagaaatcacacccgtgaatcccggcacaagcccactgcttagatacgccgcttggacaggcggactggctgctgttgttctgctgtgcctggtcatcttcctgatctgcaccgccaagcggatgagagtgaaggactacagagtggacaagagcccttacaaccagtctatgtatgccgccggactgcccgtttgataataggctggagcctcggtggccatgcttcttgccccttgggcctccccccagcccctcctccccttcctgcacccgtacccccgtggtctttgaataaagtctgagtgggcggcaaaaaaaaaaaaaaaaaaaaaaaaaaaaaaaaaaaaaaaaaaaaaaaaaaaaaaaaaaaaaaaaaaaaaaaaaaaaaaaaaaaaaaaaaaaaaaaaaaaaaaaaaaaaaa

SEQ ID NO: 118 - DNA, 1764 bp, synthetic construct
  source 1..1764: mol_type = other DNA
atgggcaccgtgaacaagcctgttgtgggcgtgctgatgggcttcggcatcatcacaggcaccctgcggatcaccaatcctgtgcgggctagcgtgctgagatacgacgacttccacatcgacgaggacaagctggacaccaacagcgtgtacgagccctactaccacagcgatcacgccgagtctagctgggtcaacagaggcgagagcagcagaaaggcctacgaccacaacagcccctacatctggccccggaacgactacgatggcttcctggaaaatgcccacgagcaccacggcgtgtacaatcaaggcagaggcatcgacagcggcgagagactgatgcagcctacacagatgagcgcccaagaggacctgggagatgataccggcatccacgtgatccccacactgaacggcgacgacagacacaagatcgtgaacgtggaccagcggcagtacggcgacgtgttcaagggcgacctgaatcctaagcctcagggccagcgcctgatcgaggtgtccgtggaagagaatcaccccttcacactgagagcccctatccagagaatctacggcgtgcgctataccgagacatggtcctttctgcccagcctgacatgtaccggggatgccgctcctgccatccagcacatttgcctgaagcacaccacctgtttccaggacgtggtggtggatgtggactgcgccgagaacaccaaagaggatcagctggccgagatcagctaccggttccagggaaagaaagaggccgaccagccttggatcgtggtcaacaccagcacactgttcgacgagctggaactggaccctcctgagattgaacccggggtgctgaaggtgctgagaaccgagaagcagtacctgggagtgtacatctggaacatgagaggcagcgacggcacctctacctacgccacctttctggtcacatggaagggcgacgagaaaacacggaaccccacaccagctgtgacccctcaacctagaggcgccgagtttcacatgtggaattaccacagccacgtgttcagcgtgggcgatacctttagcctggccatgcatctgcagtacaagatccacgaggcccctttcgacctgctgctggaatggctgtacgtgcccatcgatcctacctgccagcctatgcggctgtactccacctgtctgtatcaccccaacgctccccagtgcctgagccacatgaatagcggctgcaccttcacaagccctcacctggctcagcgagtggccagcacagtgtaccagaattgcgagcacgccgacaattacaccgcctactgtctgggcatcagccacatggaacctagcttcggcctgatcctgcacgatggcggcacaaccctgaagttcgtggatacccctgagagcctgagcggcctgtatgtgttcgtggtgtacttcaacggccacgtggaagccgtggcctacaccgtggtgtctaccgtggaccacttcgtgaacgccatcgaggaaagaggcttccctccaactgctggacagcctcctgccaccaccaagcctaaagaaatcacacccgtgaatcccggcacaagcccactgcttagatacgccgcttggacaggcggactggctgctgttgttctgctgtgcctggtcatcttcctgatctgcaccgccaagcggatgagagtgaaggactacagagtggacaagagcccttacaaccagtctatgtatgccgccggactgcccgtttga

SEQ ID NO: 119 - protein, 587 aa, synthetic construct
MGTVNKPVVGVLMGFGIITGTLRITNPVRASVLRYDDFHIDEDKLDTNSVYEPYYHSDHAESSWVNRGESSRKAYDHNSPYIWPRNDYDGFLENAHEHHGVYNQGRGIDSGERLMQPTQMSAQEDLGDDTGIHVIPTLNGDDRHKIVNVDQRQYGDVFKGDLNPKPQGQRLIEVSVEENHPFTLRAPIQRIYGVRYTETWSFLPSLTCTGDAAPAIQHICLKHTTCFQDVVVDVDCAENTKEDQLAEISYRFQGKKEADQPWIVVNTSTLFDELELDPPEIEPGVLKVLRTEKQYLGVYIWNMRGSDGTSTYATFLVTWKGDEKTRNPTPAVTPQPRGAEFHMWNYHSHVFSVGDTFSLAMHLQYKIHEAPFDLLLEWLYVPIDPTCQPMRLYSTCLYHPNAPQCLSHMNSGCTFTSPHLAQRVASTVYQNCEHADNYTAYCLGISHMEPSFGLILHDGGTTLKFVDTPESLSGLYVFVVYFNGHVEAVAYTVVSTVDHFVNAIEERGFPPTAGQPPATTKPKEITPVNPGTSPLLRYAAWTGGLAAVVLLCLVIFLICTAKRMRVKDYRVDKSPYNQSMYAAGLPV

SEQ ID NO: 120 - RNA, 2059 nt, synthetic construct
  source 1..2059: mol_type = other RNA
agactcctccccatcctctccctctgtccctctgtccctctgaccctgcactgtcccagcaccgccaccatgggcaccgtgaacaagcctgttgtgggcgtgctgatgggcttcggcatcatcacaggcaccctgcggatcaccaatcctgtgcgggctagcgtgctgagatacgacgacttccacatcgacgaggacaagctggacaccaacagcgtgtacgagccctactaccacagcgatcacgccgagtctagctgggtcaacagaggcgagagcagcagaaaggcctacgaccacaacagcccctacatctggccccggaacgactacgatggcttcctggaaaatgcccacgagcaccacggcgtgtacaatcaaggcagaggcatcgacagcggcgagagactgatgcagcctacacagatgagcgcccaagaggacctgggagatgataccggcatccacgtgatccccacactgaacggcgacgacagacacaagatcgtgaacgtggaccagcggcagtacggcgacgtgttcaagggcgacctgaatcctaagcctcagggccagcgcctgatcgaggtgtccgtggaagagaatcaccccttcacactgagagcccctatccagagaatctacggcgtgcgctataccgagacatggtcctttctgcccagcctgacatgtaccggggatgccgctcctgccatccagcacatttgcctgaagcacaccacctgtttccaggacgtggtggtggatgtggactgcgccgagaacaccaaagaggatcagctggccgagatcagctaccggttccagggaaagaaagaggccgaccagccttggatcgtggtcaacaccagcacactgttcgacgagctggaactggaccctcctgagattgaacccggggtgctgaaggtgctgagaaccgagaagcagtacctgggagtgtacatctggaacatgagaggcagcgacggcacctctacctacgccacctttctggtcacatggaagggcgacgagaaaacacggaaccccacaccagctgtgacccctcaacctagaggcgccgagtttcacatgtggaattaccacagccacgtgttcagcgtgggcgatacctttagcctggccatgcatctgcagtacaagatccacgaggcccctttcgacctgctgctggaatggctgtacgtgcccatcgatcctacctgccagcctatgcggctgtactccacctgtctgtatcaccccaacgctccccagtgcctgagccacatgaatagcggctgcaccttcacaagccctcacctggctcagcgagtggccagcacagtgtaccagaattgcgagcacgccgacaattacaccgcctactgtctgggcatcagccacatggaacctagcttcggcctgatcctgcacgatggcggcacaaccctgaagttcgtggatacccctgagagcctgagcggcctgtatgtgttcgtggtgtacttcaacggccacgtggaagccgtggcctacaccgtggtgtctaccgtggaccacttcgtgaacgccatcgaggaaagaggcttccctccaactgctggacagcctcctgccaccaccaagcctaaagaaatcacacccgtgaatcccggcacaagcccactgcttagatacgccgcttggacaggcggactggctgctgttgttctgctgtgcctggtcatcttcctgatctgcaccgccaagcggatgagagtgaaggactacagagtggacaagagcccttacaaccagtctatgtatgccgccggactgcccgtttgataataggctggagcctcggtggccatgcttcttgccccttgggcctccccccagcccctcctccccttcctgcacccgtacccccgtggtctttgaataaagtctgagtgggcggcaaaaaaaaaaaaaaaaaaaaaaaaaaaaaaaaaaaaaaaaaaaaaaaaaaaaaaaaaaaaaaaaaaaaaaaaaaaaaaaaaaaaaaaaaaaaaaaaaaaaaaaaaaaaaa

SEQ ID NO: 121 - DNA, 2059 bp, synthetic construct
  source 1..2059: mol_type = other DNA
agactcctccccatcctctccctctgtccctctgtccctctgaccctgcactgtcccagcaccgccaccatgggcaccgtgaacaagcctgttgtgggcgtgctgatgggcttcggcatcatcacaggcaccctgcggatcaccaatcctgtgcgggctagcgtgctgagatacgacgacttccacatcgacgaggacaagctggacaccaacagcgtgtacgagccctactaccacagcgatcacgccgagtctagctgggtcaacagaggcgagagcagcagaaaggcctacgaccacaacagcccctacatctggccccggaacgactacgatggcttcctggaaaatgcccacgagcaccacggcgtgtacaatcaaggcagaggcatcgacagcggcgagagactgatgcagcctacacagatgagcgcccaagaggacctgggagatgataccggcatccacgtgatccccacactgaacggcgacgacagacacaagatcgtgaacgtggaccagcggcagtacggcgacgtgttcaagggcgacctgaatcctaagcctcagggccagcgcctgatcgaggtgtccgtggaagagaatcaccccttcacactgagagcccctatccagagaatctacggcgtgcgctataccgagacatggtcctttctgcccagcctgacatgtaccggggatgccgctcctgccatccagcacatttgcctgaagcacaccacctgtttccaggacgtggtggtggatgtggactgcgccgagaacaccaaagaggatcagctggccgagatcagctaccggttccagggaaagaaagaggccgaccagccttggatcgtggtcaacaccagcacactgttcgacgagctggaactggaccctcctgagattgaacccggggtgctgaaggtgctgagaaccgagaagcagtacctgggagtgtacatctggaacatgagaggcagcgacggcacctctacctacgccacctttctggtcacatggaagggcgacgagaaaacacggaaccccacaccagctgtgacccctcaacctagaggcgccgagtttcacatgtggaattaccacagccacgtgttcagcgtgggcgatacctttagcctggccatgcatctgcagtacaagatccacgaggcccctttcgacctgctgctggaatggctgtacgtgcccatcgatcctacctgccagcctatgcggctgtactccacctgtctgtatcaccccaacgctccccagtgcctgagccacatgaatagcggctgcaccttcacaagccctcacctggctcagcgagtggccagcacagtgtaccagaattgcgagcacgccgacaattacaccgcctactgtctgggcatcagccacatggaacctagcttcggcctgatcctgcacgatggcggcacaaccctgaagttcgtggatacccctgagagcctgagcggcctgtatgtgttcgtggtgtacttcaacggccacgtggaagccgtggcctacaccgtggtgtctaccgtggaccacttcgtgaacgccatcgaggaaagaggcttccctccaactgctggacagcctcctgccaccaccaagcctaaagaaatcacacccgtgaatcccggcacaagcccactgcttagatacgccgcttggacaggcggactggctgctgttgttctgctgtgcctggtcatcttcctgatctgcaccgccaagcggatgagagtgaaggccaagagagtggacaagagcccttacaaccagtctatgtatgccgccggactgcccgtttgataataggctggagcctcggtggccatgcttcttgccccttgggcctccccccagcccctcctccccttcctgcacccgtacccccgtggtctttgaataaagtctgagtgggcggcaaaaaaaaaaaaaaaaaaaaaaaaaaaaaaaaaaaaaaaaaaaaaaaaaaaaaaaaaaaaaaaaaaaaaaaaaaaaaaaaaaaaaaaaaaaaaaaaaaaaaaaaaaaaaa

SEQ ID NO: 122 - DNA, 1764 bp, synthetic construct
  source 1..1764: mol_type = other DNA
atgggcaccgtgaacaagcctgttgtgggcgtgctgatgggcttcggcatcatcacaggcaccctgcggatcaccaatcctgtgcgggctagcgtgctgagatacgacgacttccacatcgacgaggacaagctggacaccaacagcgtgtacgagccctactaccacagcgatcacgccgagtctagctgggtcaacagaggcgagagcagcagaaaggcctacgaccacaacagcccctacatctggccccggaacgactacgatggcttcctggaaaatgcccacgagcaccacggcgtgtacaatcaaggcagaggcatcgacagcggcgagagactgatgcagcctacacagatgagcgcccaagaggacctgggagatgataccggcatccacgtgatccccacactgaacggcgacgacagacacaagatcgtgaacgtggaccagcggcagtacggcgacgtgttcaagggcgacctgaatcctaagcctcagggccagcgcctgatcgaggtgtccgtggaagagaatcaccccttcacactgagagcccctatccagagaatctacggcgtgcgctataccgagacatggtcctttctgcccagcctgacatgtaccggggatgccgctcctgccatccagcacatttgcctgaagcacaccacctgtttccaggacgtggtggtggatgtggactgcgccgagaacaccaaagaggatcagctggccgagatcagctaccggttccagggaaagaaagaggccgaccagccttggatcgtggtcaacaccagcacactgttcgacgagctggaactggaccctcctgagattgaacccggggtgctgaaggtgctgagaaccgagaagcagtacctgggagtgtacatctggaacatgagaggcagcgacggcacctctacctacgccacctttctggtcacatggaagggcgacgagaaaacacggaaccccacaccagctgtgacccctcaacctagaggcgccgagtttcacatgtggaattaccacagccacgtgttcagcgtgggcgatacctttagcctggccatgcatctgcagtacaagatccacgaggcccctttcgacctgctgctggaatggctgtacgtgcccatcgatcctacctgccagcctatgcggctgtactccacctgtctgtatcaccccaacgctccccagtgcctgagccacatgaatagcggctgcaccttcacaagccctcacctggctcagcgagtggccagcacagtgtaccagaattgcgagcacgccgacaattacaccgcctactgtctgggcatcagccacatggaacctagcttcggcctgatcctgcacgatggcggcacaaccctgaagttcgtggatacccctgagagcctgagcggcctgtatgtgttcgtggtgtacttcaacggccacgtggaagccgtggcctacaccgtggtgtctaccgtggaccacttcgtgaacgccatcgaggaaagaggcttccctccaactgctggacagcctcctgccaccaccaagcctaaagaaatcacacccgtgaatcccggcacaagcccactgcttagatacgccgcttggacaggcggactggctgctgttgttctgctgtgcctggtcatcttcctgatctgcaccgccaagcggatgagagtgaaggccaagagagtggacaagagcccttacaaccagtctatgtatgccgccggactgcccgtttga

SEQ ID NO: 123 - protein, 587 aa, synthetic construct
MGTVNKPVVGVLMGFGIITGTLRITNPVRASVLRYDDFHIDEDKLDTNSVYEPYYHSDHAESSWVNRGESSRKAYDHNSPYIWPRNDYDGFLENAHEHHGVYNQGRGIDSGERLMQPTQMSAQEDLGDDTGIHVIPTLNGDDRHKIVNVDQRQYGDVFKGDLNPKPQGQRLIEVSVEENHPFTLRAPIQRIYGVRYTETWSFLPSLTCTGDAAPAIQHICLKHTTCFQDVVVDVDCAENTKEDQLAEISYRFQGKKEADQPWIVVNTSTLFDELELDPPEIEPGVLKVLRTEKQYLGVYIWNMRGSDGTSTYATFLVTWKGDEKTRNPTPAVTPQPRGAEFHMWNYHSHVFSVGDTFSLAMHLQYKIHEAPFDLLLEWLYVPIDPTCQPMRLYSTCLYHPNAPQCLSHMNSGCTFTSPHLAQRVASTVYQNCEHADNYTAYCLGISHMEPSFGLILHDGGTTLKFVDTPESLSGLYVFVVYFNGHVEAVAYTVVSTVDHFVNAIEERGFPPTAGQPPATTKPKEITPVNPGTSPLLRYAAWTGGLAAVVLLCLVIFLICTAKRMRVKAKRVDKSPYNQSMYAAGLPV

SEQ ID NO: 124 - RNA, 2059 nt, synthetic construct
  source 1..2059: mol_type = other RNA
agactcctccccatcctctccctctgtccctctgtccctctgaccctgcactgtcccagcaccgccaccatgggcaccgtgaacaagcctgttgtgggcgtgctgatgggcttcggcatcatcacaggcaccctgcggatcaccaatcctgtgcgggctagcgtgctgagatacgacgacttccacatcgacgaggacaagctggacaccaacagcgtgtacgagccctactaccacagcgatcacgccgagtctagctgggtcaacagaggcgagagcagcagaaaggcctacgaccacaacagcccctacatctggccccggaacgactacgatggcttcctggaaaatgcccacgagcaccacggcgtgtacaatcaaggcagaggcatcgacagcggcgagagactgatgcagcctacacagatgagcgcccaagaggacctgggagatgataccggcatccacgtgatccccacactgaacggcgacgacagacacaagatcgtgaacgtggaccagcggcagtacggcgacgtgttcaagggcgacctgaatcctaagcctcagggccagcgcctgatcgaggtgtccgtggaagagaatcaccccttcacactgagagcccctatccagagaatctacggcgtgcgctataccgagacatggtcctttctgcccagcctgacatgtaccggggatgccgctcctgccatccagcacatttgcctgaagcacaccacctgtttccaggacgtggtggtggatgtggactgcgccgagaacaccaaagaggatcagctggccgagatcagctaccggttccagggaaagaaagaggccgaccagccttggatcgtggtcaacaccagcacactgttcgacgagctggaactggaccctcctgagattgaacccggggtgctgaaggtgctgagaaccgagaagcagtacctgggagtgtacatctggaacatgagaggcagcgacggcacctctacctacgccacctttctggtcacatggaagggcgacgagaaaacacggaaccccacaccagctgtgacccctcaacctagaggcgccgagtttcacatgtggaattaccacagccacgtgttcagcgtgggcgatacctttagcctggccatgcatctgcagtacaagatccacgaggcccctttcgacctgctgctggaatggctgtacgtgcccatcgatcctacctgccagcctatgcggctgtactccacctgtctgtatcaccccaacgctccccagtgcctgagccacatgaatagcggctgcaccttcacaagccctcacctggctcagcgagtggccagcacagtgtaccagaattgcgagcacgccgacaattacaccgcctactgtctgggcatcagccacatggaacctagcttcggcctgatcctgcacgatggcggcacaaccctgaagttcgtggatacccctgagagcctgagcggcctgtatgtgttcgtggtgtacttcaacggccacgtggaagccgtggcctacaccgtggtgtctaccgtggaccacttcgtgaacgccatcgaggaaagaggcttccctccaactgctggacagcctcctgccaccaccaagcctaaagaaatcacacccgtgaatcccggcacaagcccactgcttagatacgccgcttggacaggcggactggctgctgttgttctgctgtgcctggtcatcttcctgatctgcaccgccaagcggatgagagtgaaggccaagagagtggacaagagcccttacaaccagtctatgtatgccgccggactgcccgtttgataataggctggagcctcggtggccatgcttcttgccccttgggcctccccccagcccctcctccccttcctgcacccgtacccccgtggtctttgaataaagtctgagtgggcggcaaaaaaaaaaaaaaaaaaaaaaaaaaaaaaaaaaaaaaaaaaaaaaaaaaaaaaaaaaaaaaaaaaaaaaaaaaaaaaaaaaaaaaaaaaaaaaaaaaaaaaaaaaaaaa

SEQ ID NO: 125 - DNA, 2059 bp, synthetic construct
  source 1..2059: mol_type = other DNA
agactcctccccatcctctccctctgtccctctgtccctctgaccctgcactgtcccagcaccgccaccatgggcaccgtgaacaagcctgttgtgggcgtgctgatgggcttcggcatcatcacaggcaccctgcggatcaccaatcctgtgcgggctagcgtgctgagatacgacgacttccacatcgacgaggacaagctggacaccaacagcgtgtacgagccctactaccacagcgatcacgccgagtctagctgggtcaacagaggcgagagcagcagaaaggcctacgaccacaacagcccctacatctggccccggaacgactacgatggcttcctggaaaatgcccacgagcaccacggcgtgtacaatcaaggcagaggcatcgacagcggcgagagactgatgcagcctacacagatgagcgcccaagaggacctgggagatgataccggcatccacgtgatccccacactgaacggcgacgacagacacaagatcgtgaacgtggaccagcggcagtacggcgacgtgttcaagggcgacctgaatcctaagcctcagggccagcgcctgatcgaggtgtccgtggaagagaatcaccccttcacactgagagcccctatccagagaatctacggcgtgcgctataccgagacatggtcctttctgcccagcctgacatgtaccggggatgccgctcctgccatccagcacatttgcctgaagcacaccacctgtttccaggacgtggtggtggatgtggactgcgccgagaacaccaaagaggatcagctggccgagatcagctaccggttccagggaaagaaagaggccgaccagccttggatcgtggtcaacaccagcacactgttcgacgagctggaactggaccctcctgagattgaacccggggtgctgaaggtgctgagaaccgagaagcagtacctgggagtgtacatctggaacatgagaggcagcgacggcacctctacctacgccacctttctggtcacatggaagggcgacgagaaaacacggaaccccacaccagctgtgacccctcaacctagaggcgccgagtttcacatgtggaattaccacagccacgtgttcagcgtgggcgatacctttagcctggccatgcatctgcagtacaagatccacgaggcccctttcgacctgctgctggaatggctgtacgtgcccatcgatcctacctgccagcctatgcggctgtactccacctgtctgtatcaccccaacgctccccagtgcctgagccacatgaatagcggctgcaccttcacaagccctcacctggctcagcgagtggccagcacagtgtaccagaattgcgagcacgccgacaattacaccgcctactgtctgggcatcagccacatggaacctagcttcggcctgatcctgcacgatggcggcacaaccctgaagttcgtggatacccctgagagcctgagcggcctgtatgtgttcgtggtgtacttcaacggccacgtggaagccgtggcctacaccgtggtgtctaccgtggaccacttcgtgaacgccatcgaggaaagaggcttccctccaactgctggacagcctcctgccaccaccaagcctaaagaaatcacacccgtgaatcccggcacaagcccactgcttagatacgccgcttggacaggcggactggctgctgttgttctgctgtgcctggtcatcttcctgatctgcaccgccaagcggatgagagtgaaggcctatgaggtggacaagagcccttacaaccagtctatgtatgccgccggactgcccgtttgataataggctggagcctcggtggccatgcttcttgccccttgggcctccccccagcccctcctccccttcctgcacccgtacccccgtggtctttgaataaagtctgagtgggcggcaaaaaaaaaaaaaaaaaaaaaaaaaaaaaaaaaaaaaaaaaaaaaaaaaaaaaaaaaaaaaaaaaaaaaaaaaaaaaaaaaaaaaaaaaaaaaaaaaaaaaaaaaaaaaa

SEQ ID NO: 126 - DNA, 1764 bp, synthetic construct
  source 1..1764: mol_type = other DNA
atgggcaccgtgaacaagcctgttgtgggcgtgctgatgggcttcggcatcatcacaggcaccctgcggatcaccaatcctgtgcgggctagcgtgctgagatacgacgacttccacatcgacgaggacaagctggacaccaacagcgtgtacgagccctactaccacagcgatcacgccgagtctagctgggtcaacagaggcgagagcagcagaaaggcctacgaccacaacagcccctacatctggccccggaacgactacgatggcttcctggaaaatgcccacgagcaccacggcgtgtacaatcaaggcagaggcatcgacagcggcgagagactgatgcagcctacacagatgagcgcccaagaggacctgggagatgataccggcatccacgtgatccccacactgaacggcgacgacagacacaagatcgtgaacgtggaccagcggcagtacggcgacgtgttcaagggcgacctgaatcctaagcctcagggccagcgcctgatcgaggtgtccgtggaagagaatcaccccttcacactgagagcccctatccagagaatctacggcgtgcgctataccgagacatggtcctttctgcccagcctgacatgtaccggggatgccgctcctgccatccagcacatttgcctgaagcacaccacctgtttccaggacgtggtggtggatgtggactgcgccgagaacaccaaagaggatcagctggccgagatcagctaccggttccagggaaagaaagaggccgaccagccttggatcgtggtcaacaccagcacactgttcgacgagctggaactggaccctcctgagattgaacccggggtgctgaaggtgctgagaaccgagaagcagtacctgggagtgtacatctggaacatgagaggcagcgacggcacctctacctacgccacctttctggtcacatggaagggcgacgagaaaacacggaaccccacaccagctgtgacccctcaacctagaggcgccgagtttcacatgtggaattaccacagccacgtgttcagcgtgggcgatacctttagcctggccatgcatctgcagtacaagatccacgaggcccctttcgacctgctgctggaatggctgtacgtgcccatcgatcctacctgccagcctatgcggctgtactccacctgtctgtatcaccccaacgctccccagtgcctgagccacatgaatagcggctgcaccttcacaagccctcacctggctcagcgagtggccagcacagtgtaccagaattgcgagcacgccgacaattacaccgcctactgtctgggcatcagccacatggaacctagcttcggcctgatcctgcacgatggcggcacaaccctgaagttcgtggatacccctgagagcctgagcggcctgtatgtgttcgtggtgtacttcaacggccacgtggaagccgtggcctacaccgtggtgtctaccgtggaccacttcgtgaacgccatcgaggaaagaggcttccctccaactgctggacagcctcctgccaccaccaagcctaaagaaatcacacccgtgaatcccggcacaagcccactgcttagatacgccgcttggacaggcggactggctgctgttgttctgctgtgcctggtcatcttcctgatctgcaccgccaagcggatgagagtgaaggcctatgaggtggacaagagcccttacaaccagtctatgtatgccgccggactgcccgtttga

SEQ ID NO: 127 - protein, 587 aa, synthetic construct
MGTVNKPVVGVLMGFGIITGTLRITNPVRASVLRYDDFHIDEDKLDTNSVYEPYYHSDHAESSWVNRGESSRKAYDHNSPYIWPRNDYDGFLENAHEHHGVYNQGRGIDSGERLMQPTQMSAQEDLGDDTGIHVIPTLNGDDRHKIVNVDQRQYGDVFKGDLNPKPQGQRLIEVSVEENHPFTLRAPIQRIYGVRYTETWSFLPSLTCTGDAAPAIQHICLKHTTCFQDVVVDVDCAENTKEDQLAEISYRFQGKKEADQPWIVVNTSTLFDELELDPPEIEPGVLKVLRTEKQYLGVYIWNMRGSDGTSTYATFLVTWKGDEKTRNPTPAVTPQPRGAEFHMWNYHSHVFSVGDTFSLAMHLQYKIHEAPFDLLLEWLYVPIDPTCQPMRLYSTCLYHPNAPQCLSHMNSGCTFTSPHLAQRVASTVYQNCEHADNYTAYCLGISHMEPSFGLILHDGGTTLKFVDTPESLSGLYVFVVYFNGHVEAVAYTVVSTVDHFVNAIEERGFPPTAGQPPATTKPKEITPVNPGTSPLLRYAAWTGGLAAVVLLCLVIFLICTAKRMRVKAYEVDKSPYNQSMYAAGLPV

SEQ ID NO: 128 - RNA, 2059 nt, synthetic construct
  source 1..2059: mol_type = other RNA
agactcctccccatcctctccctctgtccctctgtccctctgaccctgcactgtcccagcaccgccaccatgggcaccgtgaacaagcctgttgtgggcgtgctgatgggcttcggcatcatcacaggcaccctgcggatcaccaatcctgtgcgggctagcgtgctgagatacgacgacttccacatcgacgaggacaagctggacaccaacagcgtgtacgagccctactaccacagcgatcacgccgagtctagctgggtcaacagaggcgagagcagcagaaaggcctacgaccacaacagcccctacatctggccccggaacgactacgatggcttcctggaaaatgcccacgagcaccacggcgtgtacaatcaaggcagaggcatcgacagcggcgagagactgatgcagcctacacagatgagcgcccaagaggacctgggagatgataccggcatccacgtgatccccacactgaacggcgacgacagacacaagatcgtgaacgtggaccagcggcagtacggcgacgtgttcaagggcgacctgaatcctaagcctcagggccagcgcctgatcgaggtgtccgtggaagagaatcaccccttcacactgagagcccctatccagagaatctacggcgtgcgctataccgagacatggtcctttctgcccagcctgacatgtaccggggatgccgctcctgccatccagcacatttgcctgaagcacaccacctgtttccaggacgtggtggtggatgtggactgcgccgagaacaccaaagaggatcagctggccgagatcagctaccggttccagggaaagaaagaggccgaccagccttggatcgtggtcaacaccagcacactgttcgacgagctggaactggaccctcctgagattgaacccggggtgctgaaggtgctgagaaccgagaagcagtacctgggagtgtacatctggaacatgagaggcagcgacggcacctctacctacgccacctttctggtcacatggaagggcgacgagaaaacacggaaccccacaccagctgtgacccctcaacctagaggcgccgagtttcacatgtggaattaccacagccacgtgttcagcgtgggcgatacctttagcctggccatgcatctgcagtacaagatccacgaggcccctttcgacctgctgctggaatggctgtacgtgcccatcgatcctacctgccagcctatgcggctgtactccacctgtctgtatcaccccaacgctccccagtgcctgagccacatgaatagcggctgcaccttcacaagccctcacctggctcagcgagtggccagcacagtgtaccagaattgcgagcacgccgacaattacaccgcctactgtctgggcatcagccacatggaacctagcttcggcctgatcctgcacgatggcggcacaaccctgaagttcgtggatacccctgagagcctgagcggcctgtatgtgttcgtggtgtacttcaacggccacgtggaagccgtggcctacaccgtggtgtctaccgtggaccacttcgtgaacgccatcgaggaaagaggcttccctccaactgctggacagcctcctgccaccaccaagcctaaagaaatcacacccgtgaatcccggcacaagcccactgcttagatacgccgcttggacaggcggactggctgctgttgttctgctgtgcctggtcatcttcctgatctgcaccgccaagcggatgagagtgaaggcctatgaggtggacaagagcccttacaaccagtctatgtatgccgccggactgcccgtttgataataggctggagcctcggtggccatgcttcttgccccttgggcctccccccagcccctcctccccttcctgcacccgtacccccgtggtctttgaataaagtctgagtgggcggcaaaaaaaaaaaaaaaaaaaaaaaaaaaaaaaaaaaaaaaaaaaaaaaaaaaaaaaaaaaaaaaaaaaaaaaaaaaaaaaaaaaaaaaaaaaaaaaaaaaaaaaaaaaaaa

SEQ ID NO: 129 - DNA, 2059 bp, synthetic construct
  source 1..2059: mol_type = other DNA
agactcctccccatcctctccctctgtccctctgtccctctgaccctgcactgtcccagcaccgccaccatgggcaccgtgaacaagcctgttgtgggcgtgctgatgggcttcggcatcatcacaggcaccctgcggatcaccaatcctgtgcgggctagcgtgctgagatacgacgacttccacatcgacgaggacaagctggacaccaacagcgtgtacgagccctactaccacagcgatcacgccgagtctagctgggtcaacagaggcgagagcagcagaaaggcctacgaccacaacagcccctacatctggccccggaacgactacgatggcttcctggaaaatgcccacgagcaccacggcgtgtacaatcaaggcagaggcatcgacagcggcgagagactgatgcagcctacacagatgagcgcccaagaggacctgggagatgataccggcatccacgtgatccccacactgaacggcgacgacagacacaagatcgtgaacgtggaccagcggcagtacggcgacgtgttcaagggcgacctgaatcctaagcctcagggccagcgcctgatcgaggtgtccgtggaagagaatcaccccttcacactgagagcccctatccagagaatctacggcgtgcgctataccgagacatggtcctttctgcccagcctgacatgtaccggggatgccgctcctgccatccagcacatttgcctgaagcacaccacctgtttccaggacgtggtggtggatgtggactgcgccgagaacaccaaagaggatcagctggccgagatcagctaccggttccagggaaagaaagaggccgaccagccttggatcgtggtcaacaccagcacactgttcgacgagctggaactggaccctcctgagattgaacccggggtgctgaaggtgctgagaaccgagaagcagtacctgggagtgtacatctggaacatgagaggcagcgacggcacctctacctacgccacctttctggtcacatggaagggcgacgagaaaacacggaaccccacaccagctgtgacccctcaacctagaggcgccgagtttcacatgtggaattaccacagccacgtgttcagcgtgggcgatacctttagcctggccatgcatctgcagtacaagatccacgaggcccctttcgacctgctgctggaatggctgtacgtgcccatcgatcctacctgccagcctatgcggctgtactccacctgtctgtatcaccccaacgctccccagtgcctgagccacatgaatagcggctgcaccttcacaagccctcacctggctcagcgagtggccagcacagtgtaccagaattgcgagcacgccgacaattacaccgcctactgtctgggcatcagccacatggaacctagcttcggcctgatcctgcacgatggcggcacaaccctgaagttcgtggatacccctgagagcctgagcggcctgtatgtgttcgtggtgtacttcaacggccacgtggaagccgtggcctacaccgtggtgtctaccgtggaccacttcgtgaacgccatcgaggaaagaggcttccctccaactgctggacagcctcctgccaccaccaagcctaaagaaatcacacccgtgaatcccggcacaagcccactgcttagatacgccgcttggacaggcggactggctgctgttgttctgctgtgcctggtcatcttcctgatctgcaccgccaagcggatgagagtgaaggcctaccggaaggacaagagcccttacaaccagtctatgtatgccgccggactgcccgtttgataataggctggagcctcggtggccatgcttcttgccccttgggcctccccccagcccctcctccccttcctgcacccgtacccccgtggtctttgaataaagtctgagtgggcggcaaaaaaaaaaaaaaaaaaaaaaaaaaaaaaaaaaaaaaaaaaaaaaaaaaaaaaaaaaaaaaaaaaaaaaaaaaaaaaaaaaaaaaaaaaaaaaaaaaaaaaaaaaaaaa

SEQ ID NO: 130 - DNA, 1764 bp, synthetic construct
  source 1..1764: mol_type = other DNA
atgggcaccgtgaacaagcctgttgtgggcgtgctgatgggcttcggcatcatcacaggcaccctgcggatcaccaatcctgtgcgggctagcgtgctgagatacgacgacttccacatcgacgaggacaagctggacaccaacagcgtgtacgagccctactaccacagcgatcacgccgagtctagctgggtcaacagaggcgagagcagcagaaaggcctacgaccacaacagcccctacatctggccccggaacgactacgatggcttcctggaaaatgcccacgagcaccacggcgtgtacaatcaaggcagaggcatcgacagcggcgagagactgatgcagcctacacagatgagcgcccaagaggacctgggagatgataccggcatccacgtgatccccacactgaacggcgacgacagacacaagatcgtgaacgtggaccagcggcagtacggcgacgtgttcaagggcgacctgaatcctaagcctcagggccagcgcctgatcgaggtgtccgtggaagagaatcaccccttcacactgagagcccctatccagagaatctacggcgtgcgctataccgagacatggtcctttctgcccagcctgacatgtaccggggatgccgctcctgccatccagcacatttgcctgaagcacaccacctgtttccaggacgtggtggtggatgtggactgcgccgagaacaccaaagaggatcagctggccgagatcagctaccggttccagggaaagaaagaggccgaccagccttggatcgtggtcaacaccagcacactgttcgacgagctggaactggaccctcctgagattgaacccggggtgctgaaggtgctgagaaccgagaagcagtacctgggagtgtacatctggaacatgagaggcagcgacggcacctctacctacgccacctttctggtcacatggaagggcgacgagaaaacacggaaccccacaccagctgtgacccctcaacctagaggcgccgagtttcacatgtggaattaccacagccacgtgttcagcgtgggcgatacctttagcctggccatgcatctgcagtacaagatccacgaggcccctttcgacctgctgctggaatggctgtacgtgcccatcgatcctacctgccagcctatgcggctgtactccacctgtctgtatcaccccaacgctccccagtgcctgagccacatgaatagcggctgcaccttcacaagccctcacctggctcagcgagtggccagcacagtgtaccagaattgcgagcacgccgacaattacaccgcctactgtctgggcatcagccacatggaacctagcttcggcctgatcctgcacgatggcggcacaaccctgaagttcgtggatacccctgagagcctgagcggcctgtatgtgttcgtggtgtacttcaacggccacgtggaagccgtggcctacaccgtggtgtctaccgtggaccacttcgtgaacgccatcgaggaaagaggcttccctccaactgctggacagcctcctgccaccaccaagcctaaagaaatcacacccgtgaatcccggcacaagcccactgcttagatacgccgcttggacaggcggactggctgctgttgttctgctgtgcctggtcatcttcctgatctgcaccgccaagcggatgagagtgaaggcctaccggaaggacaagagcccttacaaccagtctatgtatgccgccggactgcccgtttga

SEQ ID NO: 131 - protein, 587 aa, synthetic construct
MGTVNKPVVGVLMGFGIITGTLRITNPVRASVLRYDDFHIDEDKLDTNSVYEPYYHSDHAESSWVNRGESSRKAYDHNSPYIWPRNDYDGFLENAHEHHGVYNQGRGIDSGERLMQPTQMSAQEDLGDDTGIHVIPTLNGDDRHKIVNVDQRQYGDVFKGDLNPKPQGQRLIEVSVEENHPFTLRAPIQRIYGVRYTETWSFLPSLTCTGDAAPAIQHICLKHTTCFQDVVVDVDCAENTKEDQLAEISYRFQGKKEADQPWIVVNTSTLFDELELDPPEIEPGVLKVLRTEKQYLGVYIWNMRGSDGTSTYATFLVTWKGDEKTRNPTPAVTPQPRGAEFHMWNYHSHVFSVGDTFSLAMHLQYKIHEAPFDLLLEWLYVPIDPTCQPMRLYSTCLYHPNAPQCLSHMNSGCTFTSPHLAQRVASTVYQNCEHADNYTAYCLGISHMEPSFGLILHDGGTTLKFVDTPESLSGLYVFVVYFNGHVEAVAYTVVSTVDHFVNAIEERGFPPTAGQPPATTKPKEITPVNPGTSPLLRYAAWTGGLAAVVLLCLVIFLICTAKRMRVKAYRKDKSPYNQSMYAAGLPV

SEQ ID NO: 132 - RNA, 2059 nt, synthetic construct
  source 1..2059: mol_type = other RNA
agactcctccccatcctctccctctgtccctctgtccctctgaccctgcactgtcccagcaccgccaccatgggcaccgtgaacaagcctgttgtgggcgtgctgatgggcttcggcatcatcacaggcaccctgcggatcaccaatcctgtgcgggctagcgtgctgagatacgacgacttccacatcgacgaggacaagctggacaccaacagcgtgtacgagccctactaccacagcgatcacgccgagtctagctgggtcaacagaggcgagagcagcagaaaggcctacgaccacaacagcccctacatctggccccggaacgactacgatggcttcctggaaaatgcccacgagcaccacggcgtgtacaatcaaggcagaggcatcgacagcggcgagagactgatgcagcctacacagatgagcgcccaagaggacctgggagatgataccggcatccacgtgatccccacactgaacggcgacgacagacacaagatcgtgaacgtggaccagcggcagtacggcgacgtgttcaagggcgacctgaatcctaagcctcagggccagcgcctgatcgaggtgtccgtggaagagaatcaccccttcacactgagagcccctatccagagaatctacggcgtgcgctataccgagacatggtcctttctgcccagcctgacatgtaccggggatgccgctcctgccatccagcacatttgcctgaagcacaccacctgtttccaggacgtggtggtggatgtggactgcgccgagaacaccaaagaggatcagctggccgagatcagctaccggttccagggaaagaaagaggccgaccagccttggatcgtggtcaacaccagcacactgttcgacgagctggaactggaccctcctgagattgaacccggggtgctgaaggtgctgagaaccgagaagcagtacctgggagtgtacatctggaacatgagaggcagcgacggcacctctacctacgccacctttctggtcacatggaagggcgacgagaaaacacggaaccccacaccagctgtgacccctcaacctagaggcgccgagtttcacatgtggaattaccacagccacgtgttcagcgtgggcgatacctttagcctggccatgcatctgcagtacaagatccacgaggcccctttcgacctgctgctggaatggctgtacgtgcccatcgatcctacctgccagcctatgcggctgtactccacctgtctgtatcaccccaacgctccccagtgcctgagccacatgaatagcggctgcaccttcacaagccctcacctggctcagcgagtggccagcacagtgtaccagaattgcgagcacgccgacaattacaccgcctactgtctgggcatcagccacatggaacctagcttcggcctgatcctgcacgatggcggcacaaccctgaagttcgtggatacccctgagagcctgagcggcctgtatgtgttcgtggtgtacttcaacggccacgtggaagccgtggcctacaccgtggtgtctaccgtggaccacttcgtgaacgccatcgaggaaagaggcttccctccaactgctggacagcctcctgccaccaccaagcctaaagaaatcacacccgtgaatcccggcacaagcccactgcttagatacgccgcttggacaggcggactggctgctgttgttctgctgtgcctggtcatcttcctgatctgcaccgccaagcggatgagagtgaaggcctaccggaaggacaagagcccttacaaccagtctatgtatgccgccggactgcccgtttgataataggctggagcctcggtggccatgcttcttgccccttgggcctccccccagcccctcctccccttcctgcacccgtacccccgtggtctttgaataaagtctgagtgggcggcaaaaaaaaaaaaaaaaaaaaaaaaaaaaaaaaaaaaaaaaaaaaaaaaaaaaaaaaaaaaaaaaaaaaaaaaaaaaaaaaaaaaaaaaaaaaaaaaaaaaaaaaaaaaaa

SEQ ID NO: 133 - DNA, 2134 bp, synthetic construct
  source 1..2134: mol_type = other DNA
agactcctccccatcctctccctctgtccctctgtccctctgaccctgcactgtcccagcaccgccaccatgggcaccgtgaacaagcctgttgtgggcgtgctgatgggcttcggcatcatcacaggcaccctgcggatcaccaatcctgtgcgggctagcgtgctgagatacgacgacttccacatcgacgaggacaagctggacaccaacagcgtgtacgagccctactaccacagcgatcacgccgagtctagctgggtcaacagaggcgagagcagcagaaaggcctacgaccacaacagcccctacatctggccccggaacgactacgatggcttcctggaaaatgcccacgagcaccacggcgtgtacaatcaaggcagaggcatcgacagcggcgagagactgatgcagcctacacagatgagcgcccaagaggacctgggagatgataccggcatccacgtgatccccacactgaacggcgacgacagacacaagatcgtgaacgtggaccagcggcagtacggcgacgtgttcaagggcgacctgaatcctaagcctcagggccagcgcctgatcgaggtgtccgtggaagagaatcaccccttcacactgagagcccctatccagagaatctacggcgtgcgctataccgagacatggtcctttctgcccagcctgacatgtaccggggatgccgctcctgccatccagcacatttgcctgaagcacaccacctgtttccaggacgtggtggtggatgtggactgcgccgagaacaccaaagaggatcagctggccgagatcagctaccggttccagggaaagaaagaggccgaccagccttggatcgtggtcaacaccagcacactgttcgacgagctggaactggaccctcctgagattgaacccggggtgctgaaggtgctgagaaccgagaagcagtacctgggagtgtacatctggaacatgagaggcagcgacggcacctctacctacgccacctttctggtcacatggaagggcgacgagaaaacacggaaccccacaccagctgtgacccctcaacctagaggcgccgagtttcacatgtggaattaccacagccacgtgttcagcgtgggcgatacctttagcctggccatgcatctgcagtacaagatccacgaggcccctttcgacctgctgctggaatggctgtacgtgcccatcgatcctacctgccagcctatgcggctgtactccacctgtctgtatcaccccaacgctccccagtgcctgagccacatgaatagcggctgcaccttcacaagccctcacctggctcagcgagtggccagcacagtgtaccagaattgcgagcacgccgacaattacaccgcctactgtctgggcatcagccacatggaacctagcttcggcctgatcctgcacgatggcggcacaaccctgaagttcgtggatacccctgagagcctgagcggcctgtatgtgttcgtggtgtacttcaacggccacgtggaagccgtggcctacaccgtggtgtctaccgtggaccacttcgtgaacgccatcgaggaaagaggcttccctccaactgctggacagcctcctgccaccaccaagcctaaagaaatcacacccgtgaatcccggcacaagcccactgcttagatacgccgcttggacaggcggactggctgctgttgttctgctgtgcctggtcatcttcctgatctgcaccgccaagcggatgagagtgaaggctatgtatgccgccggactgcccgtggacgatttcgaggatagcgagagcaccgacaccgaggaagagttcggcaacgccattggaggatctcacggcggcagcagctataccgtgtacatcgacaagacccggtgataataggctggagcctcggtggccatgcttcttgccccttgggcctccccccagcccctcctccccttcctgcacccgtacccccgtggtctttgaataaagtctgagtgggcggcaaaaaaaaaaaaaaaaaaaaaaaaaaaaaaaaaaaaaaaaaaaaaaaaaaaaaaaaaaaaaaaaaaaaaaaaaaaaaaaaaaaaaaaaaaaaaaaaaaaaaaaaaaaaaa

SEQ ID NO: 134 - DNA, 1839 bp, synthetic construct
  source 1..1839: mol_type = other DNA
atgggcaccgtgaacaagcctgttgtgggcgtgctgatgggcttcggcatcatcacaggcaccctgcggatcaccaatcctgtgcgggctagcgtgctgagatacgacgacttccacatcgacgaggacaagctggacaccaacagcgtgtacgagccctactaccacagcgatcacgccgagtctagctgggtcaacagaggcgagagcagcagaaaggcctacgaccacaacagcccctacatctggccccggaacgactacgatggcttcctggaaaatgcccacgagcaccacggcgtgtacaatcaaggcagaggcatcgacagcggcgagagactgatgcagcctacacagatgagcgcccaagaggacctgggagatgataccggcatccacgtgatccccacactgaacggcgacgacagacacaagatcgtgaacgtggaccagcggcagtacggcgacgtgttcaagggcgacctgaatcctaagcctcagggccagcgcctgatcgaggtgtccgtggaagagaatcaccccttcacactgagagcccctatccagagaatctacggcgtgcgctataccgagacatggtcctttctgcccagcctgacatgtaccggggatgccgctcctgccatccagcacatttgcctgaagcacaccacctgtttccaggacgtggtggtggatgtggactgcgccgagaacaccaaagaggatcagctggccgagatcagctaccggttccagggaaagaaagaggccgaccagccttggatcgtggtcaacaccagcacactgttcgacgagctggaactggaccctcctgagattgaacccggggtgctgaaggtgctgagaaccgagaagcagtacctgggagtgtacatctggaacatgagaggcagcgacggcacctctacctacgccacctttctggtcacatggaagggcgacgagaaaacacggaaccccacaccagctgtgacccctcaacctagaggcgccgagtttcacatgtggaattaccacagccacgtgttcagcgtgggcgatacctttagcctggccatgcatctgcagtacaagatccacgaggcccctttcgacctgctgctggaatggctgtacgtgcccatcgatcctacctgccagcctatgcggctgtactccacctgtctgtatcaccccaacgctccccagtgcctgagccacatgaatagcggctgcaccttcacaagccctcacctggctcagcgagtggccagcacagtgtaccagaattgcgagcacgccgacaattacaccgcctactgtctgggcatcagccacatggaacctagcttcggcctgatcctgcacgatggcggcacaaccctgaagttcgtggatacccctgagagcctgagcggcctgtatgtgttcgtggtgtacttcaacggccacgtggaagccgtggcctacaccgtggtgtctaccgtggaccacttcgtgaacgccatcgaggaaagaggcttccctccaactgctggacagcctcctgccaccaccaagcctaaagaaatcacacccgtgaatcccggcacaagcccactgcttagatacgccgcttggacaggcggactggctgctgttgttctgctgtgcctggtcatcttcctgatctgcaccgccaagcggatgagagtgaaggctatgtatgccgccggactgcccgtggacgatttcgaggatagcgagagcaccgacaccgaggaagagttcggcaacgccattggaggatctcacggcggcagcagctataccgtgtacatcgacaagacccggtga

SEQ ID NO: 135 - protein, 612 aa, synthetic construct
MGTVNKPVVGVLMGFGIITGTLRITNPVRASVLRYDDFHIDEDKLDTNSVYEPYYHSDHAESSWVNRGESSRKAYDHNSPYIWPRNDYDGFLENAHEHHGVYNQGRGIDSGERLMQPTQMSAQEDLGDDTGIHVIPTLNGDDRHKIVNVDQRQYGDVFKGDLNPKPQGQRLIEVSVEENHPFTLRAPIQRIYGVRYTETWSFLPSLTCTGDAAPAIQHICLKHTTCFQDVVVDVDCAENTKEDQLAEISYRFQGKKEADQPWIVVNTSTLFDELELDPPEIEPGVLKVLRTEKQYLGVYIWNMRGSDGTSTYATFLVTWKGDEKTRNPTPAVTPQPRGAEFHMWNYHSHVFSVGDTFSLAMHLQYKIHEAPFDLLLEWLYVPIDPTCQPMRLYSTCLYHPNAPQCLSHMNSGCTFTSPHLAQRVASTVYQNCEHADNYTAYCLGISHMEPSFGLILHDGGTTLKFVDTPESLSGLYVFVVYFNGHVEAVAYTVVSTVDHFVNAIEERGFPPTAGQPPATTKPKEITPVNPGTSPLLRYAAWTGGLAAVVLLCLVIFLICTAKRMRVKAMYAAGLPVDDFEDSESTDTEEEFGNAIGGSHGGSSYTVYIDKTR

SEQ ID NO: 136 - RNA, 2134 nt, synthetic construct
  source 1..2134: mol_type = other RNA
agactcctccccatcctctccctctgtccctctgtccctctgaccctgcactgtcccagcaccgccaccatgggcaccgtgaacaagcctgttgtgggcgtgctgatgggcttcggcatcatcacaggcaccctgcggatcaccaatcctgtgcgggctagcgtgctgagatacgacgacttccacatcgacgaggacaagctggacaccaacagcgtgtacgagccctactaccacagcgatcacgccgagtctagctgggtcaacagaggcgagagcagcagaaaggcctacgaccacaacagcccctacatctggccccggaacgactacgatggcttcctggaaaatgcccacgagcaccacggcgtgtacaatcaaggcagaggcatcgacagcggcgagagactgatgcagcctacacagatgagcgcccaagaggacctgggagatgataccggcatccacgtgatccccacactgaacggcgacgacagacacaagatcgtgaacgtggaccagcggcagtacggcgacgtgttcaagggcgacctgaatcctaagcctcagggccagcgcctgatcgaggtgtccgtggaagagaatcaccccttcacactgagagcccctatccagagaatctacggcgtgcgctataccgagacatggtcctttctgcccagcctgacatgtaccggggatgccgctcctgccatccagcacatttgcctgaagcacaccacctgtttccaggacgtggtggtggatgtggactgcgccgagaacaccaaagaggatcagctggccgagatcagctaccggttccagggaaagaaagaggccgaccagccttggatcgtggtcaacaccagcacactgttcgacgagctggaactggaccctcctgagattgaacccggggtgctgaaggtgctgagaaccgagaagcagtacctgggagtgtacatctggaacatgagaggcagcgacggcacctctacctacgccacctttctggtcacatggaagggcgacgagaaaacacggaaccccacaccagctgtgacccctcaacctagaggcgccgagtttcacatgtggaattaccacagccacgtgttcagcgtgggcgatacctttagcctggccatgcatctgcagtacaagatccacgaggcccctttcgacctgctgctggaatggctgtacgtgcccatcgatcctacctgccagcctatgcggctgtactccacctgtctgtatcaccccaacgctccccagtgcctgagccacatgaatagcggctgcaccttcacaagccctcacctggctcagcgagtggccagcacagtgtaccagaattgcgagcacgccgacaattacaccgcctactgtctgggcatcagccacatggaacctagcttcggcctgatcctgcacgatggcggcacaaccctgaagttcgtggatacccctgagagcctgagcggcctgtatgtgttcgtggtgtacttcaacggccacgtggaagccgtggcctacaccgtggtgtctaccgtggaccacttcgtgaacgccatcgaggaaagaggcttccctccaactgctggacagcctcctgccaccaccaagcctaaagaaatcacacccgtgaatcccggcacaagcccactgcttagatacgccgcttggacaggcggactggctgctgttgttctgctgtgcctggtcatcttcctgatctgcaccgccaagcggatgagagtgaaggctatgtatgccgccggactgcccgtggacgatttcgaggatagcgagagcaccgacaccgaggaagagttcggcaacgccattggaggatctcacggcggcagcagctataccgtgtacatcgacaagacccggtgataataggctggagcctcggtggccatgcttcttgccccttgggcctccccccagcccctcctccccttcctgcacccgtacccccgtggtctttgaataaagtctgagtgggcggcaaaaaaaaaaaaaaaaaaaaaaaaaaaaaaaaaaaaaaaaaaaaaaaaaaaaaaaaaaaaaaaaaaaaaaaaaaaaaaaaaaaaaaaaaaaaaaaaaaaaaaaaaaaaaa

SEQ ID NO: 137 - DNA, 2134 bp, synthetic construct
  source 1..2134: mol_type = other DNA
agactcctccccatcctctccctctgtccctctgtccctctgaccctgcactgtcccagcaccgccaccatgggcaccgtgaacaagcctgttgtgggcgtgctgatgggcttcggcatcatcacaggcaccctgcggatcaccaatcctgtgcgggctagcgtgctgagatacgacgacttccacatcgacgaggacaagctggacaccaacagcgtgtacgagccctactaccacagcgatcacgccgagtctagctgggtcaacagaggcgagagcagcagaaaggcctacgaccacaacagcccctacatctggccccggaacgactacgatggcttcctggaaaatgcccacgagcaccacggcgtgtacaatcaaggcagaggcatcgacagcggcgagagactgatgcagcctacacagatgagcgcccaagaggacctgggagatgataccggcatccacgtgatccccacactgaacggcgacgacagacacaagatcgtgaacgtggaccagcggcagtacggcgacgtgttcaagggcgacctgaatcctaagcctcagggccagcgcctgatcgaggtgtccgtggaagagaatcaccccttcacactgagagcccctatccagagaatctacggcgtgcgctataccgagacatggtcctttctgcccagcctgacatgtaccggggatgccgctcctgccatccagcacatttgcctgaagcacaccacctgtttccaggacgtggtggtggatgtggactgcgccgagaacaccaaagaggatcagctggccgagatcagctaccggttccagggaaagaaagaggccgaccagccttggatcgtggtcaacaccagcacactgttcgacgagctggaactggaccctcctgagattgaacccggggtgctgaaggtgctgagaaccgagaagcagtacctgggagtgtacatctggaacatgagaggcagcgacggcacctctacctacgccacctttctggtcacatggaagggcgacgagaaaacacggaaccccacaccagctgtgacccctcaacctagaggcgccgagtttcacatgtggaattaccacagccacgtgttcagcgtgggcgatacctttagcctggccatgcatctgcagtacaagatccacgaggcccctttcgacctgctgctggaatggctgtacgtgcccatcgatcctacctgccagcctatgcggctgtactccacctgtctgtatcaccccaacgctccccagtgcctgagccacatgaatagcggctgcaccttcacaagccctcacctggctcagcgagtggccagcacagtgtaccagaattgcgagcacgccgacaattacaccgcctactgtctgggcatcagccacatggaacctagcttcggcctgatcctgcacgatggcggcacaaccctgaagttcgtggatacccctgagagcctgagcggcctgtatgtgttcgtggtgtacttcaacggccacgtggaagccgtggcctacaccgtggtgtctaccgtggaccacttcgtgaacgccatcgaggaaagaggcttccctccaactgctggacagcctcctgccaccaccaagcctaaagaaatcacacccgtgaatcccggcacaagcccactgcttagatacgccgcttggacaggcggactggctgctgttgttctgctgtgcctggtcatcttcctgatctgcaccgccaagcggatgagagtgaaggctatgtatgccgccggactgcccgtggacgattttgaggatgctgaagccgccgacgccgaggaagaatttggcaacgccattggcggaagccacggcggcagtagctataccgtgtacatcgacaagacccggtgataataggctggagcctcggtggccatgcttcttgccccttgggcctccccccagcccctcctccccttcctgcacccgtacccccgtggtctttgaataaagtctgagtgggcggcaaaaaaaaaaaaaaaaaaaaaaaaaaaaaaaaaaaaaaaaaaaaaaaaaaaaaaaaaaaaaaaaaaaaaaaaaaaaaaaaaaaaaaaaaaaaaaaaaaaaaaaaaaaaaa

SEQ ID NO: 138 - DNA, 1839 bp, synthetic construct
  source 1..1839: mol_type = other DNA
atgggcaccgtgaacaagcctgttgtgggcgtgctgatgggcttcggcatcatcacaggcaccctgcggatcaccaatcctgtgcgggctagcgtgctgagatacgacgacttccacatcgacgaggacaagctggacaccaacagcgtgtacgagccctactaccacagcgatcacgccgagtctagctgggtcaacagaggcgagagcagcagaaaggcctacgaccacaacagcccctacatctggccccggaacgactacgatggcttcctggaaaatgcccacgagcaccacggcgtgtacaatcaaggcagaggcatcgacagcggcgagagactgatgcagcctacacagatgagcgcccaagaggacctgggagatgataccggcatccacgtgatccccacactgaacggcgacgacagacacaagatcgtgaacgtggaccagcggcagtacggcgacgtgttcaagggcgacctgaatcctaagcctcagggccagcgcctgatcgaggtgtccgtggaagagaatcaccccttcacactgagagcccctatccagagaatctacggcgtgcgctataccgagacatggtcctttctgcccagcctgacatgtaccggggatgccgctcctgccatccagcacatttgcctgaagcacaccacctgtttccaggacgtggtggtggatgtggactgcgccgagaacaccaaagaggatcagctggccgagatcagctaccggttccagggaaagaaagaggccgaccagccttggatcgtggtcaacaccagcacactgttcgacgagctggaactggaccctcctgagattgaacccggggtgctgaaggtgctgagaaccgagaagcagtacctgggagtgtacatctggaacatgagaggcagcgacggcacctctacctacgccacctttctggtcacatggaagggcgacgagaaaacacggaaccccacaccagctgtgacccctcaacctagaggcgccgagtttcacatgtggaattaccacagccacgtgttcagcgtgggcgatacctttagcctggccatgcatctgcagtacaagatccacgaggcccctttcgacctgctgctggaatggctgtacgtgcccatcgatcctacctgccagcctatgcggctgtactccacctgtctgtatcaccccaacgctccccagtgcctgagccacatgaatagcggctgcaccttcacaagccctcacctggctcagcgagtggccagcacagtgtaccagaattgcgagcacgccgacaattacaccgcctactgtctgggcatcagccacatggaacctagcttcggcctgatcctgcacgatggcggcacaaccctgaagttcgtggatacccctgagagcctgagcggcctgtatgtgttcgtggtgtacttcaacggccacgtggaagccgtggcctacaccgtggtgtctaccgtggaccacttcgtgaacgccatcgaggaaagaggcttccctccaactgctggacagcctcctgccaccaccaagcctaaagaaatcacacccgtgaatcccggcacaagcccactgcttagatacgccgcttggacaggcggactggctgctgttgttctgctgtgcctggtcatcttcctgatctgcaccgccaagcggatgagagtgaaggctatgtatgccgccggactgcccgtggacgattttgaggatgctgaagccgccgacgccgaggaagaatttggcaacgccattggcggaagccacggcggcagtagctataccgtgtacatcgacaagacccggtga

SEQ ID NO: 139 - protein, 612 aa, synthetic construct
MGTVNKPVVGVLMGFGIITGTLRITNPVRASVLRYDDFHIDEDKLDTNSVYEPYYHSDHAESSWVNRGESSRKAYDHNSPYIWPRNDYDGFLENAHEHHGVYNQGRGIDSGERLMQPTQMSAQEDLGDDTGIHVIPTLNGDDRHKIVNVDQRQYGDVFKGDLNPKPQGQRLIEVSVEENHPFTLRAPIQRIYGVRYTETWSFLPSLTCTGDAAPAIQHICLKHTTCFQDVVVDVDCAENTKEDQLAEISYRFQGKKEADQPWIVVNTSTLFDELELDPPEIEPGVLKVLRTEKQYLGVYIWNMRGSDGTSTYATFLVTWKGDEKTRNPTPAVTPQPRGAEFHMWNYHSHVFSVGDTFSLAMHLQYKIHEAPFDLLLEWLYVPIDPTCQPMRLYSTCLYHPNAPQCLSHMNSGCTFTSPHLAQRVASTVYQNCEHADNYTAYCLGISHMEPSFGLILHDGGTTLKFVDTPESLSGLYVFVVYFNGHVEAVAYTVVSTVDHFVNAIEERGFPPTAGQPPATTKPKEITPVNPGTSPLLRYAAWTGGLAAVVLLCLVIFLICTAKRMRVKAMYAAGLPVDDFEDAEAADAEEEFGNAIGGSHGGSSYTVYIDKTR

SEQ ID NO: 140 - RNA, 2134 nt, synthetic construct
  source 1..2134: mol_type = other RNA
agactcctccccatcctctccctctgtccctctgtccctctgaccctgcactgtcccagcaccgccaccatgggcaccgtgaacaagcctgttgtgggcgtgctgatgggcttcggcatcatcacaggcaccctgcggatcaccaatcctgtgcgggctagcgtgctgagatacgacgacttccacatcgacgaggacaagctggacaccaacagcgtgtacgagccctactaccacagcgatcacgccgagtctagctgggtcaacagaggcgagagcagcagaaaggcctacgaccacaacagcccctacatctggccccggaacgactacgatggcttcctggaaaatgcccacgagcaccacggcgtgtacaatcaaggcagaggcatcgacagcggcgagagactgatgcagcctacacagatgagcgcccaagaggacctgggagatgataccggcatccacgtgatccccacactgaacggcgacgacagacacaagatcgtgaacgtggaccagcggcagtacggcgacgtgttcaagggcgacctgaatcctaagcctcagggccagcgcctgatcgaggtgtccgtggaagagaatcaccccttcacactgagagcccctatccagagaatctacggcgtgcgctataccgagacatggtcctttctgcccagcctgacatgtaccggggatgccgctcctgccatccagcacatttgcctgaagcacaccacctgtttccaggacgtggtggtggatgtggactgcgccgagaacaccaaagaggatcagctggccgagatcagctaccggttccagggaaagaaagaggccgaccagccttggatcgtggtcaacaccagcacactgttcgacgagctggaactggaccctcctgagattgaacccggggtgctgaaggtgctgagaaccgagaagcagtacctgggagtgtacatctggaacatgagaggcagcgacggcacctctacctacgccacctttctggtcacatggaagggcgacgagaaaacacggaaccccacaccagctgtgacccctcaacctagaggcgccgagtttcacatgtggaattaccacagccacgtgttcagcgtgggcgatacctttagcctggccatgcatctgcagtacaagatccacgaggcccctttcgacctgctgctggaatggctgtacgtgcccatcgatcctacctgccagcctatgcggctgtactccacctgtctgtatcaccccaacgctccccagtgcctgagccacatgaatagcggctgcaccttcacaagccctcacctggctcagcgagtggccagcacagtgtaccagaattgcgagcacgccgacaattacaccgcctactgtctgggcatcagccacatggaacctagcttcggcctgatcctgcacgatggcggcacaaccctgaagttcgtggatacccctgagagcctgagcggcctgtatgtgttcgtggtgtacttcaacggccacgtggaagccgtggcctacaccgtggtgtctaccgtggaccacttcgtgaacgccatcgaggaaagaggcttccctccaactgctggacagcctcctgccaccaccaagcctaaagaaatcacacccgtgaatcccggcacaagcccactgcttagatacgccgcttggacaggcggactggctgctgttgttctgctgtgcctggtcatcttcctgatctgcaccgccaagcggatgagagtgaaggctatgtatgccgccggactgcccgtggacgattttgaggatgctgaagccgccgacgccgaggaagaatttggcaacgccattggcggaagccacggcggcagtagctataccgtgtacatcgacaagacccggtgataataggctggagcctcggtggccatgcttcttgccccttgggcctccccccagcccctcctccccttcctgcacccgtacccccgtggtctttgaataaagtctgagtgggcggcaaaaaaaaaaaaaaaaaaaaaaaaaaaaaaaaaaaaaaaaaaaaaaaaaaaaaaaaaaaaaaaaaaaaaaaaaaaaaaaaaaaaaaaaaaaaaaaaaaaaaaaaaaaaaa

SEQ ID NO: 141 - DNA, 2167 bp, synthetic construct
  source 1..2167: mol_type = other DNA
agactcctccccatcctctccctctgtccctctgtccctctgaccctgcactgtcccagcaccgccaccatgggcaccgtgaacaagcctgttgtgggcgtgctgatgggcttcggcatcatcacaggcaccctgcggatcaccaatcctgtgcgggctagcgtgctgagatacgacgacttccacatcgacgaggacaagctggacaccaacagcgtgtacgagccctactaccacagcgatcacgccgagtctagctgggtcaacagaggcgagagcagcagaaaggcctacgaccacaacagcccctacatctggccccggaacgactacgatggcttcctggaaaatgcccacgagcaccacggcgtgtacaatcaaggcagaggcatcgacagcggcgagagactgatgcagcctacacagatgagcgcccaagaggacctgggagatgataccggcatccacgtgatccccacactgaacggcgacgacagacacaagatcgtgaacgtggaccagcggcagtacggcgacgtgttcaagggcgacctgaatcctaagcctcagggccagcgcctgatcgaggtgtccgtggaagagaatcaccccttcacactgagagcccctatccagagaatctacggcgtgcgctataccgagacatggtcctttctgcccagcctgacatgtaccggggatgccgctcctgccatccagcacatttgcctgaagcacaccacctgtttccaggacgtggtggtggatgtggactgcgccgagaacaccaaagaggatcagctggccgagatcagctaccggttccagggaaagaaagaggccgaccagccttggatcgtggtcaacaccagcacactgttcgacgagctggaactggaccctcctgagattgaacccggggtgctgaaggtgctgagaaccgagaagcagtacctgggagtgtacatctggaacatgagaggcagcgacggcacctctacctacgccacctttctggtcacatggaagggcgacgagaaaacacggaaccccacaccagctgtgacccctcaacctagaggcgccgagtttcacatgtggaattaccacagccacgtgttcagcgtgggcgatacctttagcctggccatgcatctgcagtacaagatccacgaggcccctttcgacctgctgctggaatggctgtacgtgcccatcgatcctacctgccagcctatgcggctgtactccacctgtctgtatcaccccaacgctccccagtgcctgagccacatgaatagcggctgcaccttcacaagccctcacctggctcagcgagtggccagcacagtgtaccagaattgcgagcacgccgacaattacaccgcctactgtctgggcatcagccacatggaacctagcttcggcctgatcctgcacgatggcggcacaaccctgaagttcgtggatacccctgagagcctgagcggcctgtatgtgttcgtggtgtacttcaacggccacgtggaagccgtggcctacaccgtggtgtctaccgtggaccacttcgtgaacgccatcgaggaaagaggcttccctccaactgctggacagcctcctgccaccaccaagcctaaagaaatcacacccgtgaatcccggcacaagcccactgcttagatacgccgcttggacaggcggactggctgctgttgttctgctgtgcctggtcatcttcctgatctgcaccgccaagcggatgcgcgtgaaggacaaagagaaggacaagtccccttacaaccagtctatgtatggcgccggactgcccgtggacgatttcgaggatagcgagagcaccgacaccgaggaagagttcggcaacgccattggaggatctcacggcggcagcagctataccgtgtacatcgacaagacccggtgataataggctggagcctcggtggccatgcttcttgccccttgggcctccccccagcccctcctccccttcctgcacccgtacccccgtggtctttgaataaagtctgagtgggcggcaaaaaaaaaaaaaaaaaaaaaaaaaaaaaaaaaaaaaaaaaaaaaaaaaaaaaaaaaaaaaaaaaaaaaaaaaaaaaaaaaaaaaaaaaaaaaaaaaaaaaaaaaaaaaa

SEQ ID NO: 142 - DNA, 1872 bp, synthetic construct
  source 1..1872: mol_type = other DNA
atgggcaccgtgaacaagcctgttgtgggcgtgctgatgggcttcggcatcatcacaggcaccctgcggatcaccaatcctgtgcgggctagcgtgctgagatacgacgacttccacatcgacgaggacaagctggacaccaacagcgtgtacgagccctactaccacagcgatcacgccgagtctagctgggtcaacagaggcgagagcagcagaaaggcctacgaccacaacagcccctacatctggccccggaacgactacgatggcttcctggaaaatgcccacgagcaccacggcgtgtacaatcaaggcagaggcatcgacagcggcgagagactgatgcagcctacacagatgagcgcccaagaggacctgggagatgataccggcatccacgtgatccccacactgaacggcgacgacagacacaagatcgtgaacgtggaccagcggcagtacggcgacgtgttcaagggcgacctgaatcctaagcctcagggccagcgcctgatcgaggtgtccgtggaagagaatcaccccttcacactgagagcccctatccagagaatctacggcgtgcgctataccgagacatggtcctttctgcccagcctgacatgtaccggggatgccgctcctgccatccagcacatttgcctgaagcacaccacctgtttccaggacgtggtggtggatgtggactgcgccgagaacaccaaagaggatcagctggccgagatcagctaccggttccagggaaagaaagaggccgaccagccttggatcgtggtcaacaccagcacactgttcgacgagctggaactggaccctcctgagattgaacccggggtgctgaaggtgctgagaaccgagaagcagtacctgggagtgtacatctggaacatgagaggcagcgacggcacctctacctacgccacctttctggtcacatggaagggcgacgagaaaacacggaaccccacaccagctgtgacccctcaacctagaggcgccgagtttcacatgtggaattaccacagccacgtgttcagcgtgggcgatacctttagcctggccatgcatctgcagtacaagatccacgaggcccctttcgacctgctgctggaatggctgtacgtgcccatcgatcctacctgccagcctatgcggctgtactccacctgtctgtatcaccccaacgctccccagtgcctgagccacatgaatagcggctgcaccttcacaagccctcacctggctcagcgagtggccagcacagtgtaccagaattgcgagcacgccgacaattacaccgcctactgtctgggcatcagccacatggaacctagcttcggcctgatcctgcacgatggcggcacaaccctgaagttcgtggatacccctgagagcctgagcggcctgtatgtgttcgtggtgtacttcaacggccacgtggaagccgtggcctacaccgtggtgtctaccgtggaccacttcgtgaacgccatcgaggaaagaggcttccctccaactgctggacagcctcctgccaccaccaagcctaaagaaatcacacccgtgaatcccggcacaagcccactgcttagatacgccgcttggacaggcggactggctgctgttgttctgctgtgcctggtcatcttcctgatctgcaccgccaagcggatgcgcgtgaaggacaaagagaaggacaagtccccttacaaccagtctatgtatggcgccggactgcccgtggacgatttcgaggatagcgagagcaccgacaccgaggaagagttcggcaacgccattggaggatctcacggcggcagcagctataccgtgtacatcgacaagacccggtga

SEQ ID NO: 143 - protein, 623 aa, synthetic construct
MGTVNKPVVGVLMGFGIITGTLRITNPVRASVLRYDDFHIDEDKLDTNSVYEPYYHSDHAESSWVNRGESSRKAYDHNSPYIWPRNDYDGFLENAHEHHGVYNQGRGIDSGERLMQPTQMSAQEDLGDDTGIHVIPTLNGDDRHKIVNVDQRQYGDVFKGDLNPKPQGQRLIEVSVEENHPFTLRAPIQRIYGVRYTETWSFLPSLTCTGDAAPAIQHICLKHTTCFQDVVVDVDCAENTKEDQLAEISYRFQGKKEADQPWIVVNTSTLFDELELDPPEIEPGVLKVLRTEKQYLGVYIWNMRGSDGTSTYATFLVTWKGDEKTRNPTPAVTPQPRGAEFHMWNYHSHVFSVGDTFSLAMHLQYKIHEAPFDLLLEWLYVPIDPTCQPMRLYSTCLYHPNAPQCLSHMNSGCTFTSPHLAQRVASTVYQNCEHADNYTAYCLGISHMEPSFGLILHDGGTTLKFVDTPESLSGLYVFVVYFNGHVEAVAYTVVSTVDHFVNAIEERGFPPTAGQPPATTKPKEITPVNPGTSPLLRYAAWTGGLAAVVLLCLVIFLICTAKRMRVKDKEKDKSPYNQSMYGAGLPVDDFEDSESTDTEEEFGNAIGGSHGGSSYTVYIDKTR

SEQ ID NO: 144 - RNA, 2167 nt, synthetic construct
  source 1..2167: mol_type = other RNA
agactcctccccatcctctccctctgtccctctgtccctctgaccctgcactgtcccagcaccgccaccatgggcaccgtgaacaagcctgttgtgggcgtgctgatgggcttcggcatcatcacaggcaccctgcggatcaccaatcctgtgcgggctagcgtgctgagatacgacgacttccacatcgacgaggacaagctggacaccaacagcgtgtacgagccctactaccacagcgatcacgccgagtctagctgggtcaacagaggcgagagcagcagaaaggcctacgaccacaacagcccctacatctggccccggaacgactacgatggcttcctggaaaatgcccacgagcaccacggcgtgtacaatcaaggcagaggcatcgacagcggcgagagactgatgcagcctacacagatgagcgcccaagaggacctgggagatgataccggcatccacgtgatccccacactgaacggcgacgacagacacaagatcgtgaacgtggaccagcggcagtacggcgacgtgttcaagggcgacctgaatcctaagcctcagggccagcgcctgatcgaggtgtccgtggaagagaatcaccccttcacactgagagcccctatccagagaatctacggcgtgcgctataccgagacatggtcctttctgcccagcctgacatgtaccggggatgccgctcctgccatccagcacatttgcctgaagcacaccacctgtttccaggacgtggtggtggatgtggactgcgccgagaacaccaaagaggatcagctggccgagatcagctaccggttccagggaaagaaagaggccgaccagccttggatcgtggtcaacaccagcacactgttcgacgagctggaactggaccctcctgagattgaacccggggtgctgaaggtgctgagaaccgagaagcagtacctgggagtgtacatctggaacatgagaggcagcgacggcacctctacctacgccacctttctggtcacatggaagggcgacgagaaaacacggaaccccacaccagctgtgacccctcaacctagaggcgccgagtttcacatgtggaattaccacagccacgtgttcagcgtgggcgatacctttagcctggccatgcatctgcagtacaagatccacgaggcccctttcgacctgctgctggaatggctgtacgtgcccatcgatcctacctgccagcctatgcggctgtactccacctgtctgtatcaccccaacgctccccagtgcctgagccacatgaatagcggctgcaccttcacaagccctcacctggctcagcgagtggccagcacagtgtaccagaattgcgagcacgccgacaattacaccgcctactgtctgggcatcagccacatggaacctagcttcggcctgatcctgcacgatggcggcacaaccctgaagttcgtggatacccctgagagcctgagcggcctgtatgtgttcgtggtgtacttcaacggccacgtggaagccgtggcctacaccgtggtgtctaccgtggaccacttcgtgaacgccatcgaggaaagaggcttccctccaactgctggacagcctcctgccaccaccaagcctaaagaaatcacacccgtgaatcccggcacaagcccactgcttagatacgccgcttggacaggcggactggctgctgttgttctgctgtgcctggtcatcttcctgatctgcaccgccaagcggatgcgcgtgaaggacaaagagaaggacaagtccccttacaaccagtctatgtatggcgccggactgcccgtggacgatttcgaggatagcgagagcaccgacaccgaggaagagttcggcaacgccattggaggatctcacggcggcagcagctataccgtgtacatcgacaagacccggtgataataggctggagcctcggtggccatgcttcttgccccttgggcctccccccagcccctcctccccttcctgcacccgtacccccgtggtctttgaataaagtctgagtgggcggcaaaaaaaaaaaaaaaaaaaaaaaaaaaaaaaaaaaaaaaaaaaaaaaaaaaaaaaaaaaaaaaaaaaaaaaaaaaaaaaaaaaaaaaaaaaaaaaaaaaaaaaaaaaaaa

SEQ ID NO: 145 - DNA, 2167 bp, synthetic construct
  source 1..2167: mol_type = other DNA
agactcctccccatcctctccctctgtccctctgtccctctgaccctgcactgtcccagcaccgccaccatgggcaccgtgaacaagcctgttgtgggcgtgctgatgggcttcggcatcatcacaggcaccctgcggatcaccaatcctgtgcgggctagcgtgctgagatacgacgacttccacatcgacgaggacaagctggacaccaacagcgtgtacgagccctactaccacagcgatcacgccgagtctagctgggtcaacagaggcgagagcagcagaaaggcctacgaccacaacagcccctacatctggccccggaacgactacgatggcttcctggaaaatgcccacgagcaccacggcgtgtacaatcaaggcagaggcatcgacagcggcgagagactgatgcagcctacacagatgagcgcccaagaggacctgggagatgataccggcatccacgtgatccccacactgaacggcgacgacagacacaagatcgtgaacgtggaccagcggcagtacggcgacgtgttcaagggcgacctgaatcctaagcctcagggccagcgcctgatcgaggtgtccgtggaagagaatcaccccttcacactgagagcccctatccagagaatctacggcgtgcgctataccgagacatggtcctttctgcccagcctgacatgtaccggggatgccgctcctgccatccagcacatttgcctgaagcacaccacctgtttccaggacgtggtggtggatgtggactgcgccgagaacaccaaagaggatcagctggccgagatcagctaccggttccagggaaagaaagaggccgaccagccttggatcgtggtcaacaccagcacactgttcgacgagctggaactggaccctcctgagattgaacccggggtgctgaaggtgctgagaaccgagaagcagtacctgggagtgtacatctggaacatgagaggcagcgacggcacctctacctacgccacctttctggtcacatggaagggcgacgagaaaacacggaaccccacaccagctgtgacccctcaacctagaggcgccgagtttcacatgtggaattaccacagccacgtgttcagcgtgggcgatacctttagcctggccatgcatctgcagtacaagatccacgaggcccctttcgacctgctgctggaatggctgtacgtgcccatcgatcctacctgccagcctatgcggctgtactccacctgtctgtatcaccccaacgctccccagtgcctgagccacatgaatagcggctgcaccttcacaagccctcacctggctcagcgagtggccagcacagtgtaccagaattgcgagcacgccgacaattacaccgcctactgtctgggcatcagccacatggaacctagcttcggcctgatcctgcacgatggcggcacaaccctgaagttcgtggatacccctgagagcctgagcggcctgtatgtgttcgtggtgtacttcaacggccacgtggaagccgtggcctacaccgtggtgtctaccgtggaccacttcgtgaacgccatcgaggaaagaggcttccctccaactgctggacagcctcctgccaccaccaagcctaaagaaatcacacccgtgaatcccggcacaagcccactgcttagatacgccgcttggacaggcggactggctgctgttgttctgctgtgcctggtcatcttcctgatctgcaccgccaagcggatgcgcgtgaaggacaaagagaaggacaagtccccttacaaccagtctatgtatggcgccggactgcccgtggacgattttgaggatgctgaagccgccgacgccgaggaagaatttggcaacgccattggcggaagccacggcggcagtagctataccgtgtacatcgacaagacccggtgataataggctggagcctcggtggccatgcttcttgccccttgggcctccccccagcccctcctccccttcctgcacccgtacccccgtggtctttgaataaagtctgagtgggcggcaaaaaaaaaaaaaaaaaaaaaaaaaaaaaaaaaaaaaaaaaaaaaaaaaaaaaaaaaaaaaaaaaaaaaaaaaaaaaaaaaaaaaaaaaaaaaaaaaaaaaaaaaaaaaa

SEQ ID NO: 146 - DNA, 1872 bp, synthetic construct
  source 1..1872: mol_type = other DNA
atgggcaccgtgaacaagcctgttgtgggcgtgctgatgggcttcggcatcatcacaggcaccctgcggatcaccaatcctgtgcgggctagcgtgctgagatacgacgacttccacatcgacgaggacaagctggacaccaacagcgtgtacgagccctactaccacagcgatcacgccgagtctagctgggtcaacagaggcgagagcagcagaaaggcctacgaccacaacagcccctacatctggccccggaacgactacgatggcttcctggaaaatgcccacgagcaccacggcgtgtacaatcaaggcagaggcatcgacagcggcgagagactgatgcagcctacacagatgagcgcccaagaggacctgggagatgataccggcatccacgtgatccccacactgaacggcgacgacagacacaagatcgtgaacgtggaccagcggcagtacggcgacgtgttcaagggcgacctgaatcctaagcctcagggccagcgcctgatcgaggtgtccgtggaagagaatcaccccttcacactgagagcccctatccagagaatctacggcgtgcgctataccgagacatggtcctttctgcccagcctgacatgtaccggggatgccgctcctgccatccagcacatttgcctgaagcacaccacctgtttccaggacgtggtggtggatgtggactgcgccgagaacaccaaagaggatcagctggccgagatcagctaccggttccagggaaagaaagaggccgaccagccttggatcgtggtcaacaccagcacactgttcgacgagctggaactggaccctcctgagattgaacccggggtgctgaaggtgctgagaaccgagaagcagtacctgggagtgtacatctggaacatgagaggcagcgacggcacctctacctacgccacctttctggtcacatggaagggcgacgagaaaacacggaaccccacaccagctgtgacccctcaacctagaggcgccgagtttcacatgtggaattaccacagccacgtgttcagcgtgggcgatacctttagcctggccatgcatctgcagtacaagatccacgaggcccctttcgacctgctgctggaatggctgtacgtgcccatcgatcctacctgccagcctatgcggctgtactccacctgtctgtatcaccccaacgctccccagtgcctgagccacatgaatagcggctgcaccttcacaagccctcacctggctcagcgagtggccagcacagtgtaccagaattgcgagcacgccgacaattacaccgcctactgtctgggcatcagccacatggaacctagcttcggcctgatcctgcacgatggcggcacaaccctgaagttcgtggatacccctgagagcctgagcggcctgtatgtgttcgtggtgtacttcaacggccacgtggaagccgtggcctacaccgtggtgtctaccgtggaccacttcgtgaacgccatcgaggaaagaggcttccctccaactgctggacagcctcctgccaccaccaagcctaaagaaatcacacccgtgaatcccggcacaagcccactgcttagatacgccgcttggacaggcggactggctgctgttgttctgctgtgcctggtcatcttcctgatctgcaccgccaagcggatgcgcgtgaaggacaaagagaaggacaagtccccttacaaccagtctatgtatggcgccggactgcccgtggacgattttgaggatgctgaagccgccgacgccgaggaagaatttggcaacgccattggcggaagccacggcggcagtagctataccgtgtacatcgacaagacccggtga

SEQ ID NO: 147 - protein, 623 aa, synthetic construct
MGTVNKPVVGVLMGFGIITGTLRITNPVRASVLRYDDFHIDEDKLDTNSVYEPYYHSDHAESSWVNRGESSRKAYDHNSPYIWPRNDYDGFLENAHEHHGVYNQGRGIDSGERLMQPTQMSAQEDLGDDTGIHVIPTLNGDDRHKIVNVDQRQYGDVFKGDLNPKPQGQRLIEVSVEENHPFTLRAPIQRIYGVRYTETWSFLPSLTCTGDAAPAIQHICLKHTTCFQDVVVDVDCAENTKEDQLAEISYRFQGKKEADQPWIVVNTSTLFDELELDPPEIEPGVLKVLRTEKQYLGVYIWNMRGSDGTSTYATFLVTWKGDEKTRNPTPAVTPQPRGAEFHMWNYHSHVFSVGDTFSLAMHLQYKIHEAPFDLLLEWLYVPIDPTCQPMRLYSTCLYHPNAPQCLSHMNSGCTFTSPHLAQRVASTVYQNCEHADNYTAYCLGISHMEPSFGLILHDGGTTLKFVDTPESLSGLYVFVVYFNGHVEAVAYTVVSTVDHFVNAIEERGFPPTAGQPPATTKPKEITPVNPGTSPLLRYAAWTGGLAAVVLLCLVIFLICTAKRMRVKDKEKDKSPYNQSMYGAGLPVDDFEDAEAADAEEEFGNAIGGSHGGSSYTVYIDKTR

SEQ ID NO: 148 - RNA, 2167 nt, synthetic construct
  source 1..2167: mol_type = other RNA
agactcctccccatcctctccctctgtccctctgtccctctgaccctgcactgtcccagcaccgccaccatgggcaccgtgaacaagcctgttgtgggcgtgctgatgggcttcggcatcatcacaggcaccctgcggatcaccaatcctgtgcgggctagcgtgctgagatacgacgacttccacatcgacgaggacaagctggacaccaacagcgtgtacgagccctactaccacagcgatcacgccgagtctagctgggtcaacagaggcgagagcagcagaaaggcctacgaccacaacagcccctacatctggccccggaacgactacgatggcttcctggaaaatgcccacgagcaccacggcgtgtacaatcaaggcagaggcatcgacagcggcgagagactgatgcagcctacacagatgagcgcccaagaggacctgggagatgataccggcatccacgtgatccccacactgaacggcgacgacagacacaagatcgtgaacgtggaccagcggcagtacggcgacgtgttcaagggcgacctgaatcctaagcctcagggccagcgcctgatcgaggtgtccgtggaagagaatcaccccttcacactgagagcccctatccagagaatctacggcgtgcgctataccgagacatggtcctttctgcccagcctgacatgtaccggggatgccgctcctgccatccagcacatttgcctgaagcacaccacctgtttccaggacgtggtggtggatgtggactgcgccgagaacaccaaagaggatcagctggccgagatcagctaccggttccagggaaagaaagaggccgaccagccttggatcgtggtcaacaccagcacactgttcgacgagctggaactggaccctcctgagattgaacccggggtgctgaaggtgctgagaaccgagaagcagtacctgggagtgtacatctggaacatgagaggcagcgacggcacctctacctacgccacctttctggtcacatggaagggcgacgagaaaacacggaaccccacaccagctgtgacccctcaacctagaggcgccgagtttcacatgtggaattaccacagccacgtgttcagcgtgggcgatacctttagcctggccatgcatctgcagtacaagatccacgaggcccctttcgacctgctgctggaatggctgtacgtgcccatcgatcctacctgccagcctatgcggctgtactccacctgtctgtatcaccccaacgctccccagtgcctgagccacatgaatagcggctgcaccttcacaagccctcacctggctcagcgagtggccagcacagtgtaccagaattgcgagcacgccgacaattacaccgcctactgtctgggcatcagccacatggaacctagcttcggcctgatcctgcacgatggcggcacaaccctgaagttcgtggatacccctgagagcctgagcggcctgtatgtgttcgtggtgtacttcaacggccacgtggaagccgtggcctacaccgtggtgtctaccgtggaccacttcgtgaacgccatcgaggaaagaggcttccctccaactgctggacagcctcctgccaccaccaagcctaaagaaatcacacccgtgaatcccggcacaagcccactgcttagatacgccgcttggacaggcggactggctgctgttgttctgctgtgcctggtcatcttcctgatctgcaccgccaagcggatgcgcgtgaaggacaaagagaaggacaagtccccttacaaccagtctatgtatggcgccggactgcccgtggacgattttgaggatgctgaagccgccgacgccgaggaagaatttggcaacgccattggcggaagccacggcggcagtagctataccgtgtacatcgacaagacccggtgataataggctggagcctcggtggccatgcttcttgccccttgggcctccccccagcccctcctccccttcctgcacccgtacccccgtggtctttgaataaagtctgagtgggcggcaaaaaaaaaaaaaaaaaaaaaaaaaaaaaaaaaaaaaaaaaaaaaaaaaaaaaaaaaaaaaaaaaaaaaaaaaaaaaaaaaaaaaaaaaaaaaaaaaaaaaaaaaaaaaa

SEQ ID NO: 149 - DNA, 2167 bp, synthetic construct
  source 1..2167: mol_type = other DNA
agactcctccccatcctctccctctgtccctctgtccctctgaccctgcactgtcccagcaccgccaccatgggcaccgtgaacaagcctgttgtgggcgtgctgatgggcttcggcatcatcacaggcaccctgcggatcaccaatcctgtgcgggctagcgtgctgagatacgacgacttccacatcgacgaggacaagctggacaccaacagcgtgtacgagccctactaccacagcgatcacgccgagtctagctgggtcaacagaggcgagagcagcagaaaggcctacgaccacaacagcccctacatctggccccggaacgactacgatggcttcctggaaaatgcccacgagcaccacggcgtgtacaatcaaggcagaggcatcgacagcggcgagagactgatgcagcctacacagatgagcgcccaagaggacctgggagatgataccggcatccacgtgatccccacactgaacggcgacgacagacacaagatcgtgaacgtggaccagcggcagtacggcgacgtgttcaagggcgacctgaatcctaagcctcagggccagcgcctgatcgaggtgtccgtggaagagaatcaccccttcacactgagagcccctatccagagaatctacggcgtgcgctataccgagacatggtcctttctgcccagcctgacatgtaccggggatgccgctcctgccatccagcacatttgcctgaagcacaccacctgtttccaggacgtggtggtggatgtggactgcgccgagaacaccaaagaggatcagctggccgagatcagctaccggttccagggaaagaaagaggccgaccagccttggatcgtggtcaacaccagcacactgttcgacgagctggaactggaccctcctgagattgaacccggggtgctgaaggtgctgagaaccgagaagcagtacctgggagtgtacatctggaacatgagaggcagcgacggcacctctacctacgccacctttctggtcacatggaagggcgacgagaaaacacggaaccccacaccagctgtgacccctcaacctagaggcgccgagtttcacatgtggaattaccacagccacgtgttcagcgtgggcgatacctttagcctggccatgcatctgcagtacaagatccacgaggcccctttcgacctgctgctggaatggctgtacgtgcccatcgatcctacctgccagcctatgcggctgtactccacctgtctgtatcaccccaacgctccccagtgcctgagccacatgaatagcggctgcaccttcacaagccctcacctggctcagcgagtggccagcacagtgtaccagaattgcgagcacgccgacaattacaccgcctactgtctgggcatcagccacatggaacctagcttcggcctgatcctgcacgatggcggcacaaccctgaagttcgtggatacccctgagagcctgagcggcctgtatgtgttcgtggtgtacttcaacggccacgtggaagccgtggcctacaccgtggtgtctaccgtggaccacttcgtgaacgccatcgaggaaagaggcttccctccaactgctggacagcctcctgccaccaccaagcctaaagaaatcacacccgtgaatcccggcacaagcccactgcttagatacgccgcttggacaggcggactggctgctgttgttctgctgtgcctggtcatcttcctgatctgcaccgccaagcggatgagagtgaaggcctacagagtggacaagagcccttacaaccagtctatgtatggcgccggactgcccgtggacgattttgaggatgctgaagccgccgacgccgaggaagaatttggcaacgccattggcggaagccacggcggcagtagctataccgtgtacatcgacaagacccggtgataataggctggagcctcggtggccatgcttcttgccccttgggcctccccccagcccctcctccccttcctgcacccgtacccccgtggtctttgaataaagtctgagtgggcggcaaaaaaaaaaaaaaaaaaaaaaaaaaaaaaaaaaaaaaaaaaaaaaaaaaaaaaaaaaaaaaaaaaaaaaaaaaaaaaaaaaaaaaaaaaaaaaaaaaaaaaaaaaaaaa

SEQ ID NO: 150 - DNA, 1872 bp, synthetic construct
  source 1..1872: mol_type = other DNA
atgggcaccgtgaacaagcctgttgtgggcgtgctgatgggcttcggcatcatcacaggcaccctgcggatcaccaatcctgtgcgggctagcgtgctgagatacgacgacttccacatcgacgaggacaagctggacaccaacagcgtgtacgagccctactaccacagcgatcacgccgagtctagctgggtcaacagaggcgagagcagcagaaaggcctacgaccacaacagcccctacatctggccccggaacgactacgatggcttcctggaaaatgcccacgagcaccacggcgtgtacaatcaaggcagaggcatcgacagcggcgagagactgatgcagcctacacagatgagcgcccaagaggacctgggagatgataccggcatccacgtgatccccacactgaacggcgacgacagacacaagatcgtgaacgtggaccagcggcagtacggcgacgtgttcaagggcgacctgaatcctaagcctcagggccagcgcctgatcgaggtgtccgtggaagagaatcaccccttcacactgagagcccctatccagagaatctacggcgtgcgctataccgagacatggtcctttctgcccagcctgacatgtaccggggatgccgctcctgccatccagcacatttgcctgaagcacaccacctgtttccaggacgtggtggtggatgtggactgcgccgagaacaccaaagaggatcagctggccgagatcagctaccggttccagggaaagaaagaggccgaccagccttggatcgtggtcaacaccagcacactgttcgacgagctggaactggaccctcctgagattgaacccggggtgctgaaggtgctgagaaccgagaagcagtacctgggagtgtacatctggaacatgagaggcagcgacggcacctctacctacgccacctttctggtcacatggaagggcgacgagaaaacacggaaccccacaccagctgtgacccctcaacctagaggcgccgagtttcacatgtggaattaccacagccacgtgttcagcgtgggcgatacctttagcctggccatgcatctgcagtacaagatccacgaggcccctttcgacctgctgctggaatggctgtacgtgcccatcgatcctacctgccagcctatgcggctgtactccacctgtctgtatcaccccaacgctccccagtgcctgagccacatgaatagcggctgcaccttcacaagccctcacctggctcagcgagtggccagcacagtgtaccagaattgcgagcacgccgacaattacaccgcctactgtctgggcatcagccacatggaacctagcttcggcctgatcctgcacgatggcggcacaaccctgaagttcgtggatacccctgagagcctgagcggcctgtatgtgttcgtggtgtacttcaacggccacgtggaagccgtggcctacaccgtggtgtctaccgtggaccacttcgtgaacgccatcgaggaaagaggcttccctccaactgctggacagcctcctgccaccaccaagcctaaagaaatcacacccgtgaatcccggcacaagcccactgcttagatacgccgcttggacaggcggactggctgctgttgttctgctgtgcctggtcatcttcctgatctgcaccgccaagcggatgagagtgaaggcctacagagtggacaagagcccttacaaccagtctatgtatggcgccggactgcccgtggacgattttgaggatgctgaagccgccgacgccgaggaagaatttggcaacgccattggcggaagccacggcggcagtagctataccgtgtacatcgacaagacccggtga

SEQ ID NO: 151 - protein, 623 aa, synthetic construct
MGTVNKPVVGVLMGFGIITGTLRITNPVRASVLRYDDFHIDEDKLDTNSVYEPYYHSDHAESSWVNRGESSRKAYDHNSPYIWPRNDYDGFLENAHEHHGVYNQGRGIDSGERLMQPTQMSAQEDLGDDTGIHVIPTLNGDDRHKIVNVDQRQYGDVFKGDLNPKPQGQRLIEVSVEENHPFTLRAPIQRIYGVRYTETWSFLPSLTCTGDAAPAIQHICLKHTTCFQDVVVDVDCAENTKEDQLAEISYRFQGKKEADQPWIVVNTSTLFDELELDPPEIEPGVLKVLRTEKQYLGVYIWNMRGSDGTSTYATFLVTWKGDEKTRNPTPAVTPQPRGAEFHMWNYHSHVFSVGDTFSLAMHLQYKIHEAPFDLLLEWLYVPIDPTCQPMRLYSTCLYHPNAPQCLSHMNSGCTFTSPHLAQRVASTVYQNCEHADNYTAYCLGISHMEPSFGLILHDGGTTLKFVDTPESLSGLYVFVVYFNGHVEAVAYTVVSTVDHFVNAIEERGFPPTAGQPPATTKPKEITPVNPGTSPLLRYAAWTGGLAAVVLLCLVIFLICTAKRMRVKAYRVDKSPYNQSMYGAGLPVDDFEDAEAADAEEEFGNAIGGSHGGSSYTVYIDKTR

SEQ ID NO: 152 - RNA, 2167 nt, synthetic construct
  source 1..2167: mol_type = other RNA
agactcctccccatcctctccctctgtccctctgtccctctgaccctgcactgtcccagcaccgccaccatgggcaccgtgaacaagcctgttgtgggcgtgctgatgggcttcggcatcatcacaggcaccctgcggatcaccaatcctgtgcgggctagcgtgctgagatacgacgacttccacatcgacgaggacaagctggacaccaacagcgtgtacgagccctactaccacagcgatcacgccgagtctagctgggtcaacagaggcgagagcagcagaaaggcctacgaccacaacagcccctacatctggccccggaacgactacgatggcttcctggaaaatgcccacgagcaccacggcgtgtacaatcaaggcagaggcatcgacagcggcgagagactgatgcagcctacacagatgagcgcccaagaggacctgggagatgataccggcatccacgtgatccccacactgaacggcgacgacagacacaagatcgtgaacgtggaccagcggcagtacggcgacgtgttcaagggcgacctgaatcctaagcctcagggccagcgcctgatcgaggtgtccgtggaagagaatcaccccttcacactgagagcccctatccagagaatctacggcgtgcgctataccgagacatggtcctttctgcccagcctgacatgtaccggggatgccgctcctgccatccagcacatttgcctgaagcacaccacctgtttccaggacgtggtggtggatgtggactgcgccgagaacaccaaagaggatcagctggccgagatcagctaccggttccagggaaagaaagaggccgaccagccttggatcgtggtcaacaccagcacactgttcgacgagctggaactggaccctcctgagattgaacccggggtgctgaaggtgctgagaaccgagaagcagtacctgggagtgtacatctggaacatgagaggcagcgacggcacctctacctacgccacctttctggtcacatggaagggcgacgagaaaacacggaaccccacaccagctgtgacccctcaacctagaggcgccgagtttcacatgtggaattaccacagccacgtgttcagcgtgggcgatacctttagcctggccatgcatctgcagtacaagatccacgaggcccctttcgacctgctgctggaatggctgtacgtgcccatcgatcctacctgccagcctatgcggctgtactccacctgtctgtatcaccccaacgctccccagtgcctgagccacatgaatagcggctgcaccttcacaagccctcacctggctcagcgagtggccagcacagtgtaccagaattgcgagcacgccgacaattacaccgcctactgtctgggcatcagccacatggaacctagcttcggcctgatcctgcacgatggcggcacaaccctgaagttcgtggatacccctgagagcctgagcggcctgtatgtgttcgtggtgtacttcaacggccacgtggaagccgtggcctacaccgtggtgtctaccgtggaccacttcgtgaacgccatcgaggaaagaggcttccctccaactgctggacagcctcctgccaccaccaagcctaaagaaatcacacccgtgaatcccggcacaagcccactgcttagatacgccgcttggacaggcggactggctgctgttgttctgctgtgcctggtcatcttcctgatctgcaccgccaagcggatgagagtgaaggcctacagagtggacaagagcccttacaaccagtctatgtatggcgccggactgcccgtggacgattttgaggatgctgaagccgccgacgccgaggaagaatttggcaacgccattggcggaagccacggcggcagtagctataccgtgtacatcgacaagacccggtgataataggctggagcctcggtggccatgcttcttgccccttgggcctccccccagcccctcctccccttcctgcacccgtacccccgtggtctttgaataaagtctgagtgggcggcaaaaaaaaaaaaaaaaaaaaaaaaaaaaaaaaaaaaaaaaaaaaaaaaaaaaaaaaaaaaaaaaaaaaaaaaaaaaaaaaaaaaaaaaaaaaaaaaaaaaaaaaaaaaaa

SEQ ID NO: 153 - DNA, 2044 bp, synthetic construct
  source 1..2044: mol_type = other DNA
agactcctccccatcctctccctctgtccctctgtccctctgaccctgcactgtcccagcaccgccaccatgggcaccgtgaacaagcctgttgtgggcgtgctgatgggcttcggcatcatcacaggcaccctgcggatcaccaatcctgtgcgggctagcgtgctgagatacgacgacttccacatcgacgaggacaagctggacaccaacagcgtgtacgagccctactaccacagcgatcacgccgagtctagctgggtcaacagaggcgagagcagcagaaaggcctacgaccacaacagcccctacatctggccccggaacgactacgatggcttcctggaaaatgcccacgagcaccacggcgtgtacaatcaaggcagaggcatcgacagcggcgagagactgatgcagcctacacagatgagcgcccaagaggacctgggagatgataccggcatccacgtgatccccacactgaacggcgacgacagacacaagatcgtgaacgtggaccagcggcagtacggcgacgtgttcaagggcgacctgaatcctaagcctcagggccagcgcctgatcgaggtgtccgtggaagagaatcaccccttcacactgagagcccctatccagagaatctacggcgtgcgctataccgagacatggtcctttctgcccagcctgacatgtaccggggatgccgctcctgccatccagcacatttgcctgaagcacaccacctgtttccaggacgtggtggtggatgtggactgcgccgagaacaccaaagaggatcagctggccgagatcagctaccggttccagggaaagaaagaggccgaccagccttggatcgtggtcaacaccagcacactgttcgacgagctggaactggaccctcctgagattgaacccggggtgctgaaggtgctgagaaccgagaagcagtacctgggagtgtacatctggaacatgagaggcagcgacggcacctctacctacgccacctttctggtcacatggaagggcgacgagaaaacacggaaccccacaccagctgtgacccctcaacctagaggcgccgagtttcacatgtggaattaccacagccacgtgttcagcgtgggcgatacctttagcctggccatgcatctgcagtacaagatccacgaggcccctttcgacctgctgctggaatggctgtacgtgcccatcgatcctacctgccagcctatgcggctgtactccacctgtctgtatcaccccaacgctccccagtgcctgagccacatgaatagcggctgcaccttcacaagccctcacctggctcagcgagtggccagcacagtgtaccagaattgcgagcacgccgacaattacaccgcctactgtctgggcatcagccacatggaacctagcttcggcctgatcctgcacgatggcggcacaaccctgaagttcgtggatacccctgagagcctgagcggcctgtatgtgttcgtggtgtacttcaacggccacgtggaagccgtggcctacaccgtggtgtctaccgtggaccacttcgtgaacgccatcgaggaaagaggcttccctccaactgctggacagcctcctgccaccaccaagcctaaagaaatcacacccgtgaatcccggcacaagcccactgcttagatacgccgcttggacaggcggactggctgctgttgttctgctgtgcctggtcatcttcctgatctgcaccgccaagcggatgagagtgaaggccgacgatttcgaggacagcgagagcaccgataccgaggaagaatgataataggctggagcctcggtggccatgcttcttgccccttgggcctccccccagcccctcctccccttcctgcacccgtacccccgtggtctttgaataaagtctgagtgggcggcaaaaaaaaaaaaaaaaaaaaaaaaaaaaaaaaaaaaaaaaaaaaaaaaaaaaaaaaaaaaaaaaaaaaaaaaaaaaaaaaaaaaaaaaaaaaaaaaaaaaaaaaaaaaaa

SEQ ID NO: 154 - DNA, 1749 bp, synthetic construct
  source 1..1749: mol_type = other DNA
atgggcaccgtgaacaagcctgttgtgggcgtgctgatgggcttcggcatcatcacaggcaccctgcggatcaccaatcctgtgcgggctagcgtgctgagatacgacgacttccacatcgacgaggacaagctggacaccaacagcgtgtacgagccctactaccacagcgatcacgccgagtctagctgggtcaacagaggcgagagcagcagaaaggcctacgaccacaacagcccctacatctggccccggaacgactacgatggcttcctggaaaatgcccacgagcaccacggcgtgtacaatcaaggcagaggcatcgacagcggcgagagactgatgcagcctacacagatgagcgcccaagaggacctgggagatgataccggcatccacgtgatccccacactgaacggcgacgacagacacaagatcgtgaacgtggaccagcggcagtacggcgacgtgttcaagggcgacctgaatcctaagcctcagggccagcgcctgatcgaggtgtccgtggaagagaatcaccccttcacactgagagcccctatccagagaatctacggcgtgcgctataccgagacatggtcctttctgcccagcctgacatgtaccggggatgccgctcctgccatccagcacatttgcctgaagcacaccacctgtttccaggacgtggtggtggatgtggactgcgccgagaacaccaaagaggatcagctggccgagatcagctaccggttccagggaaagaaagaggccgaccagccttggatcgtggtcaacaccagcacactgttcgacgagctggaactggaccctcctgagattgaacccggggtgctgaaggtgctgagaaccgagaagcagtacctgggagtgtacatctggaacatgagaggcagcgacggcacctctacctacgccacctttctggtcacatggaagggcgacgagaaaacacggaaccccacaccagctgtgacccctcaacctagaggcgccgagtttcacatgtggaattaccacagccacgtgttcagcgtgggcgatacctttagcctggccatgcatctgcagtacaagatccacgaggcccctttcgacctgctgctggaatggctgtacgtgcccatcgatcctacctgccagcctatgcggctgtactccacctgtctgtatcaccccaacgctccccagtgcctgagccacatgaatagcggctgcaccttcacaagccctcacctggctcagcgagtggccagcacagtgtaccagaattgcgagcacgccgacaattacaccgcctactgtctgggcatcagccacatggaacctagcttcggcctgatcctgcacgatggcggcacaaccctgaagttcgtggatacccctgagagcctgagcggcctgtatgtgttcgtggtgtacttcaacggccacgtggaagccgtggcctacaccgtggtgtctaccgtggaccacttcgtgaacgccatcgaggaaagaggcttccctccaactgctggacagcctcctgccaccaccaagcctaaagaaatcacacccgtgaatcccggcacaagcccactgcttagatacgccgcttggacaggcggactggctgctgttgttctgctgtgcctggtcatcttcctgatctgcaccgccaagcggatgagagtgaaggccgacgatttcgaggacagcgagagcaccgataccgaggaagaatga

SEQ ID NO: 155 - protein, 582 aa, synthetic construct
MGTVNKPVVGVLMGFGIITGTLRITNPVRASVLRYDDFHIDEDKLDTNSVYEPYYHSDHAESSWVNRGESSRKAYDHNSPYIWPRNDYDGFLENAHEHHGVYNQGRGIDSGERLMQPTQMSAQEDLGDDTGIHVIPTLNGDDRHKIVNVDQRQYGDVFKGDLNPKPQGQRLIEVSVEENHPFTLRAPIQRIYGVRYTETWSFLPSLTCTGDAAPAIQHICLKHTTCFQDVVVDVDCAENTKEDQLAEISYRFQGKKEADQPWIVVNTSTLFDELELDPPEIEPGVLKVLRTEKQYLGVYIWNMRGSDGTSTYATFLVTWKGDEKTRNPTPAVTPQPRGAEFHMWNYHSHVFSVGDTFSLAMHLQYKIHEAPFDLLLEWLYVPIDPTCQPMRLYSTCLYHPNAPQCLSHMNSGCTFTSPHLAQRVASTVYQNCEHADNYTAYCLGISHMEPSFGLILHDGGTTLKFVDTPESLSGLYVFVVYFNGHVEAVAYTVVSTVDHFVNAIEERGFPPTAGQPPATTKPKEITPVNPGTSPLLRYAAWTGGLAAVVLLCLVIFLICTAKRMRVKADDFEDSESTDTEEE

SEQ ID NO: 156 - RNA, 2044 nt, synthetic construct
  source 1..2044: mol_type = other RNA
agactcctccccatcctctccctctgtccctctgtccctctgaccctgcactgtcccagcaccgccaccatgggcaccgtgaacaagcctgttgtgggcgtgctgatgggcttcggcatcatcacaggcaccctgcggatcaccaatcctgtgcgggctagcgtgctgagatacgacgacttccacatcgacgaggacaagctggacaccaacagcgtgtacgagccctactaccacagcgatcacgccgagtctagctgggtcaacagaggcgagagcagcagaaaggcctacgaccacaacagcccctacatctggccccggaacgactacgatggcttcctggaaaatgcccacgagcaccacggcgtgtacaatcaaggcagaggcatcgacagcggcgagagactgatgcagcctacacagatgagcgcccaagaggacctgggagatgataccggcatccacgtgatccccacactgaacggcgacgacagacacaagatcgtgaacgtggaccagcggcagtacggcgacgtgttcaagggcgacctgaatcctaagcctcagggccagcgcctgatcgaggtgtccgtggaagagaatcaccccttcacactgagagcccctatccagagaatctacggcgtgcgctataccgagacatggtcctttctgcccagcctgacatgtaccggggatgccgctcctgccatccagcacatttgcctgaagcacaccacctgtttccaggacgtggtggtggatgtggactgcgccgagaacaccaaagaggatcagctggccgagatcagctaccggttccagggaaagaaagaggccgaccagccttggatcgtggtcaacaccagcacactgttcgacgagctggaactggaccctcctgagattgaacccggggtgctgaaggtgctgagaaccgagaagcagtacctgggagtgtacatctggaacatgagaggcagcgacggcacctctacctacgccacctttctggtcacatggaagggcgacgagaaaacacggaaccccacaccagctgtgacccctcaacctagaggcgccgagtttcacatgtggaattaccacagccacgtgttcagcgtgggcgatacctttagcctggccatgcatctgcagtacaagatccacgaggcccctttcgacctgctgctggaatggctgtacgtgcccatcgatcctacctgccagcctatgcggctgtactccacctgtctgtatcaccccaacgctccccagtgcctgagccacatgaatagcggctgcaccttcacaagccctcacctggctcagcgagtggccagcacagtgtaccagaattgcgagcacgccgacaattacaccgcctactgtctgggcatcagccacatggaacctagcttcggcctgatcctgcacgatggcggcacaaccctgaagttcgtggatacccctgagagcctgagcggcctgtatgtgttcgtggtgtacttcaacggccacgtggaagccgtggcctacaccgtggtgtctaccgtggaccacttcgtgaacgccatcgaggaaagaggcttccctccaactgctggacagcctcctgccaccaccaagcctaaagaaatcacacccgtgaatcccggcacaagcccactgcttagatacgccgcttggacaggcggactggctgctgttgttctgctgtgcctggtcatcttcctgatctgcaccgccaagcggatgagagtgaaggccgacgatttcgaggacagcgagagcaccgataccgaggaagaatgataataggctggagcctcggtggccatgcttcttgccccttgggcctccccccagcccctcctccccttcctgcacccgtacccccgtggtctttgaataaagtctgagtgggcggcaaaaaaaaaaaaaaaaaaaaaaaaaaaaaaaaaaaaaaaaaaaaaaaaaaaaaaaaaaaaaaaaaaaaaaaaaaaaaaaaaaaaaaaaaaaaaaaaaaaaaaaaaaaaaa

SEQ ID NO: 157 - DNA, 2044 bp, synthetic construct
  source 1..2044: mol_type = other DNA
agactcctccccatcctctccctctgtccctctgtccctctgaccctgcactgtcccagcaccgccaccatgggcaccgtgaacaagcctgttgtgggcgtgctgatgggcttcggcatcatcacaggcaccctgcggatcaccaatcctgtgcgggctagcgtgctgagatacgacgacttccacatcgacgaggacaagctggacaccaacagcgtgtacgagccctactaccacagcgatcacgccgagtctagctgggtcaacagaggcgagagcagcagaaaggcctacgaccacaacagcccctacatctggccccggaacgactacgatggcttcctggaaaatgcccacgagcaccacggcgtgtacaatcaaggcagaggcatcgacagcggcgagagactgatgcagcctacacagatgagcgcccaagaggacctgggagatgataccggcatccacgtgatccccacactgaacggcgacgacagacacaagatcgtgaacgtggaccagcggcagtacggcgacgtgttcaagggcgacctgaatcctaagcctcagggccagcgcctgatcgaggtgtccgtggaagagaatcaccccttcacactgagagcccctatccagagaatctacggcgtgcgctataccgagacatggtcctttctgcccagcctgacatgtaccggggatgccgctcctgccatccagcacatttgcctgaagcacaccacctgtttccaggacgtggtggtggatgtggactgcgccgagaacaccaaagaggatcagctggccgagatcagctaccggttccagggaaagaaagaggccgaccagccttggatcgtggtcaacaccagcacactgttcgacgagctggaactggaccctcctgagattgaacccggggtgctgaaggtgctgagaaccgagaagcagtacctgggagtgtacatctggaacatgagaggcagcgacggcacctctacctacgccacctttctggtcacatggaagggcgacgagaaaacacggaaccccacaccagctgtgacccctcaacctagaggcgccgagtttcacatgtggaattaccacagccacgtgttcagcgtgggcgatacctttagcctggccatgcatctgcagtacaagatccacgaggcccctttcgacctgctgctggaatggctgtacgtgcccatcgatcctacctgccagcctatgcggctgtactccacctgtctgtatcaccccaacgctccccagtgcctgagccacatgaatagcggctgcaccttcacaagccctcacctggctcagcgagtggccagcacagtgtaccagaattgcgagcacgccgacaattacaccgcctactgtctgggcatcagccacatggaacctagcttcggcctgatcctgcacgatggcggcacaaccctgaagttcgtggatacccctgagagcctgagcggcctgtatgtgttcgtggtgtacttcaacggccacgtggaagccgtggcctacaccgtggtgtctaccgtggaccacttcgtgaacgccatcgaggaaagaggcttccctccaactgctggacagcctcctgccaccaccaagcctaaagaaatcacacccgtgaatcccggcacaagcccactgcttagatacgccgcttggacaggcggactggctgctgttgttctgctgtgcctggtcatcttcctgatctgcaccgccaagcggatgagagtgaaggccgacgatttcgaggatgccgaggccgccgatgctgaggaagaatgataataggctggagcctcggtggccatgcttcttgccccttgggcctccccccagcccctcctccccttcctgcacccgtacccccgtggtctttgaataaagtctgagtgggcggcaaaaaaaaaaaaaaaaaaaaaaaaaaaaaaaaaaaaaaaaaaaaaaaaaaaaaaaaaaaaaaaaaaaaaaaaaaaaaaaaaaaaaaaaaaaaaaaaaaaaaaaaaaaaaa

SEQ ID NO: 158 - DNA, 1749 bp, synthetic construct
  source 1..1749: mol_type = other DNA
atgggcaccgtgaacaagcctgttgtgggcgtgctgatgggcttcggcatcatcacaggcaccctgcggatcaccaatcctgtgcgggctagcgtgctgagatacgacgacttccacatcgacgaggacaagctggacaccaacagcgtgtacgagccctactaccacagcgatcacgccgagtctagctgggtcaacagaggcgagagcagcagaaaggcctacgaccacaacagcccctacatctggccccggaacgactacgatggcttcctggaaaatgcccacgagcaccacggcgtgtacaatcaaggcagaggcatcgacagcggcgagagactgatgcagcctacacagatgagcgcccaagaggacctgggagatgataccggcatccacgtgatccccacactgaacggcgacgacagacacaagatcgtgaacgtggaccagcggcagtacggcgacgtgttcaagggcgacctgaatcctaagcctcagggccagcgcctgatcgaggtgtccgtggaagagaatcaccccttcacactgagagcccctatccagagaatctacggcgtgcgctataccgagacatggtcctttctgcccagcctgacatgtaccggggatgccgctcctgccatccagcacatttgcctgaagcacaccacctgtttccaggacgtggtggtggatgtggactgcgccgagaacaccaaagaggatcagctggccgagatcagctaccggttccagggaaagaaagaggccgaccagccttggatcgtggtcaacaccagcacactgttcgacgagctggaactggaccctcctgagattgaacccggggtgctgaaggtgctgagaaccgagaagcagtacctgggagtgtacatctggaacatgagaggcagcgacggcacctctacctacgccacctttctggtcacatggaagggcgacgagaaaacacggaaccccacaccagctgtgacccctcaacctagaggcgccgagtttcacatgtggaattaccacagccacgtgttcagcgtgggcgatacctttagcctggccatgcatctgcagtacaagatccacgaggcccctttcgacctgctgctggaatggctgtacgtgcccatcgatcctacctgccagcctatgcggctgtactccacctgtctgtatcaccccaacgctccccagtgcctgagccacatgaatagcggctgcaccttcacaagccctcacctggctcagcgagtggccagcacagtgtaccagaattgcgagcacgccgacaattacaccgcctactgtctgggcatcagccacatggaacctagcttcggcctgatcctgcacgatggcggcacaaccctgaagttcgtggatacccctgagagcctgagcggcctgtatgtgttcgtggtgtacttcaacggccacgtggaagccgtggcctacaccgtggtgtctaccgtggaccacttcgtgaacgccatcgaggaaagaggcttccctccaactgctggacagcctcctgccaccaccaagcctaaagaaatcacacccgtgaatcccggcacaagcccactgcttagatacgccgcttggacaggcggactggctgctgttgttctgctgtgcctggtcatcttcctgatctgcaccgccaagcggatgagagtgaaggccgacgatttcgaggatgccgaggccgccgatgctgaggaagaatga

SEQ ID NO: 159 - protein, 582 aa, synthetic construct
MGTVNKPVVGVLMGFGIITGTLRITNPVRASVLRYDDFHIDEDKLDTNSVYEPYYHSDHAESSWVNRGESSRKAYDHNSPYIWPRNDYDGFLENAHEHHGVYNQGRGIDSGERLMQPTQMSAQEDLGDDTGIHVIPTLNGDDRHKIVNVDQRQYGDVFKGDLNPKPQGQRLIEVSVEENHPFTLRAPIQRIYGVRYTETWSFLPSLTCTGDAAPAIQHICLKHTTCFQDVVVDVDCAENTKEDQLAEISYRFQGKKEADQPWIVVNTSTLFDELELDPPEIEPGVLKVLRTEKQYLGVYIWNMRGSDGTSTYATFLVTWKGDEKTRNPTPAVTPQPRGAEFHMWNYHSHVFSVGDTFSLAMHLQYKIHEAPFDLLLEWLYVPIDPTCQPMRLYSTCLYHPNAPQCLSHMNSGCTFTSPHLAQRVASTVYQNCEHADNYTAYCLGISHMEPSFGLILHDGGTTLKFVDTPESLSGLYVFVVYFNGHVEAVAYTVVSTVDHFVNAIEERGFPPTAGQPPATTKPKEITPVNPGTSPLLRYAAWTGGLAAVVLLCLVIFLICTAKRMRVKADDFEDAEAADAEEE

SEQ ID NO: 160 - RNA, 2044 nt, synthetic construct
  source 1..2044: mol_type = other RNA
agactcctccccatcctctccctctgtccctctgtccctctgaccctgcactgtcccagcaccgccaccatgggcaccgtgaacaagcctgttgtgggcgtgctgatgggcttcggcatcatcacaggcaccctgcggatcaccaatcctgtgcgggctagcgtgctgagatacgacgacttccacatcgacgaggacaagctggacaccaacagcgtgtacgagccctactaccacagcgatcacgccgagtctagctgggtcaacagaggcgagagcagcagaaaggcctacgaccacaacagcccctacatctggccccggaacgactacgatggcttcctggaaaatgcccacgagcaccacggcgtgtacaatcaaggcagaggcatcgacagcggcgagagactgatgcagcctacacagatgagcgcccaagaggacctgggagatgataccggcatccacgtgatccccacactgaacggcgacgacagacacaagatcgtgaacgtggaccagcggcagtacggcgacgtgttcaagggcgacctgaatcctaagcctcagggccagcgcctgatcgaggtgtccgtggaagagaatcaccccttcacactgagagcccctatccagagaatctacggcgtgcgctataccgagacatggtcctttctgcccagcctgacatgtaccggggatgccgctcctgccatccagcacatttgcctgaagcacaccacctgtttccaggacgtggtggtggatgtggactgcgccgagaacaccaaagaggatcagctggccgagatcagctaccggttccagggaaagaaagaggccgaccagccttggatcgtggtcaacaccagcacactgttcgacgagctggaactggaccctcctgagattgaacccggggtgctgaaggtgctgagaaccgagaagcagtacctgggagtgtacatctggaacatgagaggcagcgacggcacctctacctacgccacctttctggtcacatggaagggcgacgagaaaacacggaaccccacaccagctgtgacccctcaacctagaggcgccgagtttcacatgtggaattaccacagccacgtgttcagcgtgggcgatacctttagcctggccatgcatctgcagtacaagatccacgaggcccctttcgacctgctgctggaatggctgtacgtgcccatcgatcctacctgccagcctatgcggctgtactccacctgtctgtatcaccccaacgctccccagtgcctgagccacatgaatagcggctgcaccttcacaagccctcacctggctcagcgagtggccagcacagtgtaccagaattgcgagcacgccgacaattacaccgcctactgtctgggcatcagccacatggaacctagcttcggcctgatcctgcacgatggcggcacaaccctgaagttcgtggatacccctgagagcctgagcggcctgtatgtgttcgtggtgtacttcaacggccacgtggaagccgtggcctacaccgtggtgtctaccgtggaccacttcgtgaacgccatcgaggaaagaggcttccctccaactgctggacagcctcctgccaccaccaagcctaaagaaatcacacccgtgaatcccggcacaagcccactgcttagatacgccgcttggacaggcggactggctgctgttgttctgctgtgcctggtcatcttcctgatctgcaccgccaagcggatgagagtgaaggccgacgatttcgaggatgccgaggccgccgatgctgaggaagaatgataataggctggagcctcggtggccatgcttcttgccccttgggcctccccccagcccctcctccccttcctgcacccgtacccccgtggtctttgaataaagtctgagtgggcggcaaaaaaaaaaaaaaaaaaaaaaaaaaaaaaaaaaaaaaaaaaaaaaaaaaaaaaaaaaaaaaaaaaaaaaaaaaaaaaaaaaaaaaaaaaaaaaaaaaaaaaaaaaaaaa

SEQ ID NO: 161 - DNA, 2110 bp, synthetic construct
  source 1..2110: mol_type = other DNA
agactcctccccatcctctccctctgtccctctgtccctctgaccctgcactgtcccagcaccgccaccatgggcaccgtgaacaagcctgttgtgggcgtgctgatgggcttcggcatcatcacaggcaccctgcggatcaccaatcctgtgcgggctagcgtgctgagatacgacgacttccacatcgacgaggacaagctggacaccaacagcgtgtacgagccctactaccacagcgatcacgccgagtctagctgggtcaacagaggcgagagcagcagaaaggcctacgaccacaacagcccctacatctggccccggaacgactacgatggcttcctggaaaatgcccacgagcaccacggcgtgtacaatcaaggcagaggcatcgacagcggcgagagactgatgcagcctacacagatgagcgcccaagaggacctgggagatgataccggcatccacgtgatccccacactgaacggcgacgacagacacaagatcgtgaacgtggaccagcggcagtacggcgacgtgttcaagggcgacctgaatcctaagcctcagggccagcgcctgatcgaggtgtccgtggaagagaatcaccccttcacactgagagcccctatccagagaatctacggcgtgcgctataccgagacatggtcctttctgcccagcctgacatgtaccggggatgccgctcctgccatccagcacatttgcctgaagcacaccacctgtttccaggacgtggtggtggatgtggactgcgccgagaacaccaaagaggatcagctggccgagatcagctaccggttccagggaaagaaagaggccgaccagccttggatcgtggtcaacaccagcacactgttcgacgagctggaactggaccctcctgagattgaacccggggtgctgaaggtgctgagaaccgagaagcagtacctgggagtgtacatctggaacatgagaggcagcgacggcacctctacctacgccacctttctggtcacatggaagggcgacgagaaaacacggaaccccacaccagctgtgacccctcaacctagaggcgccgagtttcacatgtggaattaccacagccacgtgttcagcgtgggcgatacctttagcctggccatgcatctgcagtacaagatccacgaggcccctttcgacctgctgctggaatggctgtacgtgcccatcgatcctacctgccagcctatgcggctgtactccacctgtctgtatcaccccaacgctccccagtgcctgagccacatgaatagcggctgcaccttcacaagccctcacctggctcagcgagtggccagcacagtgtaccagaattgcgagcacgccgacaattacaccgcctactgtctgggcatcagccacatggaacctagcttcggcctgatcctgcacgatggcggcacaaccctgaagttcgtggatacccctgagagcctgagcggcctgtatgtgttcgtggtgtacttcaacggccacgtggaagccgtggcctacaccgtggtgtctaccgtggaccacttcgtgaacgccatcgaggaaagaggcttccctccaactgctggacagcctcctgccaccaccaagcctaaagaaatcacacccgtgaatcccggcacaagcccactgcttagatacgccgcttggacaggcggactggctgctgttgttctgctgtgcctggtcatcttcctgatctgcaccgccaagcggatgagagtgaaggccgacgatttcgaggacagcgagagcaccgataccgaggaagagttcggcaacgccattggcggatctcacggcggcagcagctataccgtgtacatcgacaagacccggtgataataggctggagcctcggtggccatgcttcttgccccttgggcctccccccagcccctcctccccttcctgcacccgtacccccgtggtctttgaataaagtctgagtgggcggcaaaaaaaaaaaaaaaaaaaaaaaaaaaaaaaaaaaaaaaaaaaaaaaaaaaaaaaaaaaaaaaaaaaaaaaaaaaaaaaaaaaaaaaaaaaaaaaaaaaaaaaaaaaaaa

SEQ ID NO: 162 - DNA, 1815 bp, synthetic construct
  source 1..1815: mol_type = other DNA
atgggcaccgtgaacaagcctgttgtgggcgtgctgatgggcttcggcatcatcacaggcaccctgcggatcaccaatcctgtgcgggctagcgtgctgagatacgacgacttccacatcgacgaggacaagctggacaccaacagcgtgtacgagccctactaccacagcgatcacgccgagtctagctgggtcaacagaggcgagagcagcagaaaggcctacgaccacaacagcccctacatctggccccggaacgactacgatggcttcctggaaaatgcccacgagcaccacggcgtgtacaatcaaggcagaggcatcgacagcggcgagagactgatgcagcctacacagatgagcgcccaagaggacctgggagatgataccggcatccacgtgatccccacactgaacggcgacgacagacacaagatcgtgaacgtggaccagcggcagtacggcgacgtgttcaagggcgacctgaatcctaagcctcagggccagcgcctgatcgaggtgtccgtggaagagaatcaccccttcacactgagagcccctatccagagaatctacggcgtgcgctataccgagacatggtcctttctgcccagcctgacatgtaccggggatgccgctcctgccatccagcacatttgcctgaagcacaccacctgtttccaggacgtggtggtggatgtggactgcgccgagaacaccaaagaggatcagctggccgagatcagctaccggttccagggaaagaaagaggccgaccagccttggatcgtggtcaacaccagcacactgttcgacgagctggaactggaccctcctgagattgaacccggggtgctgaaggtgctgagaaccgagaagcagtacctgggagtgtacatctggaacatgagaggcagcgacggcacctctacctacgccacctttctggtcacatggaagggcgacgagaaaacacggaaccccacaccagctgtgacccctcaacctagaggcgccgagtttcacatgtggaattaccacagccacgtgttcagcgtgggcgatacctttagcctggccatgcatctgcagtacaagatccacgaggcccctttcgacctgctgctggaatggctgtacgtgcccatcgatcctacctgccagcctatgcggctgtactccacctgtctgtatcaccccaacgctccccagtgcctgagccacatgaatagcggctgcaccttcacaagccctcacctggctcagcgagtggccagcacagtgtaccagaattgcgagcacgccgacaattacaccgcctactgtctgggcatcagccacatggaacctagcttcggcctgatcctgcacgatggcggcacaaccctgaagttcgtggatacccctgagagcctgagcggcctgtatgtgttcgtggtgtacttcaacggccacgtggaagccgtggcctacaccgtggtgtctaccgtggaccacttcgtgaacgccatcgaggaaagaggcttccctccaactgctggacagcctcctgccaccaccaagcctaaagaaatcacacccgtgaatcccggcacaagcccactgcttagatacgccgcttggacaggcggactggctgctgttgttctgctgtgcctggtcatcttcctgatctgcaccgccaagcggatgagagtgaaggccgacgatttcgaggacagcgagagcaccgataccgaggaagagttcggcaacgccattggcggatctcacggcggcagcagctataccgtgtacatcgacaagacccggtga

SEQ ID NO: 163 - protein, 604 aa, synthetic construct
MGTVNKPVVGVLMGFGIITGTLRITNPVRASVLRYDDFHIDEDKLDTNSVYEPYYHSDHAESSWVNRGESSRKAYDHNSPYIWPRNDYDGFLENAHEHHGVYNQGRGIDSGERLMQPTQMSAQEDLGDDTGIHVIPTLNGDDRHKIVNVDQRQYGDVFKGDLNPKPQGQRLIEVSVEENHPFTLRAPIQRIYGVRYTETWSFLPSLTCTGDAAPAIQHICLKHTTCFQDVVVDVDCAENTKEDQLAEISYRFQGKKEADQPWIVVNTSTLFDELELDPPEIEPGVLKVLRTEKQYLGVYIWNMRGSDGTSTYATFLVTWKGDEKTRNPTPAVTPQPRGAEFHMWNYHSHVFSVGDTFSLAMHLQYKIHEAPFDLLLEWLYVPIDPTCQPMRLYSTCLYHPNAPQCLSHMNSGCTFTSPHLAQRVASTVYQNCEHADNYTAYCLGISHMEPSFGLILHDGGTTLKFVDTPESLSGLYVFVVYFNGHVEAVAYTVVSTVDHFVNAIEERGFPPTAGQPPATTKPKEITPVNPGTSPLLRYAAWTGGLAAVVLLCLVIFLICTAKRMRVKADDFEDSESTDTEEEFGNAIGGSHGGSSYTVYIDKTR

SEQ ID NO: 164 - RNA, 2110 nt, synthetic construct
  source 1..2110: mol_type = other RNA
agactcctccccatcctctccctctgtccctctgtccctctgaccctgcactgtcccagcaccgccaccatgggcaccgtgaacaagcctgttgtgggcgtgctgatgggcttcggcatcatcacaggcaccctgcggatcaccaatcctgtgcgggctagcgtgctgagatacgacgacttccacatcgacgaggacaagctggacaccaacagcgtgtacgagccctactaccacagcgatcacgccgagtctagctgggtcaacagaggcgagagcagcagaaaggcctacgaccacaacagcccctacatctggccccggaacgactacgatggcttcctggaaaatgcccacgagcaccacggcgtgtacaatcaaggcagaggcatcgacagcggcgagagactgatgcagcctacacagatgagcgcccaagaggacctgggagatgataccggcatccacgtgatccccacactgaacggcgacgacagacacaagatcgtgaacgtggaccagcggcagtacggcgacgtgttcaagggcgacctgaatcctaagcctcagggccagcgcctgatcgaggtgtccgtggaagagaatcaccccttcacactgagagcccctatccagagaatctacggcgtgcgctataccgagacatggtcctttctgcccagcctgacatgtaccggggatgccgctcctgccatccagcacatttgcctgaagcacaccacctgtttccaggacgtggtggtggatgtggactgcgccgagaacaccaaagaggatcagctggccgagatcagctaccggttccagggaaagaaagaggccgaccagccttggatcgtggtcaacaccagcacactgttcgacgagctggaactggaccctcctgagattgaacccggggtgctgaaggtgctgagaaccgagaagcagtacctgggagtgtacatctggaacatgagaggcagcgacggcacctctacctacgccacctttctggtcacatggaagggcgacgagaaaacacggaaccccacaccagctgtgacccctcaacctagaggcgccgagtttcacatgtggaattaccacagccacgtgttcagcgtgggcgatacctttagcctggccatgcatctgcagtacaagatccacgaggcccctttcgacctgctgctggaatggctgtacgtgcccatcgatcctacctgccagcctatgcggctgtactccacctgtctgtatcaccccaacgctccccagtgcctgagccacatgaatagcggctgcaccttcacaagccctcacctggctcagcgagtggccagcacagtgtaccagaattgcgagcacgccgacaattacaccgcctactgtctgggcatcagccacatggaacctagcttcggcctgatcctgcacgatggcggcacaaccctgaagttcgtggatacccctgagagcctgagcggcctgtatgtgttcgtggtgtacttcaacggccacgtggaagccgtggcctacaccgtggtgtctaccgtggaccacttcgtgaacgccatcgaggaaagaggcttccctccaactgctggacagcctcctgccaccaccaagcctaaagaaatcacacccgtgaatcccggcacaagcccactgcttagatacgccgcttggacaggcggactggctgctgttgttctgctgtgcctggtcatcttcctgatctgcaccgccaagcggatgagagtgaaggccgacgatttcgaggacagcgagagcaccgataccgaggaagagttcggcaacgccattggcggatctcacggcggcagcagctataccgtgtacatcgacaagacccggtgataataggctggagcctcggtggccatgcttcttgccccttgggcctccccccagcccctcctccccttcctgcacccgtacccccgtggtctttgaataaagtctgagtgggcggcaaaaaaaaaaaaaaaaaaaaaaaaaaaaaaaaaaaaaaaaaaaaaaaaaaaaaaaaaaaaaaaaaaaaaaaaaaaaaaaaaaaaaaaaaaaaaaaaaaaaaaaaaaaaaa

SEQ ID NO: 165 - DNA, 2110 bp, synthetic construct
  source 1..2110: mol_type = other DNA
agactcctccccatcctctccctctgtccctctgtccctctgaccctgcactgtcccagcaccgccaccatgggcaccgtgaacaagcctgttgtgggcgtgctgatgggcttcggcatcatcacaggcaccctgcggatcaccaatcctgtgcgggctagcgtgctgagatacgacgacttccacatcgacgaggacaagctggacaccaacagcgtgtacgagccctactaccacagcgatcacgccgagtctagctgggtcaacagaggcgagagcagcagaaaggcctacgaccacaacagcccctacatctggccccggaacgactacgatggcttcctggaaaatgcccacgagcaccacggcgtgtacaatcaaggcagaggcatcgacagcggcgagagactgatgcagcctacacagatgagcgcccaagaggacctgggagatgataccggcatccacgtgatccccacactgaacggcgacgacagacacaagatcgtgaacgtggaccagcggcagtacggcgacgtgttcaagggcgacctgaatcctaagcctcagggccagcgcctgatcgaggtgtccgtggaagagaatcaccccttcacactgagagcccctatccagagaatctacggcgtgcgctataccgagacatggtcctttctgcccagcctgacatgtaccggggatgccgctcctgccatccagcacatttgcctgaagcacaccacctgtttccaggacgtggtggtggatgtggactgcgccgagaacaccaaagaggatcagctggccgagatcagctaccggttccagggaaagaaagaggccgaccagccttggatcgtggtcaacaccagcacactgttcgacgagctggaactggaccctcctgagattgaacccggggtgctgaaggtgctgagaaccgagaagcagtacctgggagtgtacatctggaacatgagaggcagcgacggcacctctacctacgccacctttctggtcacatggaagggcgacgagaaaacacggaaccccacaccagctgtgacccctcaacctagaggcgccgagtttcacatgtggaattaccacagccacgtgttcagcgtgggcgatacctttagcctggccatgcatctgcagtacaagatccacgaggcccctttcgacctgctgctggaatggctgtacgtgcccatcgatcctacctgccagcctatgcggctgtactccacctgtctgtatcaccccaacgctccccagtgcctgagccacatgaatagcggctgcaccttcacaagccctcacctggctcagcgagtggccagcacagtgtaccagaattgcgagcacgccgacaattacaccgcctactgtctgggcatcagccacatggaacctagcttcggcctgatcctgcacgatggcggcacaaccctgaagttcgtggatacccctgagagcctgagcggcctgtatgtgttcgtggtgtacttcaacggccacgtggaagccgtggcctacaccgtggtgtctaccgtggaccacttcgtgaacgccatcgaggaaagaggcttccctccaactgctggacagcctcctgccaccaccaagcctaaagaaatcacacccgtgaatcccggcacaagcccactgcttagatacgccgcttggacaggcggactggctgctgttgttctgctgtgcctggtcatcttcctgatctgcaccgccaagcggatgagagtgaaggccgacgatttcgaggatgccgaggccgccgatgctgaggaagaatttggcaacgccattggcggctctcacggcggcagtagctataccgtgtacatcgacaagacccggtgataataggctggagcctcggtggccatgcttcttgccccttgggcctccccccagcccctcctccccttcctgcacccgtacccccgtggtctttgaataaagtctgagtgggcggcaaaaaaaaaaaaaaaaaaaaaaaaaaaaaaaaaaaaaaaaaaaaaaaaaaaaaaaaaaaaaaaaaaaaaaaaaaaaaaaaaaaaaaaaaaaaaaaaaaaaaaaaaaaaaa

SEQ ID NO: 166 - DNA, 1815 bp, synthetic construct
  source 1..1815: mol_type = other DNA
atgggcaccgtgaacaagcctgttgtgggcgtgctgatgggcttcggcatcatcacaggcaccctgcggatcaccaatcctgtgcgggctagcgtgctgagatacgacgacttccacatcgacgaggacaagctggacaccaacagcgtgtacgagccctactaccacagcgatcacgccgagtctagctgggtcaacagaggcgagagcagcagaaaggcctacgaccacaacagcccctacatctggccccggaacgactacgatggcttcctggaaaatgcccacgagcaccacggcgtgtacaatcaaggcagaggcatcgacagcggcgagagactgatgcagcctacacagatgagcgcccaagaggacctgggagatgataccggcatccacgtgatccccacactgaacggcgacgacagacacaagatcgtgaacgtggaccagcggcagtacggcgacgtgttcaagggcgacctgaatcctaagcctcagggccagcgcctgatcgaggtgtccgtggaagagaatcaccccttcacactgagagcccctatccagagaatctacggcgtgcgctataccgagacatggtcctttctgcccagcctgacatgtaccggggatgccgctcctgccatccagcacatttgcctgaagcacaccacctgtttccaggacgtggtggtggatgtggactgcgccgagaacaccaaagaggatcagctggccgagatcagctaccggttccagggaaagaaagaggccgaccagccttggatcgtggtcaacaccagcacactgttcgacgagctggaactggaccctcctgagattgaacccggggtgctgaaggtgctgagaaccgagaagcagtacctgggagtgtacatctggaacatgagaggcagcgacggcacctctacctacgccacctttctggtcacatggaagggcgacgagaaaacacggaaccccacaccagctgtgacccctcaacctagaggcgccgagtttcacatgtggaattaccacagccacgtgttcagcgtgggcgatacctttagcctggccatgcatctgcagtacaagatccacgaggcccctttcgacctgctgctggaatggctgtacgtgcccatcgatcctacctgccagcctatgcggctgtactccacctgtctgtatcaccccaacgctccccagtgcctgagccacatgaatagcggctgcaccttcacaagccctcacctggctcagcgagtggccagcacagtgtaccagaattgcgagcacgccgacaattacaccgcctactgtctgggcatcagccacatggaacctagcttcggcctgatcctgcacgatggcggcacaaccctgaagttcgtggatacccctgagagcctgagcggcctgtatgtgttcgtggtgtacttcaacggccacgtggaagccgtggcctacaccgtggtgtctaccgtggaccacttcgtgaacgccatcgaggaaagaggcttccctccaactgctggacagcctcctgccaccaccaagcctaaagaaatcacacccgtgaatcccggcacaagcccactgcttagatacgccgcttggacaggcggactggctgctgttgttctgctgtgcctggtcatcttcctgatctgcaccgccaagcggatgagagtgaaggccgacgatttcgaggatgccgaggccgccgatgctgaggaagaatttggcaacgccattggcggctctcacggcggcagtagctataccgtgtacatcgacaagacccggtga

SEQ ID NO: 167 - protein, 604 aa, synthetic construct
MGTVNKPVVGVLMGFGIITGTLRITNPVRASVLRYDDFHIDEDKLDTNSVYEPYYHSDHAESSWVNRGESSRKAYDHNSPYIWPRNDYDGFLENAHEHHGVYNQGRGIDSGERLMQPTQMSAQEDLGDDTGIHVIPTLNGDDRHKIVNVDQRQYGDVFKGDLNPKPQGQRLIEVSVEENHPFTLRAPIQRIYGVRYTETWSFLPSLTCTGDAAPAIQHICLKHTTCFQDVVVDVDCAENTKEDQLAEISYRFQGKKEADQPWIVVNTSTLFDELELDPPEIEPGVLKVLRTEKQYLGVYIWNMRGSDGTSTYATFLVTWKGDEKTRNPTPAVTPQPRGAEFHMWNYHSHVFSVGDTFSLAMHLQYKIHEAPFDLLLEWLYVPIDPTCQPMRLYSTCLYHPNAPQCLSHMNSGCTFTSPHLAQRVASTVYQNCEHADNYTAYCLGISHMEPSFGLILHDGGTTLKFVDTPESLSGLYVFVVYFNGHVEAVAYTVVSTVDHFVNAIEERGFPPTAGQPPATTKPKEITPVNPGTSPLLRYAAWTGGLAAVVLLCLVIFLICTAKRMRVKADDFEDAEAADAEEEFGNAIGGSHGGSSYTVYIDKTR

SEQ ID NO: 168 - RNA, 2110 nt, synthetic construct
  source 1..2110: mol_type = other RNA
agactcctccccatcctctccctctgtccctctgtccctctgaccctgcactgtcccagcaccgccaccatgggcaccgtgaacaagcctgttgtgggcgtgctgatgggcttcggcatcatcacaggcaccctgcggatcaccaatcctgtgcgggctagcgtgctgagatacgacgacttccacatcgacgaggacaagctggacaccaacagcgtgtacgagccctactaccacagcgatcacgccgagtctagctgggtcaacagaggcgagagcagcagaaaggcctacgaccacaacagcccctacatctggccccggaacgactacgatggcttcctggaaaatgcccacgagcaccacggcgtgtacaatcaaggcagaggcatcgacagcggcgagagactgatgcagcctacacagatgagcgcccaagaggacctgggagatgataccggcatccacgtgatccccacactgaacggcgacgacagacacaagatcgtgaacgtggaccagcggcagtacggcgacgtgttcaagggcgacctgaatcctaagcctcagggccagcgcctgatcgaggtgtccgtggaagagaatcaccccttcacactgagagcccctatccagagaatctacggcgtgcgctataccgagacatggtcctttctgcccagcctgacatgtaccggggatgccgctcctgccatccagcacatttgcctgaagcacaccacctgtttccaggacgtggtggtggatgtggactgcgccgagaacaccaaagaggatcagctggccgagatcagctaccggttccagggaaagaaagaggccgaccagccttggatcgtggtcaacaccagcacactgttcgacgagctggaactggaccctcctgagattgaacccggggtgctgaaggtgctgagaaccgagaagcagtacctgggagtgtacatctggaacatgagaggcagcgacggcacctctacctacgccacctttctggtcacatggaagggcgacgagaaaacacggaaccccacaccagctgtgacccctcaacctagaggcgccgagtttcacatgtggaattaccacagccacgtgttcagcgtgggcgatacctttagcctggccatgcatctgcagtacaagatccacgaggcccctttcgacctgctgctggaatggctgtacgtgcccatcgatcctacctgccagcctatgcggctgtactccacctgtctgtatcaccccaacgctccccagtgcctgagccacatgaatagcggctgcaccttcacaagccctcacctggctcagcgagtggccagcacagtgtaccagaattgcgagcacgccgacaattacaccgcctactgtctgggcatcagccacatggaacctagcttcggcctgatcctgcacgatggcggcacaaccctgaagttcgtggatacccctgagagcctgagcggcctgtatgtgttcgtggtgtacttcaacggccacgtggaagccgtggcctacaccgtggtgtctaccgtggaccacttcgtgaacgccatcgaggaaagaggcttccctccaactgctggacagcctcctgccaccaccaagcctaaagaaatcacacccgtgaatcccggcacaagcccactgcttagatacgccgcttggacaggcggactggctgctgttgttctgctgtgcctggtcatcttcctgatctgcaccgccaagcggatgagagtgaaggccgacgatttcgaggatgccgaggccgccgatgctgaggaagaatttggcaacgccattggcggctctcacggcggcagtagctataccgtgtacatcgacaagacccggtgataataggctggagcctcggtggccatgcttcttgccccttgggcctccccccagcccctcctccccttcctgcacccgtacccccgtggtctttgaataaagtctgagtgggcggcaaaaaaaaaaaaaaaaaaaaaaaaaaaaaaaaaaaaaaaaaaaaaaaaaaaaaaaaaaaaaaaaaaaaaaaaaaaaaaaaaaaaaaaaaaaaaaaaaaaaaaaaaaaaaa

SEQ ID NO: 169 - DNA, 2161 bp, synthetic construct
  source 1..2161: mol_type = other DNA
agactcctccccatcctctccctctgtccctctgtccctctgaccctgcactgtcccagcaccgccaccatgggcaccgtgaacaagcctgttgtgggcgtgctgatgggcttcggcatcatcacaggcaccctgcggatcaccaatcctgtgcgggctagcgtgctgagatacgacgacttccacatcgacgaggacaagctggacaccaacagcgtgtacgagccctactaccacagcgatcacgccgagtctagctgggtcaacagaggcgagagcagcagaaaggcctacgaccacaacagcccctacatctggccccggaacgactacgatggcttcctggaaaatgcccacgagcaccacggcgtgtacaatcaaggcagaggcatcgacagcggcgagagactgatgcagcctacacagatgagcgcccaagaggacctgggagatgataccggcatccacgtgatccccacactgaacggcgacgacagacacaagatcgtgaacgtggaccagcggcagtacggcgacgtgttcaagggcgacctgaatcctaagcctcagggccagcgcctgatcgaggtgtccgtggaagagaatcaccccttcacactgagagcccctatccagagaatctacggcgtgcgctataccgagacatggtcctttctgcccagcctgacatgtaccggggatgccgctcctgccatccagcacatttgcctgaagcacaccacctgtttccaggacgtggtggtggatgtggactgcgccgagaacaccaaagaggatcagctggccgagatcagctaccggttccagggaaagaaagaggccgaccagccttggatcgtggtcaacaccagcacactgttcgacgagctggaactggaccctcctgagattgaacccggggtgctgaaggtgctgagaaccgagaagcagtacctgggagtgtacatctggaacatgagaggcagcgacggcacctctacctacgccacctttctggtcacatggaagggcgacgagaaaacacggaaccccacaccagctgtgacccctcaacctagaggcgccgagtttcacatgtggaattaccacagccacgtgttcagcgtgggcgatacctttagcctggccatgcatctgcagtacaagatccacgaggcccctttcgacctgctgctggaatggctgtacgtgcccatcgatcctacctgccagcctatgcggctgtactccacctgtctgtatcaccccaacgctccccagtgcctgagccacatgaatagcggctgcaccttcacaagccctcacctggctcagcgagtggccagcacagtgtaccagaattgcgagcacgccgacaattacaccgcctactgtctgggcatcagccacatggaacctagcttcggcctgatcctgcacgatggcggcacaaccctgaagttcgtggatacccctgagagcctgagcggcctgtatgtgttcgtggtgtacttcaacggccacgtggaagccgtggcctacaccgtggtgtctaccgtggaccacttcgtgaacgccatcgaggaaagaggcttccctccaactgctggacagcctcctgccaccaccaagcctaaagaaatcacacccgtgaatcccggcacaagcccactgcttagatacgccgcttggacaggcggactggctgctgttgttctgctgtgcctggtcatcttcctgatctgcaccgccaagcggatgagagtgaaggcctacagagtggacaagagcccttacaaccagagcatgtacgctgccggcctgcctgtggacgacttcgaggatagcgagagcaccgacaccgaggaagagttcggcaacgccattggaggatctcacggcggcagcagctataccgtgtacatcgacaagacccggtgagctggagcctcggtggccatgcttcttgccccttgggcctccccccagcccctcctccccttcctgcacccgtacccccgtggtctttgaataaagtctgagtgggcggcaaaaaaaaaaaaaaaaaaaaaaaaaaaaaaaaaaaaaaaaaaaaaaaaaaaaaaaaaaaaaaaaaaaaaaaaaaaaaaaaaaaaaaaaaaaaaaaaaaaaaaaaaaaaaa

SEQ ID NO: 170 - DNA, 1872 bp, synthetic construct
  source 1..1872: mol_type = other DNA
atgggcaccgtgaacaagcctgttgtgggcgtgctgatgggcttcggcatcatcacaggcaccctgcggatcaccaatcctgtgcgggctagcgtgctgagatacgacgacttccacatcgacgaggacaagctggacaccaacagcgtgtacgagccctactaccacagcgatcacgccgagtctagctgggtcaacagaggcgagagcagcagaaaggcctacgaccacaacagcccctacatctggccccggaacgactacgatggcttcctggaaaatgcccacgagcaccacggcgtgtacaatcaaggcagaggcatcgacagcggcgagagactgatgcagcctacacagatgagcgcccaagaggacctgggagatgataccggcatccacgtgatccccacactgaacggcgacgacagacacaagatcgtgaacgtggaccagcggcagtacggcgacgtgttcaagggcgacctgaatcctaagcctcagggccagcgcctgatcgaggtgtccgtggaagagaatcaccccttcacactgagagcccctatccagagaatctacggcgtgcgctataccgagacatggtcctttctgcccagcctgacatgtaccggggatgccgctcctgccatccagcacatttgcctgaagcacaccacctgtttccaggacgtggtggtggatgtggactgcgccgagaacaccaaagaggatcagctggccgagatcagctaccggttccagggaaagaaagaggccgaccagccttggatcgtggtcaacaccagcacactgttcgacgagctggaactggaccctcctgagattgaacccggggtgctgaaggtgctgagaaccgagaagcagtacctgggagtgtacatctggaacatgagaggcagcgacggcacctctacctacgccacctttctggtcacatggaagggcgacgagaaaacacggaaccccacaccagctgtgacccctcaacctagaggcgccgagtttcacatgtggaattaccacagccacgtgttcagcgtgggcgatacctttagcctggccatgcatctgcagtacaagatccacgaggcccctttcgacctgctgctggaatggctgtacgtgcccatcgatcctacctgccagcctatgcggctgtactccacctgtctgtatcaccccaacgctccccagtgcctgagccacatgaatagcggctgcaccttcacaagccctcacctggctcagcgagtggccagcacagtgtaccagaattgcgagcacgccgacaattacaccgcctactgtctgggcatcagccacatggaacctagcttcggcctgatcctgcacgatggcggcacaaccctgaagttcgtggatacccctgagagcctgagcggcctgtatgtgttcgtggtgtacttcaacggccacgtggaagccgtggcctacaccgtggtgtctaccgtggaccacttcgtgaacgccatcgaggaaagaggcttccctccaactgctggacagcctcctgccaccaccaagcctaaagaaatcacacccgtgaatcccggcacaagcccactgcttagatacgccgcttggacaggcggactggctgctgttgttctgctgtgcctggtcatcttcctgatctgcaccgccaagcggatgagagtgaaggcctacagagtggacaagagcccttacaaccagagcatgtacgctgccggcctgcctgtggacgacttcgaggatagcgagagcaccgacaccgaggaagagttcggcaacgccattggaggatctcacggcggcagcagctataccgtgtacatcgacaagacccggtga

SEQ ID NO: 171 - protein, 623 aa, synthetic construct
MGTVNKPVVGVLMGFGIITGTLRITNPVRASVLRYDDFHIDEDKLDTNSVYEPYYHSDHAESSWVNRGESSRKAYDHNSPYIWPRNDYDGFLENAHEHHGVYNQGRGIDSGERLMQPTQMSAQEDLGDDTGIHVIPTLNGDDRHKIVNVDQRQYGDVFKGDLNPKPQGQRLIEVSVEENHPFTLRAPIQRIYGVRYTETWSFLPSLTCTGDAAPAIQHICLKHTTCFQDVVVDVDCAENTKEDQLAEISYRFQGKKEADQPWIVVNTSTLFDELELDPPEIEPGVLKVLRTEKQYLGVYIWNMRGSDGTSTYATFLVTWKGDEKTRNPTPAVTPQPRGAEFHMWNYHSHVFSVGDTFSLAMHLQYKIHEAPFDLLLEWLYVPIDPTCQPMRLYSTCLYHPNAPQCLSHMNSGCTFTSPHLAQRVASTVYQNCEHADNYTAYCLGISHMEPSFGLILHDGGTTLKFVDTPESLSGLYVFVVYFNGHVEAVAYTVVSTVDHFVNAIEERGFPPTAGQPPATTKPKEITPVNPGTSPLLRYAAWTGGLAAVVLLCLVIFLICTAKRMRVKAYRVDKSPYNQSMYAAGLPVDDFEDSESTDTEEEFGNAIGGSHGGSSYTVYIDKTR

SEQ ID NO: 172 - RNA, 2161 nt, synthetic construct
  source 1..2161: mol_type = other RNA
agactcctccccatcctctccctctgtccctctgtccctctgaccctgcactgtcccagcaccgccaccatgggcaccgtgaacaagcctgttgtgggcgtgctgatgggcttcggcatcatcacaggcaccctgcggatcaccaatcctgtgcgggctagcgtgctgagatacgacgacttccacatcgacgaggacaagctggacaccaacagcgtgtacgagccctactaccacagcgatcacgccgagtctagctgggtcaacagaggcgagagcagcagaaaggcctacgaccacaacagcccctacatctggccccggaacgactacgatggcttcctggaaaatgcccacgagcaccacggcgtgtacaatcaaggcagaggcatcgacagcggcgagagactgatgcagcctacacagatgagcgcccaagaggacctgggagatgataccggcatccacgtgatccccacactgaacggcgacgacagacacaagatcgtgaacgtggaccagcggcagtacggcgacgtgttcaagggcgacctgaatcctaagcctcagggccagcgcctgatcgaggtgtccgtggaagagaatcaccccttcacactgagagcccctatccagagaatctacggcgtgcgctataccgagacatggtcctttctgcccagcctgacatgtaccggggatgccgctcctgccatccagcacatttgcctgaagcacaccacctgtttccaggacgtggtggtggatgtggactgcgccgagaacaccaaagaggatcagctggccgagatcagctaccggttccagggaaagaaagaggccgaccagccttggatcgtggtcaacaccagcacactgttcgacgagctggaactggaccctcctgagattgaacccggggtgctgaaggtgctgagaaccgagaagcagtacctgggagtgtacatctggaacatgagaggcagcgacggcacctctacctacgccacctttctggtcacatggaagggcgacgagaaaacacggaaccccacaccagctgtgacccctcaacctagaggcgccgagtttcacatgtggaattaccacagccacgtgttcagcgtgggcgatacctttagcctggccatgcatctgcagtacaagatccacgaggcccctttcgacctgctgctggaatggctgtacgtgcccatcgatcctacctgccagcctatgcggctgtactccacctgtctgtatcaccccaacgctccccagtgcctgagccacatgaatagcggctgcaccttcacaagccctcacctggctcagcgagtggccagcacagtgtaccagaattgcgagcacgccgacaattacaccgcctactgtctgggcatcagccacatggaacctagcttcggcctgatcctgcacgatggcggcacaaccctgaagttcgtggatacccctgagagcctgagcggcctgtatgtgttcgtggtgtacttcaacggccacgtggaagccgtggcctacaccgtggtgtctaccgtggaccacttcgtgaacgccatcgaggaaagaggcttccctccaactgctggacagcctcctgccaccaccaagcctaaagaaatcacacccgtgaatcccggcacaagcccactgcttagatacgccgcttggacaggcggactggctgctgttgttctgctgtgcctggtcatcttcctgatctgcaccgccaagcggatgagagtgaaggcctacagagtggacaagagcccttacaaccagagcatgtacgctgccggcctgcctgtggacgacttcgaggatagcgagagcaccgacaccgaggaagagttcggcaacgccattggaggatctcacggcggcagcagctataccgtgtacatcgacaagacccggtgagctggagcctcggtggccatgcttcttgccccttgggcctccccccagcccctcctccccttcctgcacccgtacccccgtggtctttgaataaagtctgagtgggcggcaaaaaaaaaaaaaaaaaaaaaaaaaaaaaaaaaaaaaaaaaaaaaaaaaaaaaaaaaaaaaaaaaaaaaaaaaaaaaaaaaaaaaaaaaaaaaaaaaaaaaaaaaaaaaa

SEQ ID NO: 173 - DNA, 46 bp, synthetic construct
  source 1..46: mol_type = other DNA
agaaataagagagaaaagaagagtaagaagaaatataagagccacc

SEQ ID NO: 174 - RNA, 69 nt, synthetic construct
  source 1..69: mol_type = other RNA
agactcctccccatcctctccctctgtccctctgtccctctgaccctgcactgtcccagcaccgccacc

SEQ ID NO: 175 - DNA, 102 bp, synthetic construct
  source 1..102: mol_type = other DNA
agcattctgtggtctgatcatcctgtggtttcgtcgccgccatcctcgtcgcgacacgctgttttcggttctcggcccgacgagccatcgccatcctacagc

SEQ ID NO: 176 - DNA, 102 bp, synthetic construct
  source 1..102: mol_type = other DNA
agcactcgcgctgccatcactcttccgccgtcttcgccgccatcctcggcgcgactcgcttctttcggttctaccaggtagagtccgccgccatcctccacc

SEQ ID NO: 177 - DNA, 102 bp, synthetic construct
  source 1..102: mol_type = other DNA
agcttgtctcgctccggggaacgctcggaaactcccggccgccgccacccgcgtctgttctgttacacaagggaagaaaagccgctgccgcactccgagtgt

SEQ ID NO: 178 - DNA, 110 bp, synthetic construct
  source 1..110: mol_type = other DNA
gctggagcctcggtggccatgcttcttgccccttgggcctccccccagcccctcctccccttcctgcacccgtacccccgtggtctttgaataaagtctgagtgggcggc

SEQ ID NO: 179 - DNA, 132 bp, synthetic construct
  source 1..132: mol_type = other DNA
gctcgctttcttgctgtccaatttctattaaaggttcctttgttccctaagtccaactactaaactgggggatattatgaagggccttgagcatctggattctgcctaataaaaaacatttattttcattgc

SEQ ID NO: 180 - DNA, 88 bp, synthetic construct
  source 1..88: mol_type = other DNA
ttctggacttctggacttctggacttctggacttctggacttctggacttctggacttctggacttctggacttctggacttctggac

SEQ ID NO: 181 - DNA, 115 bp, synthetic construct
  source 1..115: mol_type = other DNA
cctcgccccggacctgccctcccgccaggtgcacccacctgcaataaatgcagcgaagccgggacctcgccccggacctgccctcccgccaggtgcacccacctgcaataaatgc

SEQ ID NO: 182 - protein, 6 aa, synthetic construct
SESTDT

SEQ ID NO: 183 - protein, 6 aa, synthetic construct
AEAADA

SEQ ID NO: 184 - protein, 4 aa, synthetic construct
AYRV

SEQ ID NO: 185 - protein, 4 aa, synthetic construct
YAGL

SEQ ID NO: 186 - protein, 11 aa, synthetic construct
YRVDKSPYNQS

SEQ ID NO: 187 - protein, 19 aa, synthetic construct
YRVDKSPYNQSMYYAGLPV

SEQ ID NO: 188 - protein, 4 aa, synthetic construct
SSTT

SEQ ID NO: 189 - protein, 12 aa, synthetic construct
AYRVYAGLSSTT

SEQ ID NO: 190 - protein, 8 aa, synthetic construct
YAGLSSTT

SEQ ID NO: 191 - protein, 8 aa, synthetic construct
AYRVYAGL